European Patent Specification EP 3 638 316 B1, published September 2, 2026. Title: GENE THERAPY FOR OCULAR DISORDERS. Applicant: Trustees of the University of Pennsylvania. The sequence listing filed with the application follows.

SEQUENCE LISTING (46 sequences)

SEQ ID NO: 1 - DNA, 1962 bp, Artificial Sequence
  codon optimized sequence
  CDS (1)..(1962)
atggctgataccctgccctctgaattcgacgtgattgtgattggaaccggactccctgaatcgatcatcgccgcggcctgttcccggtccggtcggcgcgtgctgcacgtcgattcgagaagctactacggagggaattgggcctcattctccttctccggactgctctcctggctgaaggagtatcaggagaactccgacattgtctccgactcacctgtgtggcaggaccagatcctggaaaacgaggaagcaatagccctgagccggaaggacaagaccatccagcacgtggaggtgttctgttatgcctcccaagacctccatgaggacgtggaagaggctggagcgttgcagaagaatcatgccctcgtgacctccgctaactccaccgaggcagccgacagcgccttcctgccgaccgaggatgaatccctgtcaactatgtcgtgcgaaatgctgaccgaacagactccgagctccgaccccgaaaacgccctggaagtgaacggagcggaagtgaccggcgaaaaggagaaccattgcgacgacaagacttgtgtcccatccacttccgcggaggacatgtccgagaatgtgcctatcgccgaggacaccaccgaacagcccaagaagaacagaatcacgtacagccagatcatcaaggaggggcggaggtttaacatcgatctggtgtcgaagctgctgtacagccgcggtctgctgatcgatctgctcattaagtcgaacgtgtcgagatacgccgagttcaagaacatcacaaggattctcgccttccgggaaggaagagtggaacaagtgccgtgctcccgggccgacgtgttcaactcaaagcaacttaccatggtggaaaagcgcatgctgatgaaattcctgaccttctgcatggagtacgaaaagtaccctgatgagtacaagggttacgaagaaattactttctacgagtacctcaagacccagaagctgaccccgaatctgcagtacattgtgatgcactcaatcgcaatgacctccgaaaccgcctcctcgaccatcgacgggctcaaggccaccaagaacttcctgcactgtttggggcgctacggcaacactccgttcctcttcccgctgtacggccagggagagctgcctcagtgtttctgccggatgtgcgccgtgttcggcggaatctactgtctccgccactcggtccagtgcctggtggtggacaaggaatccaggaagtgcaaagccattattgaccagttcggacaacggatcatttccgagcactttcttgtggaggactcatacttcccggagaacatgtgctctcgggtccagtatcgacagatttccagggcggtgctcattactgaccggagcgtcctcaagaccgatagcgaccagcagatctccatcctgaccgtgccggcggaagaacccggcacttttgccgtgcgcgtgatcgagctttgctcatccaccatgacttgcatgaaaggcacttacctggtgcacctgacgtgcacctcatcgaaaaccgctagagaggacctggaatccgtcgtccaaaagctgttcgtgccttacaccgagatggaaattgaaaacgaacaagtggagaagccccgcatcctttgggccctgtactttaacatgcgcgattcctccgatatctcgcggtcctgctataacgacttgccttcgaacgtctacgtctgctccgggccagactgcggtcttggcaacgacaatgccgtgaagcaggcggaaacactgttccaagagatctgccctaacgaggatttttgcccgccccccccaaaccccgaggatatcatcttggacggagacagcctgcagccagaagcatccgagtccagcgccatcccggaggccaacagcgaaaccttcaaggagagcactaacctgggcaacctggaagagtccagcgaatga

SEQ ID NO: 2 - protein, 653 aa, Artificial Sequence
  Synthetic Construct
MADTLPSEFDVIVIGTGLPESIIAAACSRSGRRVLHVDSRSYYGGNWASFSFSGLLSWLKEYQENSDIVSDSPVWQDQILENEEAIALSRKDKTIQHVEVFCYASQDLHEDVEEAGALQKNHALVTSANSTEAADSAFLPTEDESLSTMSCEMLTEQTPSSDPENALEVNGAEVTGEKENHCDDKTCVPSTSAEDMSENVPIAEDTTEQPKKNRITYSQIIKEGRRFNIDLVSKLLYSRGLLIDLLIKSNVSRYAEFKNITRILAFREGRVEQVPCSRADVFNSKQLTMVEKRMLMKFLTFCMEYEKYPDEYKGYEEITFYEYLKTQKLTPNLQYIVMHSIAMTSETASSTIDGLKATKNFLHCLGRYGNTPFLFPLYGQGELPQCFCRMCAVFGGIYCLRHSVQCLVVDKESRKCKAIIDQFGQRIISEHFLVEDSYFPENMCSRVQYRQISRAVLITDRSVLKTDSDQQISILTVPAEEPGTFAVRVIELCSSTMTCMKGTYLVHLTCTSSKTAREDLESVVQKLFVPYTEMEIENEQVEKPRILWALYFNMRDSSDISRSCYNDLPSNVYVCSGPDCGLGNDNAVKQAETLFQEICPNEDFCPPPPNPEDIILDGDSLQPEASESSAIPEANSETFKESTNLGNLEESSE

SEQ ID NO: 3 - DNA, 1962 bp, Homo sapiens
  CDS (1)..(1962)
atggcggatactctcccttcggagtttgatgtgatcgtaatagggacgggtttgcctgaatccatcattgcagctgcatgttcaagaagtggccggagagttctgcatgttgattcaagaagctactatggaggaaactgggccagttttagcttttcaggactattgtcctggctaaaggaataccaggaaaacagtgacattgtaagtgacagtccagtgtggcaagaccagatccttgaaaatgaagaagccattgctcttagcaggaaggacaaaactattcaacatgtggaagtattttgttatgccagtcaggatttgcatgaagatgtcgaagaagctggtgcactgcagaaaaatcatgctcttgtgacatctgcaaactccacagaagctgcagattctgccttcctgcctacggaggatgagtcattaagcactatgagctgtgaaatgctcacagaacaaactccaagcagcgatccagagaatgcgctagaagtaaatggtgctgaagtgacaggggaaaaagaaaaccattgtgatgataaaacttgtgtgccatcaacttcagcagaagacatgagtgaaaatgtgcctatagcagaagataccacagagcaaccaaagaaaaacagaattacttactcacaaattattaaagaaggcaggagatttaatattgatttagtatcaaagctgctgtattctcgaggattactaattgatcttctaatcaaatctaatgttagtcgatatgcagagtttaaaaatattaccaggattcttgcatttcgagaaggacgagtggaacaggttccgtgttccagagcagatgtctttaatagcaaacaacttactatggtagaaaagcgaatgctaatgaaatttcttacattttgtatggaatatgagaaatatcctgatgaatataaaggatatgaagagatcacattttatgaatatttaaagactcaaaaattaacccccaacctccaatatattgtcatgcattcaattgcaatgacatcagagacagccagcagcaccatagatggtctcaaagctaccaaaaactttcttcactgtcttgggcggtatggcaacactccatttttgtttcctttatatggccaaggagaactcccccagtgtttctgcaggatgtgtgctgtgtttggtggaatttattgtcttcgccattcagtacagtgccttgtagtggacaaagaatccagaaaatgtaaagcaattatagatcagtttggtcagagaataatctctgagcatttcctcgtggaggacagttactttcctgagaacatgtgctcacgtgtgcaatacaggcagatctccagggcagtgctgattacagatagatctgtcctaaaaacagattcagatcaacagatttccattttgacagtgccagcagaggaaccaggaacttttgctgttcgggtcattgagttatgttcttcaacgatgacatgcatgaaaggcacctatttggttcatttgacttgcacatcttctaaaacagcaagagaagatttagaatcagttgtgcagaaattgtttgttccatatactgaaatggagatagaaaatgaacaagtagaaaagccaagaattctgtgggctctttacttcaatatgagagattcgtcagacatcagcaggagctgttataatgatttaccatccaacgtttatgtctgctctggcccagattgtggtttaggaaatgataatgcagtcaaacaggctgaaacacttttccaggaaatctgccccaatgaagatttctgtccccctccaccaaatcctgaagacattatccttgatggagacagtttacagccagaggcttcagaatccagtgccataccagaggctaactcggagactttcaaggaaagcacaaaccttggaaacctagaggagtcctctgaataa

SEQ ID NO: 4 - protein, 653 aa, Homo sapiens; identical to SEQ ID NO: 2

SEQ ID NO: 5 - DNA, 1985 bp, Artificial Sequence
  constructed plasmid
  misc_feature (1)..(8): NotI restriction site for subcloning into proviral plasmid
  misc_feature (4)..(16): Kozak consensus sequence
  CDS (13)..(1971): codon-optimized open reading frame (ORF)
  misc_feature (1972)..(1977): BclI restriction site with embedded stop codon/ site to add optional epitope tag
  misc_feature (1980)..(1985): BamHI restriction site for subcloning into proviral plasmid
gcggccgccaccatggctgataccctgccctctgaattcgacgtgattgtgattggaaccggactccctgaatcgatcatcgccgcggcctgttcccggtccggtcggcgcgtgctgcacgtcgattcgagaagctactacggagggaattgggcctcattctccttctccggactgctctcctggctgaaggagtatcaggagaactccgacattgtctccgactcacctgtgtggcaggaccagatcctggaaaacgaggaagcaatagccctgagccggaaggacaagaccatccagcacgtggaggtgttctgttatgcctcccaagacctccatgaggacgtggaagaggctggagcgttgcagaagaatcatgccctcgtgacctccgctaactccaccgaggcagccgacagcgccttcctgccgaccgaggatgaatccctgtcaactatgtcgtgcgaaatgctgaccgaacagactccgagctccgaccccgaaaacgccctggaagtgaacggagcggaagtgaccggcgaaaaggagaaccattgcgacgacaagacttgtgtcccatccacttccgcggaggacatgtccgagaatgtgcctatcgccgaggacaccaccgaacagcccaagaagaacagaatcacgtacagccagatcatcaaggaggggcggaggtttaacatcgatctggtgtcgaagctgctgtacagccgcggtctgctgatcgatctgctcattaagtcgaacgtgtcgagatacgccgagttcaagaacatcacaaggattctcgccttccgggaaggaagagtggaacaagtgccgtgctcccgggccgacgtgttcaactcaaagcaacttaccatggtggaaaagcgcatgctgatgaaattcctgaccttctgcatggagtacgaaaagtaccctgatgagtacaagggttacgaagaaattactttctacgagtacctcaagacccagaagctgaccccgaatctgcagtacattgtgatgcactcaatcgcaatgacctccgaaaccgcctcctcgaccatcgacgggctcaaggccaccaagaacttcctgcactgtttggggcgctacggcaacactccgttcctcttcccgctgtacggccagggagagctgcctcagtgtttctgccggatgtgcgccgtgttcggcggaatctactgtctccgccactcggtccagtgcctggtggtggacaaggaatccaggaagtgcaaagccattattgaccagttcggacaacggatcatttccgagcactttcttgtggaggactcatacttcccggagaacatgtgctctcgggtccagtatcgacagatttccagggcggtgctcattactgaccggagcgtcctcaagaccgatagcgaccagcagatctccatcctgaccgtgccggcggaagaacccggcacttttgccgtgcgcgtgatcgagctttgctcatccaccatgacttgcatgaaaggcacttacctggtgcacctgacgtgcacctcatcgaaaaccgctagagaggacctggaatccgtcgtccaaaagctgttcgtgccttacaccgagatggaaattgaaaacgaacaagtggagaagccccgcatcctttgggccctgtactttaacatgcgcgattcctccgatatctcgcggtcctgctataacgacttgccttcgaacgtctacgtctgctccgggccagactgcggtcttggcaacgacaatgccgtgaagcaggcggaaacactgttccaagagatctgccctaacgaggatttttgcccgccccccccaaaccccgaggatatcatcttggacggagacagcctgcagccagaagcatccgagtccagcgccatcccggaggccaacagcgaaaccttcaaggagagcactaacctgggcaacctggaagagtccagcgaatgatcataggatcc

SEQ ID NO: 6 - protein, 653 aa, Artificial Sequence; identical to SEQ ID NO: 2
  Synthetic Construct

SEQ ID NO: 7 - DNA, 9187 bp, Artificial Sequence
  constructed plasmid
  misc_feature (1)..(145): 5' ITR
  promoter (169)..(1786): CMV.CBA promoter
  misc_feature (1787)..(1794): Not I cloning site, cuts at 1789
  misc_feature (1805)..(1810): BamHI cloning site, cuts at 1806
  polyA_signal (1850)..(2052): BGH PolyA
  misc_feature (2109)..(2252): 3' ITR
  misc_feature (2571)..(6624): lambda stuffer
  misc_feature (7314)..(8126): Kanamycin resistance (complementary)
  misc_feature (8485)..(9128): Origin of replication (complementary)
tcgctcgctcactgaggccgcccgggcaaagcccgggcgtcgggcgacctttggtcgcccggcctcagtgagcgagcgagcgcgcagagagggagtggccaactccatcactaggggttcctgcggcctagtaggctcagaggcacacaggagtttctgcaaatctagtgcaggcgttacataacttacggtaaatggcccgcctggctgaccgcccaacgacccccgcccattgacgtcaataatgacgtatgttcccatagtaacgccaatagggactttccattgacgtcaatgggtggagtatttacggtaaactgcccacttggcagtacatcaagtgtatcatatgccaagtacgccccctattgacgtcaatgacggtaaatggcccgcctggcattatgcccagtacatgaccttatgggactttcctacttggcagtacatctacgtattagtcatcgctattaacatggtcgaggtgagccccacgttctgcttcactctccccatctcccccccctccccacccccaattttgtatttatttattttttaattattttgtgcagcgatgggggcggggggggggggggggcgcgcgccaggcggggcggggcggggcgaggggcggggcggggcgaggcggagaggtgcggcggcagccaatcagagcggcgcgctccgaaagtttccttttatggcgaggcggcggcggcggcggccctataaaaagcgaagcgcgcggcgggcggggagtcgctgcgacgctgccttcgccccgtgccccgctccgccgccgcctcgcgccgcccgccccggctctgactgaccgcgttactcccacaggtgagcgggcgggacggcccttctcctccgggctgtaattagcgcttggtttaatgacggcttgtttcttttctgtggctgcgtgaaagccttgaggggctccgggagggccctttgtgcggggggagcggctcggggggtgcgtgcgtgtgtgtgtgcgtggggagcgccgcgtgcggctccgcgctgcccggcggctgtgagcgctgcgggcgcggcgcggggctttgtgcgctccgcagtgtgcgcgaggggagcgcggccgggggcggtgccccgcggtgcggggggggctgcgaggggaacaaaggctgcgtgcggggtgtgtgcgtgggggggtgagcagggggtgtgggcgcgtcggtcgggctgcaaccccccctgcacccccctccccgagttgctgagcacggcccggcttcgggtgcggggctccgtacggggcgtggcgcggggctcgccgtgccgggcggggggtggcggcaggtgggggtgccgggcggggcggggccgcctcgggccggggagggctcgggggaggggcgcggcggcccccggagcgccggcggctgtcgaggcgcggcgagccgcagccattgccttttatggtaatcgtgcgagagggcgcagggacttcctttgtcccaaatctgtgcggagccgaaatctgggaggcgccgccgcaccccctctagcgggcgcggggcgaagcggtgcggcgccggcaggaaggaaatgggcggggagggccttcgtgcgtcgccgcgccgccgtccccttctccctctccagcctcggggctgtccgcggggggacggctgccttcgggggggacggggcagggcggggttcggcttctggcgtgtgaccggcggctctagacaattgtactaaccttcttctctttcctctcctgacaggttggtgtacactagcggccgcatagtactgcggatcctgcagatctcgagccgaattcctgcagcccgggggatcagcctcgactgtgccttctagttgccagccatctgttgtttgcccctcccccgtgccttccttgaccctggaaggtgccactcccactgtcctttcctaataaaatgaggaaattgcatcgcattgtctgagtaggtgtcattctattctggggggtggggtggggcaggacagcaagggggaggattgggaagacaatagcaggcatgctggggatgcggtgggctctatggcttctgaggcggaaagaaccagctggggctcgagatccactagggccgcaggaacccctagtgatggagttggccactccctctctgcgcgctcgctcgctcactgaggccgggcgaccaaaggtcgcccgacgcccgggctttgcccgggcggcctcagtgagcgagcgacctgcaggggcagcttgaaggaaatactaaggcaaaggtactgcaagtgctcgcaacattcgcttatgcggattattgccgtagtgccgcgacgccgggggcaagatgcagagattgccatggtacaggccgtgcggttgatattgccaaaacagagctgtgggggagagttgtcgagaaagagtgcggaagatgcaaaggcgtcggctattcaaggatgccagcaagcgcagcatatcgcgctgtgacgatgctaatcccaaaccttacccaacccacctggtcacgcactgttaagccgctgtatgacgctctggtggtgcaatgccacaaagaagagtcaatcgcagacaacattttgaatgcggtcacacgttagcagcatgattgccacggatggcaacatattaacggcatgatattgacttattgaataaaattgggtaaatttgactcaacgatgggttaattcgctcgttgtggtagtgagatgaaaagaggcggcgcttactaccgattccgcctagttggtcacttcgacgtatcgtctggaactccaaccatcgcaggcagagaggtctgcaaaatgcaatcccgaaacagttcgcaggtaatagttagagcctgcataacggtttcgggattttttatatctgcacaacaggtaagagcattgagtcgataatcgtgaagagtcggcgagcctggttagccagtgctctttccgttgtgctgaattaagcgaataccggaagcagaaccggatcaccaaatgcgtacaggcgtcatcgccgcccagcaacagcacaacccaaactgagccgtagccactgtctgtcctgaattcattagtaatagttacgctgcggccttttacacatgaccttcgtgaaagcgggtggcaggaggtcgcgctaacaacctcctgccgttttgcccgtgcatatcggtcacgaacaaatctgattactaaacacagtagcctggatttgttctatcagtaatcgaccttattcctaattaaatagagcaaatccccttattgggggtaagacatgaagatgccagaaaaacatgacctgttggccgccattctcgcggcaaaggaacaaggcatcggggcaatccttgcgtttgcaatggcgtaccttcgcggcagatataatggcggtgcgtttacaaaaacagtaatcgacgcaacgatgtgcgccattatcgcctggttcattcgtgaccttctcgacttcgccggactaagtagcaatctcgcttatataacgagcgtgtttatcggctacatcggtactgactcgattggttcgcttatcaaacgcttcgctgctaaaaaagccggagtagaagatggtagaaatcaataatcaacgtaaggcgttcctcgatatgctggcgtggtcggagggaactgataacggacgtcagaaaaccagaaatcatggttatgacgtcattgtaggcggagagctatttactgattactccgatcaccctcgcaaacttgtcacgctaaacccaaaactcaaatcaacaggcgccggacgctaccagcttctttcccgttggtgggatgcctaccgcaagcagcttggcctgaaagacttctctccgaaaagtcaggacgctgtggcattgcagcagattaaggagcgtggcgctttacctatgattgatcgtggtgatatccgtcaggcaatcgaccgttgcagcaatatctgggcttcactgccgggcgctggttatggtcagttcgagcataaggctgacagcctgattgcaaaattcaaagaagcgggcggaacggtcagagagattgatgtatgagcagagtcaccgcgattatctccgctctggttatctgcatcatcgtctgcctgtcatgggctgttaatcattaccgtgataacgccattacctacaaagcccagcgcgacaaaaatgccagagaactgaagctggcgaacgcggcaattactgacatgcagatgcgtcagcgtgatgttgctgcgctcgatgcaaaatacacgaaggagttagctgatgctaaagctgaaaatgatgctctgcgtgatgatgttgccgctggtcgtcgtcggttgcacatcaaagcagtctgtcagtcagtgcgtgaagccaccaccgcctccggcgtggataatgcagcctccccccgactggcagacaccgctgaacgggattatttcaccctcagagagaggctgatcactatgcaaaaacaactggaaggaacccagaagtatattaatgagcagtgcagatagagttgcccatatcgatgggcaactcatgcaattattgtgagcaatacacacgcgcttccagcggagtataaatgcctaaagtaataaaaccgagcaatccatttacgaatgtttgctgggtttctgttttaacaacattttctgcgccgccacaaattttggctgcatcgacagttttcttctgcccaattccagaaacgaagaaatgatgggtgatggtttcctttggtgctactgctgccggtttgttttgaacagtaaacgtctgttgagcacatcctgtaataagcagggccagcgcagtagcgagtagcatttttttcatggtgttattcccgatgctttttgaagttcgcagaatcgtatgtgtagaaaattaaacaaaccctaaacaatgagttgaaatttcatattgttaatatttattaatgtatgtcaggtgcgatgaatcgtcattgtattcccggattaactatgtccacagccctgacggggaacttctctgcgggagtgtccgggaataattaaaacgatgcacacagggtttagcgcgtacacgtattgcattatgccaacgccccggtgctgacacggaagaaaccggacgttatgatttagcgtggaaagatttgtgtagtgttctgaatgctctcagtaaatagtaatgaattatcaaaggtatagtaatatcttttatgttcatggatatttgtaacccatcggaaaactcctgctttagcaagattttccctgtattgctgaaatgtgatttctcttgatttcaacctatcataggacgtttctataagatgcgtgtttcttgagaatttaacatttacaacctttttaagtccttttattaacacggtgttatcgttttctaacacgatgtgaatattatctgtggctagatagtaaatataatgtgagacgttgtgacgttttagttcagaataaaacaattcacagtctaaatcttttcgcacttgatcgaatatttctttaaaaatggcaacctgagccattggtaaaaccttccatgtgatacgagggcgcgtagtttgcattatcgtttttatcgtttcaatctggtctgacctccttgtgttttgttgatgatttatgtcaaatattaggaatgttttcacttaatagtattggttgcgtaacaaagtgcggtcctgctggcattctggagggaaatacaaccgacagatgtatgtaaggccaacgtgctcaaatcttcatacagaaagatttgaagtaatattttaaccgctagatgaagagcaagcgcatggagcgacaaaatgaataaagaacaatctgctgatgatccctccgtggatctgattcgtgtaaaaaatatgcttaatagcaccatttctatgagttaccctgatgttgtaattgcatgtatagaacataaggtgtctctggaagcattcagagcaattgaggcagcgttggtgaagcacgataataatatgaaggattattccctggtggttgactgatcaccataactgctaatcattcaaactatttagtctgtgacagagccaacacgcagtctgtcactgtcaggaaagtggtaaaactgcaactcaattactgcaatgccctcgtaattaagtgaatttacaatatcgtcctgttcggagggaagaacgcgggatgttcattcttcatcacttttaattgatgtatatgctctcttttctgacgttagtctccgacggcaggcttcaatgacccaggctgagaaattcccggaccctttttgctcaagagcgatgttaatttgttcaatcatttggttaggaaagcggatgttgcgggttgttgttctgcgggttctgttcttcgttgacatgaggttgccccgtattcagtgtcgctgatttgtattgtctgaagttgtttttacgttaagttgatgcagatcaattaatacgatacctgcgtcataattgattatttgacgtggtttgatggcctccacgcacgttgtgatatgtagatgataatcattatcactttacgggtcctttccggtgatccgacaggttacggcctgatgcggtattttctccttacgcatctgtgcggtatttcacaccgcatacgtcaaagcaaccatagtacgcgccctgtagcggcgcattaagcgcggcgggtgtggtggttacgcgcagcgtgaccgctacacttgccagcgccctagcgcccgctcctttcgctttcttcccttcctttctcgccacgttcgccggctttccccgtcaagctctaaatcgggggctccctttagggttccgatttagtgctttacggcacctcgaccccaaaaaacttgatttgggtgatggttcacgtagtgggccatcgccctgatagacggtttttcgccctttgacgttggagtccacgttctttaatagtggactcttgttccaaactggaacaacactcaaccctatctcgggctattcttttgatttagacctgcaggcatgcaagcttactggccgtcgttttacaacgtcgtgactgggaaaaccctggcgttacccaacttaatcgccttgcagcacatccccctttcgccagctggcgtaatagcgaagaggcccgcaccgatcgcccttcccaacagttgcgcagcctgaatggcgaatgcgatttattcaacaaagccgccgtcccgtcaagtcagcgtaatgctctgccagtgttacaaccaattaaccaattctgattagaaaaactcatcgagcatcaaatgaaactgcaatttattcatatcaggattatcaataccatatttttgaaaaagccgtttctgtaatgaaggagaaaactcaccgaggcagttccataggatggcaagatcctggtatcggtctgcgattccgactcgtccaacatcaatacaacctattaatttcccctcgtcaaaaataaggttatcaagtgagaaatcaccatgagtgacgactgaatccggtgagaatggcaaaagcttatgcatttctttccagacttgttcaacaggccagccattacgctcgtcatcaaaatcactcgcatcaaccaaaccgttattcattcgtgattgcgcctgagcgagacgaaatacgcgatcgctgttaaaaggacaattacaaacaggaatcgaatgcaaccggcgcaggaacactgccagcgcatcaacaatattttcacctgaatcaggatattcttctaatacctggaatgctgttttcccggggatcgcagtggtgagtaaccatgcatcatcaggagtacggataaaatgcttgatggtcggaagaggcataaattccgtcagccagtttagtctgaccatctcatctgtaacatcattggcaacgctacctttgccatgtttcagaaacaactctggcgcatcgggcttcccatacaatcgatagattgtcgcacctgattgcccgacattatcgcgagcccatttatacccatataaatcagcatccatgttggaatttaatcgcggcttcgagcaagacgtttcccgttgaatatggctcataacaccccttgtattactgtttatgtaagcagacagttttattgttcatgatgatatatttttatcttgtgcaatgtaacatcagagattttgagacacaacgtggctttgttgaataaatcgaacttttgctgagttgaaggatcagatcacgcatcttcccgacaacgcagaccgttccgtggcaaagcaaaagttcaaaatcaccaactggtccacctacaacaaagctctcatcaaccgtggctccctcactttctggctggatgatggggcgattcaggcctggtatgagtcagcaacaccttcttcacgaggcagacctctcgacggatcgttccactgagcgtcagaccccgtagaaaagatcaaaggatcttcttgagatcctttttttctgcgcgtaatctgctgcttgcaaacaaaaaaaccaccgctaccagcggtggtttgtttgccggatcaagagctaccaactctttttccgaaggtaactggcttcagcagagcgcagataccaaatactgtccttctagtgtagccgtagttaggccaccacttcaagaactctgtagcaccgcctacatacctcgctctgctaatcctgttaccagtggctgctgccagtggcgataagtcgtgtcttaccgggttggactcaagacgatagttaccggataaggcgcagcggtcgggctgaacggggggttcgtgcacacagcccagcttggagcgaacgacctacaccgaactgagatacctacagcgtgagctatgagaaagcgccacgcttcccgaagggagaaaggcggacaggtatccggtaagcggcagggtcggaacaggagagcgcacgagggagcttccagggggaaacgcctggtatctttatagtcctgtcgggtttcgccacctctgacttgagcgtcgatttttgtgatgctcgtcaggggggcggagcctatggaaaaacgccagcaacgcggcctttttacggttcctggccttttgctggccttttgctcacatgtcctgcaggcagctgcgcgccagctgcgcgc

SEQ ID NO: 8 - DNA, 11148 bp, Artificial Sequence
  constructed plasmid
tcgctcgctcactgaggccgcccgggcaaagcccgggcgtcgggcgacctttggtcgcccggcctcagtgagcgagcgagcgcgcagagagggagtggccaactccatcactaggggttcctgcggcctagtaggctcagaggcacacaggagtttctgcaaatctagtgcaggcgttacataacttacggtaaatggcccgcctggctgaccgcccaacgacccccgcccattgacgtcaataatgacgtatgttcccatagtaacgccaatagggactttccattgacgtcaatgggtggagtatttacggtaaactgcccacttggcagtacatcaagtgtatcatatgccaagtacgccccctattgacgtcaatgacggtaaatggcccgcctggcattatgcccagtacatgaccttatgggactttcctacttggcagtacatctacgtattagtcatcgctattaacatggtcgaggtgagccccacgttctgcttcactctccccatctcccccccctccccacccccaattttgtatttatttattttttaattattttgtgcagcgatgggggcggggggggggggggggcgcgcgccaggcggggcggggcggggcgaggggcggggcggggcgaggcggagaggtgcggcggcagccaatcagagcggcgcgctccgaaagtttccttttatggcgaggcggcggcggcggcggccctataaaaagcgaagcgcgcggcgggcggggagtcgctgcgacgctgccttcgccccgtgccccgctccgccgccgcctcgcgccgcccgccccggctctgactgaccgcgttactcccacaggtgagcgggcgggacggcccttctcctccgggctgtaattagcgcttggtttaatgacggcttgtttcttttctgtggctgcgtgaaagccttgaggggctccgggagggccctttgtgcggggggagcggctcggggggtgcgtgcgtgtgtgtgtgcgtggggagcgccgcgtgcggctccgcgctgcccggcggctgtgagcgctgcgggcgcggcgcggggctttgtgcgctccgcagtgtgcgcgaggggagcgcggccgggggcggtgccccgcggtgcggggggggctgcgaggggaacaaaggctgcgtgcggggtgtgtgcgtgggggggtgagcagggggtgtgggcgcgtcggtcgggctgcaaccccccctgcacccccctccccgagttgctgagcacggcccggcttcgggtgcggggctccgtacggggcgtggcgcggggctcgccgtgccgggcggggggtggcggcaggtgggggtgccgggcggggcggggccgcctcgggccggggagggctcgggggaggggcgcggcggcccccggagcgccggcggctgtcgaggcgcggcgagccgcagccattgccttttatggtaatcgtgcgagagggcgcagggacttcctttgtcccaaatctgtgcggagccgaaatctgggaggcgccgccgcaccccctctagcgggcgcggggcgaagcggtgcggcgccggcaggaaggaaatgggcggggagggccttcgtgcgtcgccgcgccgccgtccccttctccctctccagcctcggggctgtccgcggggggacggctgccttcgggggggacggggcagggcggggttcggcttctggcgtgtgaccggcggctctagacaattgtactaaccttcttctctttcctctcctgacaggttggtgtacactagcggccgccaccatggctgataccctgccctctgaattcgacgtgattgtgattggaaccggactccctgaatcgatcatcgccgcggcctgttcccggtccggtcggcgcgtgctgcacgtcgattcgagaagctactacggagggaattgggcctcattctccttctccggactgctctcctggctgaaggagtatcaggagaactccgacattgtctccgactcacctgtgtggcaggaccagatcctggaaaacgaggaagcaatagccctgagccggaaggacaagaccatccagcacgtggaggtgttctgttatgcctcccaagacctccatgaggacgtggaagaggctggagcgttgcagaagaatcatgccctcgtgacctccgctaactccaccgaggcagccgacagcgccttcctgccgaccgaggatgaatccctgtcaactatgtcgtgcgaaatgctgaccgaacagactccgagctccgaccccgaaaacgccctggaagtgaacggagcggaagtgaccggcgaaaaggagaaccattgcgacgacaagacttgtgtcccatccacttccgcggaggacatgtccgagaatgtgcctatcgccgaggacaccaccgaacagcccaagaagaacagaatcacgtacagccagatcatcaaggaggggcggaggtttaacatcgatctggtgtcgaagctgctgtacagccgcggtctgctgatcgatctgctcattaagtcgaacgtgtcgagatacgccgagttcaagaacatcacaaggattctcgccttccgggaaggaagagtggaacaagtgccgtgctcccgggccgacgtgttcaactcaaagcaacttaccatggtggaaaagcgcatgctgatgaaattcctgaccttctgcatggagtacgaaaagtaccctgatgagtacaagggttacgaagaaattactttctacgagtacctcaagacccagaagctgaccccgaatctgcagtacattgtgatgcactcaatcgcaatgacctccgaaaccgcctcctcgaccatcgacgggctcaaggccaccaagaacttcctgcactgtttggggcgctacggcaacactccgttcctcttcccgctgtacggccagggagagctgcctcagtgtttctgccggatgtgcgccgtgttcggcggaatctactgtctccgccactcggtccagtgcctggtggtggacaaggaatccaggaagtgcaaagccattattgaccagttcggacaacggatcatttccgagcactttcttgtggaggactcatacttcccggagaacatgtgctctcgggtccagtatcgacagatttccagggcggtgctcattactgaccggagcgtcctcaagaccgatagcgaccagcagatctccatcctgaccgtgccggcggaagaacccggcacttttgccgtgcgcgtgatcgagctttgctcatccaccatgacttgcatgaaaggcacttacctggtgcacctgacgtgcacctcatcgaaaaccgctagagaggacctggaatccgtcgtccaaaagctgttcgtgccttacaccgagatggaaattgaaaacgaacaagtggagaagccccgcatcctttgggccctgtactttaacatgcgcgattcctccgatatctcgcggtcctgctataacgacttgccttcgaacgtctacgtctgctccgggccagactgcggtcttggcaacgacaatgccgtgaagcaggcggaaacactgttccaagagatctgccctaacgaggatttttgcccgccccccccaaaccccgaggatatcatcttggacggagacagcctgcagccagaagcatccgagtccagcgccatcccggaggccaacagcgaaaccttcaaggagagcactaacctgggcaacctggaagagtccagcgaatgatcataggatcctgcagatctcgagccgaattcctgcagcccgggggatcagcctcgactgtgccttctagttgccagccatctgttgtttgcccctcccccgtgccttccttgaccctggaaggtgccactcccactgtcctttcctaataaaatgaggaaattgcatcgcattgtctgagtaggtgtcattctattctggggggtggggtggggcaggacagcaagggggaggattgggaagacaatagcaggcatgctggggatgcggtgggctctatggcttctgaggcggaaagaaccagctggggctcgagatccactagggccgcaggaacccctagtgatggagttggccactccctctctgcgcgctcgctcgctcactgaggccgggcgaccaaaggtcgcccgacgcccgggctttgcccgggcggcctcagtgagcgagcgacctgcaggggcagcttgaaggaaatactaaggcaaaggtactgcaagtgctcgcaacattcgcttatgcggattattgccgtagtgccgcgacgccgggggcaagatgcagagattgccatggtacaggccgtgcggttgatattgccaaaacagagctgtgggggagagttgtcgagaaagagtgcggaagatgcaaaggcgtcggctattcaaggatgccagcaagcgcagcatatcgcgctgtgacgatgctaatcccaaaccttacccaacccacctggtcacgcactgttaagccgctgtatgacgctctggtggtgcaatgccacaaagaagagtcaatcgcagacaacattttgaatgcggtcacacgttagcagcatgattgccacggatggcaacatattaacggcatgatattgacttattgaataaaattgggtaaatttgactcaacgatgggttaattcgctcgttgtggtagtgagatgaaaagaggcggcgcttactaccgattccgcctagttggtcacttcgacgtatcgtctggaactccaaccatcgcaggcagagaggtctgcaaaatgcaatcccgaaacagttcgcaggtaatagttagagcctgcataacggtttcgggattttttatatctgcacaacaggtaagagcattgagtcgataatcgtgaagagtcggcgagcctggttagccagtgctctttccgttgtgctgaattaagcgaataccggaagcagaaccggatcaccaaatgcgtacaggcgtcatcgccgcccagcaacagcacaacccaaactgagccgtagccactgtctgtcctgaattcattagtaatagttacgctgcggccttttacacatgaccttcgtgaaagcgggtggcaggaggtcgcgctaacaacctcctgccgttttgcccgtgcatatcggtcacgaacaaatctgattactaaacacagtagcctggatttgttctatcagtaatcgaccttattcctaattaaatagagcaaatccccttattgggggtaagacatgaagatgccagaaaaacatgacctgttggccgccattctcgcggcaaaggaacaaggcatcggggcaatccttgcgtttgcaatggcgtaccttcgcggcagatataatggcggtgcgtttacaaaaacagtaatcgacgcaacgatgtgcgccattatcgcctggttcattcgtgaccttctcgacttcgccggactaagtagcaatctcgcttatataacgagcgtgtttatcggctacatcggtactgactcgattggttcgcttatcaaacgcttcgctgctaaaaaagccggagtagaagatggtagaaatcaataatcaacgtaaggcgttcctcgatatgctggcgtggtcggagggaactgataacggacgtcagaaaaccagaaatcatggttatgacgtcattgtaggcggagagctatttactgattactccgatcaccctcgcaaacttgtcacgctaaacccaaaactcaaatcaacaggcgccggacgctaccagcttctttcccgttggtgggatgcctaccgcaagcagcttggcctgaaagacttctctccgaaaagtcaggacgctgtggcattgcagcagattaaggagcgtggcgctttacctatgattgatcgtggtgatatccgtcaggcaatcgaccgttgcagcaatatctgggcttcactgccgggcgctggttatggtcagttcgagcataaggctgacagcctgattgcaaaattcaaagaagcgggcggaacggtcagagagattgatgtatgagcagagtcaccgcgattatctccgctctggttatctgcatcatcgtctgcctgtcatgggctgttaatcattaccgtgataacgccattacctacaaagcccagcgcgacaaaaatgccagagaactgaagctggcgaacgcggcaattactgacatgcagatgcgtcagcgtgatgttgctgcgctcgatgcaaaatacacgaaggagttagctgatgctaaagctgaaaatgatgctctgcgtgatgatgttgccgctggtcgtcgtcggttgcacatcaaagcagtctgtcagtcagtgcgtgaagccaccaccgcctccggcgtggataatgcagcctccccccgactggcagacaccgctgaacgggattatttcaccctcagagagaggctgatcactatgcaaaaacaactggaaggaacccagaagtatattaatgagcagtgcagatagagttgcccatatcgatgggcaactcatgcaattattgtgagcaatacacacgcgcttccagcggagtataaatgcctaaagtaataaaaccgagcaatccatttacgaatgtttgctgggtttctgttttaacaacattttctgcgccgccacaaattttggctgcatcgacagttttcttctgcccaattccagaaacgaagaaatgatgggtgatggtttcctttggtgctactgctgccggtttgttttgaacagtaaacgtctgttgagcacatcctgtaataagcagggccagcgcagtagcgagtagcatttttttcatggtgttattcccgatgctttttgaagttcgcagaatcgtatgtgtagaaaattaaacaaaccctaaacaatgagttgaaatttcatattgttaatatttattaatgtatgtcaggtgcgatgaatcgtcattgtattcccggattaactatgtccacagccctgacggggaacttctctgcgggagtgtccgggaataattaaaacgatgcacacagggtttagcgcgtacacgtattgcattatgccaacgccccggtgctgacacggaagaaaccggacgttatgatttagcgtggaaagatttgtgtagtgttctgaatgctctcagtaaatagtaatgaattatcaaaggtatagtaatatcttttatgttcatggatatttgtaacccatcggaaaactcctgctttagcaagattttccctgtattgctgaaatgtgatttctcttgatttcaacctatcataggacgtttctataagatgcgtgtttcttgagaatttaacatttacaacctttttaagtccttttattaacacggtgttatcgttttctaacacgatgtgaatattatctgtggctagatagtaaatataatgtgagacgttgtgacgttttagttcagaataaaacaattcacagtctaaatcttttcgcacttgatcgaatatttctttaaaaatggcaacctgagccattggtaaaaccttccatgtgatacgagggcgcgtagtttgcattatcgtttttatcgtttcaatctggtctgacctccttgtgttttgttgatgatttatgtcaaatattaggaatgttttcacttaatagtattggttgcgtaacaaagtgcggtcctgctggcattctggagggaaatacaaccgacagatgtatgtaaggccaacgtgctcaaatcttcatacagaaagatttgaagtaatattttaaccgctagatgaagagcaagcgcatggagcgacaaaatgaataaagaacaatctgctgatgatccctccgtggatctgattcgtgtaaaaaatatgcttaatagcaccatttctatgagttaccctgatgttgtaattgcatgtatagaacataaggtgtctctggaagcattcagagcaattgaggcagcgttggtgaagcacgataataatatgaaggattattccctggtggttgactgatcaccataactgctaatcattcaaactatttagtctgtgacagagccaacacgcagtctgtcactgtcaggaaagtggtaaaactgcaactcaattactgcaatgccctcgtaattaagtgaatttacaatatcgtcctgttcggagggaagaacgcgggatgttcattcttcatcacttttaattgatgtatatgctctcttttctgacgttagtctccgacggcaggcttcaatgacccaggctgagaaattcccggaccctttttgctcaagagcgatgttaatttgttcaatcatttggttaggaaagcggatgttgcgggttgttgttctgcgggttctgttcttcgttgacatgaggttgccccgtattcagtgtcgctgatttgtattgtctgaagttgtttttacgttaagttgatgcagatcaattaatacgatacctgcgtcataattgattatttgacgtggtttgatggcctccacgcacgttgtgatatgtagatgataatcattatcactttacgggtcctttccggtgatccgacaggttacggcctgatgcggtattttctccttacgcatctgtgcggtatttcacaccgcatacgtcaaagcaaccatagtacgcgccctgtagcggcgcattaagcgcggcgggtgtggtggttacgcgcagcgtgaccgctacacttgccagcgccctagcgcccgctcctttcgctttcttcccttcctttctcgccacgttcgccggctttccccgtcaagctctaaatcgggggctccctttagggttccgatttagtgctttacggcacctcgaccccaaaaaacttgatttgggtgatggttcacgtagtgggccatcgccctgatagacggtttttcgccctttgacgttggagtccacgttctttaatagtggactcttgttccaaactggaacaacactcaaccctatctcgggctattcttttgatttagacctgcaggcatgcaagcttactggccgtcgttttacaacgtcgtgactgggaaaaccctggcgttacccaacttaatcgccttgcagcacatccccctttcgccagctggcgtaatagcgaagaggcccgcaccgatcgcccttcccaacagttgcgcagcctgaatggcgaatgcgatttattcaacaaagccgccgtcccgtcaagtcagcgtaatgctctgccagtgttacaaccaattaaccaattctgattagaaaaactcatcgagcatcaaatgaaactgcaatttattcatatcaggattatcaataccatatttttgaaaaagccgtttctgtaatgaaggagaaaactcaccgaggcagttccataggatggcaagatcctggtatcggtctgcgattccgactcgtccaacatcaatacaacctattaatttcccctcgtcaaaaataaggttatcaagtgagaaatcaccatgagtgacgactgaatccggtgagaatggcaaaagcttatgcatttctttccagacttgttcaacaggccagccattacgctcgtcatcaaaatcactcgcatcaaccaaaccgttattcattcgtgattgcgcctgagcgagacgaaatacgcgatcgctgttaaaaggacaattacaaacaggaatcgaatgcaaccggcgcaggaacactgccagcgcatcaacaatattttcacctgaatcaggatattcttctaatacctggaatgctgttttcccggggatcgcagtggtgagtaaccatgcatcatcaggagtacggataaaatgcttgatggtcggaagaggcataaattccgtcagccagtttagtctgaccatctcatctgtaacatcattggcaacgctacctttgccatgtttcagaaacaactctggcgcatcgggcttcccatacaatcgatagattgtcgcacctgattgcccgacattatcgcgagcccatttatacccatataaatcagcatccatgttggaatttaatcgcggcttcgagcaagacgtttcccgttgaatatggctcataacaccccttgtattactgtttatgtaagcagacagttttattgttcatgatgatatatttttatcttgtgcaatgtaacatcagagattttgagacacaacgtggctttgttgaataaatcgaacttttgctgagttgaaggatcagatcacgcatcttcccgacaacgcagaccgttccgtggcaaagcaaaagttcaaaatcaccaactggtccacctacaacaaagctctcatcaaccgtggctccctcactttctggctggatgatggggcgattcaggcctggtatgagtcagcaacaccttcttcacgaggcagacctctcgacggatcgttccactgagcgtcagaccccgtagaaaagatcaaaggatcttcttgagatcctttttttctgcgcgtaatctgctgcttgcaaacaaaaaaaccaccgctaccagcggtggtttgtttgccggatcaagagctaccaactctttttccgaaggtaactggcttcagcagagcgcagataccaaatactgtccttctagtgtagccgtagttaggccaccacttcaagaactctgtagcaccgcctacatacctcgctctgctaatcctgttaccagtggctgctgccagtggcgataagtcgtgtcttaccgggttggactcaagacgatagttaccggataaggcgcagcggtcgggctgaacggggggttcgtgcacacagcccagcttggagcgaacgacctacaccgaactgagatacctacagcgtgagctatgagaaagcgccacgcttcccgaagggagaaaggcggacaggtatccggtaagcggcagggtcggaacaggagagcgcacgagggagcttccagggggaaacgcctggtatctttatagtcctgtcgggtttcgccacctctgacttgagcgtcgatttttgtgatgctcgtcaggggggcggagcctatggaaaaacgccagcaacgcggcctttttacggttcctggccttttgctggccttttgctcacatgtcctgcaggcagctgcgcgccagctgcgcgc

SEQ ID NO: 9 - DNA, 2085 bp, Artificial Sequence
  codon optimized sequence
  CDS (1)..(2085): codon-optimized ORF
atggctaagattaacacccagtactcacatccatcccgcactcacctcaaagtcaagacctccgatcgggatctgaaccgggctgagaatgggctgtcgcgcgcccactcgtcgtccgaggaaaccagcagcgtgctccagccgggcatcgccatggaaactagggggctggcggactccggacagggatccttcactggacagggtattgcccggctgagcagactgatcttcctgcttcgccgctgggcggccagacacgtgcaccatcaggaccagggacctgatagcttccccgaccgctttaggggagccgagctgaaagaagtgtcaagccaggagtcaaacgcgcaggccaacgtcggcagccaagagcctgcagaccggggacgctcggcatggccgctcgcaaagtgcaacactaacacttccaacaacaccgaagaggaaaagaaaaccaagaagaaggatgcaattgtggtggacccttcctccaacctgtactaccgctggttgaccgccatcgccctcccggtcttttacaattggtatctccttatctgccgggcctgcttcgacgaactgcaatcagagtacctgatgctgtggctggtgctggactatagcgccgatgtgctctacgtcctggatgtgctcgtgcgcgcccggaccggattcttggaacaaggcctgatggtgtccgacacgaatagactgtggcagcactataagaccacaacccagttcaagcttgacgtgctcagccttgtgccgactgacctggcctacctgaaagtcggaactaactacccggaagtcagattcaaccgactcctgaagttcagcaggctgttcgagttctttgaccgcaccgagactcggaccaactaccctaacatgttccggatcggaaatctggtgctctacatactgattatcatccattggaacgcctgtatctatttcgccatttcgaagttcatcggtttcggaaccgattcctgggtgtaccccaacatctcgatccccgaacacggtcgcctgtcccggaagtacatctactccctgtactggtccactctgactctgaccacgatcggggaaacccctccacccgtgaaggacgaagagtacctgttcgtggtggtggacttcctggtcggagtgttgattttcgccaccattgtgggaaacgtgggctccatgatctccaacatgaacgcgtcgagagctgagttccaagccaagatcgactccattaagcagtacatgcagttcagaaaggtcaccaaggacctggaaaccagggtcatccgctggttcgactacctgtgggccaacaaaaagactgtggacgaaaaggaagtgctgaagtcgctgccggataagctgaaggccgaaatcgccattaacgtgcaccttgacaccctgaagaaagtccggatcttccaagactgtgaagccggcctcctggtggagctcgtgctcaagctgcggcccaccgtgttcagcccgggagattacatttgcaagaagggcgatatcggcaaagagatgtacatcatcaacgagggaaagctggccgtggtcgcggacgacggcgtgacccagttcgtggtgctgtccgacggatcctacttcggtgaaatctcaatcctcaacatcaaggggtccaagtccggcaaccggagaactgccaacattcgctccatcggatacagcgacctgttttgcctgtccaaggatgacctgatggaggctctgactgagtaccctgaagcgaagaaggctttggaggaaaaggggcggcagattctgatgaaggacaatttgatcgacgaggagctcgcacgggccggcgccgaccccaaggatctcgaagagaaggtcgaacagctgggttcttcgcttgataccctgcaaacccgattcgcgcggctgctcgccgagtacaacgcgacccagatgaagatgaagcagagactgtcacagttggaatcccaagtcaagggcggaggcgacaagccgctggcggacggggaagtgcccggggacgccaccaagactgaggacaagcagcagtga

SEQ ID NO: 10 - protein, 694 aa, Artificial Sequence
  Synthetic Construct
MAKINTQYSHPSRTHLKVKTSDRDLNRAENGLSRAHSSSEETSSVLQPGIAMETRGLADSGQGSFTGQGIARLSRLIFLLRRWAARHVHHQDQGPDSFPDRFRGAELKEVSSQESNAQANVGSQEPADRGRSAWPLAKCNTNTSNNTEEEKKTKKKDAIVVDPSSNLYYRWLTAIALPVFYNWYLLICRACFDELQSEYLMLWLVLDYSADVLYVLDVLVRARTGFLEQGLMVSDTNRLWQHYKTTTQFKLDVLSLVPTDLAYLKVGTNYPEVRFNRLLKFSRLFEFFDRTETRTNYPNMFRIGNLVLYILIIIHWNACIYFAISKFIGFGTDSWVYPNISIPEHGRLSRKYIYSLYWSTLTLTTIGETPPPVKDEEYLFVVVDFLVGVLIFATIVGNVGSMISNMNASRAEFQAKIDSIKQYMQFRKVTKDLETRVIRWFDYLWANKKTVDEKEVLKSLPDKLKAEIAINVHLDTLKKVRIFQDCEAGLLVELVLKLRPTVFSPGDYICKKGDIGKEMYIINEGKLAVVADDGVTQFVVLSDGSYFGEISILNIKGSKSGNRRTANIRSIGYSDLFCLSKDDLMEALTEYPEAKKALEEKGRQILMKDNLIDEELARAGADPKDLEEKVEQLGSSLDTLQTRFARLLAEYNATQMKMKQRLSQLESQVKGGGDKPLADGEVPGDATKTEDKQQ

SEQ ID NO: 11 - DNA, 2250 bp, Artificial Sequence
  codon optimized sequence
  CDS (1)..(2250): codon-optimized ORF
atggctaagattaacacccagtactcacatccatcccgcactcacctcaaagtcaagacctccgatcgggatctgaaccgggctgagaatgggctgtcgcgcgcccactcgtcgtccgaggaaaccagcagcgtgctccagccgggcatcgccatggaaactagggggctggcggactccggacagggatccttcactggacagggtattgcccggttcgggcggattcagaagaagtcccagccggagaaggtcgtgcgggctgccagcaggggcaggccactcattggttggacacagtggtgcgctgaggatggtggagatgaatcggaaatggcactggccggctctcccggatgcagctcgggcccccaagggagactgagcagactgatcttcctgcttcgccgctgggcggccagacacgtgcaccatcaggaccagggacctgatagcttccccgaccgctttaggggagccgagctgaaagaagtgtcaagccaggagtcaaacgcgcaggccaacgtcggcagccaagagcctgcagaccggggacgctcggcatggccgctcgcaaagtgcaacactaacacttccaacaacaccgaagaggaaaagaaaaccaagaagaaggatgcaattgtggtggacccttcctccaacctgtactaccgctggttgaccgccatcgccctcccggtcttttacaattggtatctccttatctgccgggcctgcttcgacgaactgcaatcagagtacctgatgctgtggctggtgctggactatagcgccgatgtgctctacgtcctggatgtgctcgtgcgcgcccggaccggattcttggaacaaggcctgatggtgtccgacacgaatagactgtggcagcactataagaccacaacccagttcaagcttgacgtgctcagccttgtgccgactgacctggcctacctgaaagtcggaactaactacccggaagtcagattcaaccgactcctgaagttcagcaggctgttcgagttctttgaccgcaccgagactcggaccaactaccctaacatgttccggatcggaaatctggtgctctacatactgattatcatccattggaacgcctgtatctatttcgccatttcgaagttcatcggtttcggaaccgattcctgggtgtaccccaacatctcgatccccgaacacggtcgcctgtcccggaagtacatctactccctgtactggtccactctgactctgaccacgatcggggaaacccctccacccgtgaaggacgaagagtacctgttcgtggtggtggacttcctggtcggagtgttgattttcgccaccattgtgggaaacgtgggctccatgatctccaacatgaacgcgtcgagagctgagttccaagccaagatcgactccattaagcagtacatgcagttcagaaaggtcaccaaggacctggaaaccagggtcatccgctggttcgactacctgtgggccaacaaaaagactgtggacgaaaaggaagtgctgaagtcgctgccggataagctgaaggccgaaatcgccattaacgtgcaccttgacaccctgaagaaagtccggatcttccaagactgtgaagccggcctcctggtggagctcgtgctcaagctgcggcccaccgtgttcagcccgggagattacatttgcaagaagggcgatatcggcaaagagatgtacatcatcaacgagggaaagctggccgtggtcgcggacgacggcgtgacccagttcgtggtgctgtccgacggatcctacttcggtgaaatctcaatcctcaacatcaaggggtccaagtccggcaaccggagaactgccaacattcgctccatcggatacagcgacctgttttgcctgtccaaggatgacctgatggaggctctgactgagtaccctgaagcgaagaaggctttggaggaaaaggggcggcagattctgatgaaggacaatttgatcgacgaggagctcgcacgggccggcgccgaccccaaggatctcgaagagaaggtcgaacagctgggttcttcgcttgataccctgcaaacccgattcgcgcggctgctcgccgagtacaacgcgacccagatgaagatgaagcagagactgtcacagttggaatcccaagtcaagggcggaggcgacaagccgctggcggacggggaagtgcccggggacgccaccaagactgaggacaagcagcagtga

SEQ ID NO: 12 - protein, 749 aa, Artificial Sequence
  Synthetic Construct
MAKINTQYSHPSRTHLKVKTSDRDLNRAENGLSRAHSSSEETSSVLQPGIAMETRGLADSGQGSFTGQGIARFGRIQKKSQPEKVVRAASRGRPLIGWTQWCAEDGGDESEMALAGSPGCSSGPQGRLSRLIFLLRRWAARHVHHQDQGPDSFPDRFRGAELKEVSSQESNAQANVGSQEPADRGRSAWPLAKCNTNTSNNTEEEKKTKKKDAIVVDPSSNLYYRWLTAIALPVFYNWYLLICRACFDELQSEYLMLWLVLDYSADVLYVLDVLVRARTGFLEQGLMVSDTNRLWQHYKTTTQFKLDVLSLVPTDLAYLKVGTNYPEVRFNRLLKFSRLFEFFDRTETRTNYPNMFRIGNLVLYILIIIHWNACIYFAISKFIGFGTDSWVYPNISIPEHGRLSRKYIYSLYWSTLTLTTIGETPPPVKDEEYLFVVVDFLVGVLIFATIVGNVGSMISNMNASRAEFQAKIDSIKQYMQFRKVTKDLETRVIRWFDYLWANKKTVDEKEVLKSLPDKLKAEIAINVHLDTLKKVRIFQDCEAGLLVELVLKLRPTVFSPGDYICKKGDIGKEMYIINEGKLAVVADDGVTQFVVLSDGSYFGEISILNIKGSKSGNRRTANIRSIGYSDLFCLSKDDLMEALTEYPEAKKALEEKGRQILMKDNLIDEELARAGADPKDLEEKVEQLGSSLDTLQTRFARLLAEYNATQMKMKQRLSQLESQVKGGGDKPLADGEVPGDATKTEDKQQ

SEQ ID NO: 13 - DNA, 2085 bp, Homo sapiens
  CDS (1)..(2085): native open reading frame (ORF)
atggccaagatcaacacccaatactcccacccctccaggacccacctcaaggtaaagacctcagaccgggatctcaatcgcgctgaaaatggcctcagcagagcccactcgtcaagtgaggagacatcgtcagtgctgcagccggggatcgccatggagaccagaggactggctgactccgggcagggctccttcaccggccaggggatcgccaggctgtcgcgcctcatcttcttgctgcgcaggtgggctgccaggcatgtgcaccaccaggaccagggaccggactcttttcctgatcgtttccgtggagccgagcttaaggaggtgtccagccaagaaagcaatgcccaggcaaatgtgggcagccaggagccagcagacagagggagaagcgcctggcccctggccaaatgcaacactaacaccagcaacaacacggaggaggagaagaagacgaaaaagaaggatgcgatcgtggtggacccgtccagcaacctgtactaccgctggctgaccgccatcgccctgcctgtcttctataactggtatctgcttatttgcagggcctgtttcgatgagctgcagtccgagtacctgatgctgtggctggtcctggactactcggcagatgtcctgtatgtcttggatgtgcttgtacgagctcggacaggttttcttgagcaaggcttaatggtcagtgataccaacaggctgtggcagcattacaagacgaccacgcagttcaagctggatgtgttgtccctggtccccaccgacctggcttacttaaaggtgggcacaaactacccagaagtgaggttcaaccgcctactgaagttttcccggctctttgaattctttgaccgcacagagacaaggaccaactaccccaatatgttcaggattgggaacttggtcttgtacattctcatcatcatccactggaatgcctgcatctactttgccatttccaagttcattggttttgggacagactcctgggtctacccaaacatctcaatcccagagcatgggcgcctctccaggaagtacatttacagtctctactggtccaccttgacccttaccaccattggtgagaccccaccccccgtgaaagatgaggagtatctctttgtggtcgtagacttcttggtgggtgttctgatttttgccaccattgtgggcaatgtgggctccatgatctcgaatatgaatgcctcacgggcagagttccaggccaagattgattccatcaagcagtacatgcagttccgcaaggtcaccaaggacttggagacgcgggttatccggtggtttgactacctgtgggccaacaagaagacggtggatgagaaggaggtgctcaagagcctcccagacaagctgaaggctgagatcgccatcaacgtgcacctggacacgctgaagaaggttcgcatcttccaggactgtgaggcagggctgctggtggagctggtgctgaagctgcgacccactgtgttcagccctggggattatatctgcaagaagggagatattgggaaggagatgtacatcatcaacgagggcaagctggccgtggtggctgatgatggggtcacccagttcgtggtcctcagcgatggcagctacttcggggagatcagcattctgaacatcaaggggagcaagtcggggaaccgcaggacggccaacatccgcagcattggctactcagacctgttctgcctctcaaaggacgatctcatggaggccctcaccgagtaccccgaagccaagaaggccctggaggagaaaggacggcagatcctgatgaaagacaacctgatcgatgaggagctggccagggcgggcgcggaccccaaggaccttgaggagaaagtggagcagctggggtcctccctggacaccctgcagaccaggtttgcacgcctcctggctgagtacaacgccacccagatgaagatgaagcagcgtctcagccaactggaaagccaggtgaagggtggtggggacaagcccctggctgatggggaagttcccggggatgctacaaaaacagaggacaaacaacagtga

SEQ ID NO: 14 - protein, 694 aa, Homo sapiens; identical to SEQ ID NO: 10

SEQ ID NO: 15 - DNA, 2085 bp, Homo sapiens
atggccaagatcaacacccaatactcccacccctccaggacccacctcaaggtaaagacctcagaccgagatctcaatcgcgctgaaaatggcctcagcagagcccactcgtcaagtgaggagacatcgtcagtgctgcagccggggatcgccatggagaccagaggactggctgactccgggcagggctccttcaccggccaggggatcgccaggctgtcgcgcctcatcttcttgctgcgcaggtgggctgccaggcatgtgcaccaccaggaccagggaccggactcttttcctgatcgtttccgtggagccgagcttaaggaggtgtccagccaagaaagcaatgcccaggcaaatgtgggcagccaggagccagcagacagagggagaagcgcctggcccctggccaaatgcaacactaacaccagcaacaacacggaggaggagaagaagacgaaaaagaaggatgcgatcgtggtggacccgtccagcaacctgtactaccgctggctgaccgccatcgccctgcctgtcttctataactggtatctgcttatttgcagggcctgtttcgatgagctgcagtccgagtacctgatgctgtggctggtcctggactactcggcagatgtcctgtatgtcttggatgtgcttgtacgagctcggacaggttttctcgagcaaggcttaatggtcagtgataccaacaggctgtggcagcattacaagacgaccacgcagttcaagctggatgtgttgtccctggtccccaccgacctggcttacttaaaggtgggcacaaactacccagaagtgaggttcaaccgcctactgaagttttcccggctctttgaattctttgaccgcacagagacaaggaccaactaccccaatatgttcaggattgggaacttggtcttgtacattctcatcatcatccactggaatgcctgcatctactttgccatttccaagttcattggttttgggacagactcctgggtctacccaaacatctcaatcccagagcatgggcgcctctccaggaagtacatttacagtctctactggtccaccttgacccttaccaccattggtgagaccccaccccccgtgaaagatgaggagtatctctttgtggtcgtagacttcttggtgggtgttctgatttttgccaccattgtgggcaatgtgggctccatgatctcgaatatgaatgcctcacgggcagagttccaggccaagattgattccatcaagcagtacatgcagttccgcaaggtcaccaaggacttggagacgcgggttatccggtggtttgactacctgtgggccaacaagaagacggtggatgagaaggaggtgctcaagagcctcccagacaagctgaaggctgagatcgccatcaacgtgcacctggacacgctgaagaaggttcgcatcttccaggactgtgaggcagggctgctggtggagctggtgctgaagctgcgacccactgtgttcagccctggggattatatctgcaagaagggagatattgggaaggagatgtacatcatcaacgagggcaagctggccgtggtggctgatgatggggtcacccagttcgtggtcctcagcgatggcagctacttcggggagatcagcattctgaacatcaaggggagcaagtcggggaaccgcaggacggccaacatccgcagcattggctactcagacctgttctgcctctcaaaggacgatctcatggaggccctcaccgagtaccccgaagccaagaaggccctggaggagaaaggacggcagatcctgatgaaagacaacctgatcgatgaggagctggccagggcgggcgcggaccccaaggaccttgaggagaaagtggagcagctggggtcctccctggacaccctgcagaccaggtttgcacgcctcctggctgagtacaacgccacccagatgaagatgaagcagcgtctcagccaactggaaagccaggtgaagggtggtggggacaagcccctggctgatggggaagttcccggggatgctacaaaaacagaggacaaacaacagtga

SEQ ID NO: 16 - DNA, 2107 bp, Artificial Sequence
  constructed sequence
gcggccgccaccatggctaagattaacacccagtactcacatccatcccgcactcacctcaaagtcaagacctccgatcgggatctgaaccgggctgagaatgggctgtcgcgcgcccactcgtcgtccgaggaaaccagcagcgtgctccagccgggcatcgccatggaaactagggggctggcggactccggacagggatccttcactggacagggtattgcccggctgagcagactgatcttcctgcttcgccgctgggcggccagacacgtgcaccatcaggaccagggacctgatagcttccccgaccgctttaggggagccgagctgaaagaagtgtcaagccaggagtcaaacgcgcaggccaacgtcggcagccaagagcctgcagaccggggacgctcggcatggccgctcgcaaagtgcaacactaacacttccaacaacaccgaagaggaaaagaaaaccaagaagaaggatgcaattgtggtggacccttcctccaacctgtactaccgctggttgaccgccatcgccctcccggtcttttacaattggtatctccttatctgccgggcctgcttcgacgaactgcaatcagagtacctgatgctgtggctggtgctggactatagcgccgatgtgctctacgtcctggatgtgctcgtgcgcgcccggaccggattcttggaacaaggcctgatggtgtccgacacgaatagactgtggcagcactataagaccacaacccagttcaagcttgacgtgctcagccttgtgccgactgacctggcctacctgaaagtcggaactaactacccggaagtcagattcaaccgactcctgaagttcagcaggctgttcgagttctttgaccgcaccgagactcggaccaactaccctaacatgttccggatcggaaatctggtgctctacatactgattatcatccattggaacgcctgtatctatttcgccatttcgaagttcatcggtttcggaaccgattcctgggtgtaccccaacatctcgatccccgaacacggtcgcctgtcccggaagtacatctactccctgtactggtccactctgactctgaccacgatcggggaaacccctccacccgtgaaggacgaagagtacctgttcgtggtggtggacttcctggtcggagtgttgattttcgccaccattgtgggaaacgtgggctccatgatctccaacatgaacgcgtcgagagctgagttccaagccaagatcgactccattaagcagtacatgcagttcagaaaggtcaccaaggacctggaaaccagggtcatccgctggttcgactacctgtgggccaacaaaaagactgtggacgaaaaggaagtgctgaagtcgctgccggataagctgaaggccgaaatcgccattaacgtgcaccttgacaccctgaagaaagtccggatcttccaagactgtgaagccggcctcctggtggagctcgtgctcaagctgcggcccaccgtgttcagcccgggagattacatttgcaagaagggcgatatcggcaaagagatgtacatcatcaacgagggaaagctggccgtggtcgcggacgacggcgtgacccagttcgtggtgctgtccgacggatcctacttcggtgaaatctcaatcctcaacatcaaggggtccaagtccggcaaccggagaactgccaacattcgctccatcggatacagcgacctgttttgcctgtccaaggatgacctgatggaggctctgactgagtaccctgaagcgaagaaggctttggaggaaaaggggcggcagattctgatgaaggacaatttgatcgacgaggagctcgcacgggccggcgccgaccccaaggatctcgaagagaaggtcgaacagctgggttcttcgcttgataccctgcaaacccgattcgcgcggctgctcgccgagtacaacgcgacccagatgaagatgaagcagagactgtcacagttggaatcccaagtcaagggcggaggcgacaagccgctggcggacggggaagtgcccggggacgccaccaagactgaggacaagcagcagtgatcatagatct

SEQ ID NO: 17 - DNA, 2272 bp, Artificial Sequence
  constructed sequence
gcggccgccaccatggctaagattaacacccagtactcacatccatcccgcactcacctcaaagtcaagacctccgatcgggatctgaaccgggctgagaatgggctgtcgcgcgcccactcgtcgtccgaggaaaccagcagcgtgctccagccgggcatcgccatggaaactagggggctggcggactccggacagggatccttcactggacagggtattgcccggttcgggcggattcagaagaagtcccagccggagaaggtcgtgcgggctgccagcaggggcaggccactcattggttggacacagtggtgcgctgaggatggtggagatgaatcggaaatggcactggccggctctcccggatgcagctcgggcccccaagggagactgagcagactgatcttcctgcttcgccgctgggcggccagacacgtgcaccatcaggaccagggacctgatagcttccccgaccgctttaggggagccgagctgaaagaagtgtcaagccaggagtcaaacgcgcaggccaacgtcggcagccaagagcctgcagaccggggacgctcggcatggccgctcgcaaagtgcaacactaacacttccaacaacaccgaagaggaaaagaaaaccaagaagaaggatgcaattgtggtggacccttcctccaacctgtactaccgctggttgaccgccatcgccctcccggtcttttacaattggtatctccttatctgccgggcctgcttcgacgaactgcaatcagagtacctgatgctgtggctggtgctggactatagcgccgatgtgctctacgtcctggatgtgctcgtgcgcgcccggaccggattcttggaacaaggcctgatggtgtccgacacgaatagactgtggcagcactataagaccacaacccagttcaagcttgacgtgctcagccttgtgccgactgacctggcctacctgaaagtcggaactaactacccggaagtcagattcaaccgactcctgaagttcagcaggctgttcgagttctttgaccgcaccgagactcggaccaactaccctaacatgttccggatcggaaatctggtgctctacatactgattatcatccattggaacgcctgtatctatttcgccatttcgaagttcatcggtttcggaaccgattcctgggtgtaccccaacatctcgatccccgaacacggtcgcctgtcccggaagtacatctactccctgtactggtccactctgactctgaccacgatcggggaaacccctccacccgtgaaggacgaagagtacctgttcgtggtggtggacttcctggtcggagtgttgattttcgccaccattgtgggaaacgtgggctccatgatctccaacatgaacgcgtcgagagctgagttccaagccaagatcgactccattaagcagtacatgcagttcagaaaggtcaccaaggacctggaaaccagggtcatccgctggttcgactacctgtgggccaacaaaaagactgtggacgaaaaggaagtgctgaagtcgctgccggataagctgaaggccgaaatcgccattaacgtgcaccttgacaccctgaagaaagtccggatcttccaagactgtgaagccggcctcctggtggagctcgtgctcaagctgcggcccaccgtgttcagcccgggagattacatttgcaagaagggcgatatcggcaaagagatgtacatcatcaacgagggaaagctggccgtggtcgcggacgacggcgtgacccagttcgtggtgctgtccgacggatcctacttcggtgaaatctcaatcctcaacatcaaggggtccaagtccggcaaccggagaactgccaacattcgctccatcggatacagcgacctgttttgcctgtccaaggatgacctgatggaggctctgactgagtaccctgaagcgaagaaggctttggaggaaaaggggcggcagattctgatgaaggacaatttgatcgacgaggagctcgcacgggccggcgccgaccccaaggatctcgaagagaaggtcgaacagctgggttcttcgcttgataccctgcaaacccgattcgcgcggctgctcgccgagtacaacgcgacccagatgaagatgaagcagagactgtcacagttggaatcccaagtcaagggcggaggcgacaagccgctggcggacggggaagtgcccggggacgccaccaagactgaggacaagcagcagtgatcatagatct

SEQ ID NO: 18 - DNA, 2107 bp, Artificial Sequence
  constructed sequence
gcggccgccaccatggccaagatcaacacccaatactcccacccctccaggacccacctcaaggtaaagacctcagaccgggatctcaatcgcgctgaaaatggcctcagcagagcccactcgtcaagtgaggagacatcgtcagtgctgcagccggggatcgccatggagaccagaggactggctgactccgggcagggctccttcaccggccaggggatcgccaggctgtcgcgcctcatcttcttgctgcgcaggtgggctgccaggcatgtgcaccaccaggaccagggaccggactcttttcctgatcgtttccgtggagccgagcttaaggaggtgtccagccaagaaagcaatgcccaggcaaatgtgggcagccaggagccagcagacagagggagaagcgcctggcccctggccaaatgcaacactaacaccagcaacaacacggaggaggagaagaagacgaaaaagaaggatgcgatcgtggtggacccgtccagcaacctgtactaccgctggctgaccgccatcgccctgcctgtcttctataactggtatctgcttatttgcagggcctgtttcgatgagctgcagtccgagtacctgatgctgtggctggtcctggactactcggcagatgtcctgtatgtcttggatgtgcttgtacgagctcggacaggttttcttgagcaaggcttaatggtcagtgataccaacaggctgtggcagcattacaagacgaccacgcagttcaagctggatgtgttgtccctggtccccaccgacctggcttacttaaaggtgggcacaaactacccagaagtgaggttcaaccgcctactgaagttttcccggctctttgaattctttgaccgcacagagacaaggaccaactaccccaatatgttcaggattgggaacttggtcttgtacattctcatcatcatccactggaatgcctgcatctactttgccatttccaagttcattggttttgggacagactcctgggtctacccaaacatctcaatcccagagcatgggcgcctctccaggaagtacatttacagtctctactggtccaccttgacccttaccaccattggtgagaccccaccccccgtgaaagatgaggagtatctctttgtggtcgtagacttcttggtgggtgttctgatttttgccaccattgtgggcaatgtgggctccatgatctcgaatatgaatgcctcacgggcagagttccaggccaagattgattccatcaagcagtacatgcagttccgcaaggtcaccaaggacttggagacgcgggttatccggtggtttgactacctgtgggccaacaagaagacggtggatgagaaggaggtgctcaagagcctcccagacaagctgaaggctgagatcgccatcaacgtgcacctggacacgctgaagaaggttcgcatcttccaggactgtgaggcagggctgctggtggagctggtgctgaagctgcgacccactgtgttcagccctggggattatatctgcaagaagggagatattgggaaggagatgtacatcatcaacgagggcaagctggccgtggtggctgatgatggggtcacccagttcgtggtcctcagcgatggcagctacttcggggagatcagcattctgaacatcaaggggagcaagtcggggaaccgcaggacggccaacatccgcagcattggctactcagacctgttctgcctctcaaaggacgatctcatggaggccctcaccgagtaccccgaagccaagaaggccctggaggagaaaggacggcagatcctgatgaaagacaacctgatcgatgaggagctggccagggcgggcgcggaccccaaggaccttgaggagaaagtggagcagctggggtcctccctggacaccctgcagaccaggtttgcacgcctcctggctgagtacaacgccacccagatgaagatgaagcagcgtctcagccaactggaaagccaggtgaagggtggtggggacaagcccctggctgatggggaagttcccggggatgctacaaaaacagaggacaaacaacagtgatcatagatct

SEQ ID NO: 19 - DNA, 2430 bp, Homo sapiens
  CDS (1)..(2430)
atgtttaaatcgctgacaaaagtcaacaaggtgaagcctataggagagaacaatgagaatgaacaaagttctcgtcggaatgaagaaggctctcacccaagtaatcagtctcagcaaaccacagcacaggaagaaaacaaaggtgaagagaaatctctcaaaaccaagtcaactccagtcacgtctgaagagccacacaccaacatacaagacaaactctccaagaaaaattcctctggagatctgaccacaaaccctgaccctcaaaatgcagcagaaccaactggaacagtgccagagcagaaggaaatggaccccgggaaagaaggtccaaacagcccacaaaacaaaccgcctgcagctcctgttataaatgagtatgccgatgcccagctacacaacctggtgaaaagaatgcgtcaaagaacagccctctacaagaaaaagttggtagagggagatctctcctcacccgaagccagcccacaaactgcaaagcccacggctgtaccaccagtaaaagaaagcgatgataagccaacagaacattactacaggctgttgtggttcaaagtcaaaaagatgcctttaacagagtacttaaagcgaattaaacttccaaacagcatagattcatacacagatcgactctatctcctgtggctcttgcttgtcactcttgcctataactggaactgctgttttataccactgcgcctcgtcttcccatatcaaaccgcagacaacatacactactggcttattgcggacatcatatgtgatatcatctacctttatgatatgctatttatccagcccagactccagtttgtaagaggaggagacataatagtggattcaaatgagctaaggaaacactacaggacttctacaaaatttcagttggatgtcgcatcaataataccatttgatatttgctacctcttctttgggtttaatccaatgtttagagcaaataggatgttaaagtacacttcattttttgaatttaatcatcacctagagtctataatggacaaagcatatatctacagagttattcgaacaactggatacttgctgtttattctgcacattaatgcctgtgtttattactgggcttcaaactatgaaggaattggcactactagatgggtgtatgatggggaaggaaacgagtatctgagatgttattattgggcagttcgaactttaattaccattggtggccttccagaaccacaaactttatttgaaattgtttttcaactcttgaattttttttctggagtttttgtgttctccagtttaattggtcagatgagagatgtgattggagcagctacagccaatcagaactacttccgcgcctgcatggatgacaccattgcctacatgaacaattactccattcctaaacttgtgcaaaagcgagttcggacttggtatgaatatacatgggactctcaaagaatgctagatgagtctgatttgcttaagaccctaccaactacggtccagttagccctcgccattgatgtgaacttcagcatcatcagcaaagtcgacttgttcaagggttgtgatacacagatgatttatgacatgttgctaagattgaaatccgttctctatttgcctggtgactttgtctgcaaaaagggagaaattggcaaggaaatgtatatcatcaagcatggagaagtccaagttcttggaggccctgatggtactaaagttctggttactctgaaagctgggtcggtgtttggagaaatcagccttctagcagcaggaggaggaaaccgtcgaactgccaatgtggtggcccacgggtttgccaatcttttaactctagacaaaaagaccctccaagaaattctagtgcattatccagattctgaaaggatcctcatgaagaaagccagagtgcttttaaagcagaaggctaagaccgcagaagcaacccctccaagaaaagatcttgccctcctcttcccaccgaaagaagagacacccaaactgtttaaaactctcctaggaggcacaggaaaagcaagtcttgcaagactactcaaattgaagcgagagcaagcagctcagaagaaagaaaattctgaaggaggagaggaagaaggaaaagaaaatgaagataaacaaaaagaaaatgaagataaacaaaaagaaaatgaagataaaggaaaagaaaatgaagataaagataaaggaagagagccagaagagaagccactggacagacctgaatgtacagcaagtcctattgcagtggaggaagaaccccactcagttagaaggacagttttacccagagggacttctcgtcaatcactcattatcagcatggctccttctgctgagggcggagaagaggttcttactattgaagtcaaagaaaaggctaagcaataa

SEQ ID NO: 20 - protein, 809 aa, Homo sapiens
MFKSLTKVNKVKPIGENNENEQSSRRNEEGSHPSNQSQQTTAQEENKGEEKSLKTKSTPVTSEEPHTNIQDKLSKKNSSGDLTTNPDPQNAAEPTGTVPEQKEMDPGKEGPNSPQNKPPAAPVINEYADAQLHNLVKRMRQRTALYKKKLVEGDLSSPEASPQTAKPTAVPPVKESDDKPTEHYYRLLWFKVKKMPLTEYLKRIKLPNSIDSYTDRLYLLWLLLVTLAYNWNCCFIPLRLVFPYQTADNIHYWLIADIICDIIYLYDMLFIQPRLQFVRGGDIIVDSNELRKHYRTSTKFQLDVASIIPFDICYLFFGFNPMFRANRMLKYTSFFEFNHHLESIMDKAYIYRVIRTTGYLLFILHINACVYYWASNYEGIGTTRWVYDGEGNEYLRCYYWAVRTLITIGGLPEPQTLFEIVFQLLNFFSGVFVFSSLIGQMRDVIGAATANQNYFRACMDDTIAYMNNYSIPKLVQKRVRTWYEYTWDSQRMLDESDLLKTLPTTVQLALAIDVNFSIISKVDLFKGCDTQMIYDMLLRLKSVLYLPGDFVCKKGEIGKEMYIIKHGEVQVLGGPDGTKVLVTLKAGSVFGEISLLAAGGGNRRTANVVAHGFANLLTLDKKTLQEILVHYPDSERILMKKARVLLKQKAKTAEATPPRKDLALLFPPKEETPKLFKTLLGGTGKASLARLLKLKREQAAQKKENSEGGEEEGKENEDKQKENEDKQKENEDKGKENEDKDKGREPEEKPLDRPECTASPIAVEEEPHSVRRTVLPRGTSRQSLIISMAPSAEGGEEVLTIEVKEKAKQ

SEQ ID NO: 21 - DNA, 2430 bp, Artificial Sequence
  constructed sequence
  CDS (1)..(2430)
atgtttaaatcgctgacaaaagtcaacaaggtgaagcctataggagagaacaatgagaatgaacaaagttctcgtcggaatgaagaaggctctcacccaagtaatcagtctcagcaaaccacagcacaggaagaaaacaaaggtgaagagaaatctctcaaaaccaagtcaactccagtcacgtctgaagagccacacaccaacatacaagacaaactctccaagaaaaattcctctggagatctgaccacaaaccctgaccctcaaaatgcagcagaaccaactggaacagtgccagagcagaaggaaatggaccccgggaaagaaggtccaaacagcccacaaaacaaaccgccagcagctcctgttataaatgagtatgccgatgcccagctacacaacctggtgaaaagaatgcgtcaaagaacagccctctacaagaaaaagttggtagagggagatctctcctcacccgaagccagcccacaaactgcaaagcccacggctgtaccaccagtaaaagaaagcgatgataagccaacagaacattactacaggctgttgtggttcaaagtcaaaaagatgcctttaacagagtacttaaagcgaattaaacttccaaacagcatagattcatacacagatcgactctatctcctgtggctcttgcttgtcactcttgcctataactggaactgctgttttataccactgcgcctcgtcttcccatatcaaaccgcagacaacatacactactggcttattgcggacatcatctgtgatatcatctacctttatgatatgctatttatccagcccagactccagtttgtaagaggaggagacataatagtggattcaaatgagctaaggaaacactacaggacttctacaaaatttcagttggatgtcgcatcaataataccatttgatatttgctacctcttctttgggtttaatccaatgtttagagcaaataggatgttaaagtacacttcattttttgaatttaatcatcacctagagtctataatggacaaagcatatatctacagagttattcgaacaactggatacttgctgtttattctgcacattaatgcctgtgtttattactgggcttcaaactatgaaggaattggcactactagatgggtgtatgatggggaaggaaacgagtatctgagatgttattattgggcagttcgaactttaattaccattggtggccttccagaaccacaaactttatttgaaattgtttttcaactcttgaattttttttctggagtttttgtgttctccagtttaattggtcagatgagagatgtgattggagcagctacagccaatcagaactacttccgcgcctgcatggatgacaccattgcctacatgaacaattactccattcctaaacttgtgcaaaagcgagttcggacttggtatgaatatacatgggactctcaaagaatgctagatgagtctgatttgcttaagaccctaccaactacggtccagttagccctcgccattgatgtgaacttcagcatcatcagcaaagttgacttgttcaagggttgtgatacacagatgatttatgacatgttgctaagattgaaatccgttctctatttgcctggtgactttgtctgcaaaaagggagaaattggcaaggaaatgtatatcatcaagcatggagaagtccaagttcttggaggccctgatggtactaaagttctggttactctgaaagctgggtcggtgtttggagaaatcagccttctagcagcaggaggaggaaaccgtcgaactgccaatgtggtggcccacgggtttgccaatcttttaactctagacaaaaagaccctccaagaaattctagtgcattatccagattctgaaagaatcctcatgaagaaagccagagtgcttttaaagcagaaggctaagaccgcagaagcaacccctccaagaaaagatcttgccctcctcttcccaccgaaagaagagacacccaaactgtttaaaactctcctaggaggcacaggaaaagcaagtcttgcaagactactcaaattgaagcgagagcaagcagctcagaagaaagaaaattctgaaggaggagaggaagaaggaaaagaaaatgaagataaacaaaaagaaaatgaagataaacaaaaagaaaatgaagataaaggaaaagaaaatgaagataaagataaaggaagagagccagaagagaagccactggacagacctgaatgtacagcaagtcctattgcagtggaggaagaaccccactcagttagaaggacagttttacccagagggacttctcgtcaatcactcattatcagcatggctccttctgctgagggcggagaagaggttcttactattgaagtcaaagaaaaggctaagcaatga

SEQ ID NO: 22 - protein, 809 aa, Artificial Sequence; identical to SEQ ID NO: 20
  Synthetic Construct

SEQ ID NO: 23 - DNA, 2454 bp, Artificial Sequence
  constructed sequence
  misc_feature (1)..(12): modified end with NotI site and Kozak
  misc_feature (1)..(8): NotI site for subcloning
  CDS (13)..(2448): ORF with silent mutations (stop codon and restriction sites BamHI, PstI, SalI, and NdeI)
  misc_feature (2440)..(2442): modifed stop codon
  misc_feature (2440)..(2445): BclI site to facilitate addition of epitope tag
  misc_feature (2446)..(2448): additional stop codon
  misc_feature (2449)..(2454): PstI site for subcloning
gcggccgccaccatgtttaaatcgctgacaaaagtcaacaaggtgaagcctataggagagaacaatgagaatgaacaaagttctcgtcggaatgaagaaggctctcacccaagtaatcagtctcagcaaaccacagcacaggaagaaaacaaaggtgaagagaaatctctcaaaaccaagtcaactccagtcacgtctgaagagccacacaccaacatacaagacaaactctccaagaaaaattcctctggagatctgaccacaaaccctgaccctcaaaatgcagcagaaccaactggaacagtgccagagcagaaggaaatggaccccgggaaagaaggtccaaacagcccacaaaacaaaccgccagcagctcctgttataaatgagtatgccgatgcccagctacacaacctggtgaaaagaatgcgtcaaagaacagccctctacaagaaaaagttggtagagggagatctctcctcacccgaagccagcccacaaactgcaaagcccacggctgtaccaccagtaaaagaaagcgatgataagccaacagaacattactacaggctgttgtggttcaaagtcaaaaagatgcctttaacagagtacttaaagcgaattaaacttccaaacagcatagattcatacacagatcgactctatctcctgtggctcttgcttgtcactcttgcctataactggaactgctgttttataccactgcgcctcgtcttcccatatcaaaccgcagacaacatacactactggcttattgcggacatcatctgtgatatcatctacctttatgatatgctatttatccagcccagactccagtttgtaagaggaggagacataatagtggattcaaatgagctaaggaaacactacaggacttctacaaaatttcagttggatgtcgcatcaataataccatttgatatttgctacctcttctttgggtttaatccaatgtttagagcaaataggatgttaaagtacacttcattttttgaatttaatcatcacctagagtctataatggacaaagcatatatctacagagttattcgaacaactggatacttgctgtttattctgcacattaatgcctgtgtttattactgggcttcaaactatgaaggaattggcactactagatgggtgtatgatggggaaggaaacgagtatctgagatgttattattgggcagttcgaactttaattaccattggtggccttccagaaccacaaactttatttgaaattgtttttcaactcttgaattttttttctggagtttttgtgttctccagtttaattggtcagatgagagatgtgattggagcagctacagccaatcagaactacttccgcgcctgcatggatgacaccattgcctacatgaacaattactccattcctaaacttgtgcaaaagcgagttcggacttggtatgaatatacatgggactctcaaagaatgctagatgagtctgatttgcttaagaccctaccaactacggtccagttagccctcgccattgatgtgaacttcagcatcatcagcaaagttgacttgttcaagggttgtgatacacagatgatttatgacatgttgctaagattgaaatccgttctctatttgcctggtgactttgtctgcaaaaagggagaaattggcaaggaaatgtatatcatcaagcatggagaagtccaagttcttggaggccctgatggtactaaagttctggttactctgaaagctgggtcggtgtttggagaaatcagccttctagcagcaggaggaggaaaccgtcgaactgccaatgtggtggcccacgggtttgccaatcttttaactctagacaaaaagaccctccaagaaattctagtgcattatccagattctgaaagaatcctcatgaagaaagccagagtgcttttaaagcagaaggctaagaccgcagaagcaacccctccaagaaaagatcttgccctcctcttcccaccgaaagaagagacacccaaactgtttaaaactctcctaggaggcacaggaaaagcaagtcttgcaagactactcaaattgaagcgagagcaagcagctcagaagaaagaaaattctgaaggaggagaggaagaaggaaaagaaaatgaagataaacaaaaagaaaatgaagataaacaaaaagaaaatgaagataaaggaaaagaaaatgaagataaagataaaggaagagagccagaagagaagccactggacagacctgaatgtacagcaagtcctattgcagtggaggaagaaccccactcagttagaaggacagttttacccagagggacttctcgtcaatcactcattatcagcatggctccttctgctgagggcggagaagaggttcttactattgaagtcaaagaaaaggctaagcaatgatcataactgcag

SEQ ID NO: 24 - protein, 809 aa, Artificial Sequence; identical to SEQ ID NO: 20
  Synthetic Construct

SEQ ID NO: 25 - DNA, 11714 bp, Artificial Sequence
  constructed sequence
  misc_feature (1)..(130): 5' ITR
  misc_feature (241)..(544): CMV enhancer
  misc_feature (546)..(823): chicken beta-actin promoter
  misc_feature (824)..(1795): CBA exon 1 and intron
  misc_feature (1859)..(1864): kozak
  misc_feature (1865)..(3826): human codon optimized CHM (REP-1)
  misc_feature (3847)..(4054): bGH poly(A) signal
  misc_feature (4104)..(4233): 3' ITR
ctgcgcgctcgctcgctcactgaggccgcccgggcaaagcccgggcgtcgggcgacctttggtcgcccggcctcagtgagcgagcgagcgcgcagagagggagtggccaactccatcactaggggttccttgtagttaatgattaacccgccatgctacttatctacgtagcaagctagctagttattaatagtaatcaattacggggtcattagttcatagcccatatatggagttccgcgttacataacttacggtaaatggcccgcctggctgaccgcccaacgacccccgcccattgacgtcaataatgacgtatgttcccatagtaacgccaatagggactttccattgacgtcaatgggtggagtatttacggtaaactgcccacttggcagtacatcaagtgtatcatatgccaagtacgccccctattgacgtcaatgacggtaaatggcccgcctggcattatgcccagtacatgaccttatgggactttcctacttggcagtacatctacgtattagtcatcgctattaacatggtcgaggtgagccccacgttctgcttcactctccccatctcccccccctccccacccccaattttgtatttatttattttttaattattttgtgcagcgatgggggcggggggggggggggggcgcgcgccaggcggggcggggcggggcgaggggcggggcggggcgaggcggagaggtgcggcggcagccaatcagagcggcgcgctccgaaagtttccttttatggcgaggcggcggcggcggcggccctataaaaagcgaagcgcgcggcgggcggggagtcgctgcgacgctgccttcgccccgtgccccgctccgccgccgcctcgcgccgcccgccccggctctgactgaccgcgttactcccacaggtgagcgggcgggacggcccttctcctccgggctgtaattagcgcttggtttaatgacggcttgtttcttttctgtggctgcgtgaaagccttgaggggctccgggagggccctttgtgcggggggagcggctcggggggtgcgtgcgtgtgtgtgtgcgtggggagcgccgcgtgcggctccgcgctgcccggcggctgtgagcgctgcgggcgcggcgcggggctttgtgcgctccgcagtgtgcgcgaggggagcgcggccgggggcggtgccccgcggtgcggggggggctgcgaggggaacaaaggctgcgtgcggggtgtgtgcgtgggggggtgagcagggggtgtgggcgcgtcggtcgggctgcaaccccccctgcacccccctccccgagttgctgagcacggcccggcttcgggtgcggggctccgtacggggcgtggcgcggggctcgccgtgccgggcggggggtggcggcaggtgggggtgccgggcggggcggggccgcctcgggccggggagggctcgggggaggggcgcggcggcccccggagcgccggcggctgtcgaggcgcggcgagccgcagccattgccttttatggtaatcgtgcgagagggcgcagggacttcctttgtcccaaatctgtgcggagccgaaatctgggaggcgccgccgcaccccctctagcgggcgcggggcgaagcggtgcggcgccggcaggaaggaaatgggcggggagggccttcgtgcgtcgccgcgccgccgtccccttctccctctccagcctcggggctgtccgcggggggacggctgccttcgggggggacggggcagggcggggttcggcttctggcgtgtgaccggcggctctagacaattgtactaaccttcttctctttcctctcctgacaggttggtgtacactagcggccgccaccatggctgataccctgccctctgaattcgacgtgattgtgattggaaccggactccctgaatcgatcatcgccgcggcctgttcccggtccggtcggcgcgtgctgcacgtcgattcgagaagctactacggagggaattgggcctcattctccttctccggactgctctcctggctgaaggagtatcaggagaactccgacattgtctccgactcacctgtgtggcaggaccagatcctggaaaacgaggaagcaatagccctgagccggaaggacaagaccatccagcacgtggaggtgttctgttatgcctcccaagacctccatgaggacgtggaagaggctggagcgttgcagaagaatcatgccctcgtgacctccgctaactccaccgaggcagccgacagcgccttcctgccgaccgaggatgaatccctgtcaactatgtcgtgcgaaatgctgaccgaacagactccgagctccgaccccgaaaacgccctggaagtgaacggagcggaagtgaccggcgaaaaggagaaccattgcgacgacaagacttgtgtcccatccacttccgcggaggacatgtccgagaatgtgcctatcgccgaggacaccaccgaacagcccaagaagaacagaatcacgtacagccagatcatcaaggaggggcggaggtttaacatcgatctggtgtcgaagctgctgtacagccgcggtctgctgatcgatctgctcattaagtcgaacgtgtcgagatacgccgagttcaagaacatcacaaggattctcgccttccgggaaggaagagtggaacaagtgccgtgctcccgggccgacgtgttcaactcaaagcaacttaccatggtggaaaagcgcatgctgatgaaattcctgaccttctgcatggagtacgaaaagtaccctgatgagtacaagggttacgaagaaattactttctacgagtacctcaagacccagaagctgaccccgaatctgcagtacattgtgatgcactcaatcgcaatgacctccgaaaccgcctcctcgaccatcgacgggctcaaggccaccaagaacttcctgcactgtttggggcgctacggcaacactccgttcctcttcccgctgtacggccagggagagctgcctcagtgtttctgccggatgtgcgccgtgttcggcggaatctactgtctccgccactcggtccagtgcctggtggtggacaaggaatccaggaagtgcaaagccattattgaccagttcggacaacggatcatttccgagcactttcttgtggaggactcatacttcccggagaacatgtgctctcgggtccagtatcgacagatttccagggcggtgctcattactgaccggagcgtcctcaagaccgatagcgaccagcagatctccatcctgaccgtgccggcggaagaacccggcacttttgccgtgcgcgtgatcgagctttgctcatccaccatgacttgcatgaaaggcacttacctggtgcacctgacgtgcacctcatcgaaaaccgctagagaggacctggaatccgtcgtccaaaagctgttcgtgccttacaccgagatggaaattgaaaacgaacaagtggagaagccccgcatcctttgggccctgtactttaacatgcgcgattcctccgatatctcgcggtcctgctataacgacttgccttcgaacgtctacgtctgctccgggccagactgcggtcttggcaacgacaatgccgtgaagcaggcggaaacactgttccaagagatctgccctaacgaggatttttgcccgccccccccaaaccccgaggatatcatcttggacggagacagcctgcagccagaagcatccgagtccagcgccatcccggaggccaacagcgaaaccttcaaggagagcactaacctgggcaacctggaagagtccagcgaatgatcataggatctctgcctcgactgtgccttctagttgccagccatctgttgtttgcccctcccccgtgccttccttgaccctggaaggtgccactcccactgtcctttcctaataaaatgaggaaattgcatcgcattgtctgagtaggtgtcattctattctggggggtggggtggggcaggacagcaagggggaggattgggaagacaatagcaggcatgctggggactcgagttctacgtagataagtagcatggcgggttaatcattaactacaaggaacccctagtgatggagttggccactccctctctgcgcgctcgctcgctcactgaggccgggcgaccaaaggtcgcccgacgcccgggctttgcccgggcggcctcagtgagcgagcgagcgcgcagccttataaggatatggtgcactctcagtacaatctgctctgatgccgcatagttaagccagccccgacacccgccaacacccgctgacgcgccctgacgggcttgtctgctcccggcatccgcttacagacaagctgtgaccgtctccgggagctgcatgtgtcagaggttttcaccgtcatcaccgaaacgcgcgagacgaaagggcctcgtgatacgcctatttttataggttaatgtcatgataataatggtttcttagacgtcaggtggcacttttcggggaaatgtgcgcggaacccctatttgtttatttttctaaatacattcaaatatgtatccgctcatgagacaataaccctgataaatgcttcaataatattgaaaaaggaagagtatgagccatattcaacgggaaacgtcgaggccgcgattaaattccaacatggatgctgatttatatgggtataaatgggctcgcgataatgtcgggcaatcaggtgcgacaatctatcgcttgtatgggaagcccgatgcgccagagttgtttctgaaacatggcaaaggtagcgttgccaatgatgttacagatgagatggtcagactaaactggctgacggaatttatgccacttccgaccatcaagcattttatccgtactcctgatgatgcatggttactcaccactgcgatccccggaaaaacagcgttccaggtattagaagaatatcctgattcaggtgaaaatattgttgatgcgctggcagtgttcctgcgccggttgcactcgattcctgtttgtaattgtccttttaacagcgatcgcgtatttcgcctcgctcaggcgcaatcacgaatgaataacggtttggttgatgcgagtgattttgatgacgagcgtaatggctggcctgttgaacaagtctggaaagaaatgcataaacttttgccattctcaccggattcagtcgtcactcatggtgatttctcacttgataaccttatttttgacgaggggaaattaataggttgtattgatgttggacgagtcggaatcgcagaccgataccaggatcttgccatcctatggaactgcctcggtgagttttctccttcattacagaaacggctttttcaaaaatatggtattgataatcctgatatgaataaattgcagtttcatttgatgctcgatgagtttttctaaactgtcagaccaagtttactcatatatactttagattgatttaaaacttcatttttaatttaaaaggatctaggtgaagatcctttttgataatctcatgaccaaaatcccttaacgtgagttttcgttccactgagcgtcagaccccgtagaaaagatcaaaggatcttcttgagatcctttttttctgcgcgtaatctgctgcttgcaaacaaaaaaaccaccgctaccagcggtggtttgtttgccggatcaagagctaccaactctttttccgaaggtaactggcttcagcagagcgcagataccaaatactgttcttctagtgtagccgtagttaggccaccacttcaagaactctgtagcaccgcctacatacctcgctctgctaatcctgttaccagtggctgctgccagtggcgataagtcgtgtcttaccgggttggactcaagacgatagttaccggataaggcgcagcggtcgggctgaacggggggttcgtgcacacagcccagcttggagcgaacgacctacaccgaactgagatacctacagcgtgagctatgagaaagcgccacgcttcccgaagggagaaaggcggacaggtatccggtaagcggcagggtcggaacaggagagcgcacgagggagcttccagggggaaacgcctggtatctttatagtcctgtcgggtttcgccacctctgacttgagcgtcgatttttgtgatgctcgtcaggggggcggagcctatggaaaaacgccagcaacgcggcctttttacggttcctggccttttgctggccttttgctcacatgttctttcctgcgttatcccctgattctgtggataaccgtattaccgcctttgagtgagctgataccgctcgccgcagccgaacgaccgagcgcagcgagtcagtgagcgaggaagcggaagagcgcccaatacgcaaaccgcctctccccgcgcgttggccgattcattaatgcaggcgcctgttgatttgagttttgggtttagcgtgacaagtttgcgagggtgatcggagtaatcagtaaatagctctccgcctacaatgacgtcataaccatgatttctggttttctgacgtccgttatcagttccctccgaccacgccagcatatcgaggaacgccttacgttgattattgatttctaccatcttctactccggcttttttagcagcgaagcgtttgataagcgaaccaatcgagtcagtaccgatgtagccgataaacacgctcgttatataagcgagattgctacttagtccggcgaagtcgagaaggtcacgaatgaaccaggcgataatggcgcacatcgttgcgtcgattactgtttttgtaaacgcaccgccattatatctgccgcgaaggtacgccattgcaaacgcaaggattgccccgatgccttgttcctttgccgcgagaatggcggccaacaggtcatgtttttctggcatcttcatgtcttacccccaataaggggatttgctctatttaattaggaataaggtcgattactgatagaacaaatccaggctactgtgtttagtaatcagatttgttcgtgaccgatatgcacgggcaaaacggcaggaggttgttagcgcgacctcctgccacccgctttcacgaaggtcatgtgtaaaaggccgcagcgtaactattactaatgaattcaggacagacagtggctacggctcagtttgggttgtgctgttgctgggcggcgatgacgcctgtacgcatttggtgatccggttctgcttccggtattcgcttaattcagcacaacggaaagagcactggctaaccaggctcgccgactcttcacgattatcgactcaatgctcttacctgttgtgcagatataaaaaatcccgaaaccgttatgcaggctctaactattacctgcgaactgtttcgggattgcattttgcagacctctctgcctgcgatggttggagttccagacgatacgtcgaagtgaccaactaggcggaatcggtagtaagcgccgcctcttttcatctcactaccacaacgagcgaattaacccatcgttgagtcaaatttacccaattttattcaataagtcaatatcatgccgttaatatgttgccatccgtggcaatcatgctgctaacgtgtgaccgcattcaaaatgttgtctgcgattgactcttctttgtggcattgcaccaccagagcgtcatacagcggcttaacagtgcgtgaccaggtgggttgggtaaggtttgggattagcatcgtcacagcgcgatatgctgcgcttgctggcatccttgaatagccgacgcctttgcatcttccgcactctttctcgacaactctcccccacagctctgttttggcaatatcaaccgcacggcctgtaccatggcaatctctgcatcttgcccccggcgtcgcggcactacggcaataatccgcataagcgaatgttgcgagcacttgcagtacctttgccttagtatttccttcaagctttgccacaccacggtatttccccgataccttgtgtgcaaattgcatcagatagttgatagccttttgtttgtcgttctggctgagttcgtgcttaccgcagaatgcagccataccgaatccggcttgtgattgcgccatccccatagcagccatcacatcagtaccggaaagagagtcagaagccgtggcccgtggtgagtcgctcatcatcgggctttttggcgaatgaaatttagctacgctttcgagtctcatgcgccttctccctgtacctgaatcaatgttaggtttccgcagaacactgcgccggtatcgatatacatttggttggcaaacttgagtggtttcactgctggcgtatgaccaaagatgaacgtgtccgcgcctttgatttctttcacgatcccgttttgtgagttgctgattcgttcgcggttccagattacctgctgatgatcaactggctttccaaactcgtattcgtcaaagggataatcggcgtggcagataacatattttttatctttgctcaccagttcgatgattaacggaagttcatctgctttatgggcaagagctttagccagaatttctttgtcgtaatcgagattaaagaaccagccaccgccattaagcagccagtgattaacgtttccacgctctgataagccatcaatcatcatttgctcatggtttccacgtacagctctgaaccaggggaatgtgattaattccaggcattcaacgttctctgcaccacgatcaaccaaatcgcccaccgagataagcaggtcttttttgttgtcgaatccaatcgtatccagtttgttcatcaggttcgtgtagcatccgtgcagatcgccaactacccaaatatttcggtatttgctgccatcaattttttcgtaatagcgcatctctttcactccatccgcgatgaaccatgagaacgtcgttgacgatggcgtgcattttcccgtctttatcatcaacgtattttctgaccgtaccgcgactacatttcagtctgcgtgctacttctgtctgatttccgtatgcttcaacgagcatgtctggaatggtttttactgagaacgtcatgcggcctcacttctgctatttcgcaggtctttgagtttctgttggtactctgccttgatcgccttgcactcttcgatagtccagcgatggcggttatggtttgattcgatttcgtctactgcttcctgcccgatgcggctaatcagttcgacgcgatacggaacgagatttccgcttttgtgctggttgcacaccacgcattgcttgtgaatattgcgttcattaaatcggagttgaggtgccgcagcagttgtccggtaatgtccggcatcccactgagcagacgtgagcgttccgcacgagatacatggtaagtcgcggtctctttctctgatgaaggcgtttacggcttgttgggcttgtttaatccagtaactgcggggctttaaggcgagttttcgaatcttaagtttatctttctgtttctgctcctctcgtcgtcgtttcttctctgctgctttttccgctttttcgcgttctttacttcgtcgttcgagtgctatcttggttccacactctggagagcaccaccactgattagcgaatgcagggtgaaaccattcccggcattcatcgtttttacatcgtcttcgcgctggtttagccatcatcttcttcctcgtgcatcgagctattcggatcgctcatcagttctgcgcagcagtgctcacacacgtgaacttccagcacatgcagcttctgaccgcagttagcgcacgttaaagctcgctcgacgctttcttgttcgtaacttcgattttggtcaatcaccttgttttcctcgcacgacgtcttagccaccggatatcccacaggtgagccgtgtagttgaaggtttttacgtcagattcttttgggattggcttgggtttatttctggtgcgtttcgttggaaggtatttgcagttttcgcagattatgtcggtgatacttcgtcgctgtctcgccacacgtcctccttttcctgcggtagtggtaacacccctgttggtgttctttcacaccggagacaccatcgattccagtaaggttgatttggtcggaagcggttatcttctttgcattcaccgcaccgataacatcgcatcatgcagcttccctcccgaagtcgaaatcaagctgccctccaaatatttcgcatgactcagaacaagagccggtatcgaatcttttagctcgtaccatgtcctgatacagggcttgataatcattttctgaatacattttcgcgataccgtccagcgacattcttcctcggtacataatctcctttggcgtttcccgatgtccgtcacgcacatgggatcccgtgatgacctcattaaaaacacgctgcaatccctcctcatctttgcaggcaagtccgattttttgcgttgattttttaatgcagaatatgcagttaccgagatgttccggtatttgcaaatcgaatggttgttgcttccaccatgcgaggatatcttccttctcaaagtctgacagttcagcaagatatctgattccaggctttggctttagccgcttcggttcatcagctctgatgccaatccacgtggtgtaattccctcgcccgaaatggtcatcacagtatttggtgaagggaacgagttttaatctgtcagtgcagaacgcgccgccgacgtatggagtgccatatttctttaccatatcgataaatggcttcagaacaggcattcgcgtctgaatatcctttggttcccataccgtataaccatttggctgtccaagctccgggttgatatcaacctgcaatacggtgagcggtatatcccagaacttcacaacttccctgacaaaccgatatgtcattggatgttcacaacctgtatccatgaaaacgtaatgcacgtctttacctgcccgtcgcttttgctccattagccagagcaaatatgctgacgtcctgccaccggagaaactaacgacatttatcatgcagccctgtctccccatctcgctttccactccagagccagtctcgcttcgtctgaccacttaacgccacgctctgtaccgaatgcctgtataagctctaatagctccgcaaattcgcctacacgcatcctgctggttgactggcctattaccacaaagccattcccggcaaggttaggaacaacatcctgctgctttaatgctgcggtaaacacacacttccagctttctgcatccagccagcgaccatgccattcaacctgacgagagacgtcacctaagcaggcccatagcttcctgttttggtctaagctgcggttgcgttcctgaatggttactacgattggtttggttgggtctggaaggatttgctgtactgcgtgaatagcgttttgctgatgtgctggagatcgaatttcaaaggttagttttttcatgacttccctctcccccaaataaaaaggctggcacgacaggtttcccgactggaaagcgggcagtgagcgcaacgcaattaatgtgagttagctcactcattaggcaccccaggctttacactttatgcttccggctcgtatgttgtgtggaattgtgagcggataacaatttcacacaggaaacagctatgaccatgattacgccaagctgtcgactctagaggatcccctaataagg

SEQ ID NO: 26 - DNA, 6647 bp, Artificial Sequence
  constructed sequence
  misc_feature (1)..(130): 5' ITR
  misc_feature (241)..(544): CMV enhancer
  misc_feature (546)..(823): chicken beta-actin promoter
  misc_feature (824)..(1795): CBA exon 1 and intron
  misc_feature (1859)..(1864): Kozak
  misc_feature (1865)..(3826): human codon optimized CHM (REM-1)
  misc_feature (3847)..(4054): bGH poly(A) signal
  misc_feature (4104)..(4233): 3' ITR
ctgcgcgctcgctcgctcactgaggccgcccgggcaaagcccgggcgtcgggcgacctttggtcgcccggcctcagtgagcgagcgagcgcgcagagagggagtggccaactccatcactaggggttccttgtagttaatgattaacccgccatgctacttatctacgtagcaagctagctagttattaatagtaatcaattacggggtcattagttcatagcccatatatggagttccgcgttacataacttacggtaaatggcccgcctggctgaccgcccaacgacccccgcccattgacgtcaataatgacgtatgttcccatagtaacgccaatagggactttccattgacgtcaatgggtggagtatttacggtaaactgcccacttggcagtacatcaagtgtatcatatgccaagtacgccccctattgacgtcaatgacggtaaatggcccgcctggcattatgcccagtacatgaccttatgggactttcctacttggcagtacatctacgtattagtcatcgctattaacatggtcgaggtgagccccacgttctgcttcactctccccatctcccccccctccccacccccaattttgtatttatttattttttaattattttgtgcagcgatgggggcggggggggggggggggcgcgcgccaggcggggcggggcggggcgaggggcggggcggggcgaggcggagaggtgcggcggcagccaatcagagcggcgcgctccgaaagtttccttttatggcgaggcggcggcggcggcggccctataaaaagcgaagcgcgcggcgggcggggagtcgctgcgacgctgccttcgccccgtgccccgctccgccgccgcctcgcgccgcccgccccggctctgactgaccgcgttactcccacaggtgagcgggcgggacggcccttctcctccgggctgtaattagcgcttggtttaatgacggcttgtttcttttctgtggctgcgtgaaagccttgaggggctccgggagggccctttgtgcggggggagcggctcggggggtgcgtgcgtgtgtgtgtgcgtggggagcgccgcgtgcggctccgcgctgcccggcggctgtgagcgctgcgggcgcggcgcggggctttgtgcgctccgcagtgtgcgcgaggggagcgcggccgggggcggtgccccgcggtgcggggggggctgcgaggggaacaaaggctgcgtgcggggtgtgtgcgtgggggggtgagcagggggtgtgggcgcgtcggtcgggctgcaaccccccctgcacccccctccccgagttgctgagcacggcccggcttcgggtgcggggctccgtacggggcgtggcgcggggctcgccgtgccgggcggggggtggcggcaggtgggggtgccgggcggggcggggccgcctcgggccggggagggctcgggggaggggcgcggcggcccccggagcgccggcggctgtcgaggcgcggcgagccgcagccattgccttttatggtaatcgtgcgagagggcgcagggacttcctttgtcccaaatctgtgcggagccgaaatctgggaggcgccgccgcaccccctctagcgggcgcggggcgaagcggtgcggcgccggcaggaaggaaatgggcggggagggccttcgtgcgtcgccgcgccgccgtccccttctccctctccagcctcggggctgtccgcggggggacggctgccttcgggggggacggggcagggcggggttcggcttctggcgtgtgaccggcggctctagacaattgtactaaccttcttctctttcctctcctgacaggttggtgtacactagcggccgccaccatggctgataccctgccctctgaattcgacgtgattgtgattggaaccggactccctgaatcgatcatcgccgcggcctgttcccggtccggtcggcgcgtgctgcacgtcgattcgagaagctactacggagggaattgggcctcattctccttctccggactgctctcctggctgaaggagtatcaggagaactccgacattgtctccgactcacctgtgtggcaggaccagatcctggaaaacgaggaagcaatagccctgagccggaaggacaagaccatccagcacgtggaggtgttctgttatgcctcccaagacctccatgaggacgtggaagaggctggagcgttgcagaagaatcatgccctcgtgacctccgctaactccaccgaggcagccgacagcgccttcctgccgaccgaggatgaatccctgtcaactatgtcgtgcgaaatgctgaccgaacagactccgagctccgaccccgaaaacgccctggaagtgaacggagcggaagtgaccggcgaaaaggagaaccattgcgacgacaagacttgtgtcccatccacttccgcggaggacatgtccgagaatgtgcctatcgccgaggacaccaccgaacagcccaagaagaacagaatcacgtacagccagatcatcaaggaggggcggaggtttaacatcgatctggtgtcgaagctgctgtacagccgcggtctgctgatcgatctgctcattaagtcgaacgtgtcgagatacgccgagttcaagaacatcacaaggattctcgccttccgggaaggaagagtggaacaagtgccgtgctcccgggccgacgtgttcaactcaaagcaacttaccatggtggaaaagcgcatgctgatgaaattcctgaccttctgcatggagtacgaaaagtaccctgatgagtacaagggttacgaagaaattactttctacgagtacctcaagacccagaagctgaccccgaatctgcagtacattgtgatgcactcaatcgcaatgacctccgaaaccgcctcctcgaccatcgacgggctcaaggccaccaagaacttcctgcactgtttggggcgctacggcaacactccgttcctcttcccgctgtacggccagggagagctgcctcagtgtttctgccggatgtgcgccgtgttcggcggaatctactgtctccgccactcggtccagtgcctggtggtggacaaggaatccaggaagtgcaaagccattattgaccagttcggacaacggatcatttccgagcactttcttgtggaggactcatacttcccggagaacatgtgctctcgggtccagtatcgacagatttccagggcggtgctcattactgaccggagcgtcctcaagaccgatagcgaccagcagatctccatcctgaccgtgccggcggaagaacccggcacttttgccgtgcgcgtgatcgagctttgctcatccaccatgacttgcatgaaaggcacttacctggtgcacctgacgtgcacctcatcgaaaaccgctagagaggacctggaatccgtcgtccaaaagctgttcgtgccttacaccgagatggaaattgaaaacgaacaagtggagaagccccgcatcctttgggccctgtactttaacatgcgcgattcctccgatatctcgcggtcctgctataacgacttgccttcgaacgtctacgtctgctccgggccagactgcggtcttggcaacgacaatgccgtgaagcaggcggaaacactgttccaagagatctgccctaacgaggatttttgcccgccccccccaaaccccgaggatatcatcttggacggagacagcctgcagccagaagcatccgagtccagcgccatcccggaggccaacagcgaaaccttcaaggagagcactaacctgggcaacctggaagagtccagcgaatgatcataggatctctgcctcgactgtgccttctagttgccagccatctgttgtttgcccctcccccgtgccttccttgaccctggaaggtgccactcccactgtcctttcctaataaaatgaggaaattgcatcgcattgtctgagtaggtgtcattctattctggggggtggggtggggcaggacagcaagggggaggattgggaagacaatagcaggcatgctggggactcgagttctacgtagataagtagcatggcgggttaatcattaactacaaggaacccctagtgatggagttggccactccctctctgcgcgctcgctcgctcactgaggccgggcgaccaaaggtcgcccgacgcccgggctttgcccgggcggcctcagtgagcgagcgagcgcgcagccttataaggatatggtgcactctcagtacaatctgctctgatgccgcatagttaagccagccccgacacccgccaacacccgctgacgcgccctgacgggcttgtctgctcccggcatccgcttacagacaagctgtgaccgtctccgggagctgcatgtgtcagaggttttcaccgtcatcaccgaaacgcgcgagacgaaagggcctcgtgatacgcctatttttataggttaatgtcatgataataatggtttcttagacgtcaggtggcacttttcggggaaatgtgcgcggaacccctatttgtttatttttctaaatacattcaaatatgtatccgctcatgagacaataaccctgataaatgcttcaataatattgaaaaaggaagagtatgagccatattcaacgggaaacgtcgaggccgcgattaaattccaacatggatgctgatttatatgggtataaatgggctcgcgataatgtcgggcaatcaggtgcgacaatctatcgcttgtatgggaagcccgatgcgccagagttgtttctgaaacatggcaaaggtagcgttgccaatgatgttacagatgagatggtcagactaaactggctgacggaatttatgccacttccgaccatcaagcattttatccgtactcctgatgatgcatggttactcaccactgcgatccccggaaaaacagcgttccaggtattagaagaatatcctgattcaggtgaaaatattgttgatgcgctggcagtgttcctgcgccggttgcactcgattcctgtttgtaattgtccttttaacagcgatcgcgtatttcgcctcgctcaggcgcaatcacgaatgaataacggtttggttgatgcgagtgattttgatgacgagcgtaatggctggcctgttgaacaagtctggaaagaaatgcataaacttttgccattctcaccggattcagtcgtcactcatggtgatttctcacttgataaccttatttttgacgaggggaaattaataggttgtattgatgttggacgagtcggaatcgcagaccgataccaggatcttgccatcctatggaactgcctcggtgagttttctccttcattacagaaacggctttttcaaaaatatggtattgataatcctgatatgaataaattgcagtttcatttgatgctcgatgagtttttctaaactgtcagaccaagtttactcatatatactttagattgatttaaaacttcatttttaatttaaaaggatctaggtgaagatcctttttgataatctcatgaccaaaatcccttaacgtgagttttcgttccactgagcgtcagaccccgtagaaaagatcaaaggatcttcttgagatcctttttttctgcgcgtaatctgctgcttgcaaacaaaaaaaccaccgctaccagcggtggtttgtttgccggatcaagagctaccaactctttttccgaaggtaactggcttcagcagagcgcagataccaaatactgttcttctagtgtagccgtagttaggccaccacttcaagaactctgtagcaccgcctacatacctcgctctgctaatcctgttaccagtggctgctgccagtggcgataagtcgtgtcttaccgggttggactcaagacgatagttaccggataaggcgcagcggtcgggctgaacggggggttcgtgcacacagcccagcttggagcgaacgacctacaccgaactgagatacctacagcgtgagctatgagaaagcgccacgcttcccgaagggagaaaggcggacaggtatccggtaagcggcagggtcggaacaggagagcgcacgagggagcttccagggggaaacgcctggtatctttatagtcctgtcgggtttcgccacctctgacttgagcgtcgatttttgtgatgctcgtcaggggggcggagcctatggaaaaacgccagcaacgcggcctttttacggttcctggccttttgctggccttttgctcacatgttctttcctgcgttatcccctgattctgtggataaccgtattaccgcctttgagtgagctgataccgctcgccgcagccgaacgaccgagcgcagcgagtcagtgagcgaggaagcggaagagcgcccaatacgcaaaccgcctctccccgcgcgttggccgattcattaatgcagctggcacgacaggtttcccgactggaaagcgggcagtgagcgcaacgcaattaatgtgagttagctcactcattaggcaccccaggctttacactttatgcttccggctcgtatgttgtgtggaattgtgagcggataacaatttcacacaggaaacagctatgaccatgattacgccaagctgtcgactctagaggatcccctaataagg

SEQ ID NO: 27 - DNA, 11971 bp, Artificial Sequence
  constructed sequence
  misc_feature (1)..(130): 5' ITR
  misc_feature (241)..(544): CMV Enhancer
  misc_feature (546)..(823): chicken beta-actin promoter
  misc_feature (824)..(1795): CBA exon 1 and intron
  misc_feature (1859)..(1864): kozak
  misc_feature (1865)..(3826): human codon optimized CHM (REP-1)
  misc_feature (3847)..(4054): bGH poly(A) signal
  misc_feature (4104)..(4233): 3' ITR
ctgcgcgctcgctcgctcactgaggccgcccgggcaaagcccgggcgtcgggcgacctttggtcgcccggcctcagtgagcgagcgagcgcgcagagagggagtggccaactccatcactaggggttccttgtagttaatgattaacccgccatgctacttatctacgtagcaagctagctagttattaatagtaatcaattacggggtcattagttcatagcccatatatggagttccgcgttacataacttacggtaaatggcccgcctggctgaccgcccaacgacccccgcccattgacgtcaataatgacgtatgttcccatagtaacgccaatagggactttccattgacgtcaatgggtggagtatttacggtaaactgcccacttggcagtacatcaagtgtatcatatgccaagtacgccccctattgacgtcaatgacggtaaatggcccgcctggcattatgcccagtacatgaccttatgggactttcctacttggcagtacatctacgtattagtcatcgctattaacatggtcgaggtgagccccacgttctgcttcactctccccatctcccccccctccccacccccaattttgtatttatttattttttaattattttgtgcagcgatgggggcggggggggggggggggcgcgcgccaggcggggcggggcggggcgaggggcggggcggggcgaggcggagaggtgcggcggcagccaatcagagcggcgcgctccgaaagtttccttttatggcgaggcggcggcggcggcggccctataaaaagcgaagcgcgcggcgggcggggagtcgctgcgacgctgccttcgccccgtgccccgctccgccgccgcctcgcgccgcccgccccggctctgactgaccgcgttactcccacaggtgagcgggcgggacggcccttctcctccgggctgtaattagcgcttggtttaatgacggcttgtttcttttctgtggctgcgtgaaagccttgaggggctccgggagggccctttgtgcggggggagcggctcggggggtgcgtgcgtgtgtgtgtgcgtggggagcgccgcgtgcggctccgcgctgcccggcggctgtgagcgctgcgggcgcggcgcggggctttgtgcgctccgcagtgtgcgcgaggggagcgcggccgggggcggtgccccgcggtgcggggggggctgcgaggggaacaaaggctgcgtgcggggtgtgtgcgtgggggggtgagcagggggtgtgggcgcgtcggtcgggctgcaaccccccctgcacccccctccccgagttgctgagcacggcccggcttcgggtgcggggctccgtacggggcgtggcgcggggctcgccgtgccgggcggggggtggcggcaggtgggggtgccgggcggggcggggccgcctcgggccggggagggctcgggggaggggcgcggcggcccccggagcgccggcggctgtcgaggcgcggcgagccgcagccattgccttttatggtaatcgtgcgagagggcgcagggacttcctttgtcccaaatctgtgcggagccgaaatctgggaggcgccgccgcaccccctctagcgggcgcggggcgaagcggtgcggcgccggcaggaaggaaatgggcggggagggccttcgtgcgtcgccgcgccgccgtccccttctccctctccagcctcggggctgtccgcggggggacggctgccttcgggggggacggggcagggcggggttcggcttctggcgtgtgaccggcggctctagacaattgtactaaccttcttctctttcctctcctgacaggttggtgtacactagcggccgccaccatggctgataccctgccctctgaattcgacgtgattgtgattggaaccggactccctgaatcgatcatcgccgcggcctgttcccggtccggtcggcgcgtgctgcacgtcgattcgagaagctactacggagggaattgggcctcattctccttctccggactgctctcctggctgaaggagtatcaggagaactccgacattgtctccgactcacctgtgtggcaggaccagatcctggaaaacgaggaagcaatagccctgagccggaaggacaagaccatccagcacgtggaggtgttctgttatgcctcccaagacctccatgaggacgtggaagaggctggagcgttgcagaagaatcatgccctcgtgacctccgctaactccaccgaggcagccgacagcgccttcctgccgaccgaggatgaatccctgtcaactatgtcgtgcgaaatgctgaccgaacagactccgagctccgaccccgaaaacgccctggaagtgaacggagcggaagtgaccggcgaaaaggagaaccattgcgacgacaagacttgtgtcccatccacttccgcggaggacatgtccgagaatgtgcctatcgccgaggacaccaccgaacagcccaagaagaacagaatcacgtacagccagatcatcaaggaggggcggaggtttaacatcgatctggtgtcgaagctgctgtacagccgcggtctgctgatcgatctgctcattaagtcgaacgtgtcgagatacgccgagttcaagaacatcacaaggattctcgccttccgggaaggaagagtggaacaagtgccgtgctcccgggccgacgtgttcaactcaaagcaacttaccatggtggaaaagcgcatgctgatgaaattcctgaccttctgcatggagtacgaaaagtaccctgatgagtacaagggttacgaagaaattactttctacgagtacctcaagacccagaagctgaccccgaatctgcagtacattgtgatgcactcaatcgcaatgacctccgaaaccgcctcctcgaccatcgacgggctcaaggccaccaagaacttcctgcactgtttggggcgctacggcaacactccgttcctcttcccgctgtacggccagggagagctgcctcagtgtttctgccggatgtgcgccgtgttcggcggaatctactgtctccgccactcggtccagtgcctggtggtggacaaggaatccaggaagtgcaaagccattattgaccagttcggacaacggatcatttccgagcactttcttgtggaggactcatacttcccggagaacatgtgctctcgggtccagtatcgacagatttccagggcggtgctcattactgaccggagcgtcctcaagaccgatagcgaccagcagatctccatcctgaccgtgccggcggaagaacccggcacttttgccgtgcgcgtgatcgagctttgctcatccaccatgacttgcatgaaaggcacttacctggtgcacctgacgtgcacctcatcgaaaaccgctagagaggacctggaatccgtcgtccaaaagctgttcgtgccttacaccgagatggaaattgaaaacgaacaagtggagaagccccgcatcctttgggccctgtactttaacatgcgcgattcctccgatatctcgcggtcctgctataacgacttgccttcgaacgtctacgtctgctccgggccagactgcggtcttggcaacgacaatgccgtgaagcaggcggaaacactgttccaagagatctgccctaacgaggatttttgcccgccccccccaaaccccgaggatatcatcttggacggagacagcctgcagccagaagcatccgagtccagcgccatcccggaggccaacagcgaaaccttcaaggagagcactaacctgggcaacctggaagagtccagcgaatgatcataggatctctgcctcgactgtgccttctagttgccagccatctgttgtttgcccctcccccgtgccttccttgaccctggaaggtgccactcccactgtcctttcctaataaaatgaggaaattgcatcgcattgtctgagtaggtgtcattctattctggggggtggggtggggcaggacagcaagggggaggattgggaagacaatagcaggcatgctggggactcgagttctacgtagataagtagcatggcgggttaatcattaactacaaggaacccctagtgatggagttggccactccctctctgcgcgctcgctcgctcactgaggccgggcgaccaaaggtcgcccgacgcccgggctttgcccgggcggcctcagtgagcgagcgagcgcgcagccttaattaacctaataaggaaaatgaagggaagttcctatactttctagagaataggaacttctatagggagtcgaataagggcgacacaaaaggtattctaaatgcataataaatactgataacatcttatagtttgtattatattttgtattatcgttgacatgtataattttgatatcaaaaactgattttccctttattattttcgagatttattttcttaattctctttaacaaactagaaatattgtatatacaaaaaatcataaataatagatgaatagtttaattataggtgttcatcaatcgaaaaagcaacgtatcttatttaaagtgcgttgcttttttctcatttataaggttaaataattctcatatatcaagcaaagtgacaggcgcccttaaatattctgacaaatgctctttccctaaactccccccataaaaaaacccgccgaagcgggtttttacgttatttgcggattaacgattactcgttatcagaaccgcccaggatgcctggcagttccctactctcgccgctgcgctcggtcgttcggctgcgggacctcagcgctagcggagtgtatactggcttactatgttggcactgatgagggtgtcagtgaagtgcttcatgtggcaggagaaaaaaggctgcaccggtgcgtcagcagaatatgtgatacaggatatattccgcttcctcgctcactgactcgctacgctcggtcgttcgactgcggcgagcggaaatggcttacgaacggggcggagatttcctggaagatgccaggaagatacttaacagggaagtgagagggccgcggcaaagccgtttttccataggctccgcccccctgacaagcatcacgaaatctgacgctcaaatcagtggtggcgaaacccgacaggactataaagataccaggcgtttccccctggcggctccctcgtgcgctctcctgttcctgcctttcggtttaccggtgtcattccgctgttatggccgcgtttgtctcattccacgcctgacactcagttccgggtaggcagttcgctccaagctggactgtatgcacgaaccccccgttcagtccgaccgctgcgccttatccggtaactatcgtcttgagtccaacccggaaagacatgcaaaagcaccactggcagcagccactggtaattgatttagaggagttagtcttgaagtcatgcgccggttaaggctaaactgaaaggacaagttttggtgactgcgctcctccaagccagttacctcggttcaaagagttggtagctcagagaaccttcgaaaaaccgccctgcaaggcggttttttcgttttcagagcaagagattacgcgcagaccaaaacgatctcaagaagatcatcttattaagctcctttttatttgggggagagggaagtcatgaaaaaactaacctttgaaattcgatctccagcacatcagcaaaacgctattcacgcagtacagcaaatccttccagacccaaccaaaccaatcgtagtaaccattcaggaacgcaaccgcagcttagaccaaaacaggaagctatgggcctgcttaggtgacgtctctcgtcaggttgaatggcatggtcgctggctggatgcagaaagctggaagtgtgtgtttaccgcagcattaaagcagcaggatgttgttcctaaccttgccgggaatggctttgtggtaataggccagtcaaccagcaggatgcgtgtaggcgaatttgcggagctattagagcttatacaggcattcggtacagagcgtggcgttaagtggtcagacgaagcgagactggctctggagtggaaagcgagatggggagacagggctgcatgataaatgtcgttagtttctccggtggcaggacgtcagcatatttgctctggctaatggagcaaaagcgacgggcaggtaaagacgtgcattacgttttcatggatacaggttgtgaacatccaatgacatatcggtttgtcagggaagttgtgaagttctgggatataccgctcaccgtattgcaggttgatatcaacccggagcttggacagccaaatggttatacggtatgggaaccaaaggatattcagacgcgaatgcctgttctgaagccatttatcgatatggtaaagaaatatggcactccatacgtcggcggcgcgttctgcactgacagattaaaactcgttcccttcaccaaatactgtgatgaccatttcgggcgagggaattacaccacgtggattggcatcagagctgatgaaccgaagcggctaaagccaaagcctggaatcagatatcttgctgaactgtcagactttgagaaggaagatatcctcgcatggtggaagcaacaaccattcgatttgcaaataccggaacatctcggtaactgcatattctgcattaaaaaatcaacgcaaaaaatcggacttgcctgcaaagatgaggagggattgcagcgtgtttttaatgaggtcatcacgggatcccatgtgcgtgacggacatcgggaaacgccaaaggagattatgtaccgaggaagaatgtcgctggacggtatcgcgaaaatgtattcagaaaatgattatcaagccctgtatcaggacatggtacgagctaaaagattcgataccggctcttgttctgagtcatgcgaaatatttggagggcagcttgatttcgacttcgggagggaagctgcatgatgcgatgttatcggtgcggtgaatgcaaagaagataaccgcttccgaccaaatcaaccttactggaatcgatggtgtctccggtgtgaaagaacaccaacaggggtgttaccactaccgcaggaaaaggaggacgtgtggcgagacagcgacgaagtatcaccgacataatctgcgaaaactgcaaataccttccaacgaaacgcaccagaaataaacccaagccaatcccaaaagaatctgacgtaaaaaccttcaactacacggctcacctgtgggatatccggtggctaagacgtcgtgcgaggaaaacaaggtgattgaccaaaatcgaagttacgaacaagaaagcgtcgagcgagctttaacgtgcgctaactgcggtcagaagctgcatgtgctggaagttcacgtgtgtgagcactgctgcgcagaactgatgagcgatccgaatagctcgatgcacgaggaagaagatgatggctaaaccagcgcgaagacgatgtaaaaacgatgaatgccgggaatggtttcaccctgcattcgctaatcagtggtggtgctctccagagtgtggaaccaagatagcactcgaacgacgaagtaaagaacgcgaaaaagcggaaaaagcagcagagaagaaacgacgacgagaggagcagaaacagaaagataaacttaagattcgaaaactcgccttaaagccccgcagttactggattaaacaagcccaacaagccgtaaacgccttcatcagagaaagagaccgcgacttaccatgtatctcgtgcggaacgctcacgtctgctcagtgggatgccggacattaccggacaactgctgcggcacctcaactccgatttaatgaacgcaatattcacaagcaatgcgtggtgtgcaaccagcacaaaagcggaaatctcgttccgtatcgcgtcgaactgattagccgcatcgggcaggaagcagtagacgaaatcgaatcaaaccataaccgccatcgctggactatcgaagagtgcaaggcgatcaaggcagagtaccaacagaaactcaaagacctgcgaaatagcagaagtgaggccgcatgacgttctcagtaaaaaccattccagacatgctcgttgaagcatacggaaatcagacagaagtagcacgcagactgaaatgtagtcgcggtacggtcagaaaatacgttgatgataaagacgggaaaatgcacgccatcgtcaacgacgttctcatggttcatcgcggatggagtgaaagagatgcgctattacgaaaaaattgatggcagcaaataccgaaatatttgggtagttggcgatctgcacggatgctacacgaacctgatgaacaaactggatacgattggattcgacaacaaaaaagacctgcttatctcggtgggcgatttggttgatcgtggtgcagagaacgttgaatgcctggaattaatcacattcccctggttcagagctgtacgtggaaaccatgagcaaatgatgattgatggcttatcagagcgtggaaacgttaatcactggctgcttaatggcggtggctggttctttaatctcgattacgacaaagaaattctggctaaagctcttgcccataaagcagatgaacttccgttaatcatcgaactggtgagcaaagataaaaaatatgttatctgccacgccgattatccctttgacgaatacgagtttggaaagccagttgatcatcagcaggtaatctggaaccgcgaacgaatcagcaactcacaaaacgggatcgtgaaagaaatcaaaggcgcggacacgttcatctttggtcatacgccagcagtgaaaccactcaagtttgccaaccaaatgtatatcgataccggcgcagtgttctgcggaaacctaacattgattcaggtacagggagaaggcgcatgagactcgaaagcgtagctaaatttcattcgccaaaaagcccgatgatgagcgactcaccacgggccacggcttctgactctctttccggtactgatgtgatggctgctatggggatggcgcaatcacaagccggattcggtatggctgcattctgcggtaagcacgaactcagccagaacgacaaacaaaaggctatcaactatctgatgcaatttgcacacaaggtatcggggaaataccgtggtgtggcaaagcttgaaggaaatactaaggcaaaggtactgcaagtgctcgcaacattcgcttatgcggattattgccgtagtgccgcgacgccgggggcaagatgcagagattgccatggtacaggccgtgcggttgatattgccaaaacagagctgtgggggagagttgtcgagaaagagtgcggaagatgcaaaggcgtcggctattcaaggatgccagcaagcgcagcatatcgcgctgtgacgatgctaatcccaaaccttacccaacccacctggtcacgcactgttaagccgctgtatgacgctctggtggtgcaatgccacaaagaagagtcaatcgcagacaacattttgaatgcggtcacacgttagcagcatgattgccacggatggcaacatattaacggcatgatattgacttattgaataaaattgggtaaatttgactcaacgatgggttaattcgctcgttgtggtagtgagatgaaaagaggcggcgcttactaccgattccgcctagttggtcacttcgacgtatcgtctggaactccaaccatcgcaggcagagaggtctgcaaaatgcaatcccgaaacagttcgcaggtaatagttagagcctgcataacggtttcgggattttttatatctgcacaacaggtaagagcattgagtcgataatcgtgaagagtcggcgagcctggttagccagtgctctttccgttgtgctgaattaagcgaataccggaagcagaaccggatcaccaaatgcgtacaggcgtcatcgccgcccagcaacagcacaacccaaactgagccgtagccactgtctgtcctgaattcattagtaatagttacgctgcggccttttacacatgaccttcgtgaaagcgggtggcaggaggtcgcgctaacaacctcctgccgttttgcccgtgcatatcggtcacgaacaaatctgattactaaacacagtagcctggatttgttctatcagtaatcgaccttattcctaattaaatagagcaaatccccttattgggggtaagacatgaagatgccagaaaaacatgacctgttggccgccattctcgcggcaaaggaacaaggcatcggggcaatccttgcgtttgcaatggcgtaccttcgcggcagatataatggcggtgcgtttacaaaaacagtaatcgacgcaacgatgtgcgccattatcgcctggttcattcgtgaccttctcgacttcgccggactaagtagcaatctcgcttatataacgagcgtgtttatcggctacatcggtactgactcgattggttcgcttatcaaacgcttcgctgctaaaaaagccggagtagaagatggtagaaatcaataatcaacgtaaggcgttcctcgatatgctggcgtggtcggagggaactgataacggacgtcagaaaaccagaaatcatggttatgacgtcattgtaggcggagagctatttactgattactccgatcaccctcgcaaacttgtcacgctaaacccaaaactcaaatcaacaggcgcagcttttagaaaaactcatcgagcatcaaatgaaactgcaatttattcatatcaggattatcaataccatatttttgaaaaagccgtttctgtaatgaaggagaaaactcaccgaggcagttccataggatggcaagatcctggtatcggtctgcgattccgactcgtccaacatcaatacaacctattaatttcccctcgtcaaaaataaggttatcaagtgagaaatcaccatgagtgacgactgaatccggtgagaatggcaaaagtttatgcatttctttccagacttgttcaacaggccagccattacgctcgtcatcaaaatcactcgcatcaaccaaaccgttattcattcgtgattgcgcctgagcgaggcgaaatacgcgatcgctgttaaaaggacaattacaaacaggaatcgagtgcaaccggcgcaggaacactgccagcgcatcaacaatattttcacctgaatcaggatattcttctaatacctggaacgctgtttttccggggatcgcagtggtgagtaaccatgcatcatcaggagtacggataaaatgcttgatggtcggaagtggcataaattccgtcagccagtttagtctgaccatctcatctgtaacatcattggcaacgctacctttgccatgtttcagaaacaactctggcgcatcgggcttcccatacaagcgatagattgtcgcacctgattgcccgacattatcgcgagcccatttatacccatataaatcagcatccatgttggaatttaatcgcggcctcgacgtttcccgttgaatatggctcatattcttcctttttcaatattattgaagcatttatcagggttattgtctcatgagcggatacatatttgaatgtatttagaaaaataaacaaataggggtcagtgttacaaccaattaaccaattctgaacattatcgcgagcccatttatacctgaatatggctcataacaccccttgtttgcctggcggcagtagcgcggtggtcccacctgaccccatgccgaactcagaagtgaaacgccgtagcgccgatggtagtgtggggactccccatgcgagagtagggaactgccaggcatcaaataaaacgaaaggctcagtcgaaagactgggcctttcgcccgggctaattagggggtgtcgcccttattcgactctatagggaagttcctattctctagaaagtataggaacttctgaaggggggtcgatcgacttaattaagg

SEQ ID NO: 28 - DNA, 6900 bp, Artificial Sequence
  constructed sequence
  misc_feature (1)..(130): 5' ITR
  misc_feature (241)..(544): CMV enhancer
  misc_feature (546)..(823): chicken beta actin promoter
  misc_feature (824)..(1795): CBA exon 1 and intron
  misc_feature (1859)..(1864): kozak
  misc_feature (1865)..(3826): human codon optimized CHM (REP-1)
  misc_feature (3847)..(4054): bGH poly(A) signal
  misc_feature (4104)..(4233): 3' ITR
ctgcgcgctcgctcgctcactgaggccgcccgggcaaagcccgggcgtcgggcgacctttggtcgcccggcctcagtgagcgagcgagcgcgcagagagggagtggccaactccatcactaggggttccttgtagttaatgattaacccgccatgctacttatctacgtagcaagctagctagttattaatagtaatcaattacggggtcattagttcatagcccatatatggagttccgcgttacataacttacggtaaatggcccgcctggctgaccgcccaacgacccccgcccattgacgtcaataatgacgtatgttcccatagtaacgccaatagggactttccattgacgtcaatgggtggagtatttacggtaaactgcccacttggcagtacatcaagtgtatcatatgccaagtacgccccctattgacgtcaatgacggtaaatggcccgcctggcattatgcccagtacatgaccttatgggactttcctacttggcagtacatctacgtattagtcatcgctattaacatggtcgaggtgagccccacgttctgcttcactctccccatctcccccccctccccacccccaattttgtatttatttattttttaattattttgtgcagcgatgggggcggggggggggggggggcgcgcgccaggcggggcggggcggggcgaggggcggggcggggcgaggcggagaggtgcggcggcagccaatcagagcggcgcgctccgaaagtttccttttatggcgaggcggcggcggcggcggccctataaaaagcgaagcgcgcggcgggcggggagtcgctgcgacgctgccttcgccccgtgccccgctccgccgccgcctcgcgccgcccgccccggctctgactgaccgcgttactcccacaggtgagcgggcgggacggcccttctcctccgggctgtaattagcgcttggtttaatgacggcttgtttcttttctgtggctgcgtgaaagccttgaggggctccgggagggccctttgtgcggggggagcggctcggggggtgcgtgcgtgtgtgtgtgcgtggggagcgccgcgtgcggctccgcgctgcccggcggctgtgagcgctgcgggcgcggcgcggggctttgtgcgctccgcagtgtgcgcgaggggagcgcggccgggggcggtgccccgcggtgcggggggggctgcgaggggaacaaaggctgcgtgcggggtgtgtgcgtgggggggtgagcagggggtgtgggcgcgtcggtcgggctgcaaccccccctgcacccccctccccgagttgctgagcacggcccggcttcgggtgcggggctccgtacggggcgtggcgcggggctcgccgtgccgggcggggggtggcggcaggtgggggtgccgggcggggcggggccgcctcgggccggggagggctcgggggaggggcgcggcggcccccggagcgccggcggctgtcgaggcgcggcgagccgcagccattgccttttatggtaatcgtgcgagagggcgcagggacttcctttgtcccaaatctgtgcggagccgaaatctgggaggcgccgccgcaccccctctagcgggcgcggggcgaagcggtgcggcgccggcaggaaggaaatgggcggggagggccttcgtgcgtcgccgcgccgccgtccccttctccctctccagcctcggggctgtccgcggggggacggctgccttcgggggggacggggcagggcggggttcggcttctggcgtgtgaccggcggctctagacaattgtactaaccttcttctctttcctctcctgacaggttggtgtacactagcggccgccaccatggctgataccctgccctctgaattcgacgtgattgtgattggaaccggactccctgaatcgatcatcgccgcggcctgttcccggtccggtcggcgcgtgctgcacgtcgattcgagaagctactacggagggaattgggcctcattctccttctccggactgctctcctggctgaaggagtatcaggagaactccgacattgtctccgactcacctgtgtggcaggaccagatcctggaaaacgaggaagcaatagccctgagccggaaggacaagaccatccagcacgtggaggtgttctgttatgcctcccaagacctccatgaggacgtggaagaggctggagcgttgcagaagaatcatgccctcgtgacctccgctaactccaccgaggcagccgacagcgccttcctgccgaccgaggatgaatccctgtcaactatgtcgtgcgaaatgctgaccgaacagactccgagctccgaccccgaaaacgccctggaagtgaacggagcggaagtgaccggcgaaaaggagaaccattgcgacgacaagacttgtgtcccatccacttccgcggaggacatgtccgagaatgtgcctatcgccgaggacaccaccgaacagcccaagaagaacagaatcacgtacagccagatcatcaaggaggggcggaggtttaacatcgatctggtgtcgaagctgctgtacagccgcggtctgctgatcgatctgctcattaagtcgaacgtgtcgagatacgccgagttcaagaacatcacaaggattctcgccttccgggaaggaagagtggaacaagtgccgtgctcccgggccgacgtgttcaactcaaagcaacttaccatggtggaaaagcgcatgctgatgaaattcctgaccttctgcatggagtacgaaaagtaccctgatgagtacaagggttacgaagaaattactttctacgagtacctcaagacccagaagctgaccccgaatctgcagtacattgtgatgcactcaatcgcaatgacctccgaaaccgcctcctcgaccatcgacgggctcaaggccaccaagaacttcctgcactgtttggggcgctacggcaacactccgttcctcttcccgctgtacggccagggagagctgcctcagtgtttctgccggatgtgcgccgtgttcggcggaatctactgtctccgccactcggtccagtgcctggtggtggacaaggaatccaggaagtgcaaagccattattgaccagttcggacaacggatcatttccgagcactttcttgtggaggactcatacttcccggagaacatgtgctctcgggtccagtatcgacagatttccagggcggtgctcattactgaccggagcgtcctcaagaccgatagcgaccagcagatctccatcctgaccgtgccggcggaagaacccggcacttttgccgtgcgcgtgatcgagctttgctcatccaccatgacttgcatgaaaggcacttacctggtgcacctgacgtgcacctcatcgaaaaccgctagagaggacctggaatccgtcgtccaaaagctgttcgtgccttacaccgagatggaaattgaaaacgaacaagtggagaagccccgcatcctttgggccctgtactttaacatgcgcgattcctccgatatctcgcggtcctgctataacgacttgccttcgaacgtctacgtctgctccgggccagactgcggtcttggcaacgacaatgccgtgaagcaggcggaaacactgttccaagagatctgccctaacgaggatttttgcccgccccccccaaaccccgaggatatcatcttggacggagacagcctgcagccagaagcatccgagtccagcgccatcccggaggccaacagcgaaaccttcaaggagagcactaacctgggcaacctggaagagtccagcgaatgatcataggatctctgcctcgactgtgccttctagttgccagccatctgttgtttgcccctcccccgtgccttccttgaccctggaaggtgccactcccactgtcctttcctaataaaatgaggaaattgcatcgcattgtctgagtaggtgtcattctattctggggggtggggtggggcaggacagcaagggggaggattgggaagacaatagcaggcatgctggggactcgagttctacgtagataagtagcatggcgggttaatcattaactacaaggaacccctagtgatggagttggccactccctctctgcgcgctcgctcgctcactgaggccgggcgaccaaaggtcgcccgacgcccgggctttgcccgggcggcctcagtgagcgagcgagcgcgcagccttaattaacctaataaggaaaatgaagggaagttcctatactttctagagaataggaacttctatagggagtcgaataagggcgacacaaaaggtattctaaatgcataataaatactgataacatcttatagtttgtattatattttgtattatcgttgacatgtataattttgatatcaaaaactgattttccctttattattttcgagatttattttcttaattctctttaacaaactagaaatattgtatatacaaaaaatcataaataatagatgaatagtttaattataggtgttcatcaatcgaaaaagcaacgtatcttatttaaagtgcgttgcttttttctcatttataaggttaaataattctcatatatcaagcaaagtgacaggcgcccttaaatattctgacaaatgctctttccctaaactccccccataaaaaaacccgccgaagcgggtttttacgttatttgcggattaacgattactcgttatcagaaccgcccaggatgcctggcagttccctactctcgccgctgcgctcggtcgttcggctgcgggacctcagcgctagcggagtgtatactggcttactatgttggcactgatgagggtgtcagtgaagtgcttcatgtggcaggagaaaaaaggctgcaccggtgcgtcagcagaatatgtgatacaggatatattccgcttcctcgctcactgactcgctacgctcggtcgttcgactgcggcgagcggaaatggcttacgaacggggcggagatttcctggaagatgccaggaagatacttaacagggaagtgagagggccgcggcaaagccgtttttccataggctccgcccccctgacaagcatcacgaaatctgacgctcaaatcagtggtggcgaaacccgacaggactataaagataccaggcgtttccccctggcggctccctcgtgcgctctcctgttcctgcctttcggtttaccggtgtcattccgctgttatggccgcgtttgtctcattccacgcctgacactcagttccgggtaggcagttcgctccaagctggactgtatgcacgaaccccccgttcagtccgaccgctgcgccttatccggtaactatcgtcttgagtccaacccggaaagacatgcaaaagcaccactggcagcagccactggtaattgatttagaggagttagtcttgaagtcatgcgccggttaaggctaaactgaaaggacaagttttggtgactgcgctcctccaagccagttacctcggttcaaagagttggtagctcagagaaccttcgaaaaaccgccctgcaaggcggttttttcgttttcagagcaagagattacgcgcagaccaaaacgatctcaagaagatcatcttattaagcttttagaaaaactcatcgagcatcaaatgaaactgcaatttattcatatcaggattatcaataccatatttttgaaaaagccgtttctgtaatgaaggagaaaactcaccgaggcagttccataggatggcaagatcctggtatcggtctgcgattccgactcgtccaacatcaatacaacctattaatttcccctcgtcaaaaataaggttatcaagtgagaaatcaccatgagtgacgactgaatccggtgagaatggcaaaagtttatgcatttctttccagacttgttcaacaggccagccattacgctcgtcatcaaaatcactcgcatcaaccaaaccgttattcattcgtgattgcgcctgagcgaggcgaaatacgcgatcgctgttaaaaggacaattacaaacaggaatcgagtgcaaccggcgcaggaacactgccagcgcatcaacaatattttcacctgaatcaggatattcttctaatacctggaacgctgtttttccggggatcgcagtggtgagtaaccatgcatcatcaggagtacggataaaatgcttgatggtcggaagtggcataaattccgtcagccagtttagtctgaccatctcatctgtaacatcattggcaacgctacctttgccatgtttcagaaacaactctggcgcatcgggcttcccatacaagcgatagattgtcgcacctgattgcccgacattatcgcgagcccatttatacccatataaatcagcatccatgttggaatttaatcgcggcctcgacgtttcccgttgaatatggctcatattcttcctttttcaatattattgaagcatttatcagggttattgtctcatgagcggatacatatttgaatgtatttagaaaaataaacaaataggggtcagtgttacaaccaattaaccaattctgaacattatcgcgagcccatttatacctgaatatggctcataacaccccttgtttgcctggcggcagtagcgcggtggtcccacctgaccccatgccgaactcagaagtgaaacgccgtagcgccgatggtagtgtggggactccccatgcgagagtagggaactgccaggcatcaaataaaacgaaaggctcagtcgaaagactgggcctttcgcccgggctaattagggggtgtcgcccttattcgactctatagggaagttcctattctctagaaagtataggaacttctgaaggggggtcgatcgacttaattaagg

SEQ ID NO: 29 - DNA, 12074 bp, Artificial Sequence
  constructed sequence
ctgcgcgctcgctcgctcactgaggccgcccgggcaaagcccgggcgtcgggcgacctttggtcgcccggcctcagtgagcgagcgagcgcgcagagagggagtggccaactccatcactaggggttccttgtagttaatgattaacccgccatgctacttatctacgtagcaagctagctagttattaatagtaatcaattacggggtcattagttcatagcccatatatggagttccgcgttacataacttacggtaaatggcccgcctggctgaccgcccaacgacccccgcccattgacgtcaataatgacgtatgttcccatagtaacgccaatagggactttccattgacgtcaatgggtggagtatttacggtaaactgcccacttggcagtacatcaagtgtatcatatgccaagtacgccccctattgacgtcaatgacggtaaatggcccgcctggcattatgcccagtacatgaccttatgggactttcctacttggcagtacatctacgtattagtcatcgctattaacatggtcgaggtgagccccacgttctgcttcactctccccatctcccccccctccccacccccaattttgtatttatttattttttaattattttgtgcagcgatgggggcggggggggggggggggcgcgcgccaggcggggcggggcggggcgaggggcggggcggggcgaggcggagaggtgcggcggcagccaatcagagcggcgcgctccgaaagtttccttttatggcgaggcggcggcggcggcggccctataaaaagcgaagcgcgcggcgggcggggagtcgctgcgacgctgccttcgccccgtgccccgctccgccgccgcctcgcgccgcccgccccggctctgactgaccgcgttactcccacaggtgagcgggcgggacggcccttctcctccgggctgtaattagcgcttggtttaatgacggcttgtttcttttctgtggctgcgtgaaagccttgaggggctccgggagggccctttgtgcggggggagcggctcggggggtgcgtgcgtgtgtgtgtgcgtggggagcgccgcgtgcggctccgcgctgcccggcggctgtgagcgctgcgggcgcggcgcggggctttgtgcgctccgcagtgtgcgcgaggggagcgcggccgggggcggtgccccgcggtgcggggggggctgcgaggggaacaaaggctgcgtgcggggtgtgtgcgtgggggggtgagcagggggtgtgggcgcgtcggtcgggctgcaaccccccctgcacccccctccccgagttgctgagcacggcccggcttcgggtgcggggctccgtacggggcgtggcgcggggctcgccgtgccgggcggggggtggcggcaggtgggggtgccgggcggggcggggccgcctcgggccggggagggctcgggggaggggcgcggcggcccccggagcgccggcggctgtcgaggcgcggcgagccgcagccattgccttttatggtaatcgtgcgagagggcgcagggacttcctttgtcccaaatctgtgcggagccgaaatctgggaggcgccgccgcaccccctctagcgggcgcggggcgaagcggtgcggcgccggcaggaaggaaatgggcggggagggccttcgtgcgtcgccgcgccgccgtccccttctccctctccagcctcggggctgtccgcggggggacggctgccttcgggggggacggggcagggcggggttcggcttctggcgtgtgaccggcggctctagacaattgtactaaccttcttctctttcctctcctgacaggttggtgtacactagcggccgcatggcggatactctcccttcggagtttgatgtgatcgtaatagggacgggtttgcctgaatccatcattgcagctgcatgttcaagaagtggccggagagttctgcatgttgattcaagaagctactatggaggaaactgggccagttttagcttttcaggactattgtcctggctaaaggaataccaggaaaacagtgacattgtaagtgacagtccagtgtggcaagaccagatccttgaaaatgaagaagccattgctcttagcaggaaggacaaaactattcaacatgtggaagtattttgttatgccagtcaggatttgcatgaagatgtcgaagaagctggtgcactgcagaaaaatcatgctcttgtgacatctgcaaactccacagaagctgcagattctgccttcctgcctacggaggatgagtcattaagcactatgagctgtgaaatgctcacagaacaaactccaagcagcgatccagagaatgcgctagaagtaaatggtgctgaagtgacaggggaaaaagaaaaccattgtgatgataaaacttgtgtgccatcaacttcagcagaagacatgagtgaaaatgtgcctatagcagaagataccacagagcaaccaaagaaaaacagaattacttactcacaaattattaaagaaggcaggagatttaatattgatttagtatcaaagctgctgtattctcgaggattactaattgatcttctaatcaaatctaatgttagtcgatatgcagagtttaaaaatattaccaggattcttgcatttcgagaaggacgagtggaacaggttccgtgttccagagcagatgtctttaatagcaaacaacttactatggtagaaaagcgaatgctaatgaaatttcttacattttgtatggaatatgagaaatatcctgatgaatataaaggatatgaagagatcacattttatgaatatttaaagactcaaaaattaacccccaacctccaatatattgtcatgcattcaattgcaatgacatcagagacagccagcagcaccatagatggtctcaaagctaccaaaaactttcttcactgtcttgggcggtatggcaacactccatttttgtttcctttatatggccaaggagaactcccccagtgtttctgcaggatgtgtgctgtgtttggtggaatttattgtcttcgccattcagtacagtgccttgtagtggacaaagaatccagaaaatgtaaagcaattatagatcagtttggtcagagaataatctctgagcatttcctcgtggaggacagttactttcctgagaacatgtgctcacgtgtgcaatacaggcagatctccagggcagtgctgattacagatagatctgtcctaaaaacagattcagatcaacagatttccattttgacagtgccagcagaggaaccaggaacttttgctgttcgggtcattgagttatgttcttcaacgatgacatgcatgaaaggcacctatttggttcatttgacttgcacatcttctaaaacagcaagagaagatttagaatcagttgtgcagaaattgtttgttccatatactgaaatggagatagaaaatgaacaagtagaaaagccaagaattctgtgggctctttacttcaatatgagagattcgtcagacatcagcaggagctgttataatgatttaccatccaacgtttatgtctgctctggcccagattgtggtttaggaaatgataatgcagtcaaacaggctgaaacacttttccaggaaatctgccccaatgaagatttctgtccccctccaccaaatcctgaagacattatccttgatggagacagtttacagccagaggcttcagaatccagtgccataccagaggctaactcggagactttcaaggaaagcacaaaccttggaaacctagaggagtcctctgaataaggatctgcctcgactgtgccttctagttgccagccatctgttgtttgcccctcccccgtgccttccttgaccctggaaggtgccactcccactgtcctttcctaataaaatgaggaaattgcatcgcattgtctgagtaggtgtcattctattctggggggtggggtggggcaggacagcaagggggaggattgggaagacaatagcaggcatgctggggactcgagttctacgtagataagtagcatggcgggttaatcattaactacaaggaacccctagtgatggagttggccactccctctctgcgcgctcgctcgctcactgaggccgggcgaccaaaggtcgcccgacgcccgggctttgcccgggcggcctcagtgagcgagcgagcgcgcagccttaattaacctaaggaaaatgaagtgaagttcctatactttctagagaataggaacttctatagtgagtcgaataagggcgacacaaaatttattctaaatgcataataaatactgataacatcttatagtttgtattatattttgtattatcgttgacatgtataattttgatatcaaaaactgattttccctttattattttcgagatttattttcttaattctctttaacaaactagaaatattgtatatacaaaaaatcataaataatagatgaatagtttaattataggtgttcatcaatcgaaaaagcaacgtatcttatttaaagtgcgttgcttttttctcatttataaggttaaataattctcatatatcaagcaaagtgacaggcgcccttaaatattctgacaaatgctctttccctaaactccccccataaaaaaacccgccgaagcgggtttttacgttatttgcggattaacgattactcgttatcagaaccgcccagggggcccgagcttaacctttttatttgggggagagggaagtcatgaaaaaactaacctttgaaattcgatctccagcacatcagcaaaacgctattcacgcagtacagcaaatccttccagacccaaccaaaccaatcgtagtaaccattcaggaacgcaaccgcagcttagaccaaaacaggaagctatgggcctgcttaggtgacgtctctcgtcaggttgaatggcatggtcgctggctggatgcagaaagctggaagtgtgtgtttaccgcagcattaaagcagcaggatgttgttcctaaccttgccgggaatggctttgtggtaataggccagtcaaccagcaggatgcgtgtaggcgaatttgcggagctattagagcttatacaggcattcggtacagagcgtggcgttaagtggtcagacgaagcgagactggctctggagtggaaagcgagatggggagacagggctgcatgataaatgtcgttagtttctccggtggcaggacgtcagcatatttgctctggctaatggagcaaaagcgacgggcaggtaaagacgtgcattacgttttcatggatacaggttgtgaacatccaatgacatatcggtttgtcagggaagttgtgaagttctgggatataccgctcaccgtattgcaggttgatatcaacccggagcttggacagccaaatggttatacggtatgggaaccaaaggatattcagacgcgaatgcctgttctgaagccatttatcgatatggtaaagaaatatggcactccatacgtcggcggcgcgttctgcactgacagattaaaactcgttcccttcaccaaatactgtgatgaccatttcgggcgagggaattacaccacgtggattggcatcagagctgatgaaccgaagcggctaaagccaaagcctggaatcagatatcttgctgaactgtcagactttgagaaggaagatatcctcgcatggtggaagcaacaaccattcgatttgcaaataccggaacatctcggtaactgcatattctgcattaaaaaatcaacgcaaaaaatcggacttgcctgcaaagatgaggagggattgcagcgtgtttttaatgaggtcatcacgggatcccatgtgcgtgacggacatcgggaaacgccaaaggagattatgtaccgaggaagaatgtcgctggacggtatcgcgaaaatgtattcagaaaatgattatcaagccctgtatcaggacatggtacgagctaaaagattcgataccggctcttgttctgagtcatgcgaaatatttggagggcagcttgatttcgacttcgggagggaagctgcatgatgcgatgttatcggtgcggtgaatgcaaagaagataaccgcttccgaccaaatcaaccttactggaatcgatggtgtctccggtgtgaaagaacaccaacaggggtgttaccactaccgcaggaaaaggaggacgtgtggcgagacagcgacgaagtatcaccgacataatctgcgaaaactgcaaataccttccaacgaaacgcaccagaaataaacccaagccaatcccaaaagaatctgacgtaaaaaccttcaactacacggctcacctgtgggatatccggtggctaagacgtcgtgcgaggaaaacaaggtgattgaccaaaatcgaagttacgaacaagaaagcgtcgagcgagctttaacgtgcgctaactgcggtcagaagctgcatgtgctggaagttcacgtgtgtgagcactgctgcgcagaactgatgagcgatccgaatagctcgatgcacgaggaagaagatgatggctaaaccagcgcgaagacgatgtaaaaacgatgaatgccgggaatggtttcaccctgcattcgctaatcagtggtggtgctctccagagtgtggaaccaagatagcactcgaacgacgaagtaaagaacgcgaaaaagcggaaaaagcagcagagaagaaacgacgacgagaggagcagaaacagaaagataaacttaagattcgaaaactcgccttaaagccccgcagttactggattaaacaagcccaacaagccgtaaacgccttcatcagagaaagagaccgcgacttaccatgtatctcgtgcggaacgctcacgtctgctcagtgggatgccggacattaccggacaactgctgcggcacctcaactccgatttaatgaacgcaatattcacaagcaatgcgtggtgtgcaaccagcacaaaagcggaaatctcgttccgtatcgcgtcgaactgattagccgcatcgggcaggaagcagtagacgaaatcgaatcaaaccataaccgccatcgctggactatcgaagagtgcaaggcgatcaaggcagagtaccaacagaaactcaaagacctgcgaaatagcagaagtgaggccgcatgacgttctcagtaaaaaccattccagacatgctcgttgaagcatacggaaatcagacagaagtagcacgcagactgaaatgtagtcgcggtacggtcagaaaatacgttgatgataaagacgggaaaatgcacgccatcgtcaacgacgttctcatggttcatcgcggatggagtgaaagagatgcgctattacgaaaaaattgatggcagcaaataccgaaatatttgggtagttggcgatctgcacggatgctacacgaacctgatgaacaaactggatacgattggattcgacaacaaaaaagacctgcttatctcggtgggcgatttggttgatcgtggtgcagagaacgttgaatgcctggaattaatcacattcccctggttcagagctgtacgtggaaaccatgagcaaatgatgattgatggcttatcagagcgtggaaacgttaatcactggctgcttaatggcggtggctggttctttaatctcgattacgacaaagaaattctggctaaagctcttgcccataaagcagatgaacttccgttaatcatcgaactggtgagcaaagataaaaaatatgttatctgccacgccgattatccctttgacgaatacgagtttggaaagccagttgatcatcagcaggtaatctggaaccgcgaacgaatcagcaactcacaaaacgggatcgtgaaagaaatcaaaggcgcggacacgttcatctttggtcatacgccagcagtgaaaccactcaagtttgccaaccaaatgtatatcgataccggcgcagtgttctgcggaaacctaacattgattcaggtacagggagaaggcgcatgagactcgaaagcgtagctaaatttcattcgccaaaaagcccgatgatgagcgactcaccacgggccacggcttctgactctctttccggtactgatgtgatggctgctatggggatggcgcaatcacaagccggattcggtatggctgcattctgcggtaagcacgaactcagccagaacgacaaacaaaaggctatcaactatctgatgcaatttgcacacaaggtatcggggaaataccgtggtgtggcaaagcttgaaggaaatactaaggcaaaggtactgcaagtgctcgcaacattcgcttatgcggattattgccgtagtgccgcgacgccgggggcaagatgcagagattgccatggtacaggccgtgcggttgatattgccaaaacagagctgtgggggagagttgtcgagaaagagtgcggaagatgcaaaggcgtcggctattcaaggatgccagcaagcgcagcatatcgcgctgtgacgatgctaatcccaaaccttacccaacccacctggtcacgcactgttaagccgctgtatgacgctctggtggtgcaatgccacaaagaagagtcaatcgcagacaacattttgaatgcggtcacacgttagcagcatgattgccacggatggcaacatattaacggcatgatattgacttattgaataaaattgggtaaatttgactcaacgatgggttaattcgctcgttgtggtagtgagatgaaaagaggcggcgcttactaccgattccgcctagttggtcacttcgacgtatcgtctggaactccaaccatcgcaggcagagaggtctgcaaaatgcaatcccgaaacagttcgcaggtaatagttagagcctgcataacggtttcgggattttttatatctgcacaacaggtaagagcattgagtcgataatcgtgaagagtcggcgagcctggttagccagtgctctttccgttgtgctgaattaagcgaataccggaagcagaaccggatcaccaaatgcgtacaggcgtcatcgccgcccagcaacagcacaacccaaactgagccgtagccactgtctgtcctgaattcattagtaatagttacgctgcggccttttacacatgaccttcgtgaaagcgggtggcaggaggtcgcgctaacaacctcctgccgttttgcccgtgcatatcggtcacgaacaaatctgattactaaacacagtagcctggatttgttctatcagtaatcgaccttattcctaattaaatagagcaaatccccttattgggggtaagacatgaagatgccagaaaaacatgacctgttggccgccattctcgcggcaaaggaacaaggcatcggggcaatccttgcgtttgcaatggcgtaccttcgcggcagatataatggcggtgcgtttacaaaaacagtaatcgacgcaacgatgtgcgccattatcgcctggttcattcgtgaccttctcgacttcgccggactaagtagcaatctcgcttatataacgagcgtgtttatcggctacatcggtactgactcgattggttcgcttatcaaacgcttcgctgctaaaaaagccggagtagaagatggtagaaatcaataatcaacgtaaggcgttcctcgatatgctggcgtggtcggagggaactgataacggacgtcagaaaaccagaaatcatggttatgacgtcattgtaggcggagagctatttactgattactccgatcaccctcgcaaacttgtcacgctaaacccaaaactcaaatcaacaggcgcttaagactggccgtcgttttacaacacagaaagagtttgtagaaacgcaaaaaggccatccgtcaggggccttctgcttagtttgatgcctggcagttccctactctcgccttccgcttcctcgctcactgactcgctgcgctcggtcgttcggctgcggcgagcggtatcagctcactcaaaggcggtaatacggttatccacagaatcaggggataacgcaggaaagaacatgtgagcaaaaggccagcaaaaggccaggaaccgtaaaaaggccgcgttgctggcgtttttccataggctccgcccccctgacgagcatcacaaaaatcgacgctcaagtcagaggtggcgaaacccgacaggactataaagataccaggcgtttccccctggaagctccctcgtgcgctctcctgttccgaccctgccgcttaccggatacctgtccgcctttctcccttcgggaagcgtggcgctttctcatagctcacgctgtaggtatctcagttcggtgtaggtcgttcgctccaagctgggctgtgtgcacgaaccccccgttcagcccgaccgctgcgccttatccggtaactatcgtcttgagtccaacccggtaagacacgacttatcgccactggcagcagccactggtaacaggattagcagagcgaggtatgtaggcggtgctacagagttcttgaagtggtgggctaactacggctacactagaagaacagtatttggtatctgcgctctgctgaagccagttaccttcggaaaaagagttggtagctcttgatccggcaaacaaaccaccgctggtagcggtggtttttttgtttgcaagcagcagattacgcgcagaaaaaaaggatctcaagaagatcctttgatcttttctacggggtctgacgctcagtggaacgacgcgcgcgtaactcacgttaagggattttggtcatgagcttgcgccgtcccgtcaagtcagcgtaatgctctgcttttagaaaaactcatcgagcatcaaatgaaactgcaatttattcatatcaggattatcaataccatatttttgaaaaagccgtttctgtaatgaaggagaaaactcaccgaggcagttccataggatggcaagatcctggtatcggtctgcgattccgactcgtccaacatcaatacaacctattaatttcccctcgtcaaaaataaggttatcaagtgagaaatcaccatgagtgacgactgaatccggtgagaatggcaaaagtttatgcatttctttccagacttgttcaacaggccagccattacgctcgtcatcaaaatcactcgcatcaaccaaaccgttattcattcgtgattgcgcctgagcgaggcgaaatacgcgatcgctgttaaaaggacaattacaaacaggaatcgagtgcaaccggcgcaggaacactgccagcgcatcaacaatattttcacctgaatcaggatattcttctaatacctggaacgctgtttttccggggatcgcagtggtgagtaaccatgcatcatcaggagtacggataaaatgcttgatggtcggaagtggcataaattccgtcagccagtttagtctgaccatctcatctgtaacatcattggcaacgctacctttgccatgtttcagaaacaactctggcgcatcgggcttcccatacaagcgatagattgtcgcacctgattgcccgacattatcgcgagcccatttatacccatataaatcagcatccatgttggaatttaatcgcggcctcgacgtttcccgttgaatatggctcatattcttcctttttcaatattattgaagcatttatcagggttattgtctcatgagcggatacatatttgaatgtatttagaaaaataaacaaataggggtcagtgttacaaccaattaaccaattctgaacattatcgcgagcccatttatacctgaatatggctcataacaccccttgtttgcctggcggcagtagcgcggtggtcccacctgaccccatgccgaactcagaagtgaaacgccgtagcgccgatggtagtgtggggactccccatgcgagagtagggaactgccaggcatcaaataaaacgaaaggctcagtcgaaagactgggcctttcgcccgggctaattagggggtgtcgcccttattcgactctatagtgaagttcctattctctagaaagtataggaacttctgaagtggggtcgacttaattaagg

SEQ ID NO: 30 - DNA, 11041 bp, Artificial Sequence
  constructed sequence
ctgcgcgctcgctcgctcactgaggccgcccgggcaaagcccgggcgtcgggcgacctttggtcgcccggcctcagtgagcgagcgagcgcgcagagagggagtggccaactccatcactaggggttccttgtagttaatgattaacccgccatgctacttatctacgtagcaagctagcaagatccaagctcagatctcgatcgagttgggccccagaagcctggtggttgtttgtccttctcaggggaaaagtgaggcggccccttggaggaaggggccgggcagaatgatctaatcggattccaagcagctcaggggattgtctttttctagcaccttcttgccactcctaagcgtcctccgtgaccccggctgggatttagcctggtgctgtgtcagccccggtctcccaggggcttcccagtggtccccaggaaccctcgacagggcccggtctctctcgtccagcaagggcagggacgggccacaggccaagggccctcgatcgaggaactgaaaaaccagaaagttaactggtaagtttagtctttttgtcttttatttcaggtcccggatccggtggtggtgcaaatcaaagaactgctcctcagtggatgttgcctttacttctaggcctgtacggaagtgttacttctgctctaaaagctgcggaattgtacccgcggccgccaccatggccaagatcaacacccaatactcccacccctccaggacccacctcaaggtaaagacctcagaccgggatctcaatcgcgctgaaaatggcctcagcagagcccactcgtcaagtgaggagacatcgtcagtgctgcagccggggatcgccatggagaccagaggactggctgactccgggcagggctccttcaccggccaggggatcgccaggctgtcgcgcctcatcttcttgctgcgcaggtgggctgccaggcatgtgcaccaccaggaccagggaccggactcttttcctgatcgtttccgtggagccgagcttaaggaggtgtccagccaagaaagcaatgcccaggcaaatgtgggcagccaggagccagcagacagagggagaagcgcctggcccctggccaaatgcaacactaacaccagcaacaacacggaggaggagaagaagacgaaaaagaaggatgcgatcgtggtggacccgtccagcaacctgtactaccgctggctgaccgccatcgccctgcctgtcttctataactggtatctgcttatttgcagggcctgtttcgatgagctgcagtccgagtacctgatgctgtggctggtcctggactactcggcagatgtcctgtatgtcttggatgtgcttgtacgagctcggacaggttttcttgagcaaggcttaatggtcagtgataccaacaggctgtggcagcattacaagacgaccacgcagttcaagctggatgtgttgtccctggtccccaccgacctggcttacttaaaggtgggcacaaactacccagaagtgaggttcaaccgcctactgaagttttcccggctctttgaattctttgaccgcacagagacaaggaccaactaccccaatatgttcaggattgggaacttggtcttgtacattctcatcatcatccactggaatgcctgcatctactttgccatttccaagttcattggttttgggacagactcctgggtctacccaaacatctcaatcccagagcatgggcgcctctccaggaagtacatttacagtctctactggtccaccttgacccttaccaccattggtgagaccccaccccccgtgaaagatgaggagtatctctttgtggtcgtagacttcttggtgggtgttctgatttttgccaccattgtgggcaatgtgggctccatgatctcgaatatgaatgcctcacgggcagagttccaggccaagattgattccatcaagcagtacatgcagttccgcaaggtcaccaaggacttggagacgcgggttatccggtggtttgactacctgtgggccaacaagaagacggtggatgagaaggaggtgctcaagagcctcccagacaagctgaaggctgagatcgccatcaacgtgcacctggacacgctgaagaaggttcgcatcttccaggactgtgaggcagggctgctggtggagctggtgctgaagctgcgacccactgtgttcagccctggggattatatctgcaagaagggagatattgggaaggagatgtacatcatcaacgagggcaagctggccgtggtggctgatgatggggtcacccagttcgtggtcctcagcgatggcagctacttcggggagatcagcattctgaacatcaaggggagcaagtcggggaaccgcaggacggccaacatccgcagcattggctactcagacctgttctgcctctcaaaggacgatctcatggaggccctcaccgagtaccccgaagccaagaaggccctggaggagaaaggacggcagatcctgatgaaagacaacctgatcgatgaggagctggccagggcgggcgcggaccccaaggaccttgaggagaaagtggagcagctggggtcctccctggacaccctgcagaccaggtttgcacgcctcctggctgagtacaacgccacccagatgaagatgaagcagcgtctcagccaactggaaagccaggtgaagggtggtggggacaagcccctggctgatggggaagttcccggggatgctacaaaaacagaggacaaacaacagtgatcatagatcgatctgcctcgactgtgccttctagttgccagccatctgttgtttgcccctcccccgtgccttccttgaccctggaaggtgccactcccactgtcctttcctaataaaatgaggaaattgcatcgcattgtctgagtaggtgtcattctattctggggggtggggtggggcaggacagcaagggggaggattgggaagacaatagcaggcatgctggggactcgagttctacgtagataagtagcatggcgggttaatcattaactacaaggaacccctagtgatggagttggccactccctctctgcgcgctcgctcgctcactgaggccgggcgaccaaaggtcgcccgacgcccgggctttgcccgggcggcctcagtgagcgagcgagcgcgcagccttaattaacctaaggaaaatgaagtgaagttcctatactttctagagaataggaacttctatagtgagtcgaataagggcgacacaaaatttattctaaatgcataataaatactgataacatcttatagtttgtattatattttgtattatcgttgacatgtataattttgatatcaaaaactgattttccctttattattttcgagatttattttcttaattctctttaacaaactagaaatattgtatatacaaaaaatcataaataatagatgaatagtttaattataggtgttcatcaatcgaaaaagcaacgtatcttatttaaagtgcgttgcttttttctcatttataaggttaaataattctcatatatcaagcaaagtgacaggcgcccttaaatattctgacaaatgctctttccctaaactccccccataaaaaaacccgccgaagcgggtttttacgttatttgcggattaacgattactcgttatcagaaccgcccagggggcccgagcttaacctttttatttgggggagagggaagtcatgaaaaaactaacctttgaaattcgatctccagcacatcagcaaaacgctattcacgcagtacagcaaatccttccagacccaaccaaaccaatcgtagtaaccattcaggaacgcaaccgcagcttagaccaaaacaggaagctatgggcctgcttaggtgacgtctctcgtcaggttgaatggcatggtcgctggctggatgcagaaagctggaagtgtgtgtttaccgcagcattaaagcagcaggatgttgttcctaaccttgccgggaatggctttgtggtaataggccagtcaaccagcaggatgcgtgtaggcgaatttgcggagctattagagcttatacaggcattcggtacagagcgtggcgttaagtggtcagacgaagcgagactggctctggagtggaaagcgagatggggagacagggctgcatgataaatgtcgttagtttctccggtggcaggacgtcagcatatttgctctggctaatggagcaaaagcgacgggcaggtaaagacgtgcattacgttttcatggatacaggttgtgaacatccaatgacatatcggtttgtcagggaagttgtgaagttctgggatataccgctcaccgtattgcaggttgatatcaacccggagcttggacagccaaatggttatacggtatgggaaccaaaggatattcagacgcgaatgcctgttctgaagccatttatcgatatggtaaagaaatatggcactccatacgtcggcggcgcgttctgcactgacagattaaaactcgttcccttcaccaaatactgtgatgaccatttcgggcgagggaattacaccacgtggattggcatcagagctgatgaaccgaagcggctaaagccaaagcctggaatcagatatcttgctgaactgtcagactttgagaaggaagatatcctcgcatggtggaagcaacaaccattcgatttgcaaataccggaacatctcggtaactgcatattctgcattaaaaaatcaacgcaaaaaatcggacttgcctgcaaagatgaggagggattgcagcgtgtttttaatgaggtcatcacgggatcccatgtgcgtgacggacatcgggaaacgccaaaggagattatgtaccgaggaagaatgtcgctggacggtatcgcgaaaatgtattcagaaaatgattatcaagccctgtatcaggacatggtacgagctaaaagattcgataccggctcttgttctgagtcatgcgaaatatttggagggcagcttgatttcgacttcgggagggaagctgcatgatgcgatgttatcggtgcggtgaatgcaaagaagataaccgcttccgaccaaatcaaccttactggaatcgatggtgtctccggtgtgaaagaacaccaacaggggtgttaccactaccgcaggaaaaggaggacgtgtggcgagacagcgacgaagtatcaccgacataatctgcgaaaactgcaaataccttccaacgaaacgcaccagaaataaacccaagccaatcccaaaagaatctgacgtaaaaaccttcaactacacggctcacctgtgggatatccggtggctaagacgtcgtgcgaggaaaacaaggtgattgaccaaaatcgaagttacgaacaagaaagcgtcgagcgagctttaacgtgcgctaactgcggtcagaagctgcatgtgctggaagttcacgtgtgtgagcactgctgcgcagaactgatgagcgatccgaatagctcgatgcacgaggaagaagatgatggctaaaccagcgcgaagacgatgtaaaaacgatgaatgccgggaatggtttcaccctgcattcgctaatcagtggtggtgctctccagagtgtggaaccaagatagcactcgaacgacgaagtaaagaacgcgaaaaagcggaaaaagcagcagagaagaaacgacgacgagaggagcagaaacagaaagataaacttaagattcgaaaactcgccttaaagccccgcagttactggattaaacaagcccaacaagccgtaaacgccttcatcagagaaagagaccgcgacttaccatgtatctcgtgcggaacgctcacgtctgctcagtgggatgccggacattaccggacaactgctgcggcacctcaactccgatttaatgaacgcaatattcacaagcaatgcgtggtgtgcaaccagcacaaaagcggaaatctcgttccgtatcgcgtcgaactgattagccgcatcgggcaggaagcagtagacgaaatcgaatcaaaccataaccgccatcgctggactatcgaagagtgcaaggcgatcaaggcagagtaccaacagaaactcaaagacctgcgaaatagcagaagtgaggccgcatgacgttctcagtaaaaaccattccagacatgctcgttgaagcatacggaaatcagacagaagtagcacgcagactgaaatgtagtcgcggtacggtcagaaaatacgttgatgataaagacgggaaaatgcacgccatcgtcaacgacgttctcatggttcatcgcggatggagtgaaagagatgcgctattacgaaaaaattgatggcagcaaataccgaaatatttgggtagttggcgatctgcacggatgctacacgaacctgatgaacaaactggatacgattggattcgacaacaaaaaagacctgcttatctcggtgggcgatttggttgatcgtggtgcagagaacgttgaatgcctggaattaatcacattcccctggttcagagctgtacgtggaaaccatgagcaaatgatgattgatggcttatcagagcgtggaaacgttaatcactggctgcttaatggcggtggctggttctttaatctcgattacgacaaagaaattctggctaaagctcttgcccataaagcagatgaacttccgttaatcatcgaactggtgagcaaagataaaaaatatgttatctgccacgccgattatccctttgacgaatacgagtttggaaagccagttgatcatcagcaggtaatctggaaccgcgaacgaatcagcaactcacaaaacgggatcgtgaaagaaatcaaaggcgcggacacgttcatctttggtcatacgccagcagtgaaaccactcaagtttgccaaccaaatgtatatcgataccggcgcagtgttctgcggaaacctaacattgattcaggtacagggagaaggcgcatgagactcgaaagcgtagctaaatttcattcgccaaaaagcccgatgatgagcgactcaccacgggccacggcttctgactctctttccggtactgatgtgatggctgctatggggatggcgcaatcacaagccggattcggtatggctgcattctgcggtaagcacgaactcagccagaacgacaaacaaaaggctatcaactatctgatgcaatttgcacacaaggtatcggggaaataccgtggtgtggcaaagcttgaaggaaatactaaggcaaaggtactgcaagtgctcgcaacattcgcttatgcggattattgccgtagtgccgcgacgccgggggcaagatgcagagattgccatggtacaggccgtgcggttgatattgccaaaacagagctgtgggggagagttgtcgagaaagagtgcggaagatgcaaaggcgtcggctattcaaggatgccagcaagcgcagcatatcgcgctgtgacgatgctaatcccaaaccttacccaacccacctggtcacgcactgttaagccgctgtatgacgctctggtggtgcaatgccacaaagaagagtcaatcgcagacaacattttgaatgcggtcacacgttagcagcatgattgccacggatggcaacatattaacggcatgatattgacttattgaataaaattgggtaaatttgactcaacgatgggttaattcgctcgttgtggtagtgagatgaaaagaggcggcgcttactaccgattccgcctagttggtcacttcgacgtatcgtctggaactccaaccatcgcaggcagagaggtctgcaaaatgcaatcccgaaacagttcgcaggtaatagttagagcctgcataacggtttcgggattttttatatctgcacaacaggtaagagcattgagtcgataatcgtgaagagtcggcgagcctggttagccagtgctctttccgttgtgctgaattaagcgaataccggaagcagaaccggatcaccaaatgcgtacaggcgtcatcgccgcccagcaacagcacaacccaaactgagccgtagccactgtctgtcctgaattcattagtaatagttacgctgcggccttttacacatgaccttcgtgaaagcgggtggcaggaggtcgcgctaacaacctcctgccgttttgcccgtgcatatcggtcacgaacaaatctgattactaaacacagtagcctggatttgttctatcagtaatcgaccttattcctaattaaatagagcaaatccccttattgggggtaagacatgaagatgccagaaaaacatgacctgttggccgccattctcgcggcaaaggaacaaggcatcggggcaatccttgcgtttgcaatggcgtaccttcgcggcagatataatggcggtgcgtttacaaaaacagtaatcgacgcaacgatgtgcgccattatcgcctggttcattcgtgaccttctcgacttcgccggactaagtagcaatctcgcttatataacgagcgtgtttatcggctacatcggtactgactcgattggttcgcttatcaaacgcttcgctgctaaaaaagccggagtagaagatggtagaaatcaataatcaacgtaaggcgttcctcgatatgctggcgtggtcggagggaactgataacggacgtcagaaaaccagaaatcatggttatgacgtcattgtaggcggagagctatttactgattactccgatcaccctcgcaaacttgtcacgctaaacccaaaactcaaatcaacaggcgcttaagactggccgtcgttttacaacacagaaagagtttgtagaaacgcaaaaaggccatccgtcaggggccttctgcttagtttgatgcctggcagttccctactctcgccttccgcttcctcgctcactgactcgctgcgctcggtcgttcggctgcggcgagcggtatcagctcactcaaaggcggtaatacggttatccacagaatcaggggataacgcaggaaagaacatgtgagcaaaaggccagcaaaaggccaggaaccgtaaaaaggccgcgttgctggcgtttttccataggctccgcccccctgacgagcatcacaaaaatcgacgctcaagtcagaggtggcgaaacccgacaggactataaagataccaggcgtttccccctggaagctccctcgtgcgctctcctgttccgaccctgccgcttaccggatacctgtccgcctttctcccttcgggaagcgtggcgctttctcatagctcacgctgtaggtatctcagttcggtgtaggtcgttcgctccaagctgggctgtgtgcacgaaccccccgttcagcccgaccgctgcgccttatccggtaactatcgtcttgagtccaacccggtaagacacgacttatcgccactggcagcagccactggtaacaggattagcagagcgaggtatgtaggcggtgctacagagttcttgaagtggtgggctaactacggctacactagaagaacagtatttggtatctgcgctctgctgaagccagttaccttcggaaaaagagttggtagctcttgatccggcaaacaaaccaccgctggtagcggtggtttttttgtttgcaagcagcagattacgcgcagaaaaaaaggatctcaagaagatcctttgatcttttctacggggtctgacgctcagtggaacgacgcgcgcgtaactcacgttaagggattttggtcatgagcttgcgccgtcccgtcaagtcagcgtaatgctctgcttttagaaaaactcatcgagcatcaaatgaaactgcaatttattcatatcaggattatcaataccatatttttgaaaaagccgtttctgtaatgaaggagaaaactcaccgaggcagttccataggatggcaagatcctggtatcggtctgcgattccgactcgtccaacatcaatacaacctattaatttcccctcgtcaaaaataaggttatcaagtgagaaatcaccatgagtgacgactgaatccggtgagaatggcaaaagtttatgcatttctttccagacttgttcaacaggccagccattacgctcgtcatcaaaatcactcgcatcaaccaaaccgttattcattcgtgattgcgcctgagcgaggcgaaatacgcgatcgctgttaaaaggacaattacaaacaggaatcgagtgcaaccggcgcaggaacactgccagcgcatcaacaatattttcacctgaatcaggatattcttctaatacctggaacgctgtttttccggggatcgcagtggtgagtaaccatgcatcatcaggagtacggataaaatgcttgatggtcggaagtggcataaattccgtcagccagtttagtctgaccatctcatctgtaacatcattggcaacgctacctttgccatgtttcagaaacaactctggcgcatcgggcttcccatacaagcgatagattgtcgcacctgattgcccgacattatcgcgagcccatttatacccatataaatcagcatccatgttggaatttaatcgcggcctcgacgtttcccgttgaatatggctcatattcttcctttttcaatattattgaagcatttatcagggttattgtctcatgagcggatacatatttgaatgtatttagaaaaataaacaaataggggtcagtgttacaaccaattaaccaattctgaacattatcgcgagcccatttatacctgaatatggctcataacaccccttgtttgcctggcggcagtagcgcggtggtcccacctgaccccatgccgaactcagaagtgaaacgccgtagcgccgatggtagtgtggggactccccatgcgagagtagggaactgccaggcatcaaataaaacgaaaggctcagtcgaaagactgggcctttcgcccgggctaattagggggtgtcgcccttattcgactctatagtgaagttcctattctctagaaagtataggaacttctgaagtggggtcgacttaattaagg

SEQ ID NO: 31 - DNA, 11041 bp, Artificial Sequence
  constructed sequence
ctgcgcgctcgctcgctcactgaggccgcccgggcaaagcccgggcgtcgggcgacctttggtcgcccggcctcagtgagcgagcgagcgcgcagagagggagtggccaactccatcactaggggttccttgtagttaatgattaacccgccatgctacttatctacgtagcaagctagcaagatccaagctcagatctcgatcgagttgggccccagaagcctggtggttgtttgtccttctcaggggaaaagtgaggcggccccttggaggaaggggccgggcagaatgatctaatcggattccaagcagctcaggggattgtctttttctagcaccttcttgccactcctaagcgtcctccgtgaccccggctgggatttagcctggtgctgtgtcagccccggtctcccaggggcttcccagtggtccccaggaaccctcgacagggcccggtctctctcgtccagcaagggcagggacgggccacaggccaagggccctcgatcgaggaactgaaaaaccagaaagttaactggtaagtttagtctttttgtcttttatttcaggtcccggatccggtggtggtgcaaatcaaagaactgctcctcagtggatgttgcctttacttctaggcctgtacggaagtgttacttctgctctaaaagctgcggaattgtacccgcggccgccaccatggctaagattaacacccagtactcacatccatcccgcactcacctcaaagtcaagacctccgatcgggatctgaaccgggctgagaatgggctgtcgcgcgcccactcgtcgtccgaggaaaccagcagcgtgctccagccgggcatcgccatggaaactagggggctggcggactccggacagggatccttcactggacagggtattgcccggctgagcagactgatcttcctgcttcgccgctgggcggccagacacgtgcaccatcaggaccagggacctgatagcttccccgaccgctttaggggagccgagctgaaagaagtgtcaagccaggagtcaaacgcgcaggccaacgtcggcagccaagagcctgcagaccggggacgctcggcatggccgctcgcaaagtgcaacactaacacttccaacaacaccgaagaggaaaagaaaaccaagaagaaggatgcaattgtggtggacccttcctccaacctgtactaccgctggttgaccgccatcgccctcccggtcttttacaattggtatctccttatctgccgggcctgcttcgacgaactgcaatcagagtacctgatgctgtggctggtgctggactatagcgccgatgtgctctacgtcctggatgtgctcgtgcgcgcccggaccggattcttggaacaaggcctgatggtgtccgacacgaatagactgtggcagcactataagaccacaacccagttcaagcttgacgtgctcagccttgtgccgactgacctggcctacctgaaagtcggaactaactacccggaagtcagattcaaccgactcctgaagttcagcaggctgttcgagttctttgaccgcaccgagactcggaccaactaccctaacatgttccggatcggaaatctggtgctctacatactgattatcatccattggaacgcctgtatctatttcgccatttcgaagttcatcggtttcggaaccgattcctgggtgtaccccaacatctcgatccccgaacacggtcgcctgtcccggaagtacatctactccctgtactggtccactctgactctgaccacgatcggggaaacccctccacccgtgaaggacgaagagtacctgttcgtggtggtggacttcctggtcggagtgttgattttcgccaccattgtgggaaacgtgggctccatgatctccaacatgaacgcgtcgagagctgagttccaagccaagatcgactccattaagcagtacatgcagttcagaaaggtcaccaaggacctggaaaccagggtcatccgctggttcgactacctgtgggccaacaaaaagactgtggacgaaaaggaagtgctgaagtcgctgccggataagctgaaggccgaaatcgccattaacgtgcaccttgacaccctgaagaaagtccggatcttccaagactgtgaagccggcctcctggtggagctcgtgctcaagctgcggcccaccgtgttcagcccgggagattacatttgcaagaagggcgatatcggcaaagagatgtacatcatcaacgagggaaagctggccgtggtcgcggacgacggcgtgacccagttcgtggtgctgtccgacggatcctacttcggtgaaatctcaatcctcaacatcaaggggtccaagtccggcaaccggagaactgccaacattcgctccatcggatacagcgacctgttttgcctgtccaaggatgacctgatggaggctctgactgagtaccctgaagcgaagaaggctttggaggaaaaggggcggcagattctgatgaaggacaatttgatcgacgaggagctcgcacgggccggcgccgaccccaaggatctcgaagagaaggtcgaacagctgggttcttcgcttgataccctgcaaacccgattcgcgcggctgctcgccgagtacaacgcgacccagatgaagatgaagcagagactgtcacagttggaatcccaagtcaagggcggaggcgacaagccgctggcggacggggaagtgcccggggacgccaccaagactgaggacaagcagcagtgatcatagatcgatctgcctcgactgtgccttctagttgccagccatctgttgtttgcccctcccccgtgccttccttgaccctggaaggtgccactcccactgtcctttcctaataaaatgaggaaattgcatcgcattgtctgagtaggtgtcattctattctggggggtggggtggggcaggacagcaagggggaggattgggaagacaatagcaggcatgctggggactcgagttctacgtagataagtagcatggcgggttaatcattaactacaaggaacccctagtgatggagttggccactccctctctgcgcgctcgctcgctcactgaggccgggcgaccaaaggtcgcccgacgcccgggctttgcccgggcggcctcagtgagcgagcgagcgcgcagccttaattaacctaaggaaaatgaagtgaagttcctatactttctagagaataggaacttctatagtgagtcgaataagggcgacacaaaatttattctaaatgcataataaatactgataacatcttatagtttgtattatattttgtattatcgttgacatgtataattttgatatcaaaaactgattttccctttattattttcgagatttattttcttaattctctttaacaaactagaaatattgtatatacaaaaaatcataaataatagatgaatagtttaattataggtgttcatcaatcgaaaaagcaacgtatcttatttaaagtgcgttgcttttttctcatttataaggttaaataattctcatatatcaagcaaagtgacaggcgcccttaaatattctgacaaatgctctttccctaaactccccccataaaaaaacccgccgaagcgggtttttacgttatttgcggattaacgattactcgttatcagaaccgcccagggggcccgagcttaacctttttatttgggggagagggaagtcatgaaaaaactaacctttgaaattcgatctccagcacatcagcaaaacgctattcacgcagtacagcaaatccttccagacccaaccaaaccaatcgtagtaaccattcaggaacgcaaccgcagcttagaccaaaacaggaagctatgggcctgcttaggtgacgtctctcgtcaggttgaatggcatggtcgctggctggatgcagaaagctggaagtgtgtgtttaccgcagcattaaagcagcaggatgttgttcctaaccttgccgggaatggctttgtggtaataggccagtcaaccagcaggatgcgtgtaggcgaatttgcggagctattagagcttatacaggcattcggtacagagcgtggcgttaagtggtcagacgaagcgagactggctctggagtggaaagcgagatggggagacagggctgcatgataaatgtcgttagtttctccggtggcaggacgtcagcatatttgctctggctaatggagcaaaagcgacgggcaggtaaagacgtgcattacgttttcatggatacaggttgtgaacatccaatgacatatcggtttgtcagggaagttgtgaagttctgggatataccgctcaccgtattgcaggttgatatcaacccggagcttggacagccaaatggttatacggtatgggaaccaaaggatattcagacgcgaatgcctgttctgaagccatttatcgatatggtaaagaaatatggcactccatacgtcggcggcgcgttctgcactgacagattaaaactcgttcccttcaccaaatactgtgatgaccatttcgggcgagggaattacaccacgtggattggcatcagagctgatgaaccgaagcggctaaagccaaagcctggaatcagatatcttgctgaactgtcagactttgagaaggaagatatcctcgcatggtggaagcaacaaccattcgatttgcaaataccggaacatctcggtaactgcatattctgcattaaaaaatcaacgcaaaaaatcggacttgcctgcaaagatgaggagggattgcagcgtgtttttaatgaggtcatcacgggatcccatgtgcgtgacggacatcgggaaacgccaaaggagattatgtaccgaggaagaatgtcgctggacggtatcgcgaaaatgtattcagaaaatgattatcaagccctgtatcaggacatggtacgagctaaaagattcgataccggctcttgttctgagtcatgcgaaatatttggagggcagcttgatttcgacttcgggagggaagctgcatgatgcgatgttatcggtgcggtgaatgcaaagaagataaccgcttccgaccaaatcaaccttactggaatcgatggtgtctccggtgtgaaagaacaccaacaggggtgttaccactaccgcaggaaaaggaggacgtgtggcgagacagcgacgaagtatcaccgacataatctgcgaaaactgcaaataccttccaacgaaacgcaccagaaataaacccaagccaatcccaaaagaatctgacgtaaaaaccttcaactacacggctcacctgtgggatatccggtggctaagacgtcgtgcgaggaaaacaaggtgattgaccaaaatcgaagttacgaacaagaaagcgtcgagcgagctttaacgtgcgctaactgcggtcagaagctgcatgtgctggaagttcacgtgtgtgagcactgctgcgcagaactgatgagcgatccgaatagctcgatgcacgaggaagaagatgatggctaaaccagcgcgaagacgatgtaaaaacgatgaatgccgggaatggtttcaccctgcattcgctaatcagtggtggtgctctccagagtgtggaaccaagatagcactcgaacgacgaagtaaagaacgcgaaaaagcggaaaaagcagcagagaagaaacgacgacgagaggagcagaaacagaaagataaacttaagattcgaaaactcgccttaaagccccgcagttactggattaaacaagcccaacaagccgtaaacgccttcatcagagaaagagaccgcgacttaccatgtatctcgtgcggaacgctcacgtctgctcagtgggatgccggacattaccggacaactgctgcggcacctcaactccgatttaatgaacgcaatattcacaagcaatgcgtggtgtgcaaccagcacaaaagcggaaatctcgttccgtatcgcgtcgaactgattagccgcatcgggcaggaagcagtagacgaaatcgaatcaaaccataaccgccatcgctggactatcgaagagtgcaaggcgatcaaggcagagtaccaacagaaactcaaagacctgcgaaatagcagaagtgaggccgcatgacgttctcagtaaaaaccattccagacatgctcgttgaagcatacggaaatcagacagaagtagcacgcagactgaaatgtagtcgcggtacggtcagaaaatacgttgatgataaagacgggaaaatgcacgccatcgtcaacgacgttctcatggttcatcgcggatggagtgaaagagatgcgctattacgaaaaaattgatggcagcaaataccgaaatatttgggtagttggcgatctgcacggatgctacacgaacctgatgaacaaactggatacgattggattcgacaacaaaaaagacctgcttatctcggtgggcgatttggttgatcgtggtgcagagaacgttgaatgcctggaattaatcacattcccctggttcagagctgtacgtggaaaccatgagcaaatgatgattgatggcttatcagagcgtggaaacgttaatcactggctgcttaatggcggtggctggttctttaatctcgattacgacaaagaaattctggctaaagctcttgcccataaagcagatgaacttccgttaatcatcgaactggtgagcaaagataaaaaatatgttatctgccacgccgattatccctttgacgaatacgagtttggaaagccagttgatcatcagcaggtaatctggaaccgcgaacgaatcagcaactcacaaaacgggatcgtgaaagaaatcaaaggcgcggacacgttcatctttggtcatacgccagcagtgaaaccactcaagtttgccaaccaaatgtatatcgataccggcgcagtgttctgcggaaacctaacattgattcaggtacagggagaaggcgcatgagactcgaaagcgtagctaaatttcattcgccaaaaagcccgatgatgagcgactcaccacgggccacggcttctgactctctttccggtactgatgtgatggctgctatggggatggcgcaatcacaagccggattcggtatggctgcattctgcggtaagcacgaactcagccagaacgacaaacaaaaggctatcaactatctgatgcaatttgcacacaaggtatcggggaaataccgtggtgtggcaaagcttgaaggaaatactaaggcaaaggtactgcaagtgctcgcaacattcgcttatgcggattattgccgtagtgccgcgacgccgggggcaagatgcagagattgccatggtacaggccgtgcggttgatattgccaaaacagagctgtgggggagagttgtcgagaaagagtgcggaagatgcaaaggcgtcggctattcaaggatgccagcaagcgcagcatatcgcgctgtgacgatgctaatcccaaaccttacccaacccacctggtcacgcactgttaagccgctgtatgacgctctggtggtgcaatgccacaaagaagagtcaatcgcagacaacattttgaatgcggtcacacgttagcagcatgattgccacggatggcaacatattaacggcatgatattgacttattgaataaaattgggtaaatttgactcaacgatgggttaattcgctcgttgtggtagtgagatgaaaagaggcggcgcttactaccgattccgcctagttggtcacttcgacgtatcgtctggaactccaaccatcgcaggcagagaggtctgcaaaatgcaatcccgaaacagttcgcaggtaatagttagagcctgcataacggtttcgggattttttatatctgcacaacaggtaagagcattgagtcgataatcgtgaagagtcggcgagcctggttagccagtgctctttccgttgtgctgaattaagcgaataccggaagcagaaccggatcaccaaatgcgtacaggcgtcatcgccgcccagcaacagcacaacccaaactgagccgtagccactgtctgtcctgaattcattagtaatagttacgctgcggccttttacacatgaccttcgtgaaagcgggtggcaggaggtcgcgctaacaacctcctgccgttttgcccgtgcatatcggtcacgaacaaatctgattactaaacacagtagcctggatttgttctatcagtaatcgaccttattcctaattaaatagagcaaatccccttattgggggtaagacatgaagatgccagaaaaacatgacctgttggccgccattctcgcggcaaaggaacaaggcatcggggcaatccttgcgtttgcaatggcgtaccttcgcggcagatataatggcggtgcgtttacaaaaacagtaatcgacgcaacgatgtgcgccattatcgcctggttcattcgtgaccttctcgacttcgccggactaagtagcaatctcgcttatataacgagcgtgtttatcggctacatcggtactgactcgattggttcgcttatcaaacgcttcgctgctaaaaaagccggagtagaagatggtagaaatcaataatcaacgtaaggcgttcctcgatatgctggcgtggtcggagggaactgataacggacgtcagaaaaccagaaatcatggttatgacgtcattgtaggcggagagctatttactgattactccgatcaccctcgcaaacttgtcacgctaaacccaaaactcaaatcaacaggcgcttaagactggccgtcgttttacaacacagaaagagtttgtagaaacgcaaaaaggccatccgtcaggggccttctgcttagtttgatgcctggcagttccctactctcgccttccgcttcctcgctcactgactcgctgcgctcggtcgttcggctgcggcgagcggtatcagctcactcaaaggcggtaatacggttatccacagaatcaggggataacgcaggaaagaacatgtgagcaaaaggccagcaaaaggccaggaaccgtaaaaaggccgcgttgctggcgtttttccataggctccgcccccctgacgagcatcacaaaaatcgacgctcaagtcagaggtggcgaaacccgacaggactataaagataccaggcgtttccccctggaagctccctcgtgcgctctcctgttccgaccctgccgcttaccggatacctgtccgcctttctcccttcgggaagcgtggcgctttctcatagctcacgctgtaggtatctcagttcggtgtaggtcgttcgctccaagctgggctgtgtgcacgaaccccccgttcagcccgaccgctgcgccttatccggtaactatcgtcttgagtccaacccggtaagacacgacttatcgccactggcagcagccactggtaacaggattagcagagcgaggtatgtaggcggtgctacagagttcttgaagtggtgggctaactacggctacactagaagaacagtatttggtatctgcgctctgctgaagccagttaccttcggaaaaagagttggtagctcttgatccggcaaacaaaccaccgctggtagcggtggtttttttgtttgcaagcagcagattacgcgcagaaaaaaaggatctcaagaagatcctttgatcttttctacggggtctgacgctcagtggaacgacgcgcgcgtaactcacgttaagggattttggtcatgagcttgcgccgtcccgtcaagtcagcgtaatgctctgcttttagaaaaactcatcgagcatcaaatgaaactgcaatttattcatatcaggattatcaataccatatttttgaaaaagccgtttctgtaatgaaggagaaaactcaccgaggcagttccataggatggcaagatcctggtatcggtctgcgattccgactcgtccaacatcaatacaacctattaatttcccctcgtcaaaaataaggttatcaagtgagaaatcaccatgagtgacgactgaatccggtgagaatggcaaaagtttatgcatttctttccagacttgttcaacaggccagccattacgctcgtcatcaaaatcactcgcatcaaccaaaccgttattcattcgtgattgcgcctgagcgaggcgaaatacgcgatcgctgttaaaaggacaattacaaacaggaatcgagtgcaaccggcgcaggaacactgccagcgcatcaacaatattttcacctgaatcaggatattcttctaatacctggaacgctgtttttccggggatcgcagtggtgagtaaccatgcatcatcaggagtacggataaaatgcttgatggtcggaagtggcataaattccgtcagccagtttagtctgaccatctcatctgtaacatcattggcaacgctacctttgccatgtttcagaaacaactctggcgcatcgggcttcccatacaagcgatagattgtcgcacctgattgcccgacattatcgcgagcccatttatacccatataaatcagcatccatgttggaatttaatcgcggcctcgacgtttcccgttgaatatggctcatattcttcctttttcaatattattgaagcatttatcagggttattgtctcatgagcggatacatatttgaatgtatttagaaaaataaacaaataggggtcagtgttacaaccaattaaccaattctgaacattatcgcgagcccatttatacctgaatatggctcataacaccccttgtttgcctggcggcagtagcgcggtggtcccacctgaccccatgccgaactcagaagtgaaacgccgtagcgccgatggtagtgtggggactccccatgcgagagtagggaactgccaggcatcaaataaaacgaaaggctcagtcgaaagactgggcctttcgcccgggctaattagggggtgtcgcccttattcgactctatagtgaagttcctattctctagaaagtataggaacttctgaagtggggtcgacttaattaagg

SEQ ID NO: 32 - DNA, 11206 bp, Artificial Sequence
  constructed sequence
ctgcgcgctcgctcgctcactgaggccgcccgggcaaagcccgggcgtcgggcgacctttggtcgcccggcctcagtgagcgagcgagcgcgcagagagggagtggccaactccatcactaggggttccttgtagttaatgattaacccgccatgctacttatctacgtagcaagctagcaagatccaagctcagatctcgatcgagttgggccccagaagcctggtggttgtttgtccttctcaggggaaaagtgaggcggccccttggaggaaggggccgggcagaatgatctaatcggattccaagcagctcaggggattgtctttttctagcaccttcttgccactcctaagcgtcctccgtgaccccggctgggatttagcctggtgctgtgtcagccccggtctcccaggggcttcccagtggtccccaggaaccctcgacagggcccggtctctctcgtccagcaagggcagggacgggccacaggccaagggccctcgatcgaggaactgaaaaaccagaaagttaactggtaagtttagtctttttgtcttttatttcaggtcccggatccggtggtggtgcaaatcaaagaactgctcctcagtggatgttgcctttacttctaggcctgtacggaagtgttacttctgctctaaaagctgcggaattgtacccgcggccgccaccatggctaagattaacacccagtactcacatccatcccgcactcacctcaaagtcaagacctccgatcgggatctgaaccgggctgagaatgggctgtcgcgcgcccactcgtcgtccgaggaaaccagcagcgtgctccagccgggcatcgccatggaaactagggggctggcggactccggacagggatccttcactggacagggtattgcccggttcgggcggattcagaagaagtcccagccggagaaggtcgtgcgggctgccagcaggggcaggccactcattggttggacacagtggtgcgctgaggatggtggagatgaatcggaaatggcactggccggctctcccggatgcagctcgggcccccaagggagactgagcagactgatcttcctgcttcgccgctgggcggccagacacgtgcaccatcaggaccagggacctgatagcttccccgaccgctttaggggagccgagctgaaagaagtgtcaagccaggagtcaaacgcgcaggccaacgtcggcagccaagagcctgcagaccggggacgctcggcatggccgctcgcaaagtgcaacactaacacttccaacaacaccgaagaggaaaagaaaaccaagaagaaggatgcaattgtggtggacccttcctccaacctgtactaccgctggttgaccgccatcgccctcccggtcttttacaattggtatctccttatctgccgggcctgcttcgacgaactgcaatcagagtacctgatgctgtggctggtgctggactatagcgccgatgtgctctacgtcctggatgtgctcgtgcgcgcccggaccggattcttggaacaaggcctgatggtgtccgacacgaatagactgtggcagcactataagaccacaacccagttcaagcttgacgtgctcagccttgtgccgactgacctggcctacctgaaagtcggaactaactacccggaagtcagattcaaccgactcctgaagttcagcaggctgttcgagttctttgaccgcaccgagactcggaccaactaccctaacatgttccggatcggaaatctggtgctctacatactgattatcatccattggaacgcctgtatctatttcgccatttcgaagttcatcggtttcggaaccgattcctgggtgtaccccaacatctcgatccccgaacacggtcgcctgtcccggaagtacatctactccctgtactggtccactctgactctgaccacgatcggggaaacccctccacccgtgaaggacgaagagtacctgttcgtggtggtggacttcctggtcggagtgttgattttcgccaccattgtgggaaacgtgggctccatgatctccaacatgaacgcgtcgagagctgagttccaagccaagatcgactccattaagcagtacatgcagttcagaaaggtcaccaaggacctggaaaccagggtcatccgctggttcgactacctgtgggccaacaaaaagactgtggacgaaaaggaagtgctgaagtcgctgccggataagctgaaggccgaaatcgccattaacgtgcaccttgacaccctgaagaaagtccggatcttccaagactgtgaagccggcctcctggtggagctcgtgctcaagctgcggcccaccgtgttcagcccgggagattacatttgcaagaagggcgatatcggcaaagagatgtacatcatcaacgagggaaagctggccgtggtcgcggacgacggcgtgacccagttcgtggtgctgtccgacggatcctacttcggtgaaatctcaatcctcaacatcaaggggtccaagtccggcaaccggagaactgccaacattcgctccatcggatacagcgacctgttttgcctgtccaaggatgacctgatggaggctctgactgagtaccctgaagcgaagaaggctttggaggaaaaggggcggcagattctgatgaaggacaatttgatcgacgaggagctcgcacgggccggcgccgaccccaaggatctcgaagagaaggtcgaacagctgggttcttcgcttgataccctgcaaacccgattcgcgcggctgctcgccgagtacaacgcgacccagatgaagatgaagcagagactgtcacagttggaatcccaagtcaagggcggaggcgacaagccgctggcggacggggaagtgcccggggacgccaccaagactgaggacaagcagcagtgatcatagatcgatctgcctcgactgtgccttctagttgccagccatctgttgtttgcccctcccccgtgccttccttgaccctggaaggtgccactcccactgtcctttcctaataaaatgaggaaattgcatcgcattgtctgagtaggtgtcattctattctggggggtggggtggggcaggacagcaagggggaggattgggaagacaatagcaggcatgctggggactcgagttctacgtagataagtagcatggcgggttaatcattaactacaaggaacccctagtgatggagttggccactccctctctgcgcgctcgctcgctcactgaggccgggcgaccaaaggtcgcccgacgcccgggctttgcccgggcggcctcagtgagcgagcgagcgcgcagccttaattaacctaaggaaaatgaagtgaagttcctatactttctagagaataggaacttctatagtgagtcgaataagggcgacacaaaatttattctaaatgcataataaatactgataacatcttatagtttgtattatattttgtattatcgttgacatgtataattttgatatcaaaaactgattttccctttattattttcgagatttattttcttaattctctttaacaaactagaaatattgtatatacaaaaaatcataaataatagatgaatagtttaattataggtgttcatcaatcgaaaaagcaacgtatcttatttaaagtgcgttgcttttttctcatttataaggttaaataattctcatatatcaagcaaagtgacaggcgcccttaaatattctgacaaatgctctttccctaaactccccccataaaaaaacccgccgaagcgggtttttacgttatttgcggattaacgattactcgttatcagaaccgcccagggggcccgagcttaacctttttatttgggggagagggaagtcatgaaaaaactaacctttgaaattcgatctccagcacatcagcaaaacgctattcacgcagtacagcaaatccttccagacccaaccaaaccaatcgtagtaaccattcaggaacgcaaccgcagcttagaccaaaacaggaagctatgggcctgcttaggtgacgtctctcgtcaggttgaatggcatggtcgctggctggatgcagaaagctggaagtgtgtgtttaccgcagcattaaagcagcaggatgttgttcctaaccttgccgggaatggctttgtggtaataggccagtcaaccagcaggatgcgtgtaggcgaatttgcggagctattagagcttatacaggcattcggtacagagcgtggcgttaagtggtcagacgaagcgagactggctctggagtggaaagcgagatggggagacagggctgcatgataaatgtcgttagtttctccggtggcaggacgtcagcatatttgctctggctaatggagcaaaagcgacgggcaggtaaagacgtgcattacgttttcatggatacaggttgtgaacatccaatgacatatcggtttgtcagggaagttgtgaagttctgggatataccgctcaccgtattgcaggttgatatcaacccggagcttggacagccaaatggttatacggtatgggaaccaaaggatattcagacgcgaatgcctgttctgaagccatttatcgatatggtaaagaaatatggcactccatacgtcggcggcgcgttctgcactgacagattaaaactcgttcccttcaccaaatactgtgatgaccatttcgggcgagggaattacaccacgtggattggcatcagagctgatgaaccgaagcggctaaagccaaagcctggaatcagatatcttgctgaactgtcagactttgagaaggaagatatcctcgcatggtggaagcaacaaccattcgatttgcaaataccggaacatctcggtaactgcatattctgcattaaaaaatcaacgcaaaaaatcggacttgcctgcaaagatgaggagggattgcagcgtgtttttaatgaggtcatcacgggatcccatgtgcgtgacggacatcgggaaacgccaaaggagattatgtaccgaggaagaatgtcgctggacggtatcgcgaaaatgtattcagaaaatgattatcaagccctgtatcaggacatggtacgagctaaaagattcgataccggctcttgttctgagtcatgcgaaatatttggagggcagcttgatttcgacttcgggagggaagctgcatgatgcgatgttatcggtgcggtgaatgcaaagaagataaccgcttccgaccaaatcaaccttactggaatcgatggtgtctccggtgtgaaagaacaccaacaggggtgttaccactaccgcaggaaaaggaggacgtgtggcgagacagcgacgaagtatcaccgacataatctgcgaaaactgcaaataccttccaacgaaacgcaccagaaataaacccaagccaatcccaaaagaatctgacgtaaaaaccttcaactacacggctcacctgtgggatatccggtggctaagacgtcgtgcgaggaaaacaaggtgattgaccaaaatcgaagttacgaacaagaaagcgtcgagcgagctttaacgtgcgctaactgcggtcagaagctgcatgtgctggaagttcacgtgtgtgagcactgctgcgcagaactgatgagcgatccgaatagctcgatgcacgaggaagaagatgatggctaaaccagcgcgaagacgatgtaaaaacgatgaatgccgggaatggtttcaccctgcattcgctaatcagtggtggtgctctccagagtgtggaaccaagatagcactcgaacgacgaagtaaagaacgcgaaaaagcggaaaaagcagcagagaagaaacgacgacgagaggagcagaaacagaaagataaacttaagattcgaaaactcgccttaaagccccgcagttactggattaaacaagcccaacaagccgtaaacgccttcatcagagaaagagaccgcgacttaccatgtatctcgtgcggaacgctcacgtctgctcagtgggatgccggacattaccggacaactgctgcggcacctcaactccgatttaatgaacgcaatattcacaagcaatgcgtggtgtgcaaccagcacaaaagcggaaatctcgttccgtatcgcgtcgaactgattagccgcatcgggcaggaagcagtagacgaaatcgaatcaaaccataaccgccatcgctggactatcgaagagtgcaaggcgatcaaggcagagtaccaacagaaactcaaagacctgcgaaatagcagaagtgaggccgcatgacgttctcagtaaaaaccattccagacatgctcgttgaagcatacggaaatcagacagaagtagcacgcagactgaaatgtagtcgcggtacggtcagaaaatacgttgatgataaagacgggaaaatgcacgccatcgtcaacgacgttctcatggttcatcgcggatggagtgaaagagatgcgctattacgaaaaaattgatggcagcaaataccgaaatatttgggtagttggcgatctgcacggatgctacacgaacctgatgaacaaactggatacgattggattcgacaacaaaaaagacctgcttatctcggtgggcgatttggttgatcgtggtgcagagaacgttgaatgcctggaattaatcacattcccctggttcagagctgtacgtggaaaccatgagcaaatgatgattgatggcttatcagagcgtggaaacgttaatcactggctgcttaatggcggtggctggttctttaatctcgattacgacaaagaaattctggctaaagctcttgcccataaagcagatgaacttccgttaatcatcgaactggtgagcaaagataaaaaatatgttatctgccacgccgattatccctttgacgaatacgagtttggaaagccagttgatcatcagcaggtaatctggaaccgcgaacgaatcagcaactcacaaaacgggatcgtgaaagaaatcaaaggcgcggacacgttcatctttggtcatacgccagcagtgaaaccactcaagtttgccaaccaaatgtatatcgataccggcgcagtgttctgcggaaacctaacattgattcaggtacagggagaaggcgcatgagactcgaaagcgtagctaaatttcattcgccaaaaagcccgatgatgagcgactcaccacgggccacggcttctgactctctttccggtactgatgtgatggctgctatggggatggcgcaatcacaagccggattcggtatggctgcattctgcggtaagcacgaactcagccagaacgacaaacaaaaggctatcaactatctgatgcaatttgcacacaaggtatcggggaaataccgtggtgtggcaaagcttgaaggaaatactaaggcaaaggtactgcaagtgctcgcaacattcgcttatgcggattattgccgtagtgccgcgacgccgggggcaagatgcagagattgccatggtacaggccgtgcggttgatattgccaaaacagagctgtgggggagagttgtcgagaaagagtgcggaagatgcaaaggcgtcggctattcaaggatgccagcaagcgcagcatatcgcgctgtgacgatgctaatcccaaaccttacccaacccacctggtcacgcactgttaagccgctgtatgacgctctggtggtgcaatgccacaaagaagagtcaatcgcagacaacattttgaatgcggtcacacgttagcagcatgattgccacggatggcaacatattaacggcatgatattgacttattgaataaaattgggtaaatttgactcaacgatgggttaattcgctcgttgtggtagtgagatgaaaagaggcggcgcttactaccgattccgcctagttggtcacttcgacgtatcgtctggaactccaaccatcgcaggcagagaggtctgcaaaatgcaatcccgaaacagttcgcaggtaatagttagagcctgcataacggtttcgggattttttatatctgcacaacaggtaagagcattgagtcgataatcgtgaagagtcggcgagcctggttagccagtgctctttccgttgtgctgaattaagcgaataccggaagcagaaccggatcaccaaatgcgtacaggcgtcatcgccgcccagcaacagcacaacccaaactgagccgtagccactgtctgtcctgaattcattagtaatagttacgctgcggccttttacacatgaccttcgtgaaagcgggtggcaggaggtcgcgctaacaacctcctgccgttttgcccgtgcatatcggtcacgaacaaatctgattactaaacacagtagcctggatttgttctatcagtaatcgaccttattcctaattaaatagagcaaatccccttattgggggtaagacatgaagatgccagaaaaacatgacctgttggccgccattctcgcggcaaaggaacaaggcatcggggcaatccttgcgtttgcaatggcgtaccttcgcggcagatataatggcggtgcgtttacaaaaacagtaatcgacgcaacgatgtgcgccattatcgcctggttcattcgtgaccttctcgacttcgccggactaagtagcaatctcgcttatataacgagcgtgtttatcggctacatcggtactgactcgattggttcgcttatcaaacgcttcgctgctaaaaaagccggagtagaagatggtagaaatcaataatcaacgtaaggcgttcctcgatatgctggcgtggtcggagggaactgataacggacgtcagaaaaccagaaatcatggttatgacgtcattgtaggcggagagctatttactgattactccgatcaccctcgcaaacttgtcacgctaaacccaaaactcaaatcaacaggcgcttaagactggccgtcgttttacaacacagaaagagtttgtagaaacgcaaaaaggccatccgtcaggggccttctgcttagtttgatgcctggcagttccctactctcgccttccgcttcctcgctcactgactcgctgcgctcggtcgttcggctgcggcgagcggtatcagctcactcaaaggcggtaatacggttatccacagaatcaggggataacgcaggaaagaacatgtgagcaaaaggccagcaaaaggccaggaaccgtaaaaaggccgcgttgctggcgtttttccataggctccgcccccctgacgagcatcacaaaaatcgacgctcaagtcagaggtggcgaaacccgacaggactataaagataccaggcgtttccccctggaagctccctcgtgcgctctcctgttccgaccctgccgcttaccggatacctgtccgcctttctcccttcgggaagcgtggcgctttctcatagctcacgctgtaggtatctcagttcggtgtaggtcgttcgctccaagctgggctgtgtgcacgaaccccccgttcagcccgaccgctgcgccttatccggtaactatcgtcttgagtccaacccggtaagacacgacttatcgccactggcagcagccactggtaacaggattagcagagcgaggtatgtaggcggtgctacagagttcttgaagtggtgggctaactacggctacactagaagaacagtatttggtatctgcgctctgctgaagccagttaccttcggaaaaagagttggtagctcttgatccggcaaacaaaccaccgctggtagcggtggtttttttgtttgcaagcagcagattacgcgcagaaaaaaaggatctcaagaagatcctttgatcttttctacggggtctgacgctcagtggaacgacgcgcgcgtaactcacgttaagggattttggtcatgagcttgcgccgtcccgtcaagtcagcgtaatgctctgcttttagaaaaactcatcgagcatcaaatgaaactgcaatttattcatatcaggattatcaataccatatttttgaaaaagccgtttctgtaatgaaggagaaaactcaccgaggcagttccataggatggcaagatcctggtatcggtctgcgattccgactcgtccaacatcaatacaacctattaatttcccctcgtcaaaaataaggttatcaagtgagaaatcaccatgagtgacgactgaatccggtgagaatggcaaaagtttatgcatttctttccagacttgttcaacaggccagccattacgctcgtcatcaaaatcactcgcatcaaccaaaccgttattcattcgtgattgcgcctgagcgaggcgaaatacgcgatcgctgttaaaaggacaattacaaacaggaatcgagtgcaaccggcgcaggaacactgccagcgcatcaacaatattttcacctgaatcaggatattcttctaatacctggaacgctgtttttccggggatcgcagtggtgagtaaccatgcatcatcaggagtacggataaaatgcttgatggtcggaagtggcataaattccgtcagccagtttagtctgaccatctcatctgtaacatcattggcaacgctacctttgccatgtttcagaaacaactctggcgcatcgggcttcccatacaagcgatagattgtcgcacctgattgcccgacattatcgcgagcccatttatacccatataaatcagcatccatgttggaatttaatcgcggcctcgacgtttcccgttgaatatggctcatattcttcctttttcaatattattgaagcatttatcagggttattgtctcatgagcggatacatatttgaatgtatttagaaaaataaacaaataggggtcagtgttacaaccaattaaccaattctgaacattatcgcgagcccatttatacctgaatatggctcataacaccccttgtttgcctggcggcagtagcgcggtggtcccacctgaccccatgccgaactcagaagtgaaacgccgtagcgccgatggtagtgtggggactccccatgcgagagtagggaactgccaggcatcaaataaaacgaaaggctcagtcgaaagactgggcctttcgcccgggctaattagggggtgtcgcccttattcgactctatagtgaagttcctattctctagaaagtataggaacttctgaagtggggtcgacttaattaagg

SEQ ID NO: 33 - DNA, 11435 bp, Artificial Sequence
  constructed sequence
ctgcgcgctcgctcgctcactgaggccgcccgggcaaagcccgggcgtcgggcgacctttggtcgcccggcctcagtgagcgagcgagcgcgcagagagggagtggccaactccatcactaggggttccttgtagttaatgattaacccgccatgctacttatctacgtagcaagctagcctgaagagacagaaatatctctaattccatgagcggtcatacgaggcaagagaagccgcttagagcatggacttagttagtttcagggattggacagagtcaagagctggggtgaggaggttaccctcggtaggggtgacacagatgtcaaccgcctattccctccacatgcatgtcctgccagaagaacctgtccctgggctgggaatcttatattaccttcctctccaatgagaagagaagttcaaggctcacagacatgtgcatacacaagctcaatgcactcaagattcccctccaccactcctgcccccactacctacaggagattgactcctgctgtgcacataagctgggataatcagggtttctaaacatcagcttcaaaagtccaatgtccaaagtggtggggggccggggaacgaggtactctttccatacccttggcttttgtgtggcctggagccgctgatatagagattggagtgggacacgaggtattcctttcaaaaacacaaaggcctatactttgagccctcccatttcaatcccccaccatgcttcacctttaagacctccaactccactttgatcccagttctcaggttcaggcctcacaaggccaaaatcctgaagttacccttctcaaactcccttgcctttaacatcatcagaatcaacctcctacccccactctgtcccagcagcaatagcctgctaatcttttagcactaatcttttaggcactaatctgctttccaaactcttggcacctgaactatttataagcagtgttttatgcccccccaccaaagaaccctattcttttcccatgaccccaccaatcaaaacactcagaggactgtgggtataagaggctggggaggcaggcatagcagcggccgccaccatggccaagatcaacacccaatactcccacccctccaggacccacctcaaggtaaagacctcagaccgggatctcaatcgcgctgaaaatggcctcagcagagcccactcgtcaagtgaggagacatcgtcagtgctgcagccggggatcgccatggagaccagaggactggctgactccgggcagggctccttcaccggccaggggatcgccaggctgtcgcgcctcatcttcttgctgcgcaggtgggctgccaggcatgtgcaccaccaggaccagggaccggactcttttcctgatcgtttccgtggagccgagcttaaggaggtgtccagccaagaaagcaatgcccaggcaaatgtgggcagccaggagccagcagacagagggagaagcgcctggcccctggccaaatgcaacactaacaccagcaacaacacggaggaggagaagaagacgaaaaagaaggatgcgatcgtggtggacccgtccagcaacctgtactaccgctggctgaccgccatcgccctgcctgtcttctataactggtatctgcttatttgcagggcctgtttcgatgagctgcagtccgagtacctgatgctgtggctggtcctggactactcggcagatgtcctgtatgtcttggatgtgcttgtacgagctcggacaggttttcttgagcaaggcttaatggtcagtgataccaacaggctgtggcagcattacaagacgaccacgcagttcaagctggatgtgttgtccctggtccccaccgacctggcttacttaaaggtgggcacaaactacccagaagtgaggttcaaccgcctactgaagttttcccggctctttgaattctttgaccgcacagagacaaggaccaactaccccaatatgttcaggattgggaacttggtcttgtacattctcatcatcatccactggaatgcctgcatctactttgccatttccaagttcattggttttgggacagactcctgggtctacccaaacatctcaatcccagagcatgggcgcctctccaggaagtacatttacagtctctactggtccaccttgacccttaccaccattggtgagaccccaccccccgtgaaagatgaggagtatctctttgtggtcgtagacttcttggtgggtgttctgatttttgccaccattgtgggcaatgtgggctccatgatctcgaatatgaatgcctcacgggcagagttccaggccaagattgattccatcaagcagtacatgcagttccgcaaggtcaccaaggacttggagacgcgggttatccggtggtttgactacctgtgggccaacaagaagacggtggatgagaaggaggtgctcaagagcctcccagacaagctgaaggctgagatcgccatcaacgtgcacctggacacgctgaagaaggttcgcatcttccaggactgtgaggcagggctgctggtggagctggtgctgaagctgcgacccactgtgttcagccctggggattatatctgcaagaagggagatattgggaaggagatgtacatcatcaacgagggcaagctggccgtggtggctgatgatggggtcacccagttcgtggtcctcagcgatggcagctacttcggggagatcagcattctgaacatcaaggggagcaagtcggggaaccgcaggacggccaacatccgcagcattggctactcagacctgttctgcctctcaaaggacgatctcatggaggccctcaccgagtaccccgaagccaagaaggccctggaggagaaaggacggcagatcctgatgaaagacaacctgatcgatgaggagctggccagggcgggcgcggaccccaaggaccttgaggagaaagtggagcagctggggtcctccctggacaccctgcagaccaggtttgcacgcctcctggctgagtacaacgccacccagatgaagatgaagcagcgtctcagccaactggaaagccaggtgaagggtggtggggacaagcccctggctgatggggaagttcccggggatgctacaaaaacagaggacaaacaacagtgatcatagatcgatctgcctcgactgtgccttctagttgccagccatctgttgtttgcccctcccccgtgccttccttgaccctggaaggtgccactcccactgtcctttcctaataaaatgaggaaattgcatcgcattgtctgagtaggtgtcattctattctggggggtggggtggggcaggacagcaagggggaggattgggaagacaatagcaggcatgctggggactcgagttctacgtagataagtagcatggcgggttaatcattaactacaaggaacccctagtgatggagttggccactccctctctgcgcgctcgctcgctcactgaggccgggcgaccaaaggtcgcccgacgcccgggctttgcccgggcggcctcagtgagcgagcgagcgcgcagccttaattaacctaaggaaaatgaagtgaagttcctatactttctagagaataggaacttctatagtgagtcgaataagggcgacacaaaatttattctaaatgcataataaatactgataacatcttatagtttgtattatattttgtattatcgttgacatgtataattttgatatcaaaaactgattttccctttattattttcgagatttattttcttaattctctttaacaaactagaaatattgtatatacaaaaaatcataaataatagatgaatagtttaattataggtgttcatcaatcgaaaaagcaacgtatcttatttaaagtgcgttgcttttttctcatttataaggttaaataattctcatatatcaagcaaagtgacaggcgcccttaaatattctgacaaatgctctttccctaaactccccccataaaaaaacccgccgaagcgggtttttacgttatttgcggattaacgattactcgttatcagaaccgcccagggggcccgagcttaacctttttatttgggggagagggaagtcatgaaaaaactaacctttgaaattcgatctccagcacatcagcaaaacgctattcacgcagtacagcaaatccttccagacccaaccaaaccaatcgtagtaaccattcaggaacgcaaccgcagcttagaccaaaacaggaagctatgggcctgcttaggtgacgtctctcgtcaggttgaatggcatggtcgctggctggatgcagaaagctggaagtgtgtgtttaccgcagcattaaagcagcaggatgttgttcctaaccttgccgggaatggctttgtggtaataggccagtcaaccagcaggatgcgtgtaggcgaatttgcggagctattagagcttatacaggcattcggtacagagcgtggcgttaagtggtcagacgaagcgagactggctctggagtggaaagcgagatggggagacagggctgcatgataaatgtcgttagtttctccggtggcaggacgtcagcatatttgctctggctaatggagcaaaagcgacgggcaggtaaagacgtgcattacgttttcatggatacaggttgtgaacatccaatgacatatcggtttgtcagggaagttgtgaagttctgggatataccgctcaccgtattgcaggttgatatcaacccggagcttggacagccaaatggttatacggtatgggaaccaaaggatattcagacgcgaatgcctgttctgaagccatttatcgatatggtaaagaaatatggcactccatacgtcggcggcgcgttctgcactgacagattaaaactcgttcccttcaccaaatactgtgatgaccatttcgggcgagggaattacaccacgtggattggcatcagagctgatgaaccgaagcggctaaagccaaagcctggaatcagatatcttgctgaactgtcagactttgagaaggaagatatcctcgcatggtggaagcaacaaccattcgatttgcaaataccggaacatctcggtaactgcatattctgcattaaaaaatcaacgcaaaaaatcggacttgcctgcaaagatgaggagggattgcagcgtgtttttaatgaggtcatcacgggatcccatgtgcgtgacggacatcgggaaacgccaaaggagattatgtaccgaggaagaatgtcgctggacggtatcgcgaaaatgtattcagaaaatgattatcaagccctgtatcaggacatggtacgagctaaaagattcgataccggctcttgttctgagtcatgcgaaatatttggagggcagcttgatttcgacttcgggagggaagctgcatgatgcgatgttatcggtgcggtgaatgcaaagaagataaccgcttccgaccaaatcaaccttactggaatcgatggtgtctccggtgtgaaagaacaccaacaggggtgttaccactaccgcaggaaaaggaggacgtgtggcgagacagcgacgaagtatcaccgacataatctgcgaaaactgcaaataccttccaacgaaacgcaccagaaataaacccaagccaatcccaaaagaatctgacgtaaaaaccttcaactacacggctcacctgtgggatatccggtggctaagacgtcgtgcgaggaaaacaaggtgattgaccaaaatcgaagttacgaacaagaaagcgtcgagcgagctttaacgtgcgctaactgcggtcagaagctgcatgtgctggaagttcacgtgtgtgagcactgctgcgcagaactgatgagcgatccgaatagctcgatgcacgaggaagaagatgatggctaaaccagcgcgaagacgatgtaaaaacgatgaatgccgggaatggtttcaccctgcattcgctaatcagtggtggtgctctccagagtgtggaaccaagatagcactcgaacgacgaagtaaagaacgcgaaaaagcggaaaaagcagcagagaagaaacgacgacgagaggagcagaaacagaaagataaacttaagattcgaaaactcgccttaaagccccgcagttactggattaaacaagcccaacaagccgtaaacgccttcatcagagaaagagaccgcgacttaccatgtatctcgtgcggaacgctcacgtctgctcagtgggatgccggacattaccggacaactgctgcggcacctcaactccgatttaatgaacgcaatattcacaagcaatgcgtggtgtgcaaccagcacaaaagcggaaatctcgttccgtatcgcgtcgaactgattagccgcatcgggcaggaagcagtagacgaaatcgaatcaaaccataaccgccatcgctggactatcgaagagtgcaaggcgatcaaggcagagtaccaacagaaactcaaagacctgcgaaatagcagaagtgaggccgcatgacgttctcagtaaaaaccattccagacatgctcgttgaagcatacggaaatcagacagaagtagcacgcagactgaaatgtagtcgcggtacggtcagaaaatacgttgatgataaagacgggaaaatgcacgccatcgtcaacgacgttctcatggttcatcgcggatggagtgaaagagatgcgctattacgaaaaaattgatggcagcaaataccgaaatatttgggtagttggcgatctgcacggatgctacacgaacctgatgaacaaactggatacgattggattcgacaacaaaaaagacctgcttatctcggtgggcgatttggttgatcgtggtgcagagaacgttgaatgcctggaattaatcacattcccctggttcagagctgtacgtggaaaccatgagcaaatgatgattgatggcttatcagagcgtggaaacgttaatcactggctgcttaatggcggtggctggttctttaatctcgattacgacaaagaaattctggctaaagctcttgcccataaagcagatgaacttccgttaatcatcgaactggtgagcaaagataaaaaatatgttatctgccacgccgattatccctttgacgaatacgagtttggaaagccagttgatcatcagcaggtaatctggaaccgcgaacgaatcagcaactcacaaaacgggatcgtgaaagaaatcaaaggcgcggacacgttcatctttggtcatacgccagcagtgaaaccactcaagtttgccaaccaaatgtatatcgataccggcgcagtgttctgcggaaacctaacattgattcaggtacagggagaaggcgcatgagactcgaaagcgtagctaaatttcattcgccaaaaagcccgatgatgagcgactcaccacgggccacggcttctgactctctttccggtactgatgtgatggctgctatggggatggcgcaatcacaagccggattcggtatggctgcattctgcggtaagcacgaactcagccagaacgacaaacaaaaggctatcaactatctgatgcaatttgcacacaaggtatcggggaaataccgtggtgtggcaaagcttgaaggaaatactaaggcaaaggtactgcaagtgctcgcaacattcgcttatgcggattattgccgtagtgccgcgacgccgggggcaagatgcagagattgccatggtacaggccgtgcggttgatattgccaaaacagagctgtgggggagagttgtcgagaaagagtgcggaagatgcaaaggcgtcggctattcaaggatgccagcaagcgcagcatatcgcgctgtgacgatgctaatcccaaaccttacccaacccacctggtcacgcactgttaagccgctgtatgacgctctggtggtgcaatgccacaaagaagagtcaatcgcagacaacattttgaatgcggtcacacgttagcagcatgattgccacggatggcaacatattaacggcatgatattgacttattgaataaaattgggtaaatttgactcaacgatgggttaattcgctcgttgtggtagtgagatgaaaagaggcggcgcttactaccgattccgcctagttggtcacttcgacgtatcgtctggaactccaaccatcgcaggcagagaggtctgcaaaatgcaatcccgaaacagttcgcaggtaatagttagagcctgcataacggtttcgggattttttatatctgcacaacaggtaagagcattgagtcgataatcgtgaagagtcggcgagcctggttagccagtgctctttccgttgtgctgaattaagcgaataccggaagcagaaccggatcaccaaatgcgtacaggcgtcatcgccgcccagcaacagcacaacccaaactgagccgtagccactgtctgtcctgaattcattagtaatagttacgctgcggccttttacacatgaccttcgtgaaagcgggtggcaggaggtcgcgctaacaacctcctgccgttttgcccgtgcatatcggtcacgaacaaatctgattactaaacacagtagcctggatttgttctatcagtaatcgaccttattcctaattaaatagagcaaatccccttattgggggtaagacatgaagatgccagaaaaacatgacctgttggccgccattctcgcggcaaaggaacaaggcatcggggcaatccttgcgtttgcaatggcgtaccttcgcggcagatataatggcggtgcgtttacaaaaacagtaatcgacgcaacgatgtgcgccattatcgcctggttcattcgtgaccttctcgacttcgccggactaagtagcaatctcgcttatataacgagcgtgtttatcggctacatcggtactgactcgattggttcgcttatcaaacgcttcgctgctaaaaaagccggagtagaagatggtagaaatcaataatcaacgtaaggcgttcctcgatatgctggcgtggtcggagggaactgataacggacgtcagaaaaccagaaatcatggttatgacgtcattgtaggcggagagctatttactgattactccgatcaccctcgcaaacttgtcacgctaaacccaaaactcaaatcaacaggcgcttaagactggccgtcgttttacaacacagaaagagtttgtagaaacgcaaaaaggccatccgtcaggggccttctgcttagtttgatgcctggcagttccctactctcgccttccgcttcctcgctcactgactcgctgcgctcggtcgttcggctgcggcgagcggtatcagctcactcaaaggcggtaatacggttatccacagaatcaggggataacgcaggaaagaacatgtgagcaaaaggccagcaaaaggccaggaaccgtaaaaaggccgcgttgctggcgtttttccataggctccgcccccctgacgagcatcacaaaaatcgacgctcaagtcagaggtggcgaaacccgacaggactataaagataccaggcgtttccccctggaagctccctcgtgcgctctcctgttccgaccctgccgcttaccggatacctgtccgcctttctcccttcgggaagcgtggcgctttctcatagctcacgctgtaggtatctcagttcggtgtaggtcgttcgctccaagctgggctgtgtgcacgaaccccccgttcagcccgaccgctgcgccttatccggtaactatcgtcttgagtccaacccggtaagacacgacttatcgccactggcagcagccactggtaacaggattagcagagcgaggtatgtaggcggtgctacagagttcttgaagtggtgggctaactacggctacactagaagaacagtatttggtatctgcgctctgctgaagccagttaccttcggaaaaagagttggtagctcttgatccggcaaacaaaccaccgctggtagcggtggtttttttgtttgcaagcagcagattacgcgcagaaaaaaaggatctcaagaagatcctttgatcttttctacggggtctgacgctcagtggaacgacgcgcgcgtaactcacgttaagggattttggtcatgagcttgcgccgtcccgtcaagtcagcgtaatgctctgcttttagaaaaactcatcgagcatcaaatgaaactgcaatttattcatatcaggattatcaataccatatttttgaaaaagccgtttctgtaatgaaggagaaaactcaccgaggcagttccataggatggcaagatcctggtatcggtctgcgattccgactcgtccaacatcaatacaacctattaatttcccctcgtcaaaaataaggttatcaagtgagaaatcaccatgagtgacgactgaatccggtgagaatggcaaaagtttatgcatttctttccagacttgttcaacaggccagccattacgctcgtcatcaaaatcactcgcatcaaccaaaccgttattcattcgtgattgcgcctgagcgaggcgaaatacgcgatcgctgttaaaaggacaattacaaacaggaatcgagtgcaaccggcgcaggaacactgccagcgcatcaacaatattttcacctgaatcaggatattcttctaatacctggaacgctgtttttccggggatcgcagtggtgagtaaccatgcatcatcaggagtacggataaaatgcttgatggtcggaagtggcataaattccgtcagccagtttagtctgaccatctcatctgtaacatcattggcaacgctacctttgccatgtttcagaaacaactctggcgcatcgggcttcccatacaagcgatagattgtcgcacctgattgcccgacattatcgcgagcccatttatacccatataaatcagcatccatgttggaatttaatcgcggcctcgacgtttcccgttgaatatggctcatattcttcctttttcaatattattgaagcatttatcagggttattgtctcatgagcggatacatatttgaatgtatttagaaaaataaacaaataggggtcagtgttacaaccaattaaccaattctgaacattatcgcgagcccatttatacctgaatatggctcataacaccccttgtttgcctggcggcagtagcgcggtggtcccacctgaccccatgccgaactcagaagtgaaacgccgtagcgccgatggtagtgtggggactccccatgcgagagtagggaactgccaggcatcaaataaaacgaaaggctcagtcgaaagactgggcctttcgcccgggctaattagggggtgtcgcccttattcgactctatagtgaagttcctattctctagaaagtataggaacttctgaagtggggtcgacttaattaagg

SEQ ID NO: 34 - DNA, 11432 bp, Artificial Sequence
  constructed sequence
ctgcgcgctcgctcgctcactgaggccgcccgggcaaagcccgggcgtcgggcgacctttggtcgcccggcctcagtgagcgagcgagcgcgcagagagggagtggccaactccatcactaggggttccttgtagttaatgattaacccgccatgctacttatctacgtagcaagctagcctgaagagacagaaatatctctaattccatgagcggtcatacgaggcaagagaagccgcttagagcatggacttagttagtttcagggattggacagagtcaagagctggggtgaggaggttaccctcggtaggggtgacacagatgtcaaccgcctattccctccacatgcatgtcctgccagaagaacctgtccctgggctgggaatcttatattaccttcctctccaatgagaagagaagttcaaggctcacagacatgtgcatacacaagctcaatgcactcaagattcccctccaccactcctgcccccactacctacaggagattgactcctgctgtgcacataagctgggataatcagggtttctaaacatcagcttcaaaagtccaatgtccaaagtggtggggggccggggaacgaggtactctttccatacccttggcttttgtgtggcctggagccgctgatatagagattggagtgggacacgaggtattcctttcaaaaacacaaaggcctatactttgagccctcccatttcaatcccccaccatgcttcacctttaagacctccaactccactttgatcccagttctcaggttcaggcctcacaaggccaaaatcctgaagttacccttctcaaactcccttgcctttaacatcatcagaatcaacctcctacccccactctgtcccagcagcaatagcctgctaatcttttagcactaatcttttaggcactaatctgctttccaaactcttggcacctgaactatttataagcagtgttttatgcccccccaccaaagaaccctattcttttcccatgaccccaccaatcaaaacactcagaggactgtgggtataagaggctggggaggcaggcatagcagcggccgccaccatggctaagattaacacccagtactcacatccatcccgcactcacctcaaagtcaagacctccgatcgggatctgaaccgggctgagaatgggctgtcgcgcgcccactcgtcgtccgaggaaaccagcagcgtgctccagccgggcatcgccatggaaactagggggctggcggactccggacagggatccttcactggacagggtattgcccggctgagcagactgatcttcctgcttcgccgctgggcggccagacacgtgcaccatcaggaccagggacctgatagcttccccgaccgctttaggggagccgagctgaaagaagtgtcaagccaggagtcaaacgcgcaggccaacgtcggcagccaagagcctgcagaccggggacgctcggcatggccgctcgcaaagtgcaacactaacacttccaacaacaccgaagaggaaaagaaaaccaagaagaaggatgcaattgtggtggacccttcctccaacctgtactaccgctggttgaccgccatcgccctcccggtcttttacaattggtatctccttatctgccgggcctgcttcgacgaactgcaatcagagtacctgatgctgtggctggtgctggactatagcgccgatgtgctctacgtcctggatgtgctcgtgcgcgcccggaccggattcttggaacaaggcctgatggtgtccgacacgaatagactgtggcagcactataagaccacaacccagttcaagcttgacgtgctcagccttgtgccgactgacctggcctacctgaaagtcggaactaactacccggaagtcagattcaaccgactcctgaagttcagcaggctgttcgagttctttgaccgcaccgagactcggaccaactaccctaacatgttccggatcggaaatctggtgctctacatactgattatcatccattggaacgcctgtatctatttcgccatttcgaagttcatcggtttcggaaccgattcctgggtgtaccccaacatctcgatccccgaacacggtcgcctgtcccggaagtacatctactccctgtactggtccactctgactctgaccacgatcggggaaacccctccacccgtgaaggacgaagagtacctgttcgtggtggtggacttcctggtcggagtgttgattttcgccaccattgtgggaaacgtgggctccatgatctccaacatgaacgcgtcgagagctgagttccaagccaagatcgactccattaagcagtacatgcagttcagaaaggtcaccaaggacctggaaaccagggtcatccgctggttcgactacctgtgggccaacaaaaagactgtggacgaaaaggaagtgctgaagtcgctgccggataagctgaaggccgaaatcgccattaacgtgcaccttgacaccctgaagaaagtccggatcttccaagactgtgaagccggcctcctggtggagctcgtgctcaagctgcggcccaccgtgttcagcccgggagattacatttgcaagaagggcgatatcggcaaagagatgtacatcatcaacgagggaaagctggccgtggtcgcggacgacggcgtgacccagttcgtggtgctgtccgacggatcctacttcggtgaaatctcaatcctcaacatcaaggggtccaagtccggcaaccggagaactgccaacattcgctccatcggatacagcgacctgttttgcctgtccaaggatgacctgatggaggctctgactgagtaccctgaagcgaagaaggctttggaggaaaaggggcggcagattctgatgaaggacaatttgatcgacgaggagctcgcacgggccggcgccgaccccaaggatctcgaagagaaggtcgaacagctgggttcttcgcttgataccctgcaaacccgattcgcgcggctgctcgccgagtacaacgcgacccagatgaagatgaagcagagactgtcacagttggaatcccaagtcaagggcggaggcgacaagccgctggcggacggggaagtgcccggggacgccaccaagactgaggacaagcagcagtgatcatagatcctgcctcgactgtgccttctagttgccagccatctgttgtttgcccctcccccgtgccttccttgaccctggaaggtgccactcccactgtcctttcctaataaaatgaggaaattgcatcgcattgtctgagtaggtgtcattctattctggggggtggggtggggcaggacagcaagggggaggattgggaagacaatagcaggcatgctggggactcgagttctacgtagataagtagcatggcgggttaatcattaactacaaggaacccctagtgatggagttggccactccctctctgcgcgctcgctcgctcactgaggccgggcgaccaaaggtcgcccgacgcccgggctttgcccgggcggcctcagtgagcgagcgagcgcgcagccttaattaacctaaggaaaatgaagtgaagttcctatactttctagagaataggaacttctatagtgagtcgaataagggcgacacaaaatttattctaaatgcataataaatactgataacatcttatagtttgtattatattttgtattatcgttgacatgtataattttgatatcaaaaactgattttccctttattattttcgagatttattttcttaattctctttaacaaactagaaatattgtatatacaaaaaatcataaataatagatgaatagtttaattataggtgttcatcaatcgaaaaagcaacgtatcttatttaaagtgcgttgcttttttctcatttataaggttaaataattctcatatatcaagcaaagtgacaggcgcccttaaatattctgacaaatgctctttccctaaactccccccataaaaaaacccgccgaagcgggtttttacgttatttgcggattaacgattactcgttatcagaaccgcccagggggcccgagcttaacctttttatttgggggagagggaagtcatgaaaaaactaacctttgaaattcgatctccagcacatcagcaaaacgctattcacgcagtacagcaaatccttccagacccaaccaaaccaatcgtagtaaccattcaggaacgcaaccgcagcttagaccaaaacaggaagctatgggcctgcttaggtgacgtctctcgtcaggttgaatggcatggtcgctggctggatgcagaaagctggaagtgtgtgtttaccgcagcattaaagcagcaggatgttgttcctaaccttgccgggaatggctttgtggtaataggccagtcaaccagcaggatgcgtgtaggcgaatttgcggagctattagagcttatacaggcattcggtacagagcgtggcgttaagtggtcagacgaagcgagactggctctggagtggaaagcgagatggggagacagggctgcatgataaatgtcgttagtttctccggtggcaggacgtcagcatatttgctctggctaatggagcaaaagcgacgggcaggtaaagacgtgcattacgttttcatggatacaggttgtgaacatccaatgacatatcggtttgtcagggaagttgtgaagttctgggatataccgctcaccgtattgcaggttgatatcaacccggagcttggacagccaaatggttatacggtatgggaaccaaaggatattcagacgcgaatgcctgttctgaagccatttatcgatatggtaaagaaatatggcactccatacgtcggcggcgcgttctgcactgacagattaaaactcgttcccttcaccaaatactgtgatgaccatttcgggcgagggaattacaccacgtggattggcatcagagctgatgaaccgaagcggctaaagccaaagcctggaatcagatatcttgctgaactgtcagactttgagaaggaagatatcctcgcatggtggaagcaacaaccattcgatttgcaaataccggaacatctcggtaactgcatattctgcattaaaaaatcaacgcaaaaaatcggacttgcctgcaaagatgaggagggattgcagcgtgtttttaatgaggtcatcacgggatcccatgtgcgtgacggacatcgggaaacgccaaaggagattatgtaccgaggaagaatgtcgctggacggtatcgcgaaaatgtattcagaaaatgattatcaagccctgtatcaggacatggtacgagctaaaagattcgataccggctcttgttctgagtcatgcgaaatatttggagggcagcttgatttcgacttcgggagggaagctgcatgatgcgatgttatcggtgcggtgaatgcaaagaagataaccgcttccgaccaaatcaaccttactggaatcgatggtgtctccggtgtgaaagaacaccaacaggggtgttaccactaccgcaggaaaaggaggacgtgtggcgagacagcgacgaagtatcaccgacataatctgcgaaaactgcaaataccttccaacgaaacgcaccagaaataaacccaagccaatcccaaaagaatctgacgtaaaaaccttcaactacacggctcacctgtgggatatccggtggctaagacgtcgtgcgaggaaaacaaggtgattgaccaaaatcgaagttacgaacaagaaagcgtcgagcgagctttaacgtgcgctaactgcggtcagaagctgcatgtgctggaagttcacgtgtgtgagcactgctgcgcagaactgatgagcgatccgaatagctcgatgcacgaggaagaagatgatggctaaaccagcgcgaagacgatgtaaaaacgatgaatgccgggaatggtttcaccctgcattcgctaatcagtggtggtgctctccagagtgtggaaccaagatagcactcgaacgacgaagtaaagaacgcgaaaaagcggaaaaagcagcagagaagaaacgacgacgagaggagcagaaacagaaagataaacttaagattcgaaaactcgccttaaagccccgcagttactggattaaacaagcccaacaagccgtaaacgccttcatcagagaaagagaccgcgacttaccatgtatctcgtgcggaacgctcacgtctgctcagtgggatgccggacattaccggacaactgctgcggcacctcaactccgatttaatgaacgcaatattcacaagcaatgcgtggtgtgcaaccagcacaaaagcggaaatctcgttccgtatcgcgtcgaactgattagccgcatcgggcaggaagcagtagacgaaatcgaatcaaaccataaccgccatcgctggactatcgaagagtgcaaggcgatcaaggcagagtaccaacagaaactcaaagacctgcgaaatagcagaagtgaggccgcatgacgttctcagtaaaaaccattccagacatgctcgttgaagcatacggaaatcagacagaagtagcacgcagactgaaatgtagtcgcggtacggtcagaaaatacgttgatgataaagacgggaaaatgcacgccatcgtcaacgacgttctcatggttcatcgcggatggagtgaaagagatgcgctattacgaaaaaattgatggcagcaaataccgaaatatttgggtagttggcgatctgcacggatgctacacgaacctgatgaacaaactggatacgattggattcgacaacaaaaaagacctgcttatctcggtgggcgatttggttgatcgtggtgcagagaacgttgaatgcctggaattaatcacattcccctggttcagagctgtacgtggaaaccatgagcaaatgatgattgatggcttatcagagcgtggaaacgttaatcactggctgcttaatggcggtggctggttctttaatctcgattacgacaaagaaattctggctaaagctcttgcccataaagcagatgaacttccgttaatcatcgaactggtgagcaaagataaaaaatatgttatctgccacgccgattatccctttgacgaatacgagtttggaaagccagttgatcatcagcaggtaatctggaaccgcgaacgaatcagcaactcacaaaacgggatcgtgaaagaaatcaaaggcgcggacacgttcatctttggtcatacgccagcagtgaaaccactcaagtttgccaaccaaatgtatatcgataccggcgcagtgttctgcggaaacctaacattgattcaggtacagggagaaggcgcatgagactcgaaagcgtagctaaatttcattcgccaaaaagcccgatgatgagcgactcaccacgggccacggcttctgactctctttccggtactgatgtgatggctgctatggggatggcgcaatcacaagccggattcggtatggctgcattctgcggtaagcacgaactcagccagaacgacaaacaaaaggctatcaactatctgatgcaatttgcacacaaggtatcggggaaataccgtggtgtggcaaagcttgaaggaaatactaaggcaaaggtactgcaagtgctcgcaacattcgcttatgcggattattgccgtagtgccgcgacgccgggggcaagatgcagagattgccatggtacaggccgtgcggttgatattgccaaaacagagctgtgggggagagttgtcgagaaagagtgcggaagatgcaaaggcgtcggctattcaaggatgccagcaagcgcagcatatcgcgctgtgacgatgctaatcccaaaccttacccaacccacctggtcacgcactgttaagccgctgtatgacgctctggtggtgcaatgccacaaagaagagtcaatcgcagacaacattttgaatgcggtcacacgttagcagcatgattgccacggatggcaacatattaacggcatgatattgacttattgaataaaattgggtaaatttgactcaacgatgggttaattcgctcgttgtggtagtgagatgaaaagaggcggcgcttactaccgattccgcctagttggtcacttcgacgtatcgtctggaactccaaccatcgcaggcagagaggtctgcaaaatgcaatcccgaaacagttcgcaggtaatagttagagcctgcataacggtttcgggattttttatatctgcacaacaggtaagagcattgagtcgataatcgtgaagagtcggcgagcctggttagccagtgctctttccgttgtgctgaattaagcgaataccggaagcagaaccggatcaccaaatgcgtacaggcgtcatcgccgcccagcaacagcacaacccaaactgagccgtagccactgtctgtcctgaattcattagtaatagttacgctgcggccttttacacatgaccttcgtgaaagcgggtggcaggaggtcgcgctaacaacctcctgccgttttgcccgtgcatatcggtcacgaacaaatctgattactaaacacagtagcctggatttgttctatcagtaatcgaccttattcctaattaaatagagcaaatccccttattgggggtaagacatgaagatgccagaaaaacatgacctgttggccgccattctcgcggcaaaggaacaaggcatcggggcaatccttgcgtttgcaatggcgtaccttcgcggcagatataatggcggtgcgtttacaaaaacagtaatcgacgcaacgatgtgcgccattatcgcctggttcattcgtgaccttctcgacttcgccggactaagtagcaatctcgcttatataacgagcgtgtttatcggctacatcggtactgactcgattggttcgcttatcaaacgcttcgctgctaaaaaagccggagtagaagatggtagaaatcaataatcaacgtaaggcgttcctcgatatgctggcgtggtcggagggaactgataacggacgtcagaaaaccagaaatcatggttatgacgtcattgtaggcggagagctatttactgattactccgatcaccctcgcaaacttgtcacgctaaacccaaaactcaaatcaacaggcgcttaagactggccgtcgttttacaacacagaaagagtttgtagaaacgcaaaaaggccatccgtcaggggccttctgcttagtttgatgcctggcagttccctactctcgccttccgcttcctcgctcactgactcgctgcgctcggtcgttcggctgcggcgagcggtatcagctcactcaaaggcggtaatacggttatccacagaatcaggggataacgcaggaaagaacatgtgagcaaaaggccagcaaaaggccaggaaccgtaaaaaggccgcgttgctggcgtttttccataggctccgcccccctgacgagcatcacaaaaatcgacgctcaagtcagaggtggcgaaacccgacaggactataaagataccaggcgtttccccctggaagctccctcgtgcgctctcctgttccgaccctgccgcttaccggatacctgtccgcctttctcccttcgggaagcgtggcgctttctcatagctcacgctgtaggtatctcagttcggtgtaggtcgttcgctccaagctgggctgtgtgcacgaaccccccgttcagcccgaccgctgcgccttatccggtaactatcgtcttgagtccaacccggtaagacacgacttatcgccactggcagcagccactggtaacaggattagcagagcgaggtatgtaggcggtgctacagagttcttgaagtggtgggctaactacggctacactagaagaacagtatttggtatctgcgctctgctgaagccagttaccttcggaaaaagagttggtagctcttgatccggcaaacaaaccaccgctggtagcggtggtttttttgtttgcaagcagcagattacgcgcagaaaaaaaggatctcaagaagatcctttgatcttttctacggggtctgacgctcagtggaacgacgcgcgcgtaactcacgttaagggattttggtcatgagcttgcgccgtcccgtcaagtcagcgtaatgctctgcttttagaaaaactcatcgagcatcaaatgaaactgcaatttattcatatcaggattatcaataccatatttttgaaaaagccgtttctgtaatgaaggagaaaactcaccgaggcagttccataggatggcaagatcctggtatcggtctgcgattccgactcgtccaacatcaatacaacctattaatttcccctcgtcaaaaataaggttatcaagtgagaaatcaccatgagtgacgactgaatccggtgagaatggcaaaagtttatgcatttctttccagacttgttcaacaggccagccattacgctcgtcatcaaaatcactcgcatcaaccaaaccgttattcattcgtgattgcgcctgagcgaggcgaaatacgcgatcgctgttaaaaggacaattacaaacaggaatcgagtgcaaccggcgcaggaacactgccagcgcatcaacaatattttcacctgaatcaggatattcttctaatacctggaacgctgtttttccggggatcgcagtggtgagtaaccatgcatcatcaggagtacggataaaatgcttgatggtcggaagtggcataaattccgtcagccagtttagtctgaccatctcatctgtaacatcattggcaacgctacctttgccatgtttcagaaacaactctggcgcatcgggcttcccatacaagcgatagattgtcgcacctgattgcccgacattatcgcgagcccatttatacccatataaatcagcatccatgttggaatttaatcgcggcctcgacgtttcccgttgaatatggctcatattcttcctttttcaatattattgaagcatttatcagggttattgtctcatgagcggatacatatttgaatgtatttagaaaaataaacaaataggggtcagtgttacaaccaattaaccaattctgaacattatcgcgagcccatttatacctgaatatggctcataacaccccttgtttgcctggcggcagtagcgcggtggtcccacctgaccccatgccgaactcagaagtgaaacgccgtagcgccgatggtagtgtggggactccccatgcgagagtagggaactgccaggcatcaaataaaacgaaaggctcagtcgaaagactgggcctttcgcccgggctaattagggggtgtcgcccttattcgactctatagtgaagttcctattctctagaaagtataggaacttctgaagtggggtcgacttaattaagg

SEQ ID NO: 35 - DNA, 11600 bp, Artificial Sequence
  constructed sequence
ctgcgcgctcgctcgctcactgaggccgcccgggcaaagcccgggcgtcgggcgacctttggtcgcccggcctcagtgagcgagcgagcgcgcagagagggagtggccaactccatcactaggggttccttgtagttaatgattaacccgccatgctacttatctacgtagcaagctagcctgaagagacagaaatatctctaattccatgagcggtcatacgaggcaagagaagccgcttagagcatggacttagttagtttcagggattggacagagtcaagagctggggtgaggaggttaccctcggtaggggtgacacagatgtcaaccgcctattccctccacatgcatgtcctgccagaagaacctgtccctgggctgggaatcttatattaccttcctctccaatgagaagagaagttcaaggctcacagacatgtgcatacacaagctcaatgcactcaagattcccctccaccactcctgcccccactacctacaggagattgactcctgctgtgcacataagctgggataatcagggtttctaaacatcagcttcaaaagtccaatgtccaaagtggtggggggccggggaacgaggtactctttccatacccttggcttttgtgtggcctggagccgctgatatagagattggagtgggacacgaggtattcctttcaaaaacacaaaggcctatactttgagccctcccatttcaatcccccaccatgcttcacctttaagacctccaactccactttgatcccagttctcaggttcaggcctcacaaggccaaaatcctgaagttacccttctcaaactcccttgcctttaacatcatcagaatcaacctcctacccccactctgtcccagcagcaatagcctgctaatcttttagcactaatcttttaggcactaatctgctttccaaactcttggcacctgaactatttataagcagtgttttatgcccccccaccaaagaaccctattcttttcccatgaccccaccaatcaaaacactcagaggactgtgggtataagaggctggggaggcaggcatagcagcggccgccaccatggctaagattaacacccagtactcacatccatcccgcactcacctcaaagtcaagacctccgatcgggatctgaaccgggctgagaatgggctgtcgcgcgcccactcgtcgtccgaggaaaccagcagcgtgctccagccgggcatcgccatggaaactagggggctggcggactccggacagggatccttcactggacagggtattgcccggttcgggcggattcagaagaagtcccagccggagaaggtcgtgcgggctgccagcaggggcaggccactcattggttggacacagtggtgcgctgaggatggtggagatgaatcggaaatggcactggccggctctcccggatgcagctcgggcccccaagggagactgagcagactgatcttcctgcttcgccgctgggcggccagacacgtgcaccatcaggaccagggacctgatagcttccccgaccgctttaggggagccgagctgaaagaagtgtcaagccaggagtcaaacgcgcaggccaacgtcggcagccaagagcctgcagaccggggacgctcggcatggccgctcgcaaagtgcaacactaacacttccaacaacaccgaagaggaaaagaaaaccaagaagaaggatgcaattgtggtggacccttcctccaacctgtactaccgctggttgaccgccatcgccctcccggtcttttacaattggtatctccttatctgccgggcctgcttcgacgaactgcaatcagagtacctgatgctgtggctggtgctggactatagcgccgatgtgctctacgtcctggatgtgctcgtgcgcgcccggaccggattcttggaacaaggcctgatggtgtccgacacgaatagactgtggcagcactataagaccacaacccagttcaagcttgacgtgctcagccttgtgccgactgacctggcctacctgaaagtcggaactaactacccggaagtcagattcaaccgactcctgaagttcagcaggctgttcgagttctttgaccgcaccgagactcggaccaactaccctaacatgttccggatcggaaatctggtgctctacatactgattatcatccattggaacgcctgtatctatttcgccatttcgaagttcatcggtttcggaaccgattcctgggtgtaccccaacatctcgatccccgaacacggtcgcctgtcccggaagtacatctactccctgtactggtccactctgactctgaccacgatcggggaaacccctccacccgtgaaggacgaagagtacctgttcgtggtggtggacttcctggtcggagtgttgattttcgccaccattgtgggaaacgtgggctccatgatctccaacatgaacgcgtcgagagctgagttccaagccaagatcgactccattaagcagtacatgcagttcagaaaggtcaccaaggacctggaaaccagggtcatccgctggttcgactacctgtgggccaacaaaaagactgtggacgaaaaggaagtgctgaagtcgctgccggataagctgaaggccgaaatcgccattaacgtgcaccttgacaccctgaagaaagtccggatcttccaagactgtgaagccggcctcctggtggagctcgtgctcaagctgcggcccaccgtgttcagcccgggagattacatttgcaagaagggcgatatcggcaaagagatgtacatcatcaacgagggaaagctggccgtggtcgcggacgacggcgtgacccagttcgtggtgctgtccgacggatcctacttcggtgaaatctcaatcctcaacatcaaggggtccaagtccggcaaccggagaactgccaacattcgctccatcggatacagcgacctgttttgcctgtccaaggatgacctgatggaggctctgactgagtaccctgaagcgaagaaggctttggaggaaaaggggcggcagattctgatgaaggacaatttgatcgacgaggagctcgcacgggccggcgccgaccccaaggatctcgaagagaaggtcgaacagctgggttcttcgcttgataccctgcaaacccgattcgcgcggctgctcgccgagtacaacgcgacccagatgaagatgaagcagagactgtcacagttggaatcccaagtcaagggcggaggcgacaagccgctggcggacggggaagtgcccggggacgccaccaagactgaggacaagcagcagtgatcatagatcgatctgcctcgactgtgccttctagttgccagccatctgttgtttgcccctcccccgtgccttccttgaccctggaaggtgccactcccactgtcctttcctaataaaatgaggaaattgcatcgcattgtctgagtaggtgtcattctattctggggggtggggtggggcaggacagcaagggggaggattgggaagacaatagcaggcatgctggggactcgagttctacgtagataagtagcatggcgggttaatcattaactacaaggaacccctagtgatggagttggccactccctctctgcgcgctcgctcgctcactgaggccgggcgaccaaaggtcgcccgacgcccgggctttgcccgggcggcctcagtgagcgagcgagcgcgcagccttaattaacctaaggaaaatgaagtgaagttcctatactttctagagaataggaacttctatagtgagtcgaataagggcgacacaaaatttattctaaatgcataataaatactgataacatcttatagtttgtattatattttgtattatcgttgacatgtataattttgatatcaaaaactgattttccctttattattttcgagatttattttcttaattctctttaacaaactagaaatattgtatatacaaaaaatcataaataatagatgaatagtttaattataggtgttcatcaatcgaaaaagcaacgtatcttatttaaagtgcgttgcttttttctcatttataaggttaaataattctcatatatcaagcaaagtgacaggcgcccttaaatattctgacaaatgctctttccctaaactccccccataaaaaaacccgccgaagcgggtttttacgttatttgcggattaacgattactcgttatcagaaccgcccagggggcccgagcttaacctttttatttgggggagagggaagtcatgaaaaaactaacctttgaaattcgatctccagcacatcagcaaaacgctattcacgcagtacagcaaatccttccagacccaaccaaaccaatcgtagtaaccattcaggaacgcaaccgcagcttagaccaaaacaggaagctatgggcctgcttaggtgacgtctctcgtcaggttgaatggcatggtcgctggctggatgcagaaagctggaagtgtgtgtttaccgcagcattaaagcagcaggatgttgttcctaaccttgccgggaatggctttgtggtaataggccagtcaaccagcaggatgcgtgtaggcgaatttgcggagctattagagcttatacaggcattcggtacagagcgtggcgttaagtggtcagacgaagcgagactggctctggagtggaaagcgagatggggagacagggctgcatgataaatgtcgttagtttctccggtggcaggacgtcagcatatttgctctggctaatggagcaaaagcgacgggcaggtaaagacgtgcattacgttttcatggatacaggttgtgaacatccaatgacatatcggtttgtcagggaagttgtgaagttctgggatataccgctcaccgtattgcaggttgatatcaacccggagcttggacagccaaatggttatacggtatgggaaccaaaggatattcagacgcgaatgcctgttctgaagccatttatcgatatggtaaagaaatatggcactccatacgtcggcggcgcgttctgcactgacagattaaaactcgttcccttcaccaaatactgtgatgaccatttcgggcgagggaattacaccacgtggattggcatcagagctgatgaaccgaagcggctaaagccaaagcctggaatcagatatcttgctgaactgtcagactttgagaaggaagatatcctcgcatggtggaagcaacaaccattcgatttgcaaataccggaacatctcggtaactgcatattctgcattaaaaaatcaacgcaaaaaatcggacttgcctgcaaagatgaggagggattgcagcgtgtttttaatgaggtcatcacgggatcccatgtgcgtgacggacatcgggaaacgccaaaggagattatgtaccgaggaagaatgtcgctggacggtatcgcgaaaatgtattcagaaaatgattatcaagccctgtatcaggacatggtacgagctaaaagattcgataccggctcttgttctgagtcatgcgaaatatttggagggcagcttgatttcgacttcgggagggaagctgcatgatgcgatgttatcggtgcggtgaatgcaaagaagataaccgcttccgaccaaatcaaccttactggaatcgatggtgtctccggtgtgaaagaacaccaacaggggtgttaccactaccgcaggaaaaggaggacgtgtggcgagacagcgacgaagtatcaccgacataatctgcgaaaactgcaaataccttccaacgaaacgcaccagaaataaacccaagccaatcccaaaagaatctgacgtaaaaaccttcaactacacggctcacctgtgggatatccggtggctaagacgtcgtgcgaggaaaacaaggtgattgaccaaaatcgaagttacgaacaagaaagcgtcgagcgagctttaacgtgcgctaactgcggtcagaagctgcatgtgctggaagttcacgtgtgtgagcactgctgcgcagaactgatgagcgatccgaatagctcgatgcacgaggaagaagatgatggctaaaccagcgcgaagacgatgtaaaaacgatgaatgccgggaatggtttcaccctgcattcgctaatcagtggtggtgctctccagagtgtggaaccaagatagcactcgaacgacgaagtaaagaacgcgaaaaagcggaaaaagcagcagagaagaaacgacgacgagaggagcagaaacagaaagataaacttaagattcgaaaactcgccttaaagccccgcagttactggattaaacaagcccaacaagccgtaaacgccttcatcagagaaagagaccgcgacttaccatgtatctcgtgcggaacgctcacgtctgctcagtgggatgccggacattaccggacaactgctgcggcacctcaactccgatttaatgaacgcaatattcacaagcaatgcgtggtgtgcaaccagcacaaaagcggaaatctcgttccgtatcgcgtcgaactgattagccgcatcgggcaggaagcagtagacgaaatcgaatcaaaccataaccgccatcgctggactatcgaagagtgcaaggcgatcaaggcagagtaccaacagaaactcaaagacctgcgaaatagcagaagtgaggccgcatgacgttctcagtaaaaaccattccagacatgctcgttgaagcatacggaaatcagacagaagtagcacgcagactgaaatgtagtcgcggtacggtcagaaaatacgttgatgataaagacgggaaaatgcacgccatcgtcaacgacgttctcatggttcatcgcggatggagtgaaagagatgcgctattacgaaaaaattgatggcagcaaataccgaaatatttgggtagttggcgatctgcacggatgctacacgaacctgatgaacaaactggatacgattggattcgacaacaaaaaagacctgcttatctcggtgggcgatttggttgatcgtggtgcagagaacgttgaatgcctggaattaatcacattcccctggttcagagctgtacgtggaaaccatgagcaaatgatgattgatggcttatcagagcgtggaaacgttaatcactggctgcttaatggcggtggctggttctttaatctcgattacgacaaagaaattctggctaaagctcttgcccataaagcagatgaacttccgttaatcatcgaactggtgagcaaagataaaaaatatgttatctgccacgccgattatccctttgacgaatacgagtttggaaagccagttgatcatcagcaggtaatctggaaccgcgaacgaatcagcaactcacaaaacgggatcgtgaaagaaatcaaaggcgcggacacgttcatctttggtcatacgccagcagtgaaaccactcaagtttgccaaccaaatgtatatcgataccggcgcagtgttctgcggaaacctaacattgattcaggtacagggagaaggcgcatgagactcgaaagcgtagctaaatttcattcgccaaaaagcccgatgatgagcgactcaccacgggccacggcttctgactctctttccggtactgatgtgatggctgctatggggatggcgcaatcacaagccggattcggtatggctgcattctgcggtaagcacgaactcagccagaacgacaaacaaaaggctatcaactatctgatgcaatttgcacacaaggtatcggggaaataccgtggtgtggcaaagcttgaaggaaatactaaggcaaaggtactgcaagtgctcgcaacattcgcttatgcggattattgccgtagtgccgcgacgccgggggcaagatgcagagattgccatggtacaggccgtgcggttgatattgccaaaacagagctgtgggggagagttgtcgagaaagagtgcggaagatgcaaaggcgtcggctattcaaggatgccagcaagcgcagcatatcgcgctgtgacgatgctaatcccaaaccttacccaacccacctggtcacgcactgttaagccgctgtatgacgctctggtggtgcaatgccacaaagaagagtcaatcgcagacaacattttgaatgcggtcacacgttagcagcatgattgccacggatggcaacatattaacggcatgatattgacttattgaataaaattgggtaaatttgactcaacgatgggttaattcgctcgttgtggtagtgagatgaaaagaggcggcgcttactaccgattccgcctagttggtcacttcgacgtatcgtctggaactccaaccatcgcaggcagagaggtctgcaaaatgcaatcccgaaacagttcgcaggtaatagttagagcctgcataacggtttcgggattttttatatctgcacaacaggtaagagcattgagtcgataatcgtgaagagtcggcgagcctggttagccagtgctctttccgttgtgctgaattaagcgaataccggaagcagaaccggatcaccaaatgcgtacaggcgtcatcgccgcccagcaacagcacaacccaaactgagccgtagccactgtctgtcctgaattcattagtaatagttacgctgcggccttttacacatgaccttcgtgaaagcgggtggcaggaggtcgcgctaacaacctcctgccgttttgcccgtgcatatcggtcacgaacaaatctgattactaaacacagtagcctggatttgttctatcagtaatcgaccttattcctaattaaatagagcaaatccccttattgggggtaagacatgaagatgccagaaaaacatgacctgttggccgccattctcgcggcaaaggaacaaggcatcggggcaatccttgcgtttgcaatggcgtaccttcgcggcagatataatggcggtgcgtttacaaaaacagtaatcgacgcaacgatgtgcgccattatcgcctggttcattcgtgaccttctcgacttcgccggactaagtagcaatctcgcttatataacgagcgtgtttatcggctacatcggtactgactcgattggttcgcttatcaaacgcttcgctgctaaaaaagccggagtagaagatggtagaaatcaataatcaacgtaaggcgttcctcgatatgctggcgtggtcggagggaactgataacggacgtcagaaaaccagaaatcatggttatgacgtcattgtaggcggagagctatttactgattactccgatcaccctcgcaaacttgtcacgctaaacccaaaactcaaatcaacaggcgcttaagactggccgtcgttttacaacacagaaagagtttgtagaaacgcaaaaaggccatccgtcaggggccttctgcttagtttgatgcctggcagttccctactctcgccttccgcttcctcgctcactgactcgctgcgctcggtcgttcggctgcggcgagcggtatcagctcactcaaaggcggtaatacggttatccacagaatcaggggataacgcaggaaagaacatgtgagcaaaaggccagcaaaaggccaggaaccgtaaaaaggccgcgttgctggcgtttttccataggctccgcccccctgacgagcatcacaaaaatcgacgctcaagtcagaggtggcgaaacccgacaggactataaagataccaggcgtttccccctggaagctccctcgtgcgctctcctgttccgaccctgccgcttaccggatacctgtccgcctttctcccttcgggaagcgtggcgctttctcatagctcacgctgtaggtatctcagttcggtgtaggtcgttcgctccaagctgggctgtgtgcacgaaccccccgttcagcccgaccgctgcgccttatccggtaactatcgtcttgagtccaacccggtaagacacgacttatcgccactggcagcagccactggtaacaggattagcagagcgaggtatgtaggcggtgctacagagttcttgaagtggtgggctaactacggctacactagaagaacagtatttggtatctgcgctctgctgaagccagttaccttcggaaaaagagttggtagctcttgatccggcaaacaaaccaccgctggtagcggtggtttttttgtttgcaagcagcagattacgcgcagaaaaaaaggatctcaagaagatcctttgatcttttctacggggtctgacgctcagtggaacgacgcgcgcgtaactcacgttaagggattttggtcatgagcttgcgccgtcccgtcaagtcagcgtaatgctctgcttttagaaaaactcatcgagcatcaaatgaaactgcaatttattcatatcaggattatcaataccatatttttgaaaaagccgtttctgtaatgaaggagaaaactcaccgaggcagttccataggatggcaagatcctggtatcggtctgcgattccgactcgtccaacatcaatacaacctattaatttcccctcgtcaaaaataaggttatcaagtgagaaatcaccatgagtgacgactgaatccggtgagaatggcaaaagtttatgcatttctttccagacttgttcaacaggccagccattacgctcgtcatcaaaatcactcgcatcaaccaaaccgttattcattcgtgattgcgcctgagcgaggcgaaatacgcgatcgctgttaaaaggacaattacaaacaggaatcgagtgcaaccggcgcaggaacactgccagcgcatcaacaatattttcacctgaatcaggatattcttctaatacctggaacgctgtttttccggggatcgcagtggtgagtaaccatgcatcatcaggagtacggataaaatgcttgatggtcggaagtggcataaattccgtcagccagtttagtctgaccatctcatctgtaacatcattggcaacgctacctttgccatgtttcagaaacaactctggcgcatcgggcttcccatacaagcgatagattgtcgcacctgattgcccgacattatcgcgagcccatttatacccatataaatcagcatccatgttggaatttaatcgcggcctcgacgtttcccgttgaatatggctcatattcttcctttttcaatattattgaagcatttatcagggttattgtctcatgagcggatacatatttgaatgtatttagaaaaataaacaaataggggtcagtgttacaaccaattaaccaattctgaacattatcgcgagcccatttatacctgaatatggctcataacaccccttgtttgcctggcggcagtagcgcggtggtcccacctgaccccatgccgaactcagaagtgaaacgccgtagcgccgatggtagtgtggggactccccatgcgagagtagggaactgccaggcatcaaataaaacgaaaggctcagtcgaaagactgggcctttcgcccgggctaattagggggtgtcgcccttattcgactctatagtgaagttcctattctctagaaagtataggaacttctgaagtggggtcgacttaattaagg

SEQ ID NO: 36 - DNA, 12209 bp, Artificial Sequence
  constructed sequence
ctgcgcgctcgctcgctcactgaggccgcccgggcaaagcccgggcgtcgggcgacctttggtcgcccggcctcagtgagcgagcgagcgcgcagagagggagtggccaactccatcactaggggttccttgtagttaatgattaacccgccatgctacttatctacgtagcaagctagctagttattaatagtaatcaattacggggtcattagttcatagcccatatatggagttccgcgttacataacttacggtaaatggcccgcctggctgaccgcccaacgacccccgcccattgacgtcaataatgacgtatgttcccatagtaacgccaatagggactttccattgacgtcaatgggtggagtatttacggtaaactgcccacttggcagtacatcaagtgtatcatatgccaagtacgccccctattgacgtcaatgacggtaaatggcccgcctggcattatgcccagtacatgaccttatgggactttcctacttggcagtacatctacgtattagtcatcgctattaacatggtcgaggtgagccccacgttctgcttcactctccccatctcccccccctccccacccccaattttgtatttatttattttttaattattttgtgcagcgatgggggcggggggggggggggggcgcgcgccaggcggggcggggcggggcgaggggcggggcggggcgaggcggagaggtgcggcggcagccaatcagagcggcgcgctccgaaagtttccttttatggcgaggcggcggcggcggcggccctataaaaagcgaagcgcgcggcgggcggggagtcgctgcgacgctgccttcgccccgtgccccgctccgccgccgcctcgcgccgcccgccccggctctgactgaccgcgttactcccacaggtgagcgggcgggacggcccttctcctccgggctgtaattagcgcttggtttaatgacggcttgtttcttttctgtggctgcgtgaaagccttgaggggctccgggagggccctttgtgcggggggagcggctcggggggtgcgtgcgtgtgtgtgtgcgtggggagcgccgcgtgcggctccgcgctgcccggcggctgtgagcgctgcgggcgcggcgcggggctttgtgcgctccgcagtgtgcgcgaggggagcgcggccgggggcggtgccccgcggtgcggggggggctgcgaggggaacaaaggctgcgtgcggggtgtgtgcgtgggggggtgagcagggggtgtgggcgcgtcggtcgggctgcaaccccccctgcacccccctccccgagttgctgagcacggcccggcttcgggtgcggggctccgtacggggcgtggcgcggggctcgccgtgccgggcggggggtggcggcaggtgggggtgccgggcggggcggggccgcctcgggccggggagggctcgggggaggggcgcggcggcccccggagcgccggcggctgtcgaggcgcggcgagccgcagccattgccttttatggtaatcgtgcgagagggcgcagggacttcctttgtcccaaatctgtgcggagccgaaatctgggaggcgccgccgcaccccctctagcgggcgcggggcgaagcggtgcggcgccggcaggaaggaaatgggcggggagggccttcgtgcgtcgccgcgccgccgtccccttctccctctccagcctcggggctgtccgcggggggacggctgccttcgggggggacggggcagggcggggttcggcttctggcgtgtgaccggcggctctagacaattgtactaaccttcttctctttcctctcctgacaggttggtgtacactagcggccgccaccatggccaagatcaacacccaatactcccacccctccaggacccacctcaaggtaaagacctcagaccgggatctcaatcgcgctgaaaatggcctcagcagagcccactcgtcaagtgaggagacatcgtcagtgctgcagccggggatcgccatggagaccagaggactggctgactccgggcagggctccttcaccggccaggggatcgccaggctgtcgcgcctcatcttcttgctgcgcaggtgggctgccaggcatgtgcaccaccaggaccagggaccggactcttttcctgatcgtttccgtggagccgagcttaaggaggtgtccagccaagaaagcaatgcccaggcaaatgtgggcagccaggagccagcagacagagggagaagcgcctggcccctggccaaatgcaacactaacaccagcaacaacacggaggaggagaagaagacgaaaaagaaggatgcgatcgtggtggacccgtccagcaacctgtactaccgctggctgaccgccatcgccctgcctgtcttctataactggtatctgcttatttgcagggcctgtttcgatgagctgcagtccgagtacctgatgctgtggctggtcctggactactcggcagatgtcctgtatgtcttggatgtgcttgtacgagctcggacaggttttcttgagcaaggcttaatggtcagtgataccaacaggctgtggcagcattacaagacgaccacgcagttcaagctggatgtgttgtccctggtccccaccgacctggcttacttaaaggtgggcacaaactacccagaagtgaggttcaaccgcctactgaagttttcccggctctttgaattctttgaccgcacagagacaaggaccaactaccccaatatgttcaggattgggaacttggtcttgtacattctcatcatcatccactggaatgcctgcatctactttgccatttccaagttcattggttttgggacagactcctgggtctacccaaacatctcaatcccagagcatgggcgcctctccaggaagtacatttacagtctctactggtccaccttgacccttaccaccattggtgagaccccaccccccgtgaaagatgaggagtatctctttgtggtcgtagacttcttggtgggtgttctgatttttgccaccattgtgggcaatgtgggctccatgatctcgaatatgaatgcctcacgggcagagttccaggccaagattgattccatcaagcagtacatgcagttccgcaaggtcaccaaggacttggagacgcgggttatccggtggtttgactacctgtgggccaacaagaagacggtggatgagaaggaggtgctcaagagcctcccagacaagctgaaggctgagatcgccatcaacgtgcacctggacacgctgaagaaggttcgcatcttccaggactgtgaggcagggctgctggtggagctggtgctgaagctgcgacccactgtgttcagccctggggattatatctgcaagaagggagatattgggaaggagatgtacatcatcaacgagggcaagctggccgtggtggctgatgatggggtcacccagttcgtggtcctcagcgatggcagctacttcggggagatcagcattctgaacatcaaggggagcaagtcggggaaccgcaggacggccaacatccgcagcattggctactcagacctgttctgcctctcaaaggacgatctcatggaggccctcaccgagtaccccgaagccaagaaggccctggaggagaaaggacggcagatcctgatgaaagacaacctgatcgatgaggagctggccagggcgggcgcggaccccaaggaccttgaggagaaagtggagcagctggggtcctccctggacaccctgcagaccaggtttgcacgcctcctggctgagtacaacgccacccagatgaagatgaagcagcgtctcagccaactggaaagccaggtgaagggtggtggggacaagcccctggctgatggggaagttcccggggatgctacaaaaacagaggacaaacaacagtgatcatagatcgatctgcctcgactgtgccttctagttgccagccatctgttgtttgcccctcccccgtgccttccttgaccctggaaggtgccactcccactgtcctttcctaataaaatgaggaaattgcatcgcattgtctgagtaggtgtcattctattctggggggtggggtggggcaggacagcaagggggaggattgggaagacaatagcaggcatgctggggactcgagttctacgtagataagtagcatggcgggttaatcattaactacaaggaacccctagtgatggagttggccactccctctctgcgcgctcgctcgctcactgaggccgggcgaccaaaggtcgcccgacgcccgggctttgcccgggcggcctcagtgagcgagcgagcgcgcagccttaattaacctaaggaaaatgaagtgaagttcctatactttctagagaataggaacttctatagtgagtcgaataagggcgacacaaaatttattctaaatgcataataaatactgataacatcttatagtttgtattatattttgtattatcgttgacatgtataattttgatatcaaaaactgattttccctttattattttcgagatttattttcttaattctctttaacaaactagaaatattgtatatacaaaaaatcataaataatagatgaatagtttaattataggtgttcatcaatcgaaaaagcaacgtatcttatttaaagtgcgttgcttttttctcatttataaggttaaataattctcatatatcaagcaaagtgacaggcgcccttaaatattctgacaaatgctctttccctaaactccccccataaaaaaacccgccgaagcgggtttttacgttatttgcggattaacgattactcgttatcagaaccgcccagggggcccgagcttaacctttttatttgggggagagggaagtcatgaaaaaactaacctttgaaattcgatctccagcacatcagcaaaacgctattcacgcagtacagcaaatccttccagacccaaccaaaccaatcgtagtaaccattcaggaacgcaaccgcagcttagaccaaaacaggaagctatgggcctgcttaggtgacgtctctcgtcaggttgaatggcatggtcgctggctggatgcagaaagctggaagtgtgtgtttaccgcagcattaaagcagcaggatgttgttcctaaccttgccgggaatggctttgtggtaataggccagtcaaccagcaggatgcgtgtaggcgaatttgcggagctattagagcttatacaggcattcggtacagagcgtggcgttaagtggtcagacgaagcgagactggctctggagtggaaagcgagatggggagacagggctgcatgataaatgtcgttagtttctccggtggcaggacgtcagcatatttgctctggctaatggagcaaaagcgacgggcaggtaaagacgtgcattacgttttcatggatacaggttgtgaacatccaatgacatatcggtttgtcagggaagttgtgaagttctgggatataccgctcaccgtattgcaggttgatatcaacccggagcttggacagccaaatggttatacggtatgggaaccaaaggatattcagacgcgaatgcctgttctgaagccatttatcgatatggtaaagaaatatggcactccatacgtcggcggcgcgttctgcactgacagattaaaactcgttcccttcaccaaatactgtgatgaccatttcgggcgagggaattacaccacgtggattggcatcagagctgatgaaccgaagcggctaaagccaaagcctggaatcagatatcttgctgaactgtcagactttgagaaggaagatatcctcgcatggtggaagcaacaaccattcgatttgcaaataccggaacatctcggtaactgcatattctgcattaaaaaatcaacgcaaaaaatcggacttgcctgcaaagatgaggagggattgcagcgtgtttttaatgaggtcatcacgggatcccatgtgcgtgacggacatcgggaaacgccaaaggagattatgtaccgaggaagaatgtcgctggacggtatcgcgaaaatgtattcagaaaatgattatcaagccctgtatcaggacatggtacgagctaaaagattcgataccggctcttgttctgagtcatgcgaaatatttggagggcagcttgatttcgacttcgggagggaagctgcatgatgcgatgttatcggtgcggtgaatgcaaagaagataaccgcttccgaccaaatcaaccttactggaatcgatggtgtctccggtgtgaaagaacaccaacaggggtgttaccactaccgcaggaaaaggaggacgtgtggcgagacagcgacgaagtatcaccgacataatctgcgaaaactgcaaataccttccaacgaaacgcaccagaaataaacccaagccaatcccaaaagaatctgacgtaaaaaccttcaactacacggctcacctgtgggatatccggtggctaagacgtcgtgcgaggaaaacaaggtgattgaccaaaatcgaagttacgaacaagaaagcgtcgagcgagctttaacgtgcgctaactgcggtcagaagctgcatgtgctggaagttcacgtgtgtgagcactgctgcgcagaactgatgagcgatccgaatagctcgatgcacgaggaagaagatgatggctaaaccagcgcgaagacgatgtaaaaacgatgaatgccgggaatggtttcaccctgcattcgctaatcagtggtggtgctctccagagtgtggaaccaagatagcactcgaacgacgaagtaaagaacgcgaaaaagcggaaaaagcagcagagaagaaacgacgacgagaggagcagaaacagaaagataaacttaagattcgaaaactcgccttaaagccccgcagttactggattaaacaagcccaacaagccgtaaacgccttcatcagagaaagagaccgcgacttaccatgtatctcgtgcggaacgctcacgtctgctcagtgggatgccggacattaccggacaactgctgcggcacctcaactccgatttaatgaacgcaatattcacaagcaatgcgtggtgtgcaaccagcacaaaagcggaaatctcgttccgtatcgcgtcgaactgattagccgcatcgggcaggaagcagtagacgaaatcgaatcaaaccataaccgccatcgctggactatcgaagagtgcaaggcgatcaaggcagagtaccaacagaaactcaaagacctgcgaaatagcagaagtgaggccgcatgacgttctcagtaaaaaccattccagacatgctcgttgaagcatacggaaatcagacagaagtagcacgcagactgaaatgtagtcgcggtacggtcagaaaatacgttgatgataaagacgggaaaatgcacgccatcgtcaacgacgttctcatggttcatcgcggatggagtgaaagagatgcgctattacgaaaaaattgatggcagcaaataccgaaatatttgggtagttggcgatctgcacggatgctacacgaacctgatgaacaaactggatacgattggattcgacaacaaaaaagacctgcttatctcggtgggcgatttggttgatcgtggtgcagagaacgttgaatgcctggaattaatcacattcccctggttcagagctgtacgtggaaaccatgagcaaatgatgattgatggcttatcagagcgtggaaacgttaatcactggctgcttaatggcggtggctggttctttaatctcgattacgacaaagaaattctggctaaagctcttgcccataaagcagatgaacttccgttaatcatcgaactggtgagcaaagataaaaaatatgttatctgccacgccgattatccctttgacgaatacgagtttggaaagccagttgatcatcagcaggtaatctggaaccgcgaacgaatcagcaactcacaaaacgggatcgtgaaagaaatcaaaggcgcggacacgttcatctttggtcatacgccagcagtgaaaccactcaagtttgccaaccaaatgtatatcgataccggcgcagtgttctgcggaaacctaacattgattcaggtacagggagaaggcgcatgagactcgaaagcgtagctaaatttcattcgccaaaaagcccgatgatgagcgactcaccacgggccacggcttctgactctctttccggtactgatgtgatggctgctatggggatggcgcaatcacaagccggattcggtatggctgcattctgcggtaagcacgaactcagccagaacgacaaacaaaaggctatcaactatctgatgcaatttgcacacaaggtatcggggaaataccgtggtgtggcaaagcttgaaggaaatactaaggcaaaggtactgcaagtgctcgcaacattcgcttatgcggattattgccgtagtgccgcgacgccgggggcaagatgcagagattgccatggtacaggccgtgcggttgatattgccaaaacagagctgtgggggagagttgtcgagaaagagtgcggaagatgcaaaggcgtcggctattcaaggatgccagcaagcgcagcatatcgcgctgtgacgatgctaatcccaaaccttacccaacccacctggtcacgcactgttaagccgctgtatgacgctctggtggtgcaatgccacaaagaagagtcaatcgcagacaacattttgaatgcggtcacacgttagcagcatgattgccacggatggcaacatattaacggcatgatattgacttattgaataaaattgggtaaatttgactcaacgatgggttaattcgctcgttgtggtagtgagatgaaaagaggcggcgcttactaccgattccgcctagttggtcacttcgacgtatcgtctggaactccaaccatcgcaggcagagaggtctgcaaaatgcaatcccgaaacagttcgcaggtaatagttagagcctgcataacggtttcgggattttttatatctgcacaacaggtaagagcattgagtcgataatcgtgaagagtcggcgagcctggttagccagtgctctttccgttgtgctgaattaagcgaataccggaagcagaaccggatcaccaaatgcgtacaggcgtcatcgccgcccagcaacagcacaacccaaactgagccgtagccactgtctgtcctgaattcattagtaatagttacgctgcggccttttacacatgaccttcgtgaaagcgggtggcaggaggtcgcgctaacaacctcctgccgttttgcccgtgcatatcggtcacgaacaaatctgattactaaacacagtagcctggatttgttctatcagtaatcgaccttattcctaattaaatagagcaaatccccttattgggggtaagacatgaagatgccagaaaaacatgacctgttggccgccattctcgcggcaaaggaacaaggcatcggggcaatccttgcgtttgcaatggcgtaccttcgcggcagatataatggcggtgcgtttacaaaaacagtaatcgacgcaacgatgtgcgccattatcgcctggttcattcgtgaccttctcgacttcgccggactaagtagcaatctcgcttatataacgagcgtgtttatcggctacatcggtactgactcgattggttcgcttatcaaacgcttcgctgctaaaaaagccggagtagaagatggtagaaatcaataatcaacgtaaggcgttcctcgatatgctggcgtggtcggagggaactgataacggacgtcagaaaaccagaaatcatggttatgacgtcattgtaggcggagagctatttactgattactccgatcaccctcgcaaacttgtcacgctaaacccaaaactcaaatcaacaggcgcttaagactggccgtcgttttacaacacagaaagagtttgtagaaacgcaaaaaggccatccgtcaggggccttctgcttagtttgatgcctggcagttccctactctcgccttccgcttcctcgctcactgactcgctgcgctcggtcgttcggctgcggcgagcggtatcagctcactcaaaggcggtaatacggttatccacagaatcaggggataacgcaggaaagaacatgtgagcaaaaggccagcaaaaggccaggaaccgtaaaaaggccgcgttgctggcgtttttccataggctccgcccccctgacgagcatcacaaaaatcgacgctcaagtcagaggtggcgaaacccgacaggactataaagataccaggcgtttccccctggaagctccctcgtgcgctctcctgttccgaccctgccgcttaccggatacctgtccgcctttctcccttcgggaagcgtggcgctttctcatagctcacgctgtaggtatctcagttcggtgtaggtcgttcgctccaagctgggctgtgtgcacgaaccccccgttcagcccgaccgctgcgccttatccggtaactatcgtcttgagtccaacccggtaagacacgacttatcgccactggcagcagccactggtaacaggattagcagagcgaggtatgtaggcggtgctacagagttcttgaagtggtgggctaactacggctacactagaagaacagtatttggtatctgcgctctgctgaagccagttaccttcggaaaaagagttggtagctcttgatccggcaaacaaaccaccgctggtagcggtggtttttttgtttgcaagcagcagattacgcgcagaaaaaaaggatctcaagaagatcctttgatcttttctacggggtctgacgctcagtggaacgacgcgcgcgtaactcacgttaagggattttggtcatgagcttgcgccgtcccgtcaagtcagcgtaatgctctgcttttagaaaaactcatcgagcatcaaatgaaactgcaatttattcatatcaggattatcaataccatatttttgaaaaagccgtttctgtaatgaaggagaaaactcaccgaggcagttccataggatggcaagatcctggtatcggtctgcgattccgactcgtccaacatcaatacaacctattaatttcccctcgtcaaaaataaggttatcaagtgagaaatcaccatgagtgacgactgaatccggtgagaatggcaaaagtttatgcatttctttccagacttgttcaacaggccagccattacgctcgtcatcaaaatcactcgcatcaaccaaaccgttattcattcgtgattgcgcctgagcgaggcgaaatacgcgatcgctgttaaaaggacaattacaaacaggaatcgagtgcaaccggcgcaggaacactgccagcgcatcaacaatattttcacctgaatcaggatattcttctaatacctggaacgctgtttttccggggatcgcagtggtgagtaaccatgcatcatcaggagtacggataaaatgcttgatggtcggaagtggcataaattccgtcagccagtttagtctgaccatctcatctgtaacatcattggcaacgctacctttgccatgtttcagaaacaactctggcgcatcgggcttcccatacaagcgatagattgtcgcacctgattgcccgacattatcgcgagcccatttatacccatataaatcagcatccatgttggaatttaatcgcggcctcgacgtttcccgttgaatatggctcatattcttcctttttcaatattattgaagcatttatcagggttattgtctcatgagcggatacatatttgaatgtatttagaaaaataaacaaataggggtcagtgttacaaccaattaaccaattctgaacattatcgcgagcccatttatacctgaatatggctcataacaccccttgtttgcctggcggcagtagcgcggtggtcccacctgaccccatgccgaactcagaagtgaaacgccgtagcgccgatggtagtgtggggactccccatgcgagagtagggaactgccaggcatcaaataaaacgaaaggctcagtcgaaagactgggcctttcgcccgggctaattagggggtgtcgcccttattcgactctatagtgaagttcctattctctagaaagtataggaacttctgaagtggggtcgacttaattaagg

SEQ ID NO: 37 - DNA, 12209 bp, Artificial Sequence
  constructed sequence
ctgcgcgctcgctcgctcactgaggccgcccgggcaaagcccgggcgtcgggcgacctttggtcgcccggcctcagtgagcgagcgagcgcgcagagagggagtggccaactccatcactaggggttccttgtagttaatgattaacccgccatgctacttatctacgtagcaagctagctagttattaatagtaatcaattacggggtcattagttcatagcccatatatggagttccgcgttacataacttacggtaaatggcccgcctggctgaccgcccaacgacccccgcccattgacgtcaataatgacgtatgttcccatagtaacgccaatagggactttccattgacgtcaatgggtggagtatttacggtaaactgcccacttggcagtacatcaagtgtatcatatgccaagtacgccccctattgacgtcaatgacggtaaatggcccgcctggcattatgcccagtacatgaccttatgggactttcctacttggcagtacatctacgtattagtcatcgctattaacatggtcgaggtgagccccacgttctgcttcactctccccatctcccccccctccccacccccaattttgtatttatttattttttaattattttgtgcagcgatgggggcggggggggggggggggcgcgcgccaggcggggcggggcggggcgaggggcggggcggggcgaggcggagaggtgcggcggcagccaatcagagcggcgcgctccgaaagtttccttttatggcgaggcggcggcggcggcggccctataaaaagcgaagcgcgcggcgggcggggagtcgctgcgacgctgccttcgccccgtgccccgctccgccgccgcctcgcgccgcccgccccggctctgactgaccgcgttactcccacaggtgagcgggcgggacggcccttctcctccgggctgtaattagcgcttggtttaatgacggcttgtttcttttctgtggctgcgtgaaagccttgaggggctccgggagggccctttgtgcggggggagcggctcggggggtgcgtgcgtgtgtgtgtgcgtggggagcgccgcgtgcggctccgcgctgcccggcggctgtgagcgctgcgggcgcggcgcggggctttgtgcgctccgcagtgtgcgcgaggggagcgcggccgggggcggtgccccgcggtgcggggggggctgcgaggggaacaaaggctgcgtgcggggtgtgtgcgtgggggggtgagcagggggtgtgggcgcgtcggtcgggctgcaaccccccctgcacccccctccccgagttgctgagcacggcccggcttcgggtgcggggctccgtacggggcgtggcgcggggctcgccgtgccgggcggggggtggcggcaggtgggggtgccgggcggggcggggccgcctcgggccggggagggctcgggggaggggcgcggcggcccccggagcgccggcggctgtcgaggcgcggcgagccgcagccattgccttttatggtaatcgtgcgagagggcgcagggacttcctttgtcccaaatctgtgcggagccgaaatctgggaggcgccgccgcaccccctctagcgggcgcggggcgaagcggtgcggcgccggcaggaaggaaatgggcggggagggccttcgtgcgtcgccgcgccgccgtccccttctccctctccagcctcggggctgtccgcggggggacggctgccttcgggggggacggggcagggcggggttcggcttctggcgtgtgaccggcggctctagacaattgtactaaccttcttctctttcctctcctgacaggttggtgtacactagcggccgccaccatggctaagattaacacccagtactcacatccatcccgcactcacctcaaagtcaagacctccgatcgggatctgaaccgggctgagaatgggctgtcgcgcgcccactcgtcgtccgaggaaaccagcagcgtgctccagccgggcatcgccatggaaactagggggctggcggactccggacagggatccttcactggacagggtattgcccggctgagcagactgatcttcctgcttcgccgctgggcggccagacacgtgcaccatcaggaccagggacctgatagcttccccgaccgctttaggggagccgagctgaaagaagtgtcaagccaggagtcaaacgcgcaggccaacgtcggcagccaagagcctgcagaccggggacgctcggcatggccgctcgcaaagtgcaacactaacacttccaacaacaccgaagaggaaaagaaaaccaagaagaaggatgcaattgtggtggacccttcctccaacctgtactaccgctggttgaccgccatcgccctcccggtcttttacaattggtatctccttatctgccgggcctgcttcgacgaactgcaatcagagtacctgatgctgtggctggtgctggactatagcgccgatgtgctctacgtcctggatgtgctcgtgcgcgcccggaccggattcttggaacaaggcctgatggtgtccgacacgaatagactgtggcagcactataagaccacaacccagttcaagcttgacgtgctcagccttgtgccgactgacctggcctacctgaaagtcggaactaactacccggaagtcagattcaaccgactcctgaagttcagcaggctgttcgagttctttgaccgcaccgagactcggaccaactaccctaacatgttccggatcggaaatctggtgctctacatactgattatcatccattggaacgcctgtatctatttcgccatttcgaagttcatcggtttcggaaccgattcctgggtgtaccccaacatctcgatccccgaacacggtcgcctgtcccggaagtacatctactccctgtactggtccactctgactctgaccacgatcggggaaacccctccacccgtgaaggacgaagagtacctgttcgtggtggtggacttcctggtcggagtgttgattttcgccaccattgtgggaaacgtgggctccatgatctccaacatgaacgcgtcgagagctgagttccaagccaagatcgactccattaagcagtacatgcagttcagaaaggtcaccaaggacctggaaaccagggtcatccgctggttcgactacctgtgggccaacaaaaagactgtggacgaaaaggaagtgctgaagtcgctgccggataagctgaaggccgaaatcgccattaacgtgcaccttgacaccctgaagaaagtccggatcttccaagactgtgaagccggcctcctggtggagctcgtgctcaagctgcggcccaccgtgttcagcccgggagattacatttgcaagaagggcgatatcggcaaagagatgtacatcatcaacgagggaaagctggccgtggtcgcggacgacggcgtgacccagttcgtggtgctgtccgacggatcctacttcggtgaaatctcaatcctcaacatcaaggggtccaagtccggcaaccggagaactgccaacattcgctccatcggatacagcgacctgttttgcctgtccaaggatgacctgatggaggctctgactgagtaccctgaagcgaagaaggctttggaggaaaaggggcggcagattctgatgaaggacaatttgatcgacgaggagctcgcacgggccggcgccgaccccaaggatctcgaagagaaggtcgaacagctgggttcttcgcttgataccctgcaaacccgattcgcgcggctgctcgccgagtacaacgcgacccagatgaagatgaagcagagactgtcacagttggaatcccaagtcaagggcggaggcgacaagccgctggcggacggggaagtgcccggggacgccaccaagactgaggacaagcagcagtgatcatagatcgatctgcctcgactgtgccttctagttgccagccatctgttgtttgcccctcccccgtgccttccttgaccctggaaggtgccactcccactgtcctttcctaataaaatgaggaaattgcatcgcattgtctgagtaggtgtcattctattctggggggtggggtggggcaggacagcaagggggaggattgggaagacaatagcaggcatgctggggactcgagttctacgtagataagtagcatggcgggttaatcattaactacaaggaacccctagtgatggagttggccactccctctctgcgcgctcgctcgctcactgaggccgggcgaccaaaggtcgcccgacgcccgggctttgcccgggcggcctcagtgagcgagcgagcgcgcagccttaattaacctaaggaaaatgaagtgaagttcctatactttctagagaataggaacttctatagtgagtcgaataagggcgacacaaaatttattctaaatgcataataaatactgataacatcttatagtttgtattatattttgtattatcgttgacatgtataattttgatatcaaaaactgattttccctttattattttcgagatttattttcttaattctctttaacaaactagaaatattgtatatacaaaaaatcataaataatagatgaatagtttaattataggtgttcatcaatcgaaaaagcaacgtatcttatttaaagtgcgttgcttttttctcatttataaggttaaataattctcatatatcaagcaaagtgacaggcgcccttaaatattctgacaaatgctctttccctaaactccccccataaaaaaacccgccgaagcgggtttttacgttatttgcggattaacgattactcgttatcagaaccgcccagggggcccgagcttaacctttttatttgggggagagggaagtcatgaaaaaactaacctttgaaattcgatctccagcacatcagcaaaacgctattcacgcagtacagcaaatccttccagacccaaccaaaccaatcgtagtaaccattcaggaacgcaaccgcagcttagaccaaaacaggaagctatgggcctgcttaggtgacgtctctcgtcaggttgaatggcatggtcgctggctggatgcagaaagctggaagtgtgtgtttaccgcagcattaaagcagcaggatgttgttcctaaccttgccgggaatggctttgtggtaataggccagtcaaccagcaggatgcgtgtaggcgaatttgcggagctattagagcttatacaggcattcggtacagagcgtggcgttaagtggtcagacgaagcgagactggctctggagtggaaagcgagatggggagacagggctgcatgataaatgtcgttagtttctccggtggcaggacgtcagcatatttgctctggctaatggagcaaaagcgacgggcaggtaaagacgtgcattacgttttcatggatacaggttgtgaacatccaatgacatatcggtttgtcagggaagttgtgaagttctgggatataccgctcaccgtattgcaggttgatatcaacccggagcttggacagccaaatggttatacggtatgggaaccaaaggatattcagacgcgaatgcctgttctgaagccatttatcgatatggtaaagaaatatggcactccatacgtcggcggcgcgttctgcactgacagattaaaactcgttcccttcaccaaatactgtgatgaccatttcgggcgagggaattacaccacgtggattggcatcagagctgatgaaccgaagcggctaaagccaaagcctggaatcagatatcttgctgaactgtcagactttgagaaggaagatatcctcgcatggtggaagcaacaaccattcgatttgcaaataccggaacatctcggtaactgcatattctgcattaaaaaatcaacgcaaaaaatcggacttgcctgcaaagatgaggagggattgcagcgtgtttttaatgaggtcatcacgggatcccatgtgcgtgacggacatcgggaaacgccaaaggagattatgtaccgaggaagaatgtcgctggacggtatcgcgaaaatgtattcagaaaatgattatcaagccctgtatcaggacatggtacgagctaaaagattcgataccggctcttgttctgagtcatgcgaaatatttggagggcagcttgatttcgacttcgggagggaagctgcatgatgcgatgttatcggtgcggtgaatgcaaagaagataaccgcttccgaccaaatcaaccttactggaatcgatggtgtctccggtgtgaaagaacaccaacaggggtgttaccactaccgcaggaaaaggaggacgtgtggcgagacagcgacgaagtatcaccgacataatctgcgaaaactgcaaataccttccaacgaaacgcaccagaaataaacccaagccaatcccaaaagaatctgacgtaaaaaccttcaactacacggctcacctgtgggatatccggtggctaagacgtcgtgcgaggaaaacaaggtgattgaccaaaatcgaagttacgaacaagaaagcgtcgagcgagctttaacgtgcgctaactgcggtcagaagctgcatgtgctggaagttcacgtgtgtgagcactgctgcgcagaactgatgagcgatccgaatagctcgatgcacgaggaagaagatgatggctaaaccagcgcgaagacgatgtaaaaacgatgaatgccgggaatggtttcaccctgcattcgctaatcagtggtggtgctctccagagtgtggaaccaagatagcactcgaacgacgaagtaaagaacgcgaaaaagcggaaaaagcagcagagaagaaacgacgacgagaggagcagaaacagaaagataaacttaagattcgaaaactcgccttaaagccccgcagttactggattaaacaagcccaacaagccgtaaacgccttcatcagagaaagagaccgcgacttaccatgtatctcgtgcggaacgctcacgtctgctcagtgggatgccggacattaccggacaactgctgcggcacctcaactccgatttaatgaacgcaatattcacaagcaatgcgtggtgtgcaaccagcacaaaagcggaaatctcgttccgtatcgcgtcgaactgattagccgcatcgggcaggaagcagtagacgaaatcgaatcaaaccataaccgccatcgctggactatcgaagagtgcaaggcgatcaaggcagagtaccaacagaaactcaaagacctgcgaaatagcagaagtgaggccgcatgacgttctcagtaaaaaccattccagacatgctcgttgaagcatacggaaatcagacagaagtagcacgcagactgaaatgtagtcgcggtacggtcagaaaatacgttgatgataaagacgggaaaatgcacgccatcgtcaacgacgttctcatggttcatcgcggatggagtgaaagagatgcgctattacgaaaaaattgatggcagcaaataccgaaatatttgggtagttggcgatctgcacggatgctacacgaacctgatgaacaaactggatacgattggattcgacaacaaaaaagacctgcttatctcggtgggcgatttggttgatcgtggtgcagagaacgttgaatgcctggaattaatcacattcccctggttcagagctgtacgtggaaaccatgagcaaatgatgattgatggcttatcagagcgtggaaacgttaatcactggctgcttaatggcggtggctggttctttaatctcgattacgacaaagaaattctggctaaagctcttgcccataaagcagatgaacttccgttaatcatcgaactggtgagcaaagataaaaaatatgttatctgccacgccgattatccctttgacgaatacgagtttggaaagccagttgatcatcagcaggtaatctggaaccgcgaacgaatcagcaactcacaaaacgggatcgtgaaagaaatcaaaggcgcggacacgttcatctttggtcatacgccagcagtgaaaccactcaagtttgccaaccaaatgtatatcgataccggcgcagtgttctgcggaaacctaacattgattcaggtacagggagaaggcgcatgagactcgaaagcgtagctaaatttcattcgccaaaaagcccgatgatgagcgactcaccacgggccacggcttctgactctctttccggtactgatgtgatggctgctatggggatggcgcaatcacaagccggattcggtatggctgcattctgcggtaagcacgaactcagccagaacgacaaacaaaaggctatcaactatctgatgcaatttgcacacaaggtatcggggaaataccgtggtgtggcaaagcttgaaggaaatactaaggcaaaggtactgcaagtgctcgcaacattcgcttatgcggattattgccgtagtgccgcgacgccgggggcaagatgcagagattgccatggtacaggccgtgcggttgatattgccaaaacagagctgtgggggagagttgtcgagaaagagtgcggaagatgcaaaggcgtcggctattcaaggatgccagcaagcgcagcatatcgcgctgtgacgatgctaatcccaaaccttacccaacccacctggtcacgcactgttaagccgctgtatgacgctctggtggtgcaatgccacaaagaagagtcaatcgcagacaacattttgaatgcggtcacacgttagcagcatgattgccacggatggcaacatattaacggcatgatattgacttattgaataaaattgggtaaatttgactcaacgatgggttaattcgctcgttgtggtagtgagatgaaaagaggcggcgcttactaccgattccgcctagttggtcacttcgacgtatcgtctggaactccaaccatcgcaggcagagaggtctgcaaaatgcaatcccgaaacagttcgcaggtaatagttagagcctgcataacggtttcgggattttttatatctgcacaacaggtaagagcattgagtcgataatcgtgaagagtcggcgagcctggttagccagtgctctttccgttgtgctgaattaagcgaataccggaagcagaaccggatcaccaaatgcgtacaggcgtcatcgccgcccagcaacagcacaacccaaactgagccgtagccactgtctgtcctgaattcattagtaatagttacgctgcggccttttacacatgaccttcgtgaaagcgggtggcaggaggtcgcgctaacaacctcctgccgttttgcccgtgcatatcggtcacgaacaaatctgattactaaacacagtagcctggatttgttctatcagtaatcgaccttattcctaattaaatagagcaaatccccttattgggggtaagacatgaagatgccagaaaaacatgacctgttggccgccattctcgcggcaaaggaacaaggcatcggggcaatccttgcgtttgcaatggcgtaccttcgcggcagatataatggcggtgcgtttacaaaaacagtaatcgacgcaacgatgtgcgccattatcgcctggttcattcgtgaccttctcgacttcgccggactaagtagcaatctcgcttatataacgagcgtgtttatcggctacatcggtactgactcgattggttcgcttatcaaacgcttcgctgctaaaaaagccggagtagaagatggtagaaatcaataatcaacgtaaggcgttcctcgatatgctggcgtggtcggagggaactgataacggacgtcagaaaaccagaaatcatggttatgacgtcattgtaggcggagagctatttactgattactccgatcaccctcgcaaacttgtcacgctaaacccaaaactcaaatcaacaggcgcttaagactggccgtcgttttacaacacagaaagagtttgtagaaacgcaaaaaggccatccgtcaggggccttctgcttagtttgatgcctggcagttccctactctcgccttccgcttcctcgctcactgactcgctgcgctcggtcgttcggctgcggcgagcggtatcagctcactcaaaggcggtaatacggttatccacagaatcaggggataacgcaggaaagaacatgtgagcaaaaggccagcaaaaggccaggaaccgtaaaaaggccgcgttgctggcgtttttccataggctccgcccccctgacgagcatcacaaaaatcgacgctcaagtcagaggtggcgaaacccgacaggactataaagataccaggcgtttccccctggaagctccctcgtgcgctctcctgttccgaccctgccgcttaccggatacctgtccgcctttctcccttcgggaagcgtggcgctttctcatagctcacgctgtaggtatctcagttcggtgtaggtcgttcgctccaagctgggctgtgtgcacgaaccccccgttcagcccgaccgctgcgccttatccggtaactatcgtcttgagtccaacccggtaagacacgacttatcgccactggcagcagccactggtaacaggattagcagagcgaggtatgtaggcggtgctacagagttcttgaagtggtgggctaactacggctacactagaagaacagtatttggtatctgcgctctgctgaagccagttaccttcggaaaaagagttggtagctcttgatccggcaaacaaaccaccgctggtagcggtggtttttttgtttgcaagcagcagattacgcgcagaaaaaaaggatctcaagaagatcctttgatcttttctacggggtctgacgctcagtggaacgacgcgcgcgtaactcacgttaagggattttggtcatgagcttgcgccgtcccgtcaagtcagcgtaatgctctgcttttagaaaaactcatcgagcatcaaatgaaactgcaatttattcatatcaggattatcaataccatatttttgaaaaagccgtttctgtaatgaaggagaaaactcaccgaggcagttccataggatggcaagatcctggtatcggtctgcgattccgactcgtccaacatcaatacaacctattaatttcccctcgtcaaaaataaggttatcaagtgagaaatcaccatgagtgacgactgaatccggtgagaatggcaaaagtttatgcatttctttccagacttgttcaacaggccagccattacgctcgtcatcaaaatcactcgcatcaaccaaaccgttattcattcgtgattgcgcctgagcgaggcgaaatacgcgatcgctgttaaaaggacaattacaaacaggaatcgagtgcaaccggcgcaggaacactgccagcgcatcaacaatattttcacctgaatcaggatattcttctaatacctggaacgctgtttttccggggatcgcagtggtgagtaaccatgcatcatcaggagtacggataaaatgcttgatggtcggaagtggcataaattccgtcagccagtttagtctgaccatctcatctgtaacatcattggcaacgctacctttgccatgtttcagaaacaactctggcgcatcgggcttcccatacaagcgatagattgtcgcacctgattgcccgacattatcgcgagcccatttatacccatataaatcagcatccatgttggaatttaatcgcggcctcgacgtttcccgttgaatatggctcatattcttcctttttcaatattattgaagcatttatcagggttattgtctcatgagcggatacatatttgaatgtatttagaaaaataaacaaataggggtcagtgttacaaccaattaaccaattctgaacattatcgcgagcccatttatacctgaatatggctcataacaccccttgtttgcctggcggcagtagcgcggtggtcccacctgaccccatgccgaactcagaagtgaaacgccgtagcgccgatggtagtgtggggactccccatgcgagagtagggaactgccaggcatcaaataaaacgaaaggctcagtcgaaagactgggcctttcgcccgggctaattagggggtgtcgcccttattcgactctatagtgaagttcctattctctagaaagtataggaacttctgaagtggggtcgacttaattaagg

SEQ ID NO: 38 - DNA, 12374 bp, Artificial Sequence
  constructed sequence
ctgcgcgctcgctcgctcactgaggccgcccgggcaaagcccgggcgtcgggcgacctttggtcgcccggcctcagtgagcgagcgagcgcgcagagagggagtggccaactccatcactaggggttccttgtagttaatgattaacccgccatgctacttatctacgtagcaagctagctagttattaatagtaatcaattacggggtcattagttcatagcccatatatggagttccgcgttacataacttacggtaaatggcccgcctggctgaccgcccaacgacccccgcccattgacgtcaataatgacgtatgttcccatagtaacgccaatagggactttccattgacgtcaatgggtggagtatttacggtaaactgcccacttggcagtacatcaagtgtatcatatgccaagtacgccccctattgacgtcaatgacggtaaatggcccgcctggcattatgcccagtacatgaccttatgggactttcctacttggcagtacatctacgtattagtcatcgctattaacatggtcgaggtgagccccacgttctgcttcactctccccatctcccccccctccccacccccaattttgtatttatttattttttaattattttgtgcagcgatgggggcggggggggggggggggcgcgcgccaggcggggcggggcggggcgaggggcggggcggggcgaggcggagaggtgcggcggcagccaatcagagcggcgcgctccgaaagtttccttttatggcgaggcggcggcggcggcggccctataaaaagcgaagcgcgcggcgggcggggagtcgctgcgacgctgccttcgccccgtgccccgctccgccgccgcctcgcgccgcccgccccggctctgactgaccgcgttactcccacaggtgagcgggcgggacggcccttctcctccgggctgtaattagcgcttggtttaatgacggcttgtttcttttctgtggctgcgtgaaagccttgaggggctccgggagggccctttgtgcggggggagcggctcggggggtgcgtgcgtgtgtgtgtgcgtggggagcgccgcgtgcggctccgcgctgcccggcggctgtgagcgctgcgggcgcggcgcggggctttgtgcgctccgcagtgtgcgcgaggggagcgcggccgggggcggtgccccgcggtgcggggggggctgcgaggggaacaaaggctgcgtgcggggtgtgtgcgtgggggggtgagcagggggtgtgggcgcgtcggtcgggctgcaaccccccctgcacccccctccccgagttgctgagcacggcccggcttcgggtgcggggctccgtacggggcgtggcgcggggctcgccgtgccgggcggggggtggcggcaggtgggggtgccgggcggggcggggccgcctcgggccggggagggctcgggggaggggcgcggcggcccccggagcgccggcggctgtcgaggcgcggcgagccgcagccattgccttttatggtaatcgtgcgagagggcgcagggacttcctttgtcccaaatctgtgcggagccgaaatctgggaggcgccgccgcaccccctctagcgggcgcggggcgaagcggtgcggcgccggcaggaaggaaatgggcggggagggccttcgtgcgtcgccgcgccgccgtccccttctccctctccagcctcggggctgtccgcggggggacggctgccttcgggggggacggggcagggcggggttcggcttctggcgtgtgaccggcggctctagacaattgtactaaccttcttctctttcctctcctgacaggttggtgtacactagcggccgccaccatggctaagattaacacccagtactcacatccatcccgcactcacctcaaagtcaagacctccgatcgggatctgaaccgggctgagaatgggctgtcgcgcgcccactcgtcgtccgaggaaaccagcagcgtgctccagccgggcatcgccatggaaactagggggctggcggactccggacagggatccttcactggacagggtattgcccggttcgggcggattcagaagaagtcccagccggagaaggtcgtgcgggctgccagcaggggcaggccactcattggttggacacagtggtgcgctgaggatggtggagatgaatcggaaatggcactggccggctctcccggatgcagctcgggcccccaagggagactgagcagactgatcttcctgcttcgccgctgggcggccagacacgtgcaccatcaggaccagggacctgatagcttccccgaccgctttaggggagccgagctgaaagaagtgtcaagccaggagtcaaacgcgcaggccaacgtcggcagccaagagcctgcagaccggggacgctcggcatggccgctcgcaaagtgcaacactaacacttccaacaacaccgaagaggaaaagaaaaccaagaagaaggatgcaattgtggtggacccttcctccaacctgtactaccgctggttgaccgccatcgccctcccggtcttttacaattggtatctccttatctgccgggcctgcttcgacgaactgcaatcagagtacctgatgctgtggctggtgctggactatagcgccgatgtgctctacgtcctggatgtgctcgtgcgcgcccggaccggattcttggaacaaggcctgatggtgtccgacacgaatagactgtggcagcactataagaccacaacccagttcaagcttgacgtgctcagccttgtgccgactgacctggcctacctgaaagtcggaactaactacccggaagtcagattcaaccgactcctgaagttcagcaggctgttcgagttctttgaccgcaccgagactcggaccaactaccctaacatgttccggatcggaaatctggtgctctacatactgattatcatccattggaacgcctgtatctatttcgccatttcgaagttcatcggtttcggaaccgattcctgggtgtaccccaacatctcgatccccgaacacggtcgcctgtcccggaagtacatctactccctgtactggtccactctgactctgaccacgatcggggaaacccctccacccgtgaaggacgaagagtacctgttcgtggtggtggacttcctggtcggagtgttgattttcgccaccattgtgggaaacgtgggctccatgatctccaacatgaacgcgtcgagagctgagttccaagccaagatcgactccattaagcagtacatgcagttcagaaaggtcaccaaggacctggaaaccagggtcatccgctggttcgactacctgtgggccaacaaaaagactgtggacgaaaaggaagtgctgaagtcgctgccggataagctgaaggccgaaatcgccattaacgtgcaccttgacaccctgaagaaagtccggatcttccaagactgtgaagccggcctcctggtggagctcgtgctcaagctgcggcccaccgtgttcagcccgggagattacatttgcaagaagggcgatatcggcaaagagatgtacatcatcaacgagggaaagctggccgtggtcgcggacgacggcgtgacccagttcgtggtgctgtccgacggatcctacttcggtgaaatctcaatcctcaacatcaaggggtccaagtccggcaaccggagaactgccaacattcgctccatcggatacagcgacctgttttgcctgtccaaggatgacctgatggaggctctgactgagtaccctgaagcgaagaaggctttggaggaaaaggggcggcagattctgatgaaggacaatttgatcgacgaggagctcgcacgggccggcgccgaccccaaggatctcgaagagaaggtcgaacagctgggttcttcgcttgataccctgcaaacccgattcgcgcggctgctcgccgagtacaacgcgacccagatgaagatgaagcagagactgtcacagttggaatcccaagtcaagggcggaggcgacaagccgctggcggacggggaagtgcccggggacgccaccaagactgaggacaagcagcagtgatcatagatcgatctgcctcgactgtgccttctagttgccagccatctgttgtttgcccctcccccgtgccttccttgaccctggaaggtgccactcccactgtcctttcctaataaaatgaggaaattgcatcgcattgtctgagtaggtgtcattctattctggggggtggggtggggcaggacagcaagggggaggattgggaagacaatagcaggcatgctggggactcgagttctacgtagataagtagcatggcgggttaatcattaactacaaggaacccctagtgatggagttggccactccctctctgcgcgctcgctcgctcactgaggccgggcgaccaaaggtcgcccgacgcccgggctttgcccgggcggcctcagtgagcgagcgagcgcgcagccttaattaacctaaggaaaatgaagtgaagttcctatactttctagagaataggaacttctatagtgagtcgaataagggcgacacaaaatttattctaaatgcataataaatactgataacatcttatagtttgtattatattttgtattatcgttgacatgtataattttgatatcaaaaactgattttccctttattattttcgagatttattttcttaattctctttaacaaactagaaatattgtatatacaaaaaatcataaataatagatgaatagtttaattataggtgttcatcaatcgaaaaagcaacgtatcttatttaaagtgcgttgcttttttctcatttataaggttaaataattctcatatatcaagcaaagtgacaggcgcccttaaatattctgacaaatgctctttccctaaactccccccataaaaaaacccgccgaagcgggtttttacgttatttgcggattaacgattactcgttatcagaaccgcccagggggcccgagcttaacctttttatttgggggagagggaagtcatgaaaaaactaacctttgaaattcgatctccagcacatcagcaaaacgctattcacgcagtacagcaaatccttccagacccaaccaaaccaatcgtagtaaccattcaggaacgcaaccgcagcttagaccaaaacaggaagctatgggcctgcttaggtgacgtctctcgtcaggttgaatggcatggtcgctggctggatgcagaaagctggaagtgtgtgtttaccgcagcattaaagcagcaggatgttgttcctaaccttgccgggaatggctttgtggtaataggccagtcaaccagcaggatgcgtgtaggcgaatttgcggagctattagagcttatacaggcattcggtacagagcgtggcgttaagtggtcagacgaagcgagactggctctggagtggaaagcgagatggggagacagggctgcatgataaatgtcgttagtttctccggtggcaggacgtcagcatatttgctctggctaatggagcaaaagcgacgggcaggtaaagacgtgcattacgttttcatggatacaggttgtgaacatccaatgacatatcggtttgtcagggaagttgtgaagttctgggatataccgctcaccgtattgcaggttgatatcaacccggagcttggacagccaaatggttatacggtatgggaaccaaaggatattcagacgcgaatgcctgttctgaagccatttatcgatatggtaaagaaatatggcactccatacgtcggcggcgcgttctgcactgacagattaaaactcgttcccttcaccaaatactgtgatgaccatttcgggcgagggaattacaccacgtggattggcatcagagctgatgaaccgaagcggctaaagccaaagcctggaatcagatatcttgctgaactgtcagactttgagaaggaagatatcctcgcatggtggaagcaacaaccattcgatttgcaaataccggaacatctcggtaactgcatattctgcattaaaaaatcaacgcaaaaaatcggacttgcctgcaaagatgaggagggattgcagcgtgtttttaatgaggtcatcacgggatcccatgtgcgtgacggacatcgggaaacgccaaaggagattatgtaccgaggaagaatgtcgctggacggtatcgcgaaaatgtattcagaaaatgattatcaagccctgtatcaggacatggtacgagctaaaagattcgataccggctcttgttctgagtcatgcgaaatatttggagggcagcttgatttcgacttcgggagggaagctgcatgatgcgatgttatcggtgcggtgaatgcaaagaagataaccgcttccgaccaaatcaaccttactggaatcgatggtgtctccggtgtgaaagaacaccaacaggggtgttaccactaccgcaggaaaaggaggacgtgtggcgagacagcgacgaagtatcaccgacataatctgcgaaaactgcaaataccttccaacgaaacgcaccagaaataaacccaagccaatcccaaaagaatctgacgtaaaaaccttcaactacacggctcacctgtgggatatccggtggctaagacgtcgtgcgaggaaaacaaggtgattgaccaaaatcgaagttacgaacaagaaagcgtcgagcgagctttaacgtgcgctaactgcggtcagaagctgcatgtgctggaagttcacgtgtgtgagcactgctgcgcagaactgatgagcgatccgaatagctcgatgcacgaggaagaagatgatggctaaaccagcgcgaagacgatgtaaaaacgatgaatgccgggaatggtttcaccctgcattcgctaatcagtggtggtgctctccagagtgtggaaccaagatagcactcgaacgacgaagtaaagaacgcgaaaaagcggaaaaagcagcagagaagaaacgacgacgagaggagcagaaacagaaagataaacttaagattcgaaaactcgccttaaagccccgcagttactggattaaacaagcccaacaagccgtaaacgccttcatcagagaaagagaccgcgacttaccatgtatctcgtgcggaacgctcacgtctgctcagtgggatgccggacattaccggacaactgctgcggcacctcaactccgatttaatgaacgcaatattcacaagcaatgcgtggtgtgcaaccagcacaaaagcggaaatctcgttccgtatcgcgtcgaactgattagccgcatcgggcaggaagcagtagacgaaatcgaatcaaaccataaccgccatcgctggactatcgaagagtgcaaggcgatcaaggcagagtaccaacagaaactcaaagacctgcgaaatagcagaagtgaggccgcatgacgttctcagtaaaaaccattccagacatgctcgttgaagcatacggaaatcagacagaagtagcacgcagactgaaatgtagtcgcggtacggtcagaaaatacgttgatgataaagacgggaaaatgcacgccatcgtcaacgacgttctcatggttcatcgcggatggagtgaaagagatgcgctattacgaaaaaattgatggcagcaaataccgaaatatttgggtagttggcgatctgcacggatgctacacgaacctgatgaacaaactggatacgattggattcgacaacaaaaaagacctgcttatctcggtgggcgatttggttgatcgtggtgcagagaacgttgaatgcctggaattaatcacattcccctggttcagagctgtacgtggaaaccatgagcaaatgatgattgatggcttatcagagcgtggaaacgttaatcactggctgcttaatggcggtggctggttctttaatctcgattacgacaaagaaattctggctaaagctcttgcccataaagcagatgaacttccgttaatcatcgaactggtgagcaaagataaaaaatatgttatctgccacgccgattatccctttgacgaatacgagtttggaaagccagttgatcatcagcaggtaatctggaaccgcgaacgaatcagcaactcacaaaacgggatcgtgaaagaaatcaaaggcgcggacacgttcatctttggtcatacgccagcagtgaaaccactcaagtttgccaaccaaatgtatatcgataccggcgcagtgttctgcggaaacctaacattgattcaggtacagggagaaggcgcatgagactcgaaagcgtagctaaatttcattcgccaaaaagcccgatgatgagcgactcaccacgggccacggcttctgactctctttccggtactgatgtgatggctgctatggggatggcgcaatcacaagccggattcggtatggctgcattctgcggtaagcacgaactcagccagaacgacaaacaaaaggctatcaactatctgatgcaatttgcacacaaggtatcggggaaataccgtggtgtggcaaagcttgaaggaaatactaaggcaaaggtactgcaagtgctcgcaacattcgcttatgcggattattgccgtagtgccgcgacgccgggggcaagatgcagagattgccatggtacaggccgtgcggttgatattgccaaaacagagctgtgggggagagttgtcgagaaagagtgcggaagatgcaaaggcgtcggctattcaaggatgccagcaagcgcagcatatcgcgctgtgacgatgctaatcccaaaccttacccaacccacctggtcacgcactgttaagccgctgtatgacgctctggtggtgcaatgccacaaagaagagtcaatcgcagacaacattttgaatgcggtcacacgttagcagcatgattgccacggatggcaacatattaacggcatgatattgacttattgaataaaattgggtaaatttgactcaacgatgggttaattcgctcgttgtggtagtgagatgaaaagaggcggcgcttactaccgattccgcctagttggtcacttcgacgtatcgtctggaactccaaccatcgcaggcagagaggtctgcaaaatgcaatcccgaaacagttcgcaggtaatagttagagcctgcataacggtttcgggattttttatatctgcacaacaggtaagagcattgagtcgataatcgtgaagagtcggcgagcctggttagccagtgctctttccgttgtgctgaattaagcgaataccggaagcagaaccggatcaccaaatgcgtacaggcgtcatcgccgcccagcaacagcacaacccaaactgagccgtagccactgtctgtcctgaattcattagtaatagttacgctgcggccttttacacatgaccttcgtgaaagcgggtggcaggaggtcgcgctaacaacctcctgccgttttgcccgtgcatatcggtcacgaacaaatctgattactaaacacagtagcctggatttgttctatcagtaatcgaccttattcctaattaaatagagcaaatccccttattgggggtaagacatgaagatgccagaaaaacatgacctgttggccgccattctcgcggcaaaggaacaaggcatcggggcaatccttgcgtttgcaatggcgtaccttcgcggcagatataatggcggtgcgtttacaaaaacagtaatcgacgcaacgatgtgcgccattatcgcctggttcattcgtgaccttctcgacttcgccggactaagtagcaatctcgcttatataacgagcgtgtttatcggctacatcggtactgactcgattggttcgcttatcaaacgcttcgctgctaaaaaagccggagtagaagatggtagaaatcaataatcaacgtaaggcgttcctcgatatgctggcgtggtcggagggaactgataacggacgtcagaaaaccagaaatcatggttatgacgtcattgtaggcggagagctatttactgattactccgatcaccctcgcaaacttgtcacgctaaacccaaaactcaaatcaacaggcgcttaagactggccgtcgttttacaacacagaaagagtttgtagaaacgcaaaaaggccatccgtcaggggccttctgcttagtttgatgcctggcagttccctactctcgccttccgcttcctcgctcactgactcgctgcgctcggtcgttcggctgcggcgagcggtatcagctcactcaaaggcggtaatacggttatccacagaatcaggggataacgcaggaaagaacatgtgagcaaaaggccagcaaaaggccaggaaccgtaaaaaggccgcgttgctggcgtttttccataggctccgcccccctgacgagcatcacaaaaatcgacgctcaagtcagaggtggcgaaacccgacaggactataaagataccaggcgtttccccctggaagctccctcgtgcgctctcctgttccgaccctgccgcttaccggatacctgtccgcctttctcccttcgggaagcgtggcgctttctcatagctcacgctgtaggtatctcagttcggtgtaggtcgttcgctccaagctgggctgtgtgcacgaaccccccgttcagcccgaccgctgcgccttatccggtaactatcgtcttgagtccaacccggtaagacacgacttatcgccactggcagcagccactggtaacaggattagcagagcgaggtatgtaggcggtgctacagagttcttgaagtggtgggctaactacggctacactagaagaacagtatttggtatctgcgctctgctgaagccagttaccttcggaaaaagagttggtagctcttgatccggcaaacaaaccaccgctggtagcggtggtttttttgtttgcaagcagcagattacgcgcagaaaaaaaggatctcaagaagatcctttgatcttttctacggggtctgacgctcagtggaacgacgcgcgcgtaactcacgttaagggattttggtcatgagcttgcgccgtcccgtcaagtcagcgtaatgctctgcttttagaaaaactcatcgagcatcaaatgaaactgcaatttattcatatcaggattatcaataccatatttttgaaaaagccgtttctgtaatgaaggagaaaactcaccgaggcagttccataggatggcaagatcctggtatcggtctgcgattccgactcgtccaacatcaatacaacctattaatttcccctcgtcaaaaataaggttatcaagtgagaaatcaccatgagtgacgactgaatccggtgagaatggcaaaagtttatgcatttctttccagacttgttcaacaggccagccattacgctcgtcatcaaaatcactcgcatcaaccaaaccgttattcattcgtgattgcgcctgagcgaggcgaaatacgcgatcgctgttaaaaggacaattacaaacaggaatcgagtgcaaccggcgcaggaacactgccagcgcatcaacaatattttcacctgaatcaggatattcttctaatacctggaacgctgtttttccggggatcgcagtggtgagtaaccatgcatcatcaggagtacggataaaatgcttgatggtcggaagtggcataaattccgtcagccagtttagtctgaccatctcatctgtaacatcattggcaacgctacctttgccatgtttcagaaacaactctggcgcatcgggcttcccatacaagcgatagattgtcgcacctgattgcccgacattatcgcgagcccatttatacccatataaatcagcatccatgttggaatttaatcgcggcctcgacgtttcccgttgaatatggctcatattcttcctttttcaatattattgaagcatttatcagggttattgtctcatgagcggatacatatttgaatgtatttagaaaaataaacaaataggggtcagtgttacaaccaattaaccaattctgaacattatcgcgagcccatttatacctgaatatggctcataacaccccttgtttgcctggcggcagtagcgcggtggtcccacctgaccccatgccgaactcagaagtgaaacgccgtagcgccgatggtagtgtggggactccccatgcgagagtagggaactgccaggcatcaaataaaacgaaaggctcagtcgaaagactgggcctttcgcccgggctaattagggggtgtcgcccttattcgactctatagtgaagttcctattctctagaaagtataggaacttctgaagtggggtcgacttaattaagg

SEQ ID NO: 39 - DNA, 11389 bp, Artificial Sequence
  constructed sequence
ctgcgcgctcgctcgctcactgaggccgcccgggcaaagcccgggcgtcgggcgacctttggtcgcccggcctcagtgagcgagcgagcgcgcagagagggagtggccaactccatcactaggggttccttgtagttaatgattaacccgccatgctacttatctacgtagcaagctagcaagatccaagctcagatctcgatcgagttgggccccagaagcctggtggttgtttgtccttctcaggggaaaagtgaggcggccccttggaggaaggggccgggcagaatgatctaatcggattccaagcagctcaggggattgtctttttctagcaccttcttgccactcctaagcgtcctccgtgaccccggctgggatttagcctggtgctgtgtcagccccggtctcccaggggcttcccagtggtccccaggaaccctcgacagggcccggtctctctcgtccagcaagggcagggacgggccacaggccaagggccctcgatcgaggaactgaaaaaccagaaagttaactggtaagtttagtctttttgtcttttatttcaggtcccggatccggtggtggtgcaaatcaaagaactgctcctcagtggatgttgcctttacttctaggcctgtacggaagtgttacttctgctctaaaagctgcggaattgtacccggcggccgccaccatgtttaaatcgctgacaaaagtcaacaaggtgaagcctataggagagaacaatgagaatgaacaaagttctcgtcggaatgaagaaggctctcacccaagtaatcagtctcagcaaaccacagcacaggaagaaaacaaaggtgaagagaaatctctcaaaaccaagtcaactccagtcacgtctgaagagccacacaccaacatacaagacaaactctccaagaaaaattcctctggagatctgaccacaaaccctgaccctcaaaatgcagcagaaccaactggaacagtgccagagcagaaggaaatggaccccgggaaagaaggtccaaacagcccacaaaacaaaccgccagcagctcctgttataaatgagtatgccgatgcccagctacacaacctggtgaaaagaatgcgtcaaagaacagccctctacaagaaaaagttggtagagggagatctctcctcacccgaagccagcccacaaactgcaaagcccacggctgtaccaccagtaaaagaaagcgatgataagccaacagaacattactacaggctgttgtggttcaaagtcaaaaagatgcctttaacagagtacttaaagcgaattaaacttccaaacagcatagattcatacacagatcgactctatctcctgtggctcttgcttgtcactcttgcctataactggaactgctgttttataccactgcgcctcgtcttcccatatcaaaccgcagacaacatacactactggcttattgcggacatcatctgtgatatcatctacctttatgatatgctatttatccagcccagactccagtttgtaagaggaggagacataatagtggattcaaatgagctaaggaaacactacaggacttctacaaaatttcagttggatgtcgcatcaataataccatttgatatttgctacctcttctttgggtttaatccaatgtttagagcaaataggatgttaaagtacacttcattttttgaatttaatcatcacctagagtctataatggacaaagcatatatctacagagttattcgaacaactggatacttgctgtttattctgcacattaatgcctgtgtttattactgggcttcaaactatgaaggaattggcactactagatgggtgtatgatggggaaggaaacgagtatctgagatgttattattgggcagttcgaactttaattaccattggtggccttccagaaccacaaactttatttgaaattgtttttcaactcttgaattttttttctggagtttttgtgttctccagtttaattggtcagatgagagatgtgattggagcagctacagccaatcagaactacttccgcgcctgcatggatgacaccattgcctacatgaacaattactccattcctaaacttgtgcaaaagcgagttcggacttggtatgaatatacatgggactctcaaagaatgctagatgagtctgatttgcttaagaccctaccaactacggtccagttagccctcgccattgatgtgaacttcagcatcatcagcaaagttgacttgttcaagggttgtgatacacagatgatttatgacatgttgctaagattgaaatccgttctctatttgcctggtgactttgtctgcaaaaagggagaaattggcaaggaaatgtatatcatcaagcatggagaagtccaagttcttggaggccctgatggtactaaagttctggttactctgaaagctgggtcggtgtttggagaaatcagccttctagcagcaggaggaggaaaccgtcgaactgccaatgtggtggcccacgggtttgccaatcttttaactctagacaaaaagaccctccaagaaattctagtgcattatccagattctgaaagaatcctcatgaagaaagccagagtgcttttaaagcagaaggctaagaccgcagaagcaacccctccaagaaaagatcttgccctcctcttcccaccgaaagaagagacacccaaactgtttaaaactctcctaggaggcacaggaaaagcaagtcttgcaagactactcaaattgaagcgagagcaagcagctcagaagaaagaaaattctgaaggaggagaggaagaaggaaaagaaaatgaagataaacaaaaagaaaatgaagataaacaaaaagaaaatgaagataaaggaaaagaaaatgaagataaagataaaggaagagagccagaagagaagccactggacagacctgaatgtacagcaagtcctattgcagtggaggaagaaccccactcagttagaaggacagttttacccagagggacttctcgtcaatcactcattatcagcatggctccttctgctgagggcggagaagaggttcttactattgaagtcaaagaaaaggctaagcaatgatcataactgcagatctgcctcgactgtgccttctagttgccagccatctgttgtttgcccctcccccgtgccttccttgaccctggaaggtgccactcccactgtcctttcctaataaaatgaggaaattgcatcgcattgtctgagtaggtgtcattctattctggggggtggggtggggcaggacagcaagggggaggattgggaagacaatagcaggcatgctggggactcgagttctacgtagataagtagcatggcgggttaatcattaactacaaggaacccctagtgatggagttggccactccctctctgcgcgctcgctcgctcactgaggccgggcgaccaaaggtcgcccgacgcccgggctttgcccgggcggcctcagtgagcgagcgagcgcgcagccttaattaacctaaggaaaatgaagtgaagttcctatactttctagagaataggaacttctatagtgagtcgaataagggcgacacaaaatttattctaaatgcataataaatactgataacatcttatagtttgtattatattttgtattatcgttgacatgtataattttgatatcaaaaactgattttccctttattattttcgagatttattttcttaattctctttaacaaactagaaatattgtatatacaaaaaatcataaataatagatgaatagtttaattataggtgttcatcaatcgaaaaagcaacgtatcttatttaaagtgcgttgcttttttctcatttataaggttaaataattctcatatatcaagcaaagtgacaggcgcccttaaatattctgacaaatgctctttccctaaactccccccataaaaaaacccgccgaagcgggtttttacgttatttgcggattaacgattactcgttatcagaaccgcccagggggcccgagcttaacctttttatttgggggagagggaagtcatgaaaaaactaacctttgaaattcgatctccagcacatcagcaaaacgctattcacgcagtacagcaaatccttccagacccaaccaaaccaatcgtagtaaccattcaggaacgcaaccgcagcttagaccaaaacaggaagctatgggcctgcttaggtgacgtctctcgtcaggttgaatggcatggtcgctggctggatgcagaaagctggaagtgtgtgtttaccgcagcattaaagcagcaggatgttgttcctaaccttgccgggaatggctttgtggtaataggccagtcaaccagcaggatgcgtgtaggcgaatttgcggagctattagagcttatacaggcattcggtacagagcgtggcgttaagtggtcagacgaagcgagactggctctggagtggaaagcgagatggggagacagggctgcatgataaatgtcgttagtttctccggtggcaggacgtcagcatatttgctctggctaatggagcaaaagcgacgggcaggtaaagacgtgcattacgttttcatggatacaggttgtgaacatccaatgacatatcggtttgtcagggaagttgtgaagttctgggatataccgctcaccgtattgcaggttgatatcaacccggagcttggacagccaaatggttatacggtatgggaaccaaaggatattcagacgcgaatgcctgttctgaagccatttatcgatatggtaaagaaatatggcactccatacgtcggcggcgcgttctgcactgacagattaaaactcgttcccttcaccaaatactgtgatgaccatttcgggcgagggaattacaccacgtggattggcatcagagctgatgaaccgaagcggctaaagccaaagcctggaatcagatatcttgctgaactgtcagactttgagaaggaagatatcctcgcatggtggaagcaacaaccattcgatttgcaaataccggaacatctcggtaactgcatattctgcattaaaaaatcaacgcaaaaaatcggacttgcctgcaaagatgaggagggattgcagcgtgtttttaatgaggtcatcacgggatcccatgtgcgtgacggacatcgggaaacgccaaaggagattatgtaccgaggaagaatgtcgctggacggtatcgcgaaaatgtattcagaaaatgattatcaagccctgtatcaggacatggtacgagctaaaagattcgataccggctcttgttctgagtcatgcgaaatatttggagggcagcttgatttcgacttcgggagggaagctgcatgatgcgatgttatcggtgcggtgaatgcaaagaagataaccgcttccgaccaaatcaaccttactggaatcgatggtgtctccggtgtgaaagaacaccaacaggggtgttaccactaccgcaggaaaaggaggacgtgtggcgagacagcgacgaagtatcaccgacataatctgcgaaaactgcaaataccttccaacgaaacgcaccagaaataaacccaagccaatcccaaaagaatctgacgtaaaaaccttcaactacacggctcacctgtgggatatccggtggctaagacgtcgtgcgaggaaaacaaggtgattgaccaaaatcgaagttacgaacaagaaagcgtcgagcgagctttaacgtgcgctaactgcggtcagaagctgcatgtgctggaagttcacgtgtgtgagcactgctgcgcagaactgatgagcgatccgaatagctcgatgcacgaggaagaagatgatggctaaaccagcgcgaagacgatgtaaaaacgatgaatgccgggaatggtttcaccctgcattcgctaatcagtggtggtgctctccagagtgtggaaccaagatagcactcgaacgacgaagtaaagaacgcgaaaaagcggaaaaagcagcagagaagaaacgacgacgagaggagcagaaacagaaagataaacttaagattcgaaaactcgccttaaagccccgcagttactggattaaacaagcccaacaagccgtaaacgccttcatcagagaaagagaccgcgacttaccatgtatctcgtgcggaacgctcacgtctgctcagtgggatgccggacattaccggacaactgctgcggcacctcaactccgatttaatgaacgcaatattcacaagcaatgcgtggtgtgcaaccagcacaaaagcggaaatctcgttccgtatcgcgtcgaactgattagccgcatcgggcaggaagcagtagacgaaatcgaatcaaaccataaccgccatcgctggactatcgaagagtgcaaggcgatcaaggcagagtaccaacagaaactcaaagacctgcgaaatagcagaagtgaggccgcatgacgttctcagtaaaaaccattccagacatgctcgttgaagcatacggaaatcagacagaagtagcacgcagactgaaatgtagtcgcggtacggtcagaaaatacgttgatgataaagacgggaaaatgcacgccatcgtcaacgacgttctcatggttcatcgcggatggagtgaaagagatgcgctattacgaaaaaattgatggcagcaaataccgaaatatttgggtagttggcgatctgcacggatgctacacgaacctgatgaacaaactggatacgattggattcgacaacaaaaaagacctgcttatctcggtgggcgatttggttgatcgtggtgcagagaacgttgaatgcctggaattaatcacattcccctggttcagagctgtacgtggaaaccatgagcaaatgatgattgatggcttatcagagcgtggaaacgttaatcactggctgcttaatggcggtggctggttctttaatctcgattacgacaaagaaattctggctaaagctcttgcccataaagcagatgaacttccgttaatcatcgaactggtgagcaaagataaaaaatatgttatctgccacgccgattatccctttgacgaatacgagtttggaaagccagttgatcatcagcaggtaatctggaaccgcgaacgaatcagcaactcacaaaacgggatcgtgaaagaaatcaaaggcgcggacacgttcatctttggtcatacgccagcagtgaaaccactcaagtttgccaaccaaatgtatatcgataccggcgcagtgttctgcggaaacctaacattgattcaggtacagggagaaggcgcatgagactcgaaagcgtagctaaatttcattcgccaaaaagcccgatgatgagcgactcaccacgggccacggcttctgactctctttccggtactgatgtgatggctgctatggggatggcgcaatcacaagccggattcggtatggctgcattctgcggtaagcacgaactcagccagaacgacaaacaaaaggctatcaactatctgatgcaatttgcacacaaggtatcggggaaataccgtggtgtggcaaagcttgaaggaaatactaaggcaaaggtactgcaagtgctcgcaacattcgcttatgcggattattgccgtagtgccgcgacgccgggggcaagatgcagagattgccatggtacaggccgtgcggttgatattgccaaaacagagctgtgggggagagttgtcgagaaagagtgcggaagatgcaaaggcgtcggctattcaaggatgccagcaagcgcagcatatcgcgctgtgacgatgctaatcccaaaccttacccaacccacctggtcacgcactgttaagccgctgtatgacgctctggtggtgcaatgccacaaagaagagtcaatcgcagacaacattttgaatgcggtcacacgttagcagcatgattgccacggatggcaacatattaacggcatgatattgacttattgaataaaattgggtaaatttgactcaacgatgggttaattcgctcgttgtggtagtgagatgaaaagaggcggcgcttactaccgattccgcctagttggtcacttcgacgtatcgtctggaactccaaccatcgcaggcagagaggtctgcaaaatgcaatcccgaaacagttcgcaggtaatagttagagcctgcataacggtttcgggattttttatatctgcacaacaggtaagagcattgagtcgataatcgtgaagagtcggcgagcctggttagccagtgctctttccgttgtgctgaattaagcgaataccggaagcagaaccggatcaccaaatgcgtacaggcgtcatcgccgcccagcaacagcacaacccaaactgagccgtagccactgtctgtcctgaattcattagtaatagttacgctgcggccttttacacatgaccttcgtgaaagcgggtggcaggaggtcgcgctaacaacctcctgccgttttgcccgtgcatatcggtcacgaacaaatctgattactaaacacagtagcctggatttgttctatcagtaatcgaccttattcctaattaaatagagcaaatccccttattgggggtaagacatgaagatgccagaaaaacatgacctgttggccgccattctcgcggcaaaggaacaaggcatcggggcaatccttgcgtttgcaatggcgtaccttcgcggcagatataatggcggtgcgtttacaaaaacagtaatcgacgcaacgatgtgcgccattatcgcctggttcattcgtgaccttctcgacttcgccggactaagtagcaatctcgcttatataacgagcgtgtttatcggctacatcggtactgactcgattggttcgcttatcaaacgcttcgctgctaaaaaagccggagtagaagatggtagaaatcaataatcaacgtaaggcgttcctcgatatgctggcgtggtcggagggaactgataacggacgtcagaaaaccagaaatcatggttatgacgtcattgtaggcggagagctatttactgattactccgatcaccctcgcaaacttgtcacgctaaacccaaaactcaaatcaacaggcgcttaagactggccgtcgttttacaacacagaaagagtttgtagaaacgcaaaaaggccatccgtcaggggccttctgcttagtttgatgcctggcagttccctactctcgccttccgcttcctcgctcactgactcgctgcgctcggtcgttcggctgcggcgagcggtatcagctcactcaaaggcggtaatacggttatccacagaatcaggggataacgcaggaaagaacatgtgagcaaaaggccagcaaaaggccaggaaccgtaaaaaggccgcgttgctggcgtttttccataggctccgcccccctgacgagcatcacaaaaatcgacgctcaagtcagaggtggcgaaacccgacaggactataaagataccaggcgtttccccctggaagctccctcgtgcgctctcctgttccgaccctgccgcttaccggatacctgtccgcctttctcccttcgggaagcgtggcgctttctcatagctcacgctgtaggtatctcagttcggtgtaggtcgttcgctccaagctgggctgtgtgcacgaaccccccgttcagcccgaccgctgcgccttatccggtaactatcgtcttgagtccaacccggtaagacacgacttatcgccactggcagcagccactggtaacaggattagcagagcgaggtatgtaggcggtgctacagagttcttgaagtggtgggctaactacggctacactagaagaacagtatttggtatctgcgctctgctgaagccagttaccttcggaaaaagagttggtagctcttgatccggcaaacaaaccaccgctggtagcggtggtttttttgtttgcaagcagcagattacgcgcagaaaaaaaggatctcaagaagatcctttgatcttttctacggggtctgacgctcagtggaacgacgcgcgcgtaactcacgttaagggattttggtcatgagcttgcgccgtcccgtcaagtcagcgtaatgctctgcttttagaaaaactcatcgagcatcaaatgaaactgcaatttattcatatcaggattatcaataccatatttttgaaaaagccgtttctgtaatgaaggagaaaactcaccgaggcagttccataggatggcaagatcctggtatcggtctgcgattccgactcgtccaacatcaatacaacctattaatttcccctcgtcaaaaataaggttatcaagtgagaaatcaccatgagtgacgactgaatccggtgagaatggcaaaagtttatgcatttctttccagacttgttcaacaggccagccattacgctcgtcatcaaaatcactcgcatcaaccaaaccgttattcattcgtgattgcgcctgagcgaggcgaaatacgcgatcgctgttaaaaggacaattacaaacaggaatcgagtgcaaccggcgcaggaacactgccagcgcatcaacaatattttcacctgaatcaggatattcttctaatacctggaacgctgtttttccggggatcgcagtggtgagtaaccatgcatcatcaggagtacggataaaatgcttgatggtcggaagtggcataaattccgtcagccagtttagtctgaccatctcatctgtaacatcattggcaacgctacctttgccatgtttcagaaacaactctggcgcatcgggcttcccatacaagcgatagattgtcgcacctgattgcccgacattatcgcgagcccatttatacccatataaatcagcatccatgttggaatttaatcgcggcctcgacgtttcccgttgaatatggctcatattcttcctttttcaatattattgaagcatttatcagggttattgtctcatgagcggatacatatttgaatgtatttagaaaaataaacaaataggggtcagtgttacaaccaattaaccaattctgaacattatcgcgagcccatttatacctgaatatggctcataacaccccttgtttgcctggcggcagtagcgcggtggtcccacctgaccccatgccgaactcagaagtgaaacgccgtagcgccgatggtagtgtggggactccccatgcgagagtagggaactgccaggcatcaaataaaacgaaaggctcagtcgaaagactgggcctttcgcccgggctaattagggggtgtcgcccttattcgactctatagtgaagttcctattctctagaaagtataggaacttctgaagtggggtcgacttaattaagg

SEQ ID NO: 40 - DNA, 11388 bp, Artificial Sequence
  constructed sequence
ctgcgcgctcgctcgctcactgaggccgcccgggcaaagcccgggcgtcgggcgacctttggtcgcccggcctcagtgagcgagcgagcgcgcagagagggagtggccaactccatcactaggggttccttgtagttaatgattaacccgccatgctacttatctacgtagcaagctagcaagatccaagctcagatctcgatcgagttgggccccagaagcctggtggttgtttgtccttctcaggggaaaagtgaggcggccccttggaggaaggggccgggcagaatgatctaatcggattccaagcagctcaggggattgtctttttctagcaccttcttgccactcctaagcgtcctccgtgaccccggctgggatttagcctggtgctgtgtcagccccggtctcccaggggcttcccagtggtccccaggaaccctcgacagggcccggtctctctcgtccagcaagggcagggacgggccacaggccaagggccctcgatcgaggaactgaaaaaccagaaagttaactggtaagtttagtctttttgtcttttatttcaggtcccggatccggtggtggtgcaaatcaaagaactgctcctcagtggatgttgcctttacttctaggcctgtacggaagtgttacttctgctctaaaagctgcggaattgtacccgcggccgccaccatgttcaagtccctcaccaaagtcaacaaggtcaagcccatcggagagaacaacgagaatgagcagagctctcggcgcaacgaagaaggatcccatccgtcgaaccagtcacagcagactaccgcacaggaggagaacaagggagaagaaaagtcgctcaagactaagtccacccccgtgacctcggaagaaccgcacacgaacattcaggacaagctgtccaagaagaactcctccggcgatctcacgactaacccggacccccagaatgccgctgaacctactgggaccgtgcctgagcaaaaggagatggaccccggaaaggagggtcctaactccccccaaaacaagcccccggccgcgccggtcatcaatgagtacgcggacgcgcaactgcataacctcgtgaagcggatgcggcaaagaaccgccctctacaagaagaaactggtggagggcgacctgagctcacctgaagccagcccacagaccgccaaacccaccgccgtgccgcctgtgaaggagtccgatgacaagcctaccgagcactactaccgcctgctgtggttcaaggtcaagaagatgcccctgaccgaatacctcaagcggatcaagctgccgaacagcatcgacagctacaccgaccggctttacttgctctggctgctgcttgtgaccctggcttacaactggaactgttgtttcattcccctgcggctggtgttcccttaccaaaccgcggataacattcactactggctgattgccgacatcatttgcgacatcatctacctgtacgatatgctttttatccaaccgcggctgcaattcgtccgcgggggagacatcattgtggactccaacgagctgcgcaagcattaccggacctcgacaaagttccagctggatgtggcctccatcatcccgttcgatatctgttacctgttctttggcttcaacccgatgttcagggcgaacaggatgctgaagtacacttccttcttcgaattcaaccaccacctggagtccatcatggacaaggcttacatctaccgcgtgatccggaccactggttacctcctgttcatcctgcacatcaacgcctgcgtctattactgggcctcaaactacgaaggcattggtaccacccgctgggtgtacgacggggagggaaacgagtatctgcgctgctactactgggccgtgcgaaccctcataactattggcggcctcccggaaccgcagaccctgttcgagatcgtgttccaactcctcaacttcttctcgggagtgttcgtgttttcaagcttgattggacagatgcgggacgtgatcggtgcagcaactgccaaccagaactactttcgcgcctgcatggacgacactatcgcgtacatgaacaactattcgatccccaagctggtgcagaaacgcgtgcggacttggtatgagtacacttgggactcccagagaatgcttgacgagtccgatctgctcaagaccctgcctactaccgtgcagctggcactcgccatcgatgtgaacttctccattatctcgaaagtcgatctgttcaagggctgcgacacccagatgatctacgacatgctgctgagactcaagtccgtgttgtacctccctggcgacttcgtgtgcaagaagggcgaaatcgggaaggagatgtacattatcaagcacggagaagtccaggtgctggggggaccagacggtaccaaggtccttgtcaccctgaaggccgggtccgtgttcggcgaaatttccctgttggccgccggcggtggcaacaggagaaccgcaaatgtggtggcccacggcttcgcaaaccttctgaccctggacaagaaaaccctccaggaaatcctcgtgcactacccggatagcgagcggatcctgatgaagaaagcccgggtgctgctgaagcaaaaggccaagaccgccgaagccaccccgcctcggaaggacctggctctgctgttcccacccaaggaggagactcccaaactgtttaagaccctcttgggcgggacgggaaaggcctccctcgctcgcttgcttaagttgaagagggagcaggccgcgcagaagaaggaaaactccgaaggaggggaagaagagggaaaggaaaacgaagataagcagaaggagaacgaggataagcaaaaggaaaatgaggacaaggggaaagaaaacgaggacaaggataagggtcgcgaacctgaagagaagccgctggatcggccagagtgcactgcctcgcctatcgcggtcgaagaggaaccccatagcgtgcgcagaaccgtgctgcctagaggcacatcgaggcagtcactgattatctctatggcaccaagcgccgagggaggagaggaagtgctcaccatcgaggtcaaggaaaaagcgaagcagtgatcataactgcagatctgcctcgactgtgccttctagttgccagccatctgttgtttgcccctcccccgtgccttccttgaccctggaaggtgccactcccactgtcctttcctaataaaatgaggaaattgcatcgcattgtctgagtaggtgtcattctattctggggggtggggtggggcaggacagcaagggggaggattgggaagacaatagcaggcatgctggggactcgagttctacgtagataagtagcatggcgggttaatcattaactacaaggaacccctagtgatggagttggccactccctctctgcgcgctcgctcgctcactgaggccgggcgaccaaaggtcgcccgacgcccgggctttgcccgggcggcctcagtgagcgagcgagcgcgcagccttaattaacctaaggaaaatgaagtgaagttcctatactttctagagaataggaacttctatagtgagtcgaataagggcgacacaaaatttattctaaatgcataataaatactgataacatcttatagtttgtattatattttgtattatcgttgacatgtataattttgatatcaaaaactgattttccctttattattttcgagatttattttcttaattctctttaacaaactagaaatattgtatatacaaaaaatcataaataatagatgaatagtttaattataggtgttcatcaatcgaaaaagcaacgtatcttatttaaagtgcgttgcttttttctcatttataaggttaaataattctcatatatcaagcaaagtgacaggcgcccttaaatattctgacaaatgctctttccctaaactccccccataaaaaaacccgccgaagcgggtttttacgttatttgcggattaacgattactcgttatcagaaccgcccagggggcccgagcttaacctttttatttgggggagagggaagtcatgaaaaaactaacctttgaaattcgatctccagcacatcagcaaaacgctattcacgcagtacagcaaatccttccagacccaaccaaaccaatcgtagtaaccattcaggaacgcaaccgcagcttagaccaaaacaggaagctatgggcctgcttaggtgacgtctctcgtcaggttgaatggcatggtcgctggctggatgcagaaagctggaagtgtgtgtttaccgcagcattaaagcagcaggatgttgttcctaaccttgccgggaatggctttgtggtaataggccagtcaaccagcaggatgcgtgtaggcgaatttgcggagctattagagcttatacaggcattcggtacagagcgtggcgttaagtggtcagacgaagcgagactggctctggagtggaaagcgagatggggagacagggctgcatgataaatgtcgttagtttctccggtggcaggacgtcagcatatttgctctggctaatggagcaaaagcgacgggcaggtaaagacgtgcattacgttttcatggatacaggttgtgaacatccaatgacatatcggtttgtcagggaagttgtgaagttctgggatataccgctcaccgtattgcaggttgatatcaacccggagcttggacagccaaatggttatacggtatgggaaccaaaggatattcagacgcgaatgcctgttctgaagccatttatcgatatggtaaagaaatatggcactccatacgtcggcggcgcgttctgcactgacagattaaaactcgttcccttcaccaaatactgtgatgaccatttcgggcgagggaattacaccacgtggattggcatcagagctgatgaaccgaagcggctaaagccaaagcctggaatcagatatcttgctgaactgtcagactttgagaaggaagatatcctcgcatggtggaagcaacaaccattcgatttgcaaataccggaacatctcggtaactgcatattctgcattaaaaaatcaacgcaaaaaatcggacttgcctgcaaagatgaggagggattgcagcgtgtttttaatgaggtcatcacgggatcccatgtgcgtgacggacatcgggaaacgccaaaggagattatgtaccgaggaagaatgtcgctggacggtatcgcgaaaatgtattcagaaaatgattatcaagccctgtatcaggacatggtacgagctaaaagattcgataccggctcttgttctgagtcatgcgaaatatttggagggcagcttgatttcgacttcgggagggaagctgcatgatgcgatgttatcggtgcggtgaatgcaaagaagataaccgcttccgaccaaatcaaccttactggaatcgatggtgtctccggtgtgaaagaacaccaacaggggtgttaccactaccgcaggaaaaggaggacgtgtggcgagacagcgacgaagtatcaccgacataatctgcgaaaactgcaaataccttccaacgaaacgcaccagaaataaacccaagccaatcccaaaagaatctgacgtaaaaaccttcaactacacggctcacctgtgggatatccggtggctaagacgtcgtgcgaggaaaacaaggtgattgaccaaaatcgaagttacgaacaagaaagcgtcgagcgagctttaacgtgcgctaactgcggtcagaagctgcatgtgctggaagttcacgtgtgtgagcactgctgcgcagaactgatgagcgatccgaatagctcgatgcacgaggaagaagatgatggctaaaccagcgcgaagacgatgtaaaaacgatgaatgccgggaatggtttcaccctgcattcgctaatcagtggtggtgctctccagagtgtggaaccaagatagcactcgaacgacgaagtaaagaacgcgaaaaagcggaaaaagcagcagagaagaaacgacgacgagaggagcagaaacagaaagataaacttaagattcgaaaactcgccttaaagccccgcagttactggattaaacaagcccaacaagccgtaaacgccttcatcagagaaagagaccgcgacttaccatgtatctcgtgcggaacgctcacgtctgctcagtgggatgccggacattaccggacaactgctgcggcacctcaactccgatttaatgaacgcaatattcacaagcaatgcgtggtgtgcaaccagcacaaaagcggaaatctcgttccgtatcgcgtcgaactgattagccgcatcgggcaggaagcagtagacgaaatcgaatcaaaccataaccgccatcgctggactatcgaagagtgcaaggcgatcaaggcagagtaccaacagaaactcaaagacctgcgaaatagcagaagtgaggccgcatgacgttctcagtaaaaaccattccagacatgctcgttgaagcatacggaaatcagacagaagtagcacgcagactgaaatgtagtcgcggtacggtcagaaaatacgttgatgataaagacgggaaaatgcacgccatcgtcaacgacgttctcatggttcatcgcggatggagtgaaagagatgcgctattacgaaaaaattgatggcagcaaataccgaaatatttgggtagttggcgatctgcacggatgctacacgaacctgatgaacaaactggatacgattggattcgacaacaaaaaagacctgcttatctcggtgggcgatttggttgatcgtggtgcagagaacgttgaatgcctggaattaatcacattcccctggttcagagctgtacgtggaaaccatgagcaaatgatgattgatggcttatcagagcgtggaaacgttaatcactggctgcttaatggcggtggctggttctttaatctcgattacgacaaagaaattctggctaaagctcttgcccataaagcagatgaacttccgttaatcatcgaactggtgagcaaagataaaaaatatgttatctgccacgccgattatccctttgacgaatacgagtttggaaagccagttgatcatcagcaggtaatctggaaccgcgaacgaatcagcaactcacaaaacgggatcgtgaaagaaatcaaaggcgcggacacgttcatctttggtcatacgccagcagtgaaaccactcaagtttgccaaccaaatgtatatcgataccggcgcagtgttctgcggaaacctaacattgattcaggtacagggagaaggcgcatgagactcgaaagcgtagctaaatttcattcgccaaaaagcccgatgatgagcgactcaccacgggccacggcttctgactctctttccggtactgatgtgatggctgctatggggatggcgcaatcacaagccggattcggtatggctgcattctgcggtaagcacgaactcagccagaacgacaaacaaaaggctatcaactatctgatgcaatttgcacacaaggtatcggggaaataccgtggtgtggcaaagcttgaaggaaatactaaggcaaaggtactgcaagtgctcgcaacattcgcttatgcggattattgccgtagtgccgcgacgccgggggcaagatgcagagattgccatggtacaggccgtgcggttgatattgccaaaacagagctgtgggggagagttgtcgagaaagagtgcggaagatgcaaaggcgtcggctattcaaggatgccagcaagcgcagcatatcgcgctgtgacgatgctaatcccaaaccttacccaacccacctggtcacgcactgttaagccgctgtatgacgctctggtggtgcaatgccacaaagaagagtcaatcgcagacaacattttgaatgcggtcacacgttagcagcatgattgccacggatggcaacatattaacggcatgatattgacttattgaataaaattgggtaaatttgactcaacgatgggttaattcgctcgttgtggtagtgagatgaaaagaggcggcgcttactaccgattccgcctagttggtcacttcgacgtatcgtctggaactccaaccatcgcaggcagagaggtctgcaaaatgcaatcccgaaacagttcgcaggtaatagttagagcctgcataacggtttcgggattttttatatctgcacaacaggtaagagcattgagtcgataatcgtgaagagtcggcgagcctggttagccagtgctctttccgttgtgctgaattaagcgaataccggaagcagaaccggatcaccaaatgcgtacaggcgtcatcgccgcccagcaacagcacaacccaaactgagccgtagccactgtctgtcctgaattcattagtaatagttacgctgcggccttttacacatgaccttcgtgaaagcgggtggcaggaggtcgcgctaacaacctcctgccgttttgcccgtgcatatcggtcacgaacaaatctgattactaaacacagtagcctggatttgttctatcagtaatcgaccttattcctaattaaatagagcaaatccccttattgggggtaagacatgaagatgccagaaaaacatgacctgttggccgccattctcgcggcaaaggaacaaggcatcggggcaatccttgcgtttgcaatggcgtaccttcgcggcagatataatggcggtgcgtttacaaaaacagtaatcgacgcaacgatgtgcgccattatcgcctggttcattcgtgaccttctcgacttcgccggactaagtagcaatctcgcttatataacgagcgtgtttatcggctacatcggtactgactcgattggttcgcttatcaaacgcttcgctgctaaaaaagccggagtagaagatggtagaaatcaataatcaacgtaaggcgttcctcgatatgctggcgtggtcggagggaactgataacggacgtcagaaaaccagaaatcatggttatgacgtcattgtaggcggagagctatttactgattactccgatcaccctcgcaaacttgtcacgctaaacccaaaactcaaatcaacaggcgcttaagactggccgtcgttttacaacacagaaagagtttgtagaaacgcaaaaaggccatccgtcaggggccttctgcttagtttgatgcctggcagttccctactctcgccttccgcttcctcgctcactgactcgctgcgctcggtcgttcggctgcggcgagcggtatcagctcactcaaaggcggtaatacggttatccacagaatcaggggataacgcaggaaagaacatgtgagcaaaaggccagcaaaaggccaggaaccgtaaaaaggccgcgttgctggcgtttttccataggctccgcccccctgacgagcatcacaaaaatcgacgctcaagtcagaggtggcgaaacccgacaggactataaagataccaggcgtttccccctggaagctccctcgtgcgctctcctgttccgaccctgccgcttaccggatacctgtccgcctttctcccttcgggaagcgtggcgctttctcatagctcacgctgtaggtatctcagttcggtgtaggtcgttcgctccaagctgggctgtgtgcacgaaccccccgttcagcccgaccgctgcgccttatccggtaactatcgtcttgagtccaacccggtaagacacgacttatcgccactggcagcagccactggtaacaggattagcagagcgaggtatgtaggcggtgctacagagttcttgaagtggtgggctaactacggctacactagaagaacagtatttggtatctgcgctctgctgaagccagttaccttcggaaaaagagttggtagctcttgatccggcaaacaaaccaccgctggtagcggtggtttttttgtttgcaagcagcagattacgcgcagaaaaaaaggatctcaagaagatcctttgatcttttctacggggtctgacgctcagtggaacgacgcgcgcgtaactcacgttaagggattttggtcatgagcttgcgccgtcccgtcaagtcagcgtaatgctctgcttttagaaaaactcatcgagcatcaaatgaaactgcaatttattcatatcaggattatcaataccatatttttgaaaaagccgtttctgtaatgaaggagaaaactcaccgaggcagttccataggatggcaagatcctggtatcggtctgcgattccgactcgtccaacatcaatacaacctattaatttcccctcgtcaaaaataaggttatcaagtgagaaatcaccatgagtgacgactgaatccggtgagaatggcaaaagtttatgcatttctttccagacttgttcaacaggccagccattacgctcgtcatcaaaatcactcgcatcaaccaaaccgttattcattcgtgattgcgcctgagcgaggcgaaatacgcgatcgctgttaaaaggacaattacaaacaggaatcgagtgcaaccggcgcaggaacactgccagcgcatcaacaatattttcacctgaatcaggatattcttctaatacctggaacgctgtttttccggggatcgcagtggtgagtaaccatgcatcatcaggagtacggataaaatgcttgatggtcggaagtggcataaattccgtcagccagtttagtctgaccatctcatctgtaacatcattggcaacgctacctttgccatgtttcagaaacaactctggcgcatcgggcttcccatacaagcgatagattgtcgcacctgattgcccgacattatcgcgagcccatttatacccatataaatcagcatccatgttggaatttaatcgcggcctcgacgtttcccgttgaatatggctcatattcttcctttttcaatattattgaagcatttatcagggttattgtctcatgagcggatacatatttgaatgtatttagaaaaataaacaaataggggtcagtgttacaaccaattaaccaattctgaacattatcgcgagcccatttatacctgaatatggctcataacaccccttgtttgcctggcggcagtagcgcggtggtcccacctgaccccatgccgaactcagaagtgaaacgccgtagcgccgatggtagtgtggggactccccatgcgagagtagggaactgccaggcatcaaataaaacgaaaggctcagtcgaaagactgggcctttcgcccgggctaattagggggtgtcgcccttattcgactctatagtgaagttcctattctctagaaagtataggaacttctgaagtggggtcgacttaattaagg

SEQ ID NO: 41 - DNA, 11782 bp, Artificial Sequence
  constructed sequence
ctgcgcgctcgctcgctcactgaggccgcccgggcaaagcccgggcgtcgggcgacctttggtcgcccggcctcagtgagcgagcgagcgcgcagagagggagtggccaactccatcactaggggttccttgtagttaatgattaacccgccatgctacttatctacgtagcaagctagcctgaagagacagaaatatctctaattccatgagcggtcatacgaggcaagagaagccgcttagagcatggacttagttagtttcagggattggacagagtcaagagctggggtgaggaggttaccctcggtaggggtgacacagatgtcaaccgcctattccctccacatgcatgtcctgccagaagaacctgtccctgggctgggaatcttatattaccttcctctccaatgagaagagaagttcaaggctcacagacatgtgcatacacaagctcaatgcactcaagattcccctccaccactcctgcccccactacctacaggagattgactcctgctgtgcacataagctgggataatcagggtttctaaacatcagcttcaaaagtccaatgtccaaagtggtggggggccggggaacgaggtactctttccatacccttggcttttgtgtggcctggagccgctgatatagagattggagtgggacacgaggtattcctttcaaaaacacaaaggcctatactttgagccctcccatttcaatcccccaccatgcttcacctttaagacctccaactccactttgatcccagttctcaggttcaggcctcacaaggccaaaatcctgaagttacccttctcaaactcccttgcctttaacatcatcagaatcaacctcctacccccactctgtcccagcagcaatagcctgctaatcttttagcactaatcttttaggcactaatctgctttccaaactcttggcacctgaactatttataagcagtgttttatgcccccccaccaaagaaccctattcttttcccatgaccccaccaatcaaaacactcagaggactgtgggtataagaggctggggaggcaggcatagcagcggccgccaccatgtttaaatcgctgacaaaagtcaacaaggtgaagcctataggagagaacaatgagaatgaacaaagttctcgtcggaatgaagaaggctctcacccaagtaatcagtctcagcaaaccacagcacaggaagaaaacaaaggtgaagagaaatctctcaaaaccaagtcaactccagtcacgtctgaagagccacacaccaacatacaagacaaactctccaagaaaaattcctctggagatctgaccacaaaccctgaccctcaaaatgcagcagaaccaactggaacagtgccagagcagaaggaaatggaccccgggaaagaaggtccaaacagcccacaaaacaaaccgccagcagctcctgttataaatgagtatgccgatgcccagctacacaacctggtgaaaagaatgcgtcaaagaacagccctctacaagaaaaagttggtagagggagatctctcctcacccgaagccagcccacaaactgcaaagcccacggctgtaccaccagtaaaagaaagcgatgataagccaacagaacattactacaggctgttgtggttcaaagtcaaaaagatgcctttaacagagtacttaaagcgaattaaacttccaaacagcatagattcatacacagatcgactctatctcctgtggctcttgcttgtcactcttgcctataactggaactgctgttttataccactgcgcctcgtcttcccatatcaaaccgcagacaacatacactactggcttattgcggacatcatctgtgatatcatctacctttatgatatgctatttatccagcccagactccagtttgtaagaggaggagacataatagtggattcaaatgagctaaggaaacactacaggacttctacaaaatttcagttggatgtcgcatcaataataccatttgatatttgctacctcttctttgggtttaatccaatgtttagagcaaataggatgttaaagtacacttcattttttgaatttaatcatcacctagagtctataatggacaaagcatatatctacagagttattcgaacaactggatacttgctgtttattctgcacattaatgcctgtgtttattactgggcttcaaactatgaaggaattggcactactagatgggtgtatgatggggaaggaaacgagtatctgagatgttattattgggcagttcgaactttaattaccattggtggccttccagaaccacaaactttatttgaaattgtttttcaactcttgaattttttttctggagtttttgtgttctccagtttaattggtcagatgagagatgtgattggagcagctacagccaatcagaactacttccgcgcctgcatggatgacaccattgcctacatgaacaattactccattcctaaacttgtgcaaaagcgagttcggacttggtatgaatatacatgggactctcaaagaatgctagatgagtctgatttgcttaagaccctaccaactacggtccagttagccctcgccattgatgtgaacttcagcatcatcagcaaagttgacttgttcaagggttgtgatacacagatgatttatgacatgttgctaagattgaaatccgttctctatttgcctggtgactttgtctgcaaaaagggagaaattggcaaggaaatgtatatcatcaagcatggagaagtccaagttcttggaggccctgatggtactaaagttctggttactctgaaagctgggtcggtgtttggagaaatcagccttctagcagcaggaggaggaaaccgtcgaactgccaatgtggtggcccacgggtttgccaatcttttaactctagacaaaaagaccctccaagaaattctagtgcattatccagattctgaaagaatcctcatgaagaaagccagagtgcttttaaagcagaaggctaagaccgcagaagcaacccctccaagaaaagatcttgccctcctcttcccaccgaaagaagagacacccaaactgtttaaaactctcctaggaggcacaggaaaagcaagtcttgcaagactactcaaattgaagcgagagcaagcagctcagaagaaagaaaattctgaaggaggagaggaagaaggaaaagaaaatgaagataaacaaaaagaaaatgaagataaacaaaaagaaaatgaagataaaggaaaagaaaatgaagataaagataaaggaagagagccagaagagaagccactggacagacctgaatgtacagcaagtcctattgcagtggaggaagaaccccactcagttagaaggacagttttacccagagggacttctcgtcaatcactcattatcagcatggctccttctgctgagggcggagaagaggttcttactattgaagtcaaagaaaaggctaagcaatgatcataactgcagatctgcctcgactgtgccttctagttgccagccatctgttgtttgcccctcccccgtgccttccttgaccctggaaggtgccactcccactgtcctttcctaataaaatgaggaaattgcatcgcattgtctgagtaggtgtcattctattctggggggtggggtggggcaggacagcaagggggaggattgggaagacaatagcaggcatgctggggactcgagttctacgtagataagtagcatggcgggttaatcattaactacaaggaacccctagtgatggagttggccactccctctctgcgcgctcgctcgctcactgaggccgggcgaccaaaggtcgcccgacgcccgggctttgcccgggcggcctcagtgagcgagcgagcgcgcagccttaattaacctaaggaaaatgaagtgaagttcctatactttctagagaataggaacttctatagtgagtcgaataagggcgacacaaaatttattctaaatgcataataaatactgataacatcttatagtttgtattatattttgtattatcgttgacatgtataattttgatatcaaaaactgattttccctttattattttcgagatttattttcttaattctctttaacaaactagaaatattgtatatacaaaaaatcataaataatagatgaatagtttaattataggtgttcatcaatcgaaaaagcaacgtatcttatttaaagtgcgttgcttttttctcatttataaggttaaataattctcatatatcaagcaaagtgacaggcgcccttaaatattctgacaaatgctctttccctaaactccccccataaaaaaacccgccgaagcgggtttttacgttatttgcggattaacgattactcgttatcagaaccgcccagggggcccgagcttaacctttttatttgggggagagggaagtcatgaaaaaactaacctttgaaattcgatctccagcacatcagcaaaacgctattcacgcagtacagcaaatccttccagacccaaccaaaccaatcgtagtaaccattcaggaacgcaaccgcagcttagaccaaaacaggaagctatgggcctgcttaggtgacgtctctcgtcaggttgaatggcatggtcgctggctggatgcagaaagctggaagtgtgtgtttaccgcagcattaaagcagcaggatgttgttcctaaccttgccgggaatggctttgtggtaataggccagtcaaccagcaggatgcgtgtaggcgaatttgcggagctattagagcttatacaggcattcggtacagagcgtggcgttaagtggtcagacgaagcgagactggctctggagtggaaagcgagatggggagacagggctgcatgataaatgtcgttagtttctccggtggcaggacgtcagcatatttgctctggctaatggagcaaaagcgacgggcaggtaaagacgtgcattacgttttcatggatacaggttgtgaacatccaatgacatatcggtttgtcagggaagttgtgaagttctgggatataccgctcaccgtattgcaggttgatatcaacccggagcttggacagccaaatggttatacggtatgggaaccaaaggatattcagacgcgaatgcctgttctgaagccatttatcgatatggtaaagaaatatggcactccatacgtcggcggcgcgttctgcactgacagattaaaactcgttcccttcaccaaatactgtgatgaccatttcgggcgagggaattacaccacgtggattggcatcagagctgatgaaccgaagcggctaaagccaaagcctggaatcagatatcttgctgaactgtcagactttgagaaggaagatatcctcgcatggtggaagcaacaaccattcgatttgcaaataccggaacatctcggtaactgcatattctgcattaaaaaatcaacgcaaaaaatcggacttgcctgcaaagatgaggagggattgcagcgtgtttttaatgaggtcatcacgggatcccatgtgcgtgacggacatcgggaaacgccaaaggagattatgtaccgaggaagaatgtcgctggacggtatcgcgaaaatgtattcagaaaatgattatcaagccctgtatcaggacatggtacgagctaaaagattcgataccggctcttgttctgagtcatgcgaaatatttggagggcagcttgatttcgacttcgggagggaagctgcatgatgcgatgttatcggtgcggtgaatgcaaagaagataaccgcttccgaccaaatcaaccttactggaatcgatggtgtctccggtgtgaaagaacaccaacaggggtgttaccactaccgcaggaaaaggaggacgtgtggcgagacagcgacgaagtatcaccgacataatctgcgaaaactgcaaataccttccaacgaaacgcaccagaaataaacccaagccaatcccaaaagaatctgacgtaaaaaccttcaactacacggctcacctgtgggatatccggtggctaagacgtcgtgcgaggaaaacaaggtgattgaccaaaatcgaagttacgaacaagaaagcgtcgagcgagctttaacgtgcgctaactgcggtcagaagctgcatgtgctggaagttcacgtgtgtgagcactgctgcgcagaactgatgagcgatccgaatagctcgatgcacgaggaagaagatgatggctaaaccagcgcgaagacgatgtaaaaacgatgaatgccgggaatggtttcaccctgcattcgctaatcagtggtggtgctctccagagtgtggaaccaagatagcactcgaacgacgaagtaaagaacgcgaaaaagcggaaaaagcagcagagaagaaacgacgacgagaggagcagaaacagaaagataaacttaagattcgaaaactcgccttaaagccccgcagttactggattaaacaagcccaacaagccgtaaacgccttcatcagagaaagagaccgcgacttaccatgtatctcgtgcggaacgctcacgtctgctcagtgggatgccggacattaccggacaactgctgcggcacctcaactccgatttaatgaacgcaatattcacaagcaatgcgtggtgtgcaaccagcacaaaagcggaaatctcgttccgtatcgcgtcgaactgattagccgcatcgggcaggaagcagtagacgaaatcgaatcaaaccataaccgccatcgctggactatcgaagagtgcaaggcgatcaaggcagagtaccaacagaaactcaaagacctgcgaaatagcagaagtgaggccgcatgacgttctcagtaaaaaccattccagacatgctcgttgaagcatacggaaatcagacagaagtagcacgcagactgaaatgtagtcgcggtacggtcagaaaatacgttgatgataaagacgggaaaatgcacgccatcgtcaacgacgttctcatggttcatcgcggatggagtgaaagagatgcgctattacgaaaaaattgatggcagcaaataccgaaatatttgggtagttggcgatctgcacggatgctacacgaacctgatgaacaaactggatacgattggattcgacaacaaaaaagacctgcttatctcggtgggcgatttggttgatcgtggtgcagagaacgttgaatgcctggaattaatcacattcccctggttcagagctgtacgtggaaaccatgagcaaatgatgattgatggcttatcagagcgtggaaacgttaatcactggctgcttaatggcggtggctggttctttaatctcgattacgacaaagaaattctggctaaagctcttgcccataaagcagatgaacttccgttaatcatcgaactggtgagcaaagataaaaaatatgttatctgccacgccgattatccctttgacgaatacgagtttggaaagccagttgatcatcagcaggtaatctggaaccgcgaacgaatcagcaactcacaaaacgggatcgtgaaagaaatcaaaggcgcggacacgttcatctttggtcatacgccagcagtgaaaccactcaagtttgccaaccaaatgtatatcgataccggcgcagtgttctgcggaaacctaacattgattcaggtacagggagaaggcgcatgagactcgaaagcgtagctaaatttcattcgccaaaaagcccgatgatgagcgactcaccacgggccacggcttctgactctctttccggtactgatgtgatggctgctatggggatggcgcaatcacaagccggattcggtatggctgcattctgcggtaagcacgaactcagccagaacgacaaacaaaaggctatcaactatctgatgcaatttgcacacaaggtatcggggaaataccgtggtgtggcaaagcttgaaggaaatactaaggcaaaggtactgcaagtgctcgcaacattcgcttatgcggattattgccgtagtgccgcgacgccgggggcaagatgcagagattgccatggtacaggccgtgcggttgatattgccaaaacagagctgtgggggagagttgtcgagaaagagtgcggaagatgcaaaggcgtcggctattcaaggatgccagcaagcgcagcatatcgcgctgtgacgatgctaatcccaaaccttacccaacccacctggtcacgcactgttaagccgctgtatgacgctctggtggtgcaatgccacaaagaagagtcaatcgcagacaacattttgaatgcggtcacacgttagcagcatgattgccacggatggcaacatattaacggcatgatattgacttattgaataaaattgggtaaatttgactcaacgatgggttaattcgctcgttgtggtagtgagatgaaaagaggcggcgcttactaccgattccgcctagttggtcacttcgacgtatcgtctggaactccaaccatcgcaggcagagaggtctgcaaaatgcaatcccgaaacagttcgcaggtaatagttagagcctgcataacggtttcgggattttttatatctgcacaacaggtaagagcattgagtcgataatcgtgaagagtcggcgagcctggttagccagtgctctttccgttgtgctgaattaagcgaataccggaagcagaaccggatcaccaaatgcgtacaggcgtcatcgccgcccagcaacagcacaacccaaactgagccgtagccactgtctgtcctgaattcattagtaatagttacgctgcggccttttacacatgaccttcgtgaaagcgggtggcaggaggtcgcgctaacaacctcctgccgttttgcccgtgcatatcggtcacgaacaaatctgattactaaacacagtagcctggatttgttctatcagtaatcgaccttattcctaattaaatagagcaaatccccttattgggggtaagacatgaagatgccagaaaaacatgacctgttggccgccattctcgcggcaaaggaacaaggcatcggggcaatccttgcgtttgcaatggcgtaccttcgcggcagatataatggcggtgcgtttacaaaaacagtaatcgacgcaacgatgtgcgccattatcgcctggttcattcgtgaccttctcgacttcgccggactaagtagcaatctcgcttatataacgagcgtgtttatcggctacatcggtactgactcgattggttcgcttatcaaacgcttcgctgctaaaaaagccggagtagaagatggtagaaatcaataatcaacgtaaggcgttcctcgatatgctggcgtggtcggagggaactgataacggacgtcagaaaaccagaaatcatggttatgacgtcattgtaggcggagagctatttactgattactccgatcaccctcgcaaacttgtcacgctaaacccaaaactcaaatcaacaggcgcttaagactggccgtcgttttacaacacagaaagagtttgtagaaacgcaaaaaggccatccgtcaggggccttctgcttagtttgatgcctggcagttccctactctcgccttccgcttcctcgctcactgactcgctgcgctcggtcgttcggctgcggcgagcggtatcagctcactcaaaggcggtaatacggttatccacagaatcaggggataacgcaggaaagaacatgtgagcaaaaggccagcaaaaggccaggaaccgtaaaaaggccgcgttgctggcgtttttccataggctccgcccccctgacgagcatcacaaaaatcgacgctcaagtcagaggtggcgaaacccgacaggactataaagataccaggcgtttccccctggaagctccctcgtgcgctctcctgttccgaccctgccgcttaccggatacctgtccgcctttctcccttcgggaagcgtggcgctttctcatagctcacgctgtaggtatctcagttcggtgtaggtcgttcgctccaagctgggctgtgtgcacgaaccccccgttcagcccgaccgctgcgccttatccggtaactatcgtcttgagtccaacccggtaagacacgacttatcgccactggcagcagccactggtaacaggattagcagagcgaggtatgtaggcggtgctacagagttcttgaagtggtgggctaactacggctacactagaagaacagtatttggtatctgcgctctgctgaagccagttaccttcggaaaaagagttggtagctcttgatccggcaaacaaaccaccgctggtagcggtggtttttttgtttgcaagcagcagattacgcgcagaaaaaaaggatctcaagaagatcctttgatcttttctacggggtctgacgctcagtggaacgacgcgcgcgtaactcacgttaagggattttggtcatgagcttgcgccgtcccgtcaagtcagcgtaatgctctgcttttagaaaaactcatcgagcatcaaatgaaactgcaatttattcatatcaggattatcaataccatatttttgaaaaagccgtttctgtaatgaaggagaaaactcaccgaggcagttccataggatggcaagatcctggtatcggtctgcgattccgactcgtccaacatcaatacaacctattaatttcccctcgtcaaaaataaggttatcaagtgagaaatcaccatgagtgacgactgaatccggtgagaatggcaaaagtttatgcatttctttccagacttgttcaacaggccagccattacgctcgtcatcaaaatcactcgcatcaaccaaaccgttattcattcgtgattgcgcctgagcgaggcgaaatacgcgatcgctgttaaaaggacaattacaaacaggaatcgagtgcaaccggcgcaggaacactgccagcgcatcaacaatattttcacctgaatcaggatattcttctaatacctggaacgctgtttttccggggatcgcagtggtgagtaaccatgcatcatcaggagtacggataaaatgcttgatggtcggaagtggcataaattccgtcagccagtttagtctgaccatctcatctgtaacatcattggcaacgctacctttgccatgtttcagaaacaactctggcgcatcgggcttcccatacaagcgatagattgtcgcacctgattgcccgacattatcgcgagcccatttatacccatataaatcagcatccatgttggaatttaatcgcggcctcgacgtttcccgttgaatatggctcatattcttcctttttcaatattattgaagcatttatcagggttattgtctcatgagcggatacatatttgaatgtatttagaaaaataaacaaataggggtcagtgttacaaccaattaaccaattctgaacattatcgcgagcccatttatacctgaatatggctcataacaccccttgtttgcctggcggcagtagcgcggtggtcccacctgaccccatgccgaactcagaagtgaaacgccgtagcgccgatggtagtgtggggactccccatgcgagagtagggaactgccaggcatcaaataaaacgaaaggctcagtcgaaagactgggcctttcgcccgggctaattagggggtgtcgcccttattcgactctatagtgaagttcctattctctagaaagtataggaacttctgaagtggggtcgacttaattaagg

SEQ ID NO: 42 - DNA, 11782 bp, Artificial Sequence
  constructed sequence
ctgcgcgctcgctcgctcactgaggccgcccgggcaaagcccgggcgtcgggcgacctttggtcgcccggcctcagtgagcgagcgagcgcgcagagagggagtggccaactccatcactaggggttccttgtagttaatgattaacccgccatgctacttatctacgtagcaagctagcctgaagagacagaaatatctctaattccatgagcggtcatacgaggcaagagaagccgcttagagcatggacttagttagtttcagggattggacagagtcaagagctggggtgaggaggttaccctcggtaggggtgacacagatgtcaaccgcctattccctccacatgcatgtcctgccagaagaacctgtccctgggctgggaatcttatattaccttcctctccaatgagaagagaagttcaaggctcacagacatgtgcatacacaagctcaatgcactcaagattcccctccaccactcctgcccccactacctacaggagattgactcctgctgtgcacataagctgggataatcagggtttctaaacatcagcttcaaaagtccaatgtccaaagtggtggggggccggggaacgaggtactctttccatacccttggcttttgtgtggcctggagccgctgatatagagattggagtgggacacgaggtattcctttcaaaaacacaaaggcctatactttgagccctcccatttcaatcccccaccatgcttcacctttaagacctccaactccactttgatcccagttctcaggttcaggcctcacaaggccaaaatcctgaagttacccttctcaaactcccttgcctttaacatcatcagaatcaacctcctacccccactctgtcccagcagcaatagcctgctaatcttttagcactaatcttttaggcactaatctgctttccaaactcttggcacctgaactatttataagcagtgttttatgcccccccaccaaagaaccctattcttttcccatgaccccaccaatcaaaacactcagaggactgtgggtataagaggctggggaggcaggcatagcagcggccgccaccatgttcaagtccctcaccaaagtcaacaaggtcaagcccatcggagagaacaacgagaatgagcagagctctcggcgcaacgaagaaggatcccatccgtcgaaccagtcacagcagactaccgcacaggaggagaacaagggagaagaaaagtcgctcaagactaagtccacccccgtgacctcggaagaaccgcacacgaacattcaggacaagctgtccaagaagaactcctccggcgatctcacgactaacccggacccccagaatgccgctgaacctactgggaccgtgcctgagcaaaaggagatggaccccggaaaggagggtcctaactccccccaaaacaagcccccggccgcgccggtcatcaatgagtacgcggacgcgcaactgcataacctcgtgaagcggatgcggcaaagaaccgccctctacaagaagaaactggtggagggcgacctgagctcacctgaagccagcccacagaccgccaaacccaccgccgtgccgcctgtgaaggagtccgatgacaagcctaccgagcactactaccgcctgctgtggttcaaggtcaagaagatgcccctgaccgaatacctcaagcggatcaagctgccgaacagcatcgacagctacaccgaccggctttacttgctctggctgctgcttgtgaccctggcttacaactggaactgttgtttcattcccctgcggctggtgttcccttaccaaaccgcggataacattcactactggctgattgccgacatcatttgcgacatcatctacctgtacgatatgctttttatccaaccgcggctgcaattcgtccgcgggggagacatcattgtggactccaacgagctgcgcaagcattaccggacctcgacaaagttccagctggatgtggcctccatcatcccgttcgatatctgttacctgttctttggcttcaacccgatgttcagggcgaacaggatgctgaagtacacttccttcttcgaattcaaccaccacctggagtccatcatggacaaggcttacatctaccgcgtgatccggaccactggttacctcctgttcatcctgcacatcaacgcctgcgtctattactgggcctcaaactacgaaggcattggtaccacccgctgggtgtacgacggggagggaaacgagtatctgcgctgctactactgggccgtgcgaaccctcataactattggcggcctcccggaaccgcagaccctgttcgagatcgtgttccaactcctcaacttcttctcgggagtgttcgtgttttcaagcttgattggacagatgcgggacgtgatcggtgcagcaactgccaaccagaactactttcgcgcctgcatggacgacactatcgcgtacatgaacaactattcgatccccaagctggtgcagaaacgcgtgcggacttggtatgagtacacttgggactcccagagaatgcttgacgagtccgatctgctcaagaccctgcctactaccgtgcagctggcactcgccatcgatgtgaacttctccattatctcgaaagtcgatctgttcaagggctgcgacacccagatgatctacgacatgctgctgagactcaagtccgtgttgtacctccctggcgacttcgtgtgcaagaagggcgaaatcgggaaggagatgtacattatcaagcacggagaagtccaggtgctggggggaccagacggtaccaaggtccttgtcaccctgaaggccgggtccgtgttcggcgaaatttccctgttggccgccggcggtggcaacaggagaaccgcaaatgtggtggcccacggcttcgcaaaccttctgaccctggacaagaaaaccctccaggaaatcctcgtgcactacccggatagcgagcggatcctgatgaagaaagcccgggtgctgctgaagcaaaaggccaagaccgccgaagccaccccgcctcggaaggacctggctctgctgttcccacccaaggaggagactcccaaactgtttaagaccctcttgggcgggacgggaaaggcctccctcgctcgcttgcttaagttgaagagggagcaggccgcgcagaagaaggaaaactccgaaggaggggaagaagagggaaaggaaaacgaagataagcagaaggagaacgaggataagcaaaaggaaaatgaggacaaggggaaagaaaacgaggacaaggataagggtcgcgaacctgaagagaagccgctggatcggccagagtgcactgcctcgcctatcgcggtcgaagaggaaccccatagcgtgcgcagaaccgtgctgcctagaggcacatcgaggcagtcactgattatctctatggcaccaagcgccgagggaggagaggaagtgctcaccatcgaggtcaaggaaaaagcgaagcagtgatcataactgcagatctgcctcgactgtgccttctagttgccagccatctgttgtttgcccctcccccgtgccttccttgaccctggaaggtgccactcccactgtcctttcctaataaaatgaggaaattgcatcgcattgtctgagtaggtgtcattctattctggggggtggggtggggcaggacagcaagggggaggattgggaagacaatagcaggcatgctggggactcgagttctacgtagataagtagcatggcgggttaatcattaactacaaggaacccctagtgatggagttggccactccctctctgcgcgctcgctcgctcactgaggccgggcgaccaaaggtcgcccgacgcccgggctttgcccgggcggcctcagtgagcgagcgagcgcgcagccttaattaacctaaggaaaatgaagtgaagttcctatactttctagagaataggaacttctatagtgagtcgaataagggcgacacaaaatttattctaaatgcataataaatactgataacatcttatagtttgtattatattttgtattatcgttgacatgtataattttgatatcaaaaactgattttccctttattattttcgagatttattttcttaattctctttaacaaactagaaatattgtatatacaaaaaatcataaataatagatgaatagtttaattataggtgttcatcaatcgaaaaagcaacgtatcttatttaaagtgcgttgcttttttctcatttataaggttaaataattctcatatatcaagcaaagtgacaggcgcccttaaatattctgacaaatgctctttccctaaactccccccataaaaaaacccgccgaagcgggtttttacgttatttgcggattaacgattactcgttatcagaaccgcccagggggcccgagcttaacctttttatttgggggagagggaagtcatgaaaaaactaacctttgaaattcgatctccagcacatcagcaaaacgctattcacgcagtacagcaaatccttccagacccaaccaaaccaatcgtagtaaccattcaggaacgcaaccgcagcttagaccaaaacaggaagctatgggcctgcttaggtgacgtctctcgtcaggttgaatggcatggtcgctggctggatgcagaaagctggaagtgtgtgtttaccgcagcattaaagcagcaggatgttgttcctaaccttgccgggaatggctttgtggtaataggccagtcaaccagcaggatgcgtgtaggcgaatttgcggagctattagagcttatacaggcattcggtacagagcgtggcgttaagtggtcagacgaagcgagactggctctggagtggaaagcgagatggggagacagggctgcatgataaatgtcgttagtttctccggtggcaggacgtcagcatatttgctctggctaatggagcaaaagcgacgggcaggtaaagacgtgcattacgttttcatggatacaggttgtgaacatccaatgacatatcggtttgtcagggaagttgtgaagttctgggatataccgctcaccgtattgcaggttgatatcaacccggagcttggacagccaaatggttatacggtatgggaaccaaaggatattcagacgcgaatgcctgttctgaagccatttatcgatatggtaaagaaatatggcactccatacgtcggcggcgcgttctgcactgacagattaaaactcgttcccttcaccaaatactgtgatgaccatttcgggcgagggaattacaccacgtggattggcatcagagctgatgaaccgaagcggctaaagccaaagcctggaatcagatatcttgctgaactgtcagactttgagaaggaagatatcctcgcatggtggaagcaacaaccattcgatttgcaaataccggaacatctcggtaactgcatattctgcattaaaaaatcaacgcaaaaaatcggacttgcctgcaaagatgaggagggattgcagcgtgtttttaatgaggtcatcacgggatcccatgtgcgtgacggacatcgggaaacgccaaaggagattatgtaccgaggaagaatgtcgctggacggtatcgcgaaaatgtattcagaaaatgattatcaagccctgtatcaggacatggtacgagctaaaagattcgataccggctcttgttctgagtcatgcgaaatatttggagggcagcttgatttcgacttcgggagggaagctgcatgatgcgatgttatcggtgcggtgaatgcaaagaagataaccgcttccgaccaaatcaaccttactggaatcgatggtgtctccggtgtgaaagaacaccaacaggggtgttaccactaccgcaggaaaaggaggacgtgtggcgagacagcgacgaagtatcaccgacataatctgcgaaaactgcaaataccttccaacgaaacgcaccagaaataaacccaagccaatcccaaaagaatctgacgtaaaaaccttcaactacacggctcacctgtgggatatccggtggctaagacgtcgtgcgaggaaaacaaggtgattgaccaaaatcgaagttacgaacaagaaagcgtcgagcgagctttaacgtgcgctaactgcggtcagaagctgcatgtgctggaagttcacgtgtgtgagcactgctgcgcagaactgatgagcgatccgaatagctcgatgcacgaggaagaagatgatggctaaaccagcgcgaagacgatgtaaaaacgatgaatgccgggaatggtttcaccctgcattcgctaatcagtggtggtgctctccagagtgtggaaccaagatagcactcgaacgacgaagtaaagaacgcgaaaaagcggaaaaagcagcagagaagaaacgacgacgagaggagcagaaacagaaagataaacttaagattcgaaaactcgccttaaagccccgcagttactggattaaacaagcccaacaagccgtaaacgccttcatcagagaaagagaccgcgacttaccatgtatctcgtgcggaacgctcacgtctgctcagtgggatgccggacattaccggacaactgctgcggcacctcaactccgatttaatgaacgcaatattcacaagcaatgcgtggtgtgcaaccagcacaaaagcggaaatctcgttccgtatcgcgtcgaactgattagccgcatcgggcaggaagcagtagacgaaatcgaatcaaaccataaccgccatcgctggactatcgaagagtgcaaggcgatcaaggcagagtaccaacagaaactcaaagacctgcgaaatagcagaagtgaggccgcatgacgttctcagtaaaaaccattccagacatgctcgttgaagcatacggaaatcagacagaagtagcacgcagactgaaatgtagtcgcggtacggtcagaaaatacgttgatgataaagacgggaaaatgcacgccatcgtcaacgacgttctcatggttcatcgcggatggagtgaaagagatgcgctattacgaaaaaattgatggcagcaaataccgaaatatttgggtagttggcgatctgcacggatgctacacgaacctgatgaacaaactggatacgattggattcgacaacaaaaaagacctgcttatctcggtgggcgatttggttgatcgtggtgcagagaacgttgaatgcctggaattaatcacattcccctggttcagagctgtacgtggaaaccatgagcaaatgatgattgatggcttatcagagcgtggaaacgttaatcactggctgcttaatggcggtggctggttctttaatctcgattacgacaaagaaattctggctaaagctcttgcccataaagcagatgaacttccgttaatcatcgaactggtgagcaaagataaaaaatatgttatctgccacgccgattatccctttgacgaatacgagtttggaaagccagttgatcatcagcaggtaatctggaaccgcgaacgaatcagcaactcacaaaacgggatcgtgaaagaaatcaaaggcgcggacacgttcatctttggtcatacgccagcagtgaaaccactcaagtttgccaaccaaatgtatatcgataccggcgcagtgttctgcggaaacctaacattgattcaggtacagggagaaggcgcatgagactcgaaagcgtagctaaatttcattcgccaaaaagcccgatgatgagcgactcaccacgggccacggcttctgactctctttccggtactgatgtgatggctgctatggggatggcgcaatcacaagccggattcggtatggctgcattctgcggtaagcacgaactcagccagaacgacaaacaaaaggctatcaactatctgatgcaatttgcacacaaggtatcggggaaataccgtggtgtggcaaagcttgaaggaaatactaaggcaaaggtactgcaagtgctcgcaacattcgcttatgcggattattgccgtagtgccgcgacgccgggggcaagatgcagagattgccatggtacaggccgtgcggttgatattgccaaaacagagctgtgggggagagttgtcgagaaagagtgcggaagatgcaaaggcgtcggctattcaaggatgccagcaagcgcagcatatcgcgctgtgacgatgctaatcccaaaccttacccaacccacctggtcacgcactgttaagccgctgtatgacgctctggtggtgcaatgccacaaagaagagtcaatcgcagacaacattttgaatgcggtcacacgttagcagcatgattgccacggatggcaacatattaacggcatgatattgacttattgaataaaattgggtaaatttgactcaacgatgggttaattcgctcgttgtggtagtgagatgaaaagaggcggcgcttactaccgattccgcctagttggtcacttcgacgtatcgtctggaactccaaccatcgcaggcagagaggtctgcaaaatgcaatcccgaaacagttcgcaggtaatagttagagcctgcataacggtttcgggattttttatatctgcacaacaggtaagagcattgagtcgataatcgtgaagagtcggcgagcctggttagccagtgctctttccgttgtgctgaattaagcgaataccggaagcagaaccggatcaccaaatgcgtacaggcgtcatcgccgcccagcaacagcacaacccaaactgagccgtagccactgtctgtcctgaattcattagtaatagttacgctgcggccttttacacatgaccttcgtgaaagcgggtggcaggaggtcgcgctaacaacctcctgccgttttgcccgtgcatatcggtcacgaacaaatctgattactaaacacagtagcctggatttgttctatcagtaatcgaccttattcctaattaaatagagcaaatccccttattgggggtaagacatgaagatgccagaaaaacatgacctgttggccgccattctcgcggcaaaggaacaaggcatcggggcaatccttgcgtttgcaatggcgtaccttcgcggcagatataatggcggtgcgtttacaaaaacagtaatcgacgcaacgatgtgcgccattatcgcctggttcattcgtgaccttctcgacttcgccggactaagtagcaatctcgcttatataacgagcgtgtttatcggctacatcggtactgactcgattggttcgcttatcaaacgcttcgctgctaaaaaagccggagtagaagatggtagaaatcaataatcaacgtaaggcgttcctcgatatgctggcgtggtcggagggaactgataacggacgtcagaaaaccagaaatcatggttatgacgtcattgtaggcggagagctatttactgattactccgatcaccctcgcaaacttgtcacgctaaacccaaaactcaaatcaacaggcgcttaagactggccgtcgttttacaacacagaaagagtttgtagaaacgcaaaaaggccatccgtcaggggccttctgcttagtttgatgcctggcagttccctactctcgccttccgcttcctcgctcactgactcgctgcgctcggtcgttcggctgcggcgagcggtatcagctcactcaaaggcggtaatacggttatccacagaatcaggggataacgcaggaaagaacatgtgagcaaaaggccagcaaaaggccaggaaccgtaaaaaggccgcgttgctggcgtttttccataggctccgcccccctgacgagcatcacaaaaatcgacgctcaagtcagaggtggcgaaacccgacaggactataaagataccaggcgtttccccctggaagctccctcgtgcgctctcctgttccgaccctgccgcttaccggatacctgtccgcctttctcccttcgggaagcgtggcgctttctcatagctcacgctgtaggtatctcagttcggtgtaggtcgttcgctccaagctgggctgtgtgcacgaaccccccgttcagcccgaccgctgcgccttatccggtaactatcgtcttgagtccaacccggtaagacacgacttatcgccactggcagcagccactggtaacaggattagcagagcgaggtatgtaggcggtgctacagagttcttgaagtggtgggctaactacggctacactagaagaacagtatttggtatctgcgctctgctgaagccagttaccttcggaaaaagagttggtagctcttgatccggcaaacaaaccaccgctggtagcggtggtttttttgtttgcaagcagcagattacgcgcagaaaaaaaggatctcaagaagatcctttgatcttttctacggggtctgacgctcagtggaacgacgcgcgcgtaactcacgttaagggattttggtcatgagcttgcgccgtcccgtcaagtcagcgtaatgctctgcttttagaaaaactcatcgagcatcaaatgaaactgcaatttattcatatcaggattatcaataccatatttttgaaaaagccgtttctgtaatgaaggagaaaactcaccgaggcagttccataggatggcaagatcctggtatcggtctgcgattccgactcgtccaacatcaatacaacctattaatttcccctcgtcaaaaataaggttatcaagtgagaaatcaccatgagtgacgactgaatccggtgagaatggcaaaagtttatgcatttctttccagacttgttcaacaggccagccattacgctcgtcatcaaaatcactcgcatcaaccaaaccgttattcattcgtgattgcgcctgagcgaggcgaaatacgcgatcgctgttaaaaggacaattacaaacaggaatcgagtgcaaccggcgcaggaacactgccagcgcatcaacaatattttcacctgaatcaggatattcttctaatacctggaacgctgtttttccggggatcgcagtggtgagtaaccatgcatcatcaggagtacggataaaatgcttgatggtcggaagtggcataaattccgtcagccagtttagtctgaccatctcatctgtaacatcattggcaacgctacctttgccatgtttcagaaacaactctggcgcatcgggcttcccatacaagcgatagattgtcgcacctgattgcccgacattatcgcgagcccatttatacccatataaatcagcatccatgttggaatttaatcgcggcctcgacgtttcccgttgaatatggctcatattcttcctttttcaatattattgaagcatttatcagggttattgtctcatgagcggatacatatttgaatgtatttagaaaaataaacaaataggggtcagtgttacaaccaattaaccaattctgaacattatcgcgagcccatttatacctgaatatggctcataacaccccttgtttgcctggcggcagtagcgcggtggtcccacctgaccccatgccgaactcagaagtgaaacgccgtagcgccgatggtagtgtggggactccccatgcgagagtagggaactgccaggcatcaaataaaacgaaaggctcagtcgaaagactgggcctttcgcccgggctaattagggggtgtcgcccttattcgactctatagtgaagttcctattctctagaaagtataggaacttctgaagtggggtcgacttaattaagg

SEQ ID NO: 43 - DNA, 12556 bp, Artificial Sequence
  constructed sequence
ctgcgcgctcgctcgctcactgaggccgcccgggcaaagcccgggcgtcgggcgacctttggtcgcccggcctcagtgagcgagcgagcgcgcagagagggagtggccaactccatcactaggggttccttgtagttaatgattaacccgccatgctacttatctacgtagcaagctagctagttattaatagtaatcaattacggggtcattagttcatagcccatatatggagttccgcgttacataacttacggtaaatggcccgcctggctgaccgcccaacgacccccgcccattgacgtcaataatgacgtatgttcccatagtaacgccaatagggactttccattgacgtcaatgggtggagtatttacggtaaactgcccacttggcagtacatcaagtgtatcatatgccaagtacgccccctattgacgtcaatgacggtaaatggcccgcctggcattatgcccagtacatgaccttatgggactttcctacttggcagtacatctacgtattagtcatcgctattaacatggtcgaggtgagccccacgttctgcttcactctccccatctcccccccctccccacccccaattttgtatttatttattttttaattattttgtgcagcgatgggggcggggggggggggggggcgcgcgccaggcggggcggggcggggcgaggggcggggcggggcgaggcggagaggtgcggcggcagccaatcagagcggcgcgctccgaaagtttccttttatggcgaggcggcggcggcggcggccctataaaaagcgaagcgcgcggcgggcggggagtcgctgcgacgctgccttcgccccgtgccccgctccgccgccgcctcgcgccgcccgccccggctctgactgaccgcgttactcccacaggtgagcgggcgggacggcccttctcctccgggctgtaattagcgcttggtttaatgacggcttgtttcttttctgtggctgcgtgaaagccttgaggggctccgggagggccctttgtgcggggggagcggctcggggggtgcgtgcgtgtgtgtgtgcgtggggagcgccgcgtgcggctccgcgctgcccggcggctgtgagcgctgcgggcgcggcgcggggctttgtgcgctccgcagtgtgcgcgaggggagcgcggccgggggcggtgccccgcggtgcggggggggctgcgaggggaacaaaggctgcgtgcggggtgtgtgcgtgggggggtgagcagggggtgtgggcgcgtcggtcgggctgcaaccccccctgcacccccctccccgagttgctgagcacggcccggcttcgggtgcggggctccgtacggggcgtggcgcggggctcgccgtgccgggcggggggtggcggcaggtgggggtgccgggcggggcggggccgcctcgggccggggagggctcgggggaggggcgcggcggcccccggagcgccggcggctgtcgaggcgcggcgagccgcagccattgccttttatggtaatcgtgcgagagggcgcagggacttcctttgtcccaaatctgtgcggagccgaaatctgggaggcgccgccgcaccccctctagcgggcgcggggcgaagcggtgcggcgccggcaggaaggaaatgggcggggagggccttcgtgcgtcgccgcgccgccgtccccttctccctctccagcctcggggctgtccgcggggggacggctgccttcgggggggacggggcagggcggggttcggcttctggcgtgtgaccggcggctctagacaattgtactaaccttcttctctttcctctcctgacaggttggtgtacactagcggccgccaccatgtttaaatcgctgacaaaagtcaacaaggtgaagcctataggagagaacaatgagaatgaacaaagttctcgtcggaatgaagaaggctctcacccaagtaatcagtctcagcaaaccacagcacaggaagaaaacaaaggtgaagagaaatctctcaaaaccaagtcaactccagtcacgtctgaagagccacacaccaacatacaagacaaactctccaagaaaaattcctctggagatctgaccacaaaccctgaccctcaaaatgcagcagaaccaactggaacagtgccagagcagaaggaaatggaccccgggaaagaaggtccaaacagcccacaaaacaaaccgccagcagctcctgttataaatgagtatgccgatgcccagctacacaacctggtgaaaagaatgcgtcaaagaacagccctctacaagaaaaagttggtagagggagatctctcctcacccgaagccagcccacaaactgcaaagcccacggctgtaccaccagtaaaagaaagcgatgataagccaacagaacattactacaggctgttgtggttcaaagtcaaaaagatgcctttaacagagtacttaaagcgaattaaacttccaaacagcatagattcatacacagatcgactctatctcctgtggctcttgcttgtcactcttgcctataactggaactgctgttttataccactgcgcctcgtcttcccatatcaaaccgcagacaacatacactactggcttattgcggacatcatctgtgatatcatctacctttatgatatgctatttatccagcccagactccagtttgtaagaggaggagacataatagtggattcaaatgagctaaggaaacactacaggacttctacaaaatttcagttggatgtcgcatcaataataccatttgatatttgctacctcttctttgggtttaatccaatgtttagagcaaataggatgttaaagtacacttcattttttgaatttaatcatcacctagagtctataatggacaaagcatatatctacagagttattcgaacaactggatacttgctgtttattctgcacattaatgcctgtgtttattactgggcttcaaactatgaaggaattggcactactagatgggtgtatgatggggaaggaaacgagtatctgagatgttattattgggcagttcgaactttaattaccattggtggccttccagaaccacaaactttatttgaaattgtttttcaactcttgaattttttttctggagtttttgtgttctccagtttaattggtcagatgagagatgtgattggagcagctacagccaatcagaactacttccgcgcctgcatggatgacaccattgcctacatgaacaattactccattcctaaacttgtgcaaaagcgagttcggacttggtatgaatatacatgggactctcaaagaatgctagatgagtctgatttgcttaagaccctaccaactacggtccagttagccctcgccattgatgtgaacttcagcatcatcagcaaagttgacttgttcaagggttgtgatacacagatgatttatgacatgttgctaagattgaaatccgttctctatttgcctggtgactttgtctgcaaaaagggagaaattggcaaggaaatgtatatcatcaagcatggagaagtccaagttcttggaggccctgatggtactaaagttctggttactctgaaagctgggtcggtgtttggagaaatcagccttctagcagcaggaggaggaaaccgtcgaactgccaatgtggtggcccacgggtttgccaatcttttaactctagacaaaaagaccctccaagaaattctagtgcattatccagattctgaaagaatcctcatgaagaaagccagagtgcttttaaagcagaaggctaagaccgcagaagcaacccctccaagaaaagatcttgccctcctcttcccaccgaaagaagagacacccaaactgtttaaaactctcctaggaggcacaggaaaagcaagtcttgcaagactactcaaattgaagcgagagcaagcagctcagaagaaagaaaattctgaaggaggagaggaagaaggaaaagaaaatgaagataaacaaaaagaaaatgaagataaacaaaaagaaaatgaagataaaggaaaagaaaatgaagataaagataaaggaagagagccagaagagaagccactggacagacctgaatgtacagcaagtcctattgcagtggaggaagaaccccactcagttagaaggacagttttacccagagggacttctcgtcaatcactcattatcagcatggctccttctgctgagggcggagaagaggttcttactattgaagtcaaagaaaaggctaagcaatgatcataactgcagatctgcctcgactgtgccttctagttgccagccatctgttgtttgcccctcccccgtgccttccttgaccctggaaggtgccactcccactgtcctttcctaataaaatgaggaaattgcatcgcattgtctgagtaggtgtcattctattctggggggtggggtggggcaggacagcaagggggaggattgggaagacaatagcaggcatgctggggactcgagttctacgtagataagtagcatggcgggttaatcattaactacaaggaacccctagtgatggagttggccactccctctctgcgcgctcgctcgctcactgaggccgggcgaccaaaggtcgcccgacgcccgggctttgcccgggcggcctcagtgagcgagcgagcgcgcagccttaattaacctaaggaaaatgaagtgaagttcctatactttctagagaataggaacttctatagtgagtcgaataagggcgacacaaaatttattctaaatgcataataaatactgataacatcttatagtttgtattatattttgtattatcgttgacatgtataattttgatatcaaaaactgattttccctttattattttcgagatttattttcttaattctctttaacaaactagaaatattgtatatacaaaaaatcataaataatagatgaatagtttaattataggtgttcatcaatcgaaaaagcaacgtatcttatttaaagtgcgttgcttttttctcatttataaggttaaataattctcatatatcaagcaaagtgacaggcgcccttaaatattctgacaaatgctctttccctaaactccccccataaaaaaacccgccgaagcgggtttttacgttatttgcggattaacgattactcgttatcagaaccgcccagggggcccgagcttaacctttttatttgggggagagggaagtcatgaaaaaactaacctttgaaattcgatctccagcacatcagcaaaacgctattcacgcagtacagcaaatccttccagacccaaccaaaccaatcgtagtaaccattcaggaacgcaaccgcagcttagaccaaaacaggaagctatgggcctgcttaggtgacgtctctcgtcaggttgaatggcatggtcgctggctggatgcagaaagctggaagtgtgtgtttaccgcagcattaaagcagcaggatgttgttcctaaccttgccgggaatggctttgtggtaataggccagtcaaccagcaggatgcgtgtaggcgaatttgcggagctattagagcttatacaggcattcggtacagagcgtggcgttaagtggtcagacgaagcgagactggctctggagtggaaagcgagatggggagacagggctgcatgataaatgtcgttagtttctccggtggcaggacgtcagcatatttgctctggctaatggagcaaaagcgacgggcaggtaaagacgtgcattacgttttcatggatacaggttgtgaacatccaatgacatatcggtttgtcagggaagttgtgaagttctgggatataccgctcaccgtattgcaggttgatatcaacccggagcttggacagccaaatggttatacggtatgggaaccaaaggatattcagacgcgaatgcctgttctgaagccatttatcgatatggtaaagaaatatggcactccatacgtcggcggcgcgttctgcactgacagattaaaactcgttcccttcaccaaatactgtgatgaccatttcgggcgagggaattacaccacgtggattggcatcagagctgatgaaccgaagcggctaaagccaaagcctggaatcagatatcttgctgaactgtcagactttgagaaggaagatatcctcgcatggtggaagcaacaaccattcgatttgcaaataccggaacatctcggtaactgcatattctgcattaaaaaatcaacgcaaaaaatcggacttgcctgcaaagatgaggagggattgcagcgtgtttttaatgaggtcatcacgggatcccatgtgcgtgacggacatcgggaaacgccaaaggagattatgtaccgaggaagaatgtcgctggacggtatcgcgaaaatgtattcagaaaatgattatcaagccctgtatcaggacatggtacgagctaaaagattcgataccggctcttgttctgagtcatgcgaaatatttggagggcagcttgatttcgacttcgggagggaagctgcatgatgcgatgttatcggtgcggtgaatgcaaagaagataaccgcttccgaccaaatcaaccttactggaatcgatggtgtctccggtgtgaaagaacaccaacaggggtgttaccactaccgcaggaaaaggaggacgtgtggcgagacagcgacgaagtatcaccgacataatctgcgaaaactgcaaataccttccaacgaaacgcaccagaaataaacccaagccaatcccaaaagaatctgacgtaaaaaccttcaactacacggctcacctgtgggatatccggtggctaagacgtcgtgcgaggaaaacaaggtgattgaccaaaatcgaagttacgaacaagaaagcgtcgagcgagctttaacgtgcgctaactgcggtcagaagctgcatgtgctggaagttcacgtgtgtgagcactgctgcgcagaactgatgagcgatccgaatagctcgatgcacgaggaagaagatgatggctaaaccagcgcgaagacgatgtaaaaacgatgaatgccgggaatggtttcaccctgcattcgctaatcagtggtggtgctctccagagtgtggaaccaagatagcactcgaacgacgaagtaaagaacgcgaaaaagcggaaaaagcagcagagaagaaacgacgacgagaggagcagaaacagaaagataaacttaagattcgaaaactcgccttaaagccccgcagttactggattaaacaagcccaacaagccgtaaacgccttcatcagagaaagagaccgcgacttaccatgtatctcgtgcggaacgctcacgtctgctcagtgggatgccggacattaccggacaactgctgcggcacctcaactccgatttaatgaacgcaatattcacaagcaatgcgtggtgtgcaaccagcacaaaagcggaaatctcgttccgtatcgcgtcgaactgattagccgcatcgggcaggaagcagtagacgaaatcgaatcaaaccataaccgccatcgctggactatcgaagagtgcaaggcgatcaaggcagagtaccaacagaaactcaaagacctgcgaaatagcagaagtgaggccgcatgacgttctcagtaaaaaccattccagacatgctcgttgaagcatacggaaatcagacagaagtagcacgcagactgaaatgtagtcgcggtacggtcagaaaatacgttgatgataaagacgggaaaatgcacgccatcgtcaacgacgttctcatggttcatcgcggatggagtgaaagagatgcgctattacgaaaaaattgatggcagcaaataccgaaatatttgggtagttggcgatctgcacggatgctacacgaacctgatgaacaaactggatacgattggattcgacaacaaaaaagacctgcttatctcggtgggcgatttggttgatcgtggtgcagagaacgttgaatgcctggaattaatcacattcccctggttcagagctgtacgtggaaaccatgagcaaatgatgattgatggcttatcagagcgtggaaacgttaatcactggctgcttaatggcggtggctggttctttaatctcgattacgacaaagaaattctggctaaagctcttgcccataaagcagatgaacttccgttaatcatcgaactggtgagcaaagataaaaaatatgttatctgccacgccgattatccctttgacgaatacgagtttggaaagccagttgatcatcagcaggtaatctggaaccgcgaacgaatcagcaactcacaaaacgggatcgtgaaagaaatcaaaggcgcggacacgttcatctttggtcatacgccagcagtgaaaccactcaagtttgccaaccaaatgtatatcgataccggcgcagtgttctgcggaaacctaacattgattcaggtacagggagaaggcgcatgagactcgaaagcgtagctaaatttcattcgccaaaaagcccgatgatgagcgactcaccacgggccacggcttctgactctctttccggtactgatgtgatggctgctatggggatggcgcaatcacaagccggattcggtatggctgcattctgcggtaagcacgaactcagccagaacgacaaacaaaaggctatcaactatctgatgcaatttgcacacaaggtatcggggaaataccgtggtgtggcaaagcttgaaggaaatactaaggcaaaggtactgcaagtgctcgcaacattcgcttatgcggattattgccgtagtgccgcgacgccgggggcaagatgcagagattgccatggtacaggccgtgcggttgatattgccaaaacagagctgtgggggagagttgtcgagaaagagtgcggaagatgcaaaggcgtcggctattcaaggatgccagcaagcgcagcatatcgcgctgtgacgatgctaatcccaaaccttacccaacccacctggtcacgcactgttaagccgctgtatgacgctctggtggtgcaatgccacaaagaagagtcaatcgcagacaacattttgaatgcggtcacacgttagcagcatgattgccacggatggcaacatattaacggcatgatattgacttattgaataaaattgggtaaatttgactcaacgatgggttaattcgctcgttgtggtagtgagatgaaaagaggcggcgcttactaccgattccgcctagttggtcacttcgacgtatcgtctggaactccaaccatcgcaggcagagaggtctgcaaaatgcaatcccgaaacagttcgcaggtaatagttagagcctgcataacggtttcgggattttttatatctgcacaacaggtaagagcattgagtcgataatcgtgaagagtcggcgagcctggttagccagtgctctttccgttgtgctgaattaagcgaataccggaagcagaaccggatcaccaaatgcgtacaggcgtcatcgccgcccagcaacagcacaacccaaactgagccgtagccactgtctgtcctgaattcattagtaatagttacgctgcggccttttacacatgaccttcgtgaaagcgggtggcaggaggtcgcgctaacaacctcctgccgttttgcccgtgcatatcggtcacgaacaaatctgattactaaacacagtagcctggatttgttctatcagtaatcgaccttattcctaattaaatagagcaaatccccttattgggggtaagacatgaagatgccagaaaaacatgacctgttggccgccattctcgcggcaaaggaacaaggcatcggggcaatccttgcgtttgcaatggcgtaccttcgcggcagatataatggcggtgcgtttacaaaaacagtaatcgacgcaacgatgtgcgccattatcgcctggttcattcgtgaccttctcgacttcgccggactaagtagcaatctcgcttatataacgagcgtgtttatcggctacatcggtactgactcgattggttcgcttatcaaacgcttcgctgctaaaaaagccggagtagaagatggtagaaatcaataatcaacgtaaggcgttcctcgatatgctggcgtggtcggagggaactgataacggacgtcagaaaaccagaaatcatggttatgacgtcattgtaggcggagagctatttactgattactccgatcaccctcgcaaacttgtcacgctaaacccaaaactcaaatcaacaggcgcttaagactggccgtcgttttacaacacagaaagagtttgtagaaacgcaaaaaggccatccgtcaggggccttctgcttagtttgatgcctggcagttccctactctcgccttccgcttcctcgctcactgactcgctgcgctcggtcgttcggctgcggcgagcggtatcagctcactcaaaggcggtaatacggttatccacagaatcaggggataacgcaggaaagaacatgtgagcaaaaggccagcaaaaggccaggaaccgtaaaaaggccgcgttgctggcgtttttccataggctccgcccccctgacgagcatcacaaaaatcgacgctcaagtcagaggtggcgaaacccgacaggactataaagataccaggcgtttccccctggaagctccctcgtgcgctctcctgttccgaccctgccgcttaccggatacctgtccgcctttctcccttcgggaagcgtggcgctttctcatagctcacgctgtaggtatctcagttcggtgtaggtcgttcgctccaagctgggctgtgtgcacgaaccccccgttcagcccgaccgctgcgccttatccggtaactatcgtcttgagtccaacccggtaagacacgacttatcgccactggcagcagccactggtaacaggattagcagagcgaggtatgtaggcggtgctacagagttcttgaagtggtgggctaactacggctacactagaagaacagtatttggtatctgcgctctgctgaagccagttaccttcggaaaaagagttggtagctcttgatccggcaaacaaaccaccgctggtagcggtggtttttttgtttgcaagcagcagattacgcgcagaaaaaaaggatctcaagaagatcctttgatcttttctacggggtctgacgctcagtggaacgacgcgcgcgtaactcacgttaagggattttggtcatgagcttgcgccgtcccgtcaagtcagcgtaatgctctgcttttagaaaaactcatcgagcatcaaatgaaactgcaatttattcatatcaggattatcaataccatatttttgaaaaagccgtttctgtaatgaaggagaaaactcaccgaggcagttccataggatggcaagatcctggtatcggtctgcgattccgactcgtccaacatcaatacaacctattaatttcccctcgtcaaaaataaggttatcaagtgagaaatcaccatgagtgacgactgaatccggtgagaatggcaaaagtttatgcatttctttccagacttgttcaacaggccagccattacgctcgtcatcaaaatcactcgcatcaaccaaaccgttattcattcgtgattgcgcctgagcgaggcgaaatacgcgatcgctgttaaaaggacaattacaaacaggaatcgagtgcaaccggcgcaggaacactgccagcgcatcaacaatattttcacctgaatcaggatattcttctaatacctggaacgctgtttttccggggatcgcagtggtgagtaaccatgcatcatcaggagtacggataaaatgcttgatggtcggaagtggcataaattccgtcagccagtttagtctgaccatctcatctgtaacatcattggcaacgctacctttgccatgtttcagaaacaactctggcgcatcgggcttcccatacaagcgatagattgtcgcacctgattgcccgacattatcgcgagcccatttatacccatataaatcagcatccatgttggaatttaatcgcggcctcgacgtttcccgttgaatatggctcatattcttcctttttcaatattattgaagcatttatcagggttattgtctcatgagcggatacatatttgaatgtatttagaaaaataaacaaataggggtcagtgttacaaccaattaaccaattctgaacattatcgcgagcccatttatacctgaatatggctcataacaccccttgtttgcctggcggcagtagcgcggtggtcccacctgaccccatgccgaactcagaagtgaaacgccgtagcgccgatggtagtgtggggactccccatgcgagagtagggaactgccaggcatcaaataaaacgaaaggctcagtcgaaagactgggcctttcgcccgggctaattagggggtgtcgcccttattcgactctatagtgaagttcctattctctagaaagtataggaacttctgaagtggggtcgacttaattaagg

SEQ ID NO: 44 - DNA, 12556 bp, Artificial Sequence
  constructed sequence
ctgcgcgctcgctcgctcactgaggccgcccgggcaaagcccgggcgtcgggcgacctttggtcgcccggcctcagtgagcgagcgagcgcgcagagagggagtggccaactccatcactaggggttccttgtagttaatgattaacccgccatgctacttatctacgtagcaagctagctagttattaatagtaatcaattacggggtcattagttcatagcccatatatggagttccgcgttacataacttacggtaaatggcccgcctggctgaccgcccaacgacccccgcccattgacgtcaataatgacgtatgttcccatagtaacgccaatagggactttccattgacgtcaatgggtggagtatttacggtaaactgcccacttggcagtacatcaagtgtatcatatgccaagtacgccccctattgacgtcaatgacggtaaatggcccgcctggcattatgcccagtacatgaccttatgggactttcctacttggcagtacatctacgtattagtcatcgctattaacatggtcgaggtgagccccacgttctgcttcactctccccatctcccccccctccccacccccaattttgtatttatttattttttaattattttgtgcagcgatgggggcggggggggggggggggcgcgcgccaggcggggcggggcggggcgaggggcggggcggggcgaggcggagaggtgcggcggcagccaatcagagcggcgcgctccgaaagtttccttttatggcgaggcggcggcggcggcggccctataaaaagcgaagcgcgcggcgggcggggagtcgctgcgacgctgccttcgccccgtgccccgctccgccgccgcctcgcgccgcccgccccggctctgactgaccgcgttactcccacaggtgagcgggcgggacggcccttctcctccgggctgtaattagcgcttggtttaatgacggcttgtttcttttctgtggctgcgtgaaagccttgaggggctccgggagggccctttgtgcggggggagcggctcggggggtgcgtgcgtgtgtgtgtgcgtggggagcgccgcgtgcggctccgcgctgcccggcggctgtgagcgctgcgggcgcggcgcggggctttgtgcgctccgcagtgtgcgcgaggggagcgcggccgggggcggtgccccgcggtgcggggggggctgcgaggggaacaaaggctgcgtgcggggtgtgtgcgtgggggggtgagcagggggtgtgggcgcgtcggtcgggctgcaaccccccctgcacccccctccccgagttgctgagcacggcccggcttcgggtgcggggctccgtacggggcgtggcgcggggctcgccgtgccgggcggggggtggcggcaggtgggggtgccgggcggggcggggccgcctcgggccggggagggctcgggggaggggcgcggcggcccccggagcgccggcggctgtcgaggcgcggcgagccgcagccattgccttttatggtaatcgtgcgagagggcgcagggacttcctttgtcccaaatctgtgcggagccgaaatctgggaggcgccgccgcaccccctctagcgggcgcggggcgaagcggtgcggcgccggcaggaaggaaatgggcggggagggccttcgtgcgtcgccgcgccgccgtccccttctccctctccagcctcggggctgtccgcggggggacggctgccttcgggggggacggggcagggcggggttcggcttctggcgtgtgaccggcggctctagacaattgtactaaccttcttctctttcctctcctgacaggttggtgtacactagcggccgccaccatgttcaagtccctcaccaaagtcaacaaggtcaagcccatcggagagaacaacgagaatgagcagagctctcggcgcaacgaagaaggatcccatccgtcgaaccagtcacagcagactaccgcacaggaggagaacaagggagaagaaaagtcgctcaagactaagtccacccccgtgacctcggaagaaccgcacacgaacattcaggacaagctgtccaagaagaactcctccggcgatctcacgactaacccggacccccagaatgccgctgaacctactgggaccgtgcctgagcaaaaggagatggaccccggaaaggagggtcctaactccccccaaaacaagcccccggccgcgccggtcatcaatgagtacgcggacgcgcaactgcataacctcgtgaagcggatgcggcaaagaaccgccctctacaagaagaaactggtggagggcgacctgagctcacctgaagccagcccacagaccgccaaacccaccgccgtgccgcctgtgaaggagtccgatgacaagcctaccgagcactactaccgcctgctgtggttcaaggtcaagaagatgcccctgaccgaatacctcaagcggatcaagctgccgaacagcatcgacagctacaccgaccggctttacttgctctggctgctgcttgtgaccctggcttacaactggaactgttgtttcattcccctgcggctggtgttcccttaccaaaccgcggataacattcactactggctgattgccgacatcatttgcgacatcatctacctgtacgatatgctttttatccaaccgcggctgcaattcgtccgcgggggagacatcattgtggactccaacgagctgcgcaagcattaccggacctcgacaaagttccagctggatgtggcctccatcatcccgttcgatatctgttacctgttctttggcttcaacccgatgttcagggcgaacaggatgctgaagtacacttccttcttcgaattcaaccaccacctggagtccatcatggacaaggcttacatctaccgcgtgatccggaccactggttacctcctgttcatcctgcacatcaacgcctgcgtctattactgggcctcaaactacgaaggcattggtaccacccgctgggtgtacgacggggagggaaacgagtatctgcgctgctactactgggccgtgcgaaccctcataactattggcggcctcccggaaccgcagaccctgttcgagatcgtgttccaactcctcaacttcttctcgggagtgttcgtgttttcaagcttgattggacagatgcgggacgtgatcggtgcagcaactgccaaccagaactactttcgcgcctgcatggacgacactatcgcgtacatgaacaactattcgatccccaagctggtgcagaaacgcgtgcggacttggtatgagtacacttgggactcccagagaatgcttgacgagtccgatctgctcaagaccctgcctactaccgtgcagctggcactcgccatcgatgtgaacttctccattatctcgaaagtcgatctgttcaagggctgcgacacccagatgatctacgacatgctgctgagactcaagtccgtgttgtacctccctggcgacttcgtgtgcaagaagggcgaaatcgggaaggagatgtacattatcaagcacggagaagtccaggtgctggggggaccagacggtaccaaggtccttgtcaccctgaaggccgggtccgtgttcggcgaaatttccctgttggccgccggcggtggcaacaggagaaccgcaaatgtggtggcccacggcttcgcaaaccttctgaccctggacaagaaaaccctccaggaaatcctcgtgcactacccggatagcgagcggatcctgatgaagaaagcccgggtgctgctgaagcaaaaggccaagaccgccgaagccaccccgcctcggaaggacctggctctgctgttcccacccaaggaggagactcccaaactgtttaagaccctcttgggcgggacgggaaaggcctccctcgctcgcttgcttaagttgaagagggagcaggccgcgcagaagaaggaaaactccgaaggaggggaagaagagggaaaggaaaacgaagataagcagaaggagaacgaggataagcaaaaggaaaatgaggacaaggggaaagaaaacgaggacaaggataagggtcgcgaacctgaagagaagccgctggatcggccagagtgcactgcctcgcctatcgcggtcgaagaggaaccccatagcgtgcgcagaaccgtgctgcctagaggcacatcgaggcagtcactgattatctctatggcaccaagcgccgagggaggagaggaagtgctcaccatcgaggtcaaggaaaaagcgaagcagtgatcataactgcagatctgcctcgactgtgccttctagttgccagccatctgttgtttgcccctcccccgtgccttccttgaccctggaaggtgccactcccactgtcctttcctaataaaatgaggaaattgcatcgcattgtctgagtaggtgtcattctattctggggggtggggtggggcaggacagcaagggggaggattgggaagacaatagcaggcatgctggggactcgagttctacgtagataagtagcatggcgggttaatcattaactacaaggaacccctagtgatggagttggccactccctctctgcgcgctcgctcgctcactgaggccgggcgaccaaaggtcgcccgacgcccgggctttgcccgggcggcctcagtgagcgagcgagcgcgcagccttaattaacctaaggaaaatgaagtgaagttcctatactttctagagaataggaacttctatagtgagtcgaataagggcgacacaaaatttattctaaatgcataataaatactgataacatcttatagtttgtattatattttgtattatcgttgacatgtataattttgatatcaaaaactgattttccctttattattttcgagatttattttcttaattctctttaacaaactagaaatattgtatatacaaaaaatcataaataatagatgaatagtttaattataggtgttcatcaatcgaaaaagcaacgtatcttatttaaagtgcgttgcttttttctcatttataaggttaaataattctcatatatcaagcaaagtgacaggcgcccttaaatattctgacaaatgctctttccctaaactccccccataaaaaaacccgccgaagcgggtttttacgttatttgcggattaacgattactcgttatcagaaccgcccagggggcccgagcttaacctttttatttgggggagagggaagtcatgaaaaaactaacctttgaaattcgatctccagcacatcagcaaaacgctattcacgcagtacagcaaatccttccagacccaaccaaaccaatcgtagtaaccattcaggaacgcaaccgcagcttagaccaaaacaggaagctatgggcctgcttaggtgacgtctctcgtcaggttgaatggcatggtcgctggctggatgcagaaagctggaagtgtgtgtttaccgcagcattaaagcagcaggatgttgttcctaaccttgccgggaatggctttgtggtaataggccagtcaaccagcaggatgcgtgtaggcgaatttgcggagctattagagcttatacaggcattcggtacagagcgtggcgttaagtggtcagacgaagcgagactggctctggagtggaaagcgagatggggagacagggctgcatgataaatgtcgttagtttctccggtggcaggacgtcagcatatttgctctggctaatggagcaaaagcgacgggcaggtaaagacgtgcattacgttttcatggatacaggttgtgaacatccaatgacatatcggtttgtcagggaagttgtgaagttctgggatataccgctcaccgtattgcaggttgatatcaacccggagcttggacagccaaatggttatacggtatgggaaccaaaggatattcagacgcgaatgcctgttctgaagccatttatcgatatggtaaagaaatatggcactccatacgtcggcggcgcgttctgcactgacagattaaaactcgttcccttcaccaaatactgtgatgaccatttcgggcgagggaattacaccacgtggattggcatcagagctgatgaaccgaagcggctaaagccaaagcctggaatcagatatcttgctgaactgtcagactttgagaaggaagatatcctcgcatggtggaagcaacaaccattcgatttgcaaataccggaacatctcggtaactgcatattctgcattaaaaaatcaacgcaaaaaatcggacttgcctgcaaagatgaggagggattgcagcgtgtttttaatgaggtcatcacgggatcccatgtgcgtgacggacatcgggaaacgccaaaggagattatgtaccgaggaagaatgtcgctggacggtatcgcgaaaatgtattcagaaaatgattatcaagccctgtatcaggacatggtacgagctaaaagattcgataccggctcttgttctgagtcatgcgaaatatttggagggcagcttgatttcgacttcgggagggaagctgcatgatgcgatgttatcggtgcggtgaatgcaaagaagataaccgcttccgaccaaatcaaccttactggaatcgatggtgtctccggtgtgaaagaacaccaacaggggtgttaccactaccgcaggaaaaggaggacgtgtggcgagacagcgacgaagtatcaccgacataatctgcgaaaactgcaaataccttccaacgaaacgcaccagaaataaacccaagccaatcccaaaagaatctgacgtaaaaaccttcaactacacggctcacctgtgggatatccggtggctaagacgtcgtgcgaggaaaacaaggtgattgaccaaaatcgaagttacgaacaagaaagcgtcgagcgagctttaacgtgcgctaactgcggtcagaagctgcatgtgctggaagttcacgtgtgtgagcactgctgcgcagaactgatgagcgatccgaatagctcgatgcacgaggaagaagatgatggctaaaccagcgcgaagacgatgtaaaaacgatgaatgccgggaatggtttcaccctgcattcgctaatcagtggtggtgctctccagagtgtggaaccaagatagcactcgaacgacgaagtaaagaacgcgaaaaagcggaaaaagcagcagagaagaaacgacgacgagaggagcagaaacagaaagataaacttaagattcgaaaactcgccttaaagccccgcagttactggattaaacaagcccaacaagccgtaaacgccttcatcagagaaagagaccgcgacttaccatgtatctcgtgcggaacgctcacgtctgctcagtgggatgccggacattaccggacaactgctgcggcacctcaactccgatttaatgaacgcaatattcacaagcaatgcgtggtgtgcaaccagcacaaaagcggaaatctcgttccgtatcgcgtcgaactgattagccgcatcgggcaggaagcagtagacgaaatcgaatcaaaccataaccgccatcgctggactatcgaagagtgcaaggcgatcaaggcagagtaccaacagaaactcaaagacctgcgaaatagcagaagtgaggccgcatgacgttctcagtaaaaaccattccagacatgctcgttgaagcatacggaaatcagacagaagtagcacgcagactgaaatgtagtcgcggtacggtcagaaaatacgttgatgataaagacgggaaaatgcacgccatcgtcaacgacgttctcatggttcatcgcggatggagtgaaagagatgcgctattacgaaaaaattgatggcagcaaataccgaaatatttgggtagttggcgatctgcacggatgctacacgaacctgatgaacaaactggatacgattggattcgacaacaaaaaagacctgcttatctcggtgggcgatttggttgatcgtggtgcagagaacgttgaatgcctggaattaatcacattcccctggttcagagctgtacgtggaaaccatgagcaaatgatgattgatggcttatcagagcgtggaaacgttaatcactggctgcttaatggcggtggctggttctttaatctcgattacgacaaagaaattctggctaaagctcttgcccataaagcagatgaacttccgttaatcatcgaactggtgagcaaagataaaaaatatgttatctgccacgccgattatccctttgacgaatacgagtttggaaagccagttgatcatcagcaggtaatctggaaccgcgaacgaatcagcaactcacaaaacgggatcgtgaaagaaatcaaaggcgcggacacgttcatctttggtcatacgccagcagtgaaaccactcaagtttgccaaccaaatgtatatcgataccggcgcagtgttctgcggaaacctaacattgattcaggtacagggagaaggcgcatgagactcgaaagcgtagctaaatttcattcgccaaaaagcccgatgatgagcgactcaccacgggccacggcttctgactctctttccggtactgatgtgatggctgctatggggatggcgcaatcacaagccggattcggtatggctgcattctgcggtaagcacgaactcagccagaacgacaaacaaaaggctatcaactatctgatgcaatttgcacacaaggtatcggggaaataccgtggtgtggcaaagcttgaaggaaatactaaggcaaaggtactgcaagtgctcgcaacattcgcttatgcggattattgccgtagtgccgcgacgccgggggcaagatgcagagattgccatggtacaggccgtgcggttgatattgccaaaacagagctgtgggggagagttgtcgagaaagagtgcggaagatgcaaaggcgtcggctattcaaggatgccagcaagcgcagcatatcgcgctgtgacgatgctaatcccaaaccttacccaacccacctggtcacgcactgttaagccgctgtatgacgctctggtggtgcaatgccacaaagaagagtcaatcgcagacaacattttgaatgcggtcacacgttagcagcatgattgccacggatggcaacatattaacggcatgatattgacttattgaataaaattgggtaaatttgactcaacgatgggttaattcgctcgttgtggtagtgagatgaaaagaggcggcgcttactaccgattccgcctagttggtcacttcgacgtatcgtctggaactccaaccatcgcaggcagagaggtctgcaaaatgcaatcccgaaacagttcgcaggtaatagttagagcctgcataacggtttcgggattttttatatctgcacaacaggtaagagcattgagtcgataatcgtgaagagtcggcgagcctggttagccagtgctctttccgttgtgctgaattaagcgaataccggaagcagaaccggatcaccaaatgcgtacaggcgtcatcgccgcccagcaacagcacaacccaaactgagccgtagccactgtctgtcctgaattcattagtaatagttacgctgcggccttttacacatgaccttcgtgaaagcgggtggcaggaggtcgcgctaacaacctcctgccgttttgcccgtgcatatcggtcacgaacaaatctgattactaaacacagtagcctggatttgttctatcagtaatcgaccttattcctaattaaatagagcaaatccccttattgggggtaagacatgaagatgccagaaaaacatgacctgttggccgccattctcgcggcaaaggaacaaggcatcggggcaatccttgcgtttgcaatggcgtaccttcgcggcagatataatggcggtgcgtttacaaaaacagtaatcgacgcaacgatgtgcgccattatcgcctggttcattcgtgaccttctcgacttcgccggactaagtagcaatctcgcttatataacgagcgtgtttatcggctacatcggtactgactcgattggttcgcttatcaaacgcttcgctgctaaaaaagccggagtagaagatggtagaaatcaataatcaacgtaaggcgttcctcgatatgctggcgtggtcggagggaactgataacggacgtcagaaaaccagaaatcatggttatgacgtcattgtaggcggagagctatttactgattactccgatcaccctcgcaaacttgtcacgctaaacccaaaactcaaatcaacaggcgcttaagactggccgtcgttttacaacacagaaagagtttgtagaaacgcaaaaaggccatccgtcaggggccttctgcttagtttgatgcctggcagttccctactctcgccttccgcttcctcgctcactgactcgctgcgctcggtcgttcggctgcggcgagcggtatcagctcactcaaaggcggtaatacggttatccacagaatcaggggataacgcaggaaagaacatgtgagcaaaaggccagcaaaaggccaggaaccgtaaaaaggccgcgttgctggcgtttttccataggctccgcccccctgacgagcatcacaaaaatcgacgctcaagtcagaggtggcgaaacccgacaggactataaagataccaggcgtttccccctggaagctccctcgtgcgctctcctgttccgaccctgccgcttaccggatacctgtccgcctttctcccttcgggaagcgtggcgctttctcatagctcacgctgtaggtatctcagttcggtgtaggtcgttcgctccaagctgggctgtgtgcacgaaccccccgttcagcccgaccgctgcgccttatccggtaactatcgtcttgagtccaacccggtaagacacgacttatcgccactggcagcagccactggtaacaggattagcagagcgaggtatgtaggcggtgctacagagttcttgaagtggtgggctaactacggctacactagaagaacagtatttggtatctgcgctctgctgaagccagttaccttcggaaaaagagttggtagctcttgatccggcaaacaaaccaccgctggtagcggtggtttttttgtttgcaagcagcagattacgcgcagaaaaaaaggatctcaagaagatcctttgatcttttctacggggtctgacgctcagtggaacgacgcgcgcgtaactcacgttaagggattttggtcatgagcttgcgccgtcccgtcaagtcagcgtaatgctctgcttttagaaaaactcatcgagcatcaaatgaaactgcaatttattcatatcaggattatcaataccatatttttgaaaaagccgtttctgtaatgaaggagaaaactcaccgaggcagttccataggatggcaagatcctggtatcggtctgcgattccgactcgtccaacatcaatacaacctattaatttcccctcgtcaaaaataaggttatcaagtgagaaatcaccatgagtgacgactgaatccggtgagaatggcaaaagtttatgcatttctttccagacttgttcaacaggccagccattacgctcgtcatcaaaatcactcgcatcaaccaaaccgttattcattcgtgattgcgcctgagcgaggcgaaatacgcgatcgctgttaaaaggacaattacaaacaggaatcgagtgcaaccggcgcaggaacactgccagcgcatcaacaatattttcacctgaatcaggatattcttctaatacctggaacgctgtttttccggggatcgcagtggtgagtaaccatgcatcatcaggagtacggataaaatgcttgatggtcggaagtggcataaattccgtcagccagtttagtctgaccatctcatctgtaacatcattggcaacgctacctttgccatgtttcagaaacaactctggcgcatcgggcttcccatacaagcgatagattgtcgcacctgattgcccgacattatcgcgagcccatttatacccatataaatcagcatccatgttggaatttaatcgcggcctcgacgtttcccgttgaatatggctcatattcttcctttttcaatattattgaagcatttatcagggttattgtctcatgagcggatacatatttgaatgtatttagaaaaataaacaaataggggtcagtgttacaaccaattaaccaattctgaacattatcgcgagcccatttatacctgaatatggctcataacaccccttgtttgcctggcggcagtagcgcggtggtcccacctgaccccatgccgaactcagaagtgaaacgccgtagcgccgatggtagtgtggggactccccatgcgagagtagggaactgccaggcatcaaataaaacgaaaggctcagtcgaaagactgggcctttcgcccgggctaattagggggtgtcgcccttattcgactctatagtgaagttcctattctctagaaagtataggaacttctgaagtggggtcgacttaattaagg

SEQ ID NO: 45 - DNA, 2450 bp, Artificial Sequence
  constructed sequence
gccgccaccatgttcaagtccctcaccaaagtcaacaaggtcaagcccatcggagagaacaacgagaatgagcagagctctcggcgcaacgaagaaggatcccatccgtcgaaccagtcacagcagactaccgcacaggaggagaacaagggagaagaaaagtcgctcaagactaagtccacccccgtgacctcggaagaaccgcacacgaacattcaggacaagctgtccaagaagaactcctccggcgatctcacgactaacccggacccccagaatgccgctgaacctactgggaccgtgcctgagcaaaaggagatggaccccggaaaggagggtcctaactccccccaaaacaagcccccggccgcgccggtcatcaatgagtacgcggacgcgcaactgcataacctcgtgaagcggatgcggcaaagaaccgccctctacaagaagaaactggtggagggcgacctgagctcacctgaagccagcccacagaccgccaaacccaccgccgtgccgcctgtgaaggagtccgatgacaagcctaccgagcactactaccgcctgctgtggttcaaggtcaagaagatgcccctgaccgaatacctcaagcggatcaagctgccgaacagcatcgacagctacaccgaccggctttacttgctctggctgctgcttgtgaccctggcttacaactggaactgttgtttcattcccctgcggctggtgttcccttaccaaaccgcggataacattcactactggctgattgccgacatcatttgcgacatcatctacctgtacgatatgctttttatccaaccgcggctgcaattcgtccgcgggggagacatcattgtggactccaacgagctgcgcaagcattaccggacctcgacaaagttccagctggatgtggcctccatcatcccgttcgatatctgttacctgttctttggcttcaacccgatgttcagggcgaacaggatgctgaagtacacttccttcttcgaattcaaccaccacctggagtccatcatggacaaggcttacatctaccgcgtgatccggaccactggttacctcctgttcatcctgcacatcaacgcctgcgtctattactgggcctcaaactacgaaggcattggtaccacccgctgggtgtacgacggggagggaaacgagtatctgcgctgctactactgggccgtgcgaaccctcataactattggcggcctcccggaaccgcagaccctgttcgagatcgtgttccaactcctcaacttcttctcgggagtgttcgtgttttcaagcttgattggacagatgcgggacgtgatcggtgcagcaactgccaaccagaactactttcgcgcctgcatggacgacactatcgcgtacatgaacaactattcgatccccaagctggtgcagaaacgcgtgcggacttggtatgagtacacttgggactcccagagaatgcttgacgagtccgatctgctcaagaccctgcctactaccgtgcagctggcactcgccatcgatgtgaacttctccattatctcgaaagtcgatctgttcaagggctgcgacacccagatgatctacgacatgctgctgagactcaagtccgtgttgtacctccctggcgacttcgtgtgcaagaagggcgaaatcgggaaggagatgtacattatcaagcacggagaagtccaggtgctggggggaccagacggtaccaaggtccttgtcaccctgaaggccgggtccgtgttcggcgaaatttccctgttggccgccggcggtggcaacaggagaaccgcaaatgtggtggcccacggcttcgcaaaccttctgaccctggacaagaaaaccctccaggaaatcctcgtgcactacccggatagcgagcggatcctgatgaagaaagcccgggtgctgctgaagcaaaaggccaagaccgccgaagccaccccgcctcggaaggacctggctctgctgttcccacccaaggaggagactcccaaactgtttaagaccctcttgggcgggacgggaaaggcctccctcgctcgcttgcttaagttgaagagggagcaggccgcgcagaagaaggaaaactccgaaggaggggaagaagagggaaaggaaaacgaagataagcagaaggagaacgaggataagcaaaaggaaaatgaggacaaggggaaagaaaacgaggacaaggataagggtcgcgaacctgaagagaagccgctggatcggccagagtgcactgcctcgcctatcgcggtcgaagaggaaccccatagcgtgcgcagaaccgtgctgcctagaggcacatcgaggcagtcactgattatctctatggcaccaagcgccgagggaggagaggaagtgctcaccatcgaggtcaaggaaaaagcgaagcagtgatcataactgca

SEQ ID NO: 46 - DNA, 12006 bp, Artificial Sequence
  constructed sequence
ctgcgcgctcgctcgctcactgaggccgcccgggcaaagcccgggcgtcgggcgacctttggtcgcccggcctcagtgagcgagcgagcgcgcagagagggagtggccaactccatcactaggggttccttgtagttaatgattaacccgccatgctacttatctacgtagcaagctagcctgaagagacagaaatatctctaattccatgagcggtcatacgaggcaagagaagccgcttagagcatggacttagttagtttcagggattggacagagtcaagagctggggtgaggaggttaccctcggtaggggtgacacagatgtcaaccgcctattccctccacatgcatgtcctgccagaagaacctgtccctgggctgggaatcttatattaccttcctctccaatgagaagagaagttcaaggctcacagacatgtgcatacacaagctcaatgcactcaagattcccctccaccactcctgcccccactacctacaggagattgactcctgctgtgcacataagctgggataatcagggtttctaaacatcagcttcaaaagtccaatgtccaaagtggtggggggccggggaacgaggtactctttccatacccttggcttttgtgtggcctggagccgctgatatagagattggagtgggacacgaggtattcctttcaaaaacacaaaggcctatactttgagccctcccatttcaatcccccaccatgcttcacctttaagacctccaactccactttgatcccagttctcaggttcaggcctcacaaggccaaaatcctgaagttacccttctcaaactcccttgcctttaacatcatcagaatcaacctcctacccccactctgtcccagcagcaatagcctgctaatcttttagcactaatcttttaggcactaatctgctttccaaactcttggcacctgaactatttataagcagtgttttatgcccccccaccaaagaaccctattcttttcccatgaccccaccaatcaaaacactcagaggactgtgggtataagaggctggggaggcaggcatagcagcggccgccaccatggccaagatcaacacccaatactcccacccctccaggacccacctcaaggtaaagacctcagaccgggatctcaatcgcgctgaaaatggcctcagcagagcccactcgtcaagtgaggagacatcgtcagtgctgcagccggggatcgccatggagaccagaggactggctgactccgggcagggctccttcaccggccaggggatcgccaggctgtcgcgcctcatcttcttgctgcgcaggtgggctgccaggcatgtgcaccaccaggaccagggaccggactcttttcctgatcgtttccgtggagccgagcttaaggaggtgtccagccaagaaagcaatgcccaggcaaatgtgggcagccaggagccagcagacagagggagaagcgcctggcccctggccaaatgcaacactaacaccagcaacaacacggaggaggagaagaagacgaaaaagaaggatgcgatcgtggtggacccgtccagcaacctgtactaccgctggctgaccgccatcgccctgcctgtcttctataactggtatctgcttatttgcagggcctgtttcgatgagctgcagtccgagtacctgatgctgtggctggtcctggactactcggcagatgtcctgtatgtcttggatgtgcttgtacgagctcggacaggttttcttgagcaaggcttaatggtcagtgataccaacaggctgtggcagcattacaagacgaccacgcagttcaagctggatgtgttgtccctggtccccaccgacctggcttacttaaaggtgggcacaaactacccagaagtgaggttcaaccgcctactgaagttttcccggctctttgaattctttgaccgcacagagacaaggaccaactaccccaatatgttcaggattgggaacttggtcttgtacattctcatcatcatccactggaatgcctgcatctactttgccatttccaagttcattggttttgggacagactcctgggtctacccaaacatctcaatcccagagcatgggcgcctctccaggaagtacatttacagtctctactggtccaccttgacccttaccaccattggtgagaccccaccccccgtgaaagatgaggagtatctctttgtggtcgtagacttcttggtgggtgttctgatttttgccaccattgtgggcaatgtgggctccatgatctcgaatatgaatgcctcacgggcagagttccaggccaagattgattccatcaagcagtacatgcagttccgcaaggtcaccaaggacttggagacgcgggttatccggtggtttgactacctgtgggccaacaagaagacggtggatgagaaggaggtgctcaagagcctcccagacaagctgaaggctgagatcgccatcaacgtgcacctggacacgctgaagaaggttcgcatcttccaggactgtgaggcagggctgctggtggagctggtgctgaagctgcgacccactgtgttcagccctggggattatatctgcaagaagggagatattgggaaggagatgtacatcatcaacgagggcaagctggccgtggtggctgatgatggggtcacccagttcgtggtcctcagcgatggcagctacttcggggagatcagcattctgaacatcaaggggagcaagtcggggaaccgcaggacggccaacatccgcagcattggctactcagacctgttctgcctctcaaaggacgatctcatggaggccctcaccgagtaccccgaagccaagaaggccctggaggagaaaggacggcagatcctgatgaaagacaacctgatcgatgaggagctggccagggcgggcgcggaccccaaggaccttgaggagaaagtggagcagctggggtcctccctggacaccctgcagaccaggtttgcacgcctcctggctgagtacaacgccacccagatgaagatgaagcagcgtctcagccaactggaaagccaggtgaagggtggtggggacaagcccctggctgatggggaagttcccggggatgctacaaaaacagaggacaaacaacagtgatcatagggccgcatagtactgcggatccgatccaatcaacctctggattacaaaatttgtgaaagattgactggtattcttaactatgttgctccttttacgctatgtggatacgctgctttaatgcctttgtatcatgctattgcttcccgtatggctttcattttctcctccttgtataaatcctggttgctgtctctttatgaggagttgtggcccgttgtcaggcaacgtggcgtggtgtgcactgtgtttgctgacgcaacccccactggttggggcattgccaccacctgtcagctcctttccgggactttcgctttccccctccctattgccacggcggaactcatcgccgcctgccttgcccgctgctggacaggggctcggctgttgggcactgacaattccgtggtgttgtcggggaaatcatcgtcctttccttggctgctcgcctgtgttgccacctggattctgcgcgggacgtccttctgctacgtcccttcggccctcaatccagcggaccttccttcccgcggcctgctgccggctctgcggcctcttccgcgtcttcgagatcgatctgcctcgactgtgccttctagttgccagccatctgttgtttgcccctcccccgtgccttccttgaccctggaaggtgccactcccactgtcctttcctaataaaatgaggaaattgcatcgcattgtctgagtaggtgtcattctattctggggggtggggtggggcaggacagcaagggggaggattgggaagacaatagcaggcatgctggggactcgagttctacgtagataagtagcatggcgggttaatcattaactacaaggaacccctagtgatggagttggccactccctctctgcgcgctcgctcgctcactgaggccgggcgaccaaaggtcgcccgacgcccgggctttgcccgggcggcctcagtgagcgagcgagcgcgcagccttaattaacctaaggaaaatgaagtgaagttcctatactttctagagaataggaacttctatagtgagtcgaataagggcgacacaaaatttattctaaatgcataataaatactgataacatcttatagtttgtattatattttgtattatcgttgacatgtataattttgatatcaaaaactgattttccctttattattttcgagatttattttcttaattctctttaacaaactagaaatattgtatatacaaaaaatcataaataatagatgaatagtttaattataggtgttcatcaatcgaaaaagcaacgtatcttatttaaagtgcgttgcttttttctcatttataaggttaaataattctcatatatcaagcaaagtgacaggcgcccttaaatattctgacaaatgctctttccctaaactccccccataaaaaaacccgccgaagcgggtttttacgttatttgcggattaacgattactcgttatcagaaccgcccagggggcccgagcttaacctttttatttgggggagagggaagtcatgaaaaaactaacctttgaaattcgatctccagcacatcagcaaaacgctattcacgcagtacagcaaatccttccagacccaaccaaaccaatcgtagtaaccattcaggaacgcaaccgcagcttagaccaaaacaggaagctatgggcctgcttaggtgacgtctctcgtcaggttgaatggcatggtcgctggctggatgcagaaagctggaagtgtgtgtttaccgcagcattaaagcagcaggatgttgttcctaaccttgccgggaatggctttgtggtaataggccagtcaaccagcaggatgcgtgtaggcgaatttgcggagctattagagcttatacaggcattcggtacagagcgtggcgttaagtggtcagacgaagcgagactggctctggagtggaaagcgagatggggagacagggctgcatgataaatgtcgttagtttctccggtggcaggacgtcagcatatttgctctggctaatggagcaaaagcgacgggcaggtaaagacgtgcattacgttttcatggatacaggttgtgaacatccaatgacatatcggtttgtcagggaagttgtgaagttctgggatataccgctcaccgtattgcaggttgatatcaacccggagcttggacagccaaatggttatacggtatgggaaccaaaggatattcagacgcgaatgcctgttctgaagccatttatcgatatggtaaagaaatatggcactccatacgtcggcggcgcgttctgcactgacagattaaaactcgttcccttcaccaaatactgtgatgaccatttcgggcgagggaattacaccacgtggattggcatcagagctgatgaaccgaagcggctaaagccaaagcctggaatcagatatcttgctgaactgtcagactttgagaaggaagatatcctcgcatggtggaagcaacaaccattcgatttgcaaataccggaacatctcggtaactgcatattctgcattaaaaaatcaacgcaaaaaatcggacttgcctgcaaagatgaggagggattgcagcgtgtttttaatgaggtcatcacgggatcccatgtgcgtgacggacatcgggaaacgccaaaggagattatgtaccgaggaagaatgtcgctggacggtatcgcgaaaatgtattcagaaaatgattatcaagccctgtatcaggacatggtacgagctaaaagattcgataccggctcttgttctgagtcatgcgaaatatttggagggcagcttgatttcgacttcgggagggaagctgcatgatgcgatgttatcggtgcggtgaatgcaaagaagataaccgcttccgaccaaatcaaccttactggaatcgatggtgtctccggtgtgaaagaacaccaacaggggtgttaccactaccgcaggaaaaggaggacgtgtggcgagacagcgacgaagtatcaccgacataatctgcgaaaactgcaaataccttccaacgaaacgcaccagaaataaacccaagccaatcccaaaagaatctgacgtaaaaaccttcaactacacggctcacctgtgggatatccggtggctaagacgtcgtgcgaggaaaacaaggtgattgaccaaaatcgaagttacgaacaagaaagcgtcgagcgagctttaacgtgcgctaactgcggtcagaagctgcatgtgctggaagttcacgtgtgtgagcactgctgcgcagaactgatgagcgatccgaatagctcgatgcacgaggaagaagatgatggctaaaccagcgcgaagacgatgtaaaaacgatgaatgccgggaatggtttcaccctgcattcgctaatcagtggtggtgctctccagagtgtggaaccaagatagcactcgaacgacgaagtaaagaacgcgaaaaagcggaaaaagcagcagagaagaaacgacgacgagaggagcagaaacagaaagataaacttaagattcgaaaactcgccttaaagccccgcagttactggattaaacaagcccaacaagccgtaaacgccttcatcagagaaagagaccgcgacttaccatgtatctcgtgcggaacgctcacgtctgctcagtgggatgccggacattaccggacaactgctgcggcacctcaactccgatttaatgaacgcaatattcacaagcaatgcgtggtgtgcaaccagcacaaaagcggaaatctcgttccgtatcgcgtcgaactgattagccgcatcgggcaggaagcagtagacgaaatcgaatcaaaccataaccgccatcgctggactatcgaagagtgcaaggcgatcaaggcagagtaccaacagaaactcaaagacctgcgaaatagcagaagtgaggccgcatgacgttctcagtaaaaaccattccagacatgctcgttgaagcatacggaaatcagacagaagtagcacgcagactgaaatgtagtcgcggtacggtcagaaaatacgttgatgataaagacgggaaaatgcacgccatcgtcaacgacgttctcatggttcatcgcggatggagtgaaagagatgcgctattacgaaaaaattgatggcagcaaataccgaaatatttgggtagttggcgatctgcacggatgctacacgaacctgatgaacaaactggatacgattggattcgacaacaaaaaagacctgcttatctcggtgggcgatttggttgatcgtggtgcagagaacgttgaatgcctggaattaatcacattcccctggttcagagctgtacgtggaaaccatgagcaaatgatgattgatggcttatcagagcgtggaaacgttaatcactggctgcttaatggcggtggctggttctttaatctcgattacgacaaagaaattctggctaaagctcttgcccataaagcagatgaacttccgttaatcatcgaactggtgagcaaagataaaaaatatgttatctgccacgccgattatccctttgacgaatacgagtttggaaagccagttgatcatcagcaggtaatctggaaccgcgaacgaatcagcaactcacaaaacgggatcgtgaaagaaatcaaaggcgcggacacgttcatctttggtcatacgccagcagtgaaaccactcaagtttgccaaccaaatgtatatcgataccggcgcagtgttctgcggaaacctaacattgattcaggtacagggagaaggcgcatgagactcgaaagcgtagctaaatttcattcgccaaaaagcccgatgatgagcgactcaccacgggccacggcttctgactctctttccggtactgatgtgatggctgctatggggatggcgcaatcacaagccggattcggtatggctgcattctgcggtaagcacgaactcagccagaacgacaaacaaaaggctatcaactatctgatgcaatttgcacacaaggtatcggggaaataccgtggtgtggcaaagcttgaaggaaatactaaggcaaaggtactgcaagtgctcgcaacattcgcttatgcggattattgccgtagtgccgcgacgccgggggcaagatgcagagattgccatggtacaggccgtgcggttgatattgccaaaacagagctgtgggggagagttgtcgagaaagagtgcggaagatgcaaaggcgtcggctattcaaggatgccagcaagcgcagcatatcgcgctgtgacgatgctaatcccaaaccttacccaacccacctggtcacgcactgttaagccgctgtatgacgctctggtggtgcaatgccacaaagaagagtcaatcgcagacaacattttgaatgcggtcacacgttagcagcatgattgccacggatggcaacatattaacggcatgatattgacttattgaataaaattgggtaaatttgactcaacgatgggttaattcgctcgttgtggtagtgagatgaaaagaggcggcgcttactaccgattccgcctagttggtcacttcgacgtatcgtctggaactccaaccatcgcaggcagagaggtctgcaaaatgcaatcccgaaacagttcgcaggtaatagttagagcctgcataacggtttcgggattttttatatctgcacaacaggtaagagcattgagtcgataatcgtgaagagtcggcgagcctggttagccagtgctctttccgttgtgctgaattaagcgaataccggaagcagaaccggatcaccaaatgcgtacaggcgtcatcgccgcccagcaacagcacaacccaaactgagccgtagccactgtctgtcctgaattcattagtaatagttacgctgcggccttttacacatgaccttcgtgaaagcgggtggcaggaggtcgcgctaacaacctcctgccgttttgcccgtgcatatcggtcacgaacaaatctgattactaaacacagtagcctggatttgttctatcagtaatcgaccttattcctaattaaatagagcaaatccccttattgggggtaagacatgaagatgccagaaaaacatgacctgttggccgccattctcgcggcaaaggaacaaggcatcggggcaatccttgcgtttgcaatggcgtaccttcgcggcagatataatggcggtgcgtttacaaaaacagtaatcgacgcaacgatgtgcgccattatcgcctggttcattcgtgaccttctcgacttcgccggactaagtagcaatctcgcttatataacgagcgtgtttatcggctacatcggtactgactcgattggttcgcttatcaaacgcttcgctgctaaaaaagccggagtagaagatggtagaaatcaataatcaacgtaaggcgttcctcgatatgctggcgtggtcggagggaactgataacggacgtcagaaaaccagaaatcatggttatgacgtcattgtaggcggagagctatttactgattactccgatcaccctcgcaaacttgtcacgctaaacccaaaactcaaatcaacaggcgcttaagactggccgtcgttttacaacacagaaagagtttgtagaaacgcaaaaaggccatccgtcaggggccttctgcttagtttgatgcctggcagttccctactctcgccttccgcttcctcgctcactgactcgctgcgctcggtcgttcggctgcggcgagcggtatcagctcactcaaaggcggtaatacggttatccacagaatcaggggataacgcaggaaagaacatgtgagcaaaaggccagcaaaaggccaggaaccgtaaaaaggccgcgttgctggcgtttttccataggctccgcccccctgacgagcatcacaaaaatcgacgctcaagtcagaggtggcgaaacccgacaggactataaagataccaggcgtttccccctggaagctccctcgtgcgctctcctgttccgaccctgccgcttaccggatacctgtccgcctttctcccttcgggaagcgtggcgctttctcatagctcacgctgtaggtatctcagttcggtgtaggtcgttcgctccaagctgggctgtgtgcacgaaccccccgttcagcccgaccgctgcgccttatccggtaactatcgtcttgagtccaacccggtaagacacgacttatcgccactggcagcagccactggtaacaggattagcagagcgaggtatgtaggcggtgctacagagttcttgaagtggtgggctaactacggctacactagaagaacagtatttggtatctgcgctctgctgaagccagttaccttcggaaaaagagttggtagctcttgatccggcaaacaaaccaccgctggtagcggtggtttttttgtttgcaagcagcagattacgcgcagaaaaaaaggatctcaagaagatcctttgatcttttctacggggtctgacgctcagtggaacgacgcgcgcgtaactcacgttaagggattttggtcatgagcttgcgccgtcccgtcaagtcagcgtaatgctctgcttttagaaaaactcatcgagcatcaaatgaaactgcaatttattcatatcaggattatcaataccatatttttgaaaaagccgtttctgtaatgaaggagaaaactcaccgaggcagttccataggatggcaagatcctggtatcggtctgcgattccgactcgtccaacatcaatacaacctattaatttcccctcgtcaaaaataaggttatcaagtgagaaatcaccatgagtgacgactgaatccggtgagaatggcaaaagtttatgcatttctttccagacttgttcaacaggccagccattacgctcgtcatcaaaatcactcgcatcaaccaaaccgttattcattcgtgattgcgcctgagcgaggcgaaatacgcgatcgctgttaaaaggacaattacaaacaggaatcgagtgcaaccggcgcaggaacactgccagcgcatcaacaatattttcacctgaatcaggatattcttctaatacctggaacgctgtttttccggggatcgcagtggtgagtaaccatgcatcatcaggagtacggataaaatgcttgatggtcggaagtggcataaattccgtcagccagtttagtctgaccatctcatctgtaacatcattggcaacgctacctttgccatgtttcagaaacaactctggcgcatcgggcttcccatacaagcgatagattgtcgcacctgattgcccgacattatcgcgagcccatttatacccatataaatcagcatccatgttggaatttaatcgcggcctcgacgtttcccgttgaatatggctcatattcttcctttttcaatattattgaagcatttatcagggttattgtctcatgagcggatacatatttgaatgtatttagaaaaataaacaaataggggtcagtgttacaaccaattaaccaattctgaacattatcgcgagcccatttatacctgaatatggctcataacaccccttgtttgcctggcggcagtagcgcggtggtcccacctgaccccatgccgaactcagaagtgaaacgccgtagcgccgatggtagtgtggggactccccatgcgagagtagggaactgccaggcatcaaataaaacgaaaggctcagtcgaaagactgggcctttcgcccgggctaattagggggtgtcgcccttattcgactctatagtgaagttcctattctctagaaagtataggaacttctgaagtggggtcgacttaattaagg